European Patent Application EP 4 692 344 A1, published February 11, 2026. Title: SELF AMPLIFYING RNA CONSTRUCT AND USE THEREOF. Applicant: 주식회사 마이크로유니. The sequence listing filed with the application follows.

SEQUENCE LISTING (197 sequences)

SEQ ID NO: 1 - DNA, 743 bp, synthetic construct
  source 1..743: mol_type = other DNA
  misc_feature 1..743: note = nucleotide sequence of 5' UTR
ttaaaacagcctgtgggttgtacccacccacagggcccactgggcgctagcactctggtatcacggtacctttgtgtgcctgttttatatcccctttccccgattgtaacttagaagatgtacacactgatcaatagcgggcatagcacaccagctatgtcttgatcaagcactcctgtatccccggaccaagtatcaatagactgctcacgcggttgaaggagaaaacgttcgtcacccggctaactacttcgagaaacccagtagtatcatgaaagttgcgaggcgtttcgttcagcacacccccagtgtagatcgggtcgatgagtcaccgcatcccccacgggcgaccgtggcggtggctgcgctggcggcctgcctacggggcaacccgtaggacgcttcaatacagacatggtgcgaagagtcgattgagctagttagtagtcctccggcccctgaatgcggctaatcctaactgcggagcacatgccctcaacccagggggtattgtgtcgtaacgggcaactctgcagcggaaccgactactttgggtgtccgtgtttccttttatccttatactggctgcttatggtgacaattgaaagattgttgccatatagctattggattggccatccagtgtctaatagagctgttatttacctctttgttggatttataccactcaacctaaaagaagttaaaacactacagctcattttacaactgaatacagcaaa

SEQ ID NO: 2 - DNA, 450 bp, synthetic construct
  source 1..450: mol_type = other DNA
  misc_feature 1..450: note = nucleotide sequence coding 2A protease
ggttcatgtgggcaacaatcaggagctgtgtacgtgggcaattacaggattgtaaacagacacctggcaacgagccacgattggcaaaattgcgtgtgggaggactacaacagggatctcctggtcagcacaacaactgctcatggttgtgatactatagcacggtgccaatgtactgctggcgtgtacttttgtgcatctagaaacaagcactacccagtgagcttcgagggtccaggtctagtgaaagttcaggagggcgagtactaccccgagagataccagtcgcacgtactccttgcagttggattttcagaaccgggtgattgtggaggtattttgaggtgtgaacatggagtcattgggctcgttaccatgggtggtgagggtgtagtaggcttcgctgacgtgcgggatcttttgtggttggaagacgacgccatggagcag

SEQ ID NO: 3 - DNA, 297 bp, synthetic construct
  source 1..297: mol_type = other DNA
  misc_feature 1..297: note = nucleotide sequence coding 2B
ggtgttagagattatgtagagcaactgggaaatgcatttggctcaggtttcactaaccaaatctgtgagcaagttaacctccttaaagaatctctgatagggcaggattccatattggaaaaatccctgaaggccctggttaaaatcatatcagccctggtgatagtggttaggaaccacgacgacctgattacagtgactgccacactagctttaatcggttgcgcatcatctccatggcgatggctcaaacaaaaagtgtgtcaatactacggaatccccatggcagaaaggcag

SEQ ID NO: 4 - DNA, 987 bp, synthetic construct
  source 1..987: mol_type = other DNA
  misc_feature 1..987: note = nucleotide sequence coding 2C
aataacggttggttaaagaaattcactgaaatgaccaacgcctgcaagggcatggagtggattgctgttaaaattcaaaagttcatcgagtggctcaaagtaaagattctgcctgaagtgaaggagaaacatgagttccttaccagattgaagcaattgccactccttgaaagtcaaattgccaccattgagcaaagcgcaccctcacaaagtgatcaagagcagcttttttcgaatgttcagtacttcgcccattactgcaggaagtatgcacctctgtatgctgccgaagcaaaaagagtgttctcattagaaaagaaaatgagtaattacatacagttcaagtccaaatgccgcattgagcctgtatgcttactccttcacggtagtccaggggctggcaagtcagtagctaccaacctgatagggagatcccttgcagagaagctcaatagctctgtgtactctttaccaccagatccagatcattttgatgggtacaaacagcaggcagtggtgatcatggatgatctctgtcaaaaccccgatgggaaggacgtgtccttgttttgccaaatggtgtctagtgtagattttgtgccacccatggcggcgctggaagaaaaaggcattctctttacgtccccgtttgtgttggcatcaaccaacgcggggtccatcaatgcaccaacagtgtcagacagcagagcacttgccagaaggtttcactttgacatgaatattgaggtgatttcgatgtacagccagaatggtaaaattaacatgcccatgtctgttaagacatgtgatgatgaatgctgcccggtcaatttcaaaaagtgttgcccactagtgtgtggcaaggccatccagtttattgacaggagaaaccaagttagatattcactggacatgctggttactgagatgtttagagagtacaaccacagacacagtgtgggtgctaccctcgaggctttgttccaa

SEQ ID NO: 5 - DNA, 267 bp, synthetic construct
  source 1..267: mol_type = other DNA
  misc_feature 1..267: note = nucleotide sequence coding 3A
ggaccaccagtatacagggaaatcaaaatcagtgtggccccggaaacaccccctccaccagcaattgctgaccttctaaaatctgtagacagtgaggcaataagggagtactgcaaggaaaggggttggcttgtgccagaggtcagctccactctacaaattgaaaaacatgttagcagggcatttatttgcttgcaagcgctaactacatttgtttcagtggctggtataatctacatcatttacaagttgtttgccggctttcag

SEQ ID NO: 6 - DNA, 66 bp, synthetic construct
  source 1..66: mol_type = other DNA
  misc_feature 1..66: note = nucleotide sequence coding 3B
ggtgcatacactggaatgcccaaccagaaacccaaggtgcccaccttaagacaagctaaggtgcaa

SEQ ID NO: 7 - DNA, 549 bp, synthetic construct
  source 1..549: mol_type = other DNA
  misc_feature 1..549: note = nucleotide sequence coding 3C
ggtccggcatttgaatttgccgtagcaatgatgaaaaggaacgccagcacagtcaagacagaatacggtgagttcacgatgcttggcatctatgataaatgggcagtgctgccgcgccacgccaagcctggaccaactattttaatgaatgatcaggaggttggtgtgctcgatgccaaagagttagttgataaagacggaaccaacctggagctgacactattgaagcttaaccgcaatgaaaagttcagagacatcagaggttttcttgcaagggaagaagttgaggtaagtgaggctgttttggcaataaacacgagcaagttcccaagcatgtacatccctgtgggccaagtcaccgattacggatttttaaatctaggtggcaccccaacaaagagaatgctcatgtacaacttccctaccagagcgggacagtgtggtggtgtccttatgtcaacaggaaaggtccttggcatacacgtgggaggaaatggtcaccaaggcttctctgctgctctcctcagacactacttcaacgaggaacag

SEQ ID NO: 8 - DNA, 1386 bp, synthetic construct
  source 1..1386: mol_type = other DNA
  misc_feature 1..1386: note = nucleotide sequence coding 3D
ggcgaaatagagtttattgagagctctaaagatgcaggatttcctgtgatcaacacccctaataaaaccaaactggaaccaagtgtgtttcatcaggtttttgagggcaacaaagaaccagcagtcctaagaaacggagacccgcgacttaaagccaactttgaggaagcgatattttccaagtacatcggaaatgtgaacacacatgtggacgagtacatgatagaagctgttgatcactacgctggacagctggcaactctggacatcagtacagaacctatgaagcttgaggatgctgtttatggcactgaaggcttggaagcattggacttgaccactagcgcaggatatccttatgtcgccttgggcatcaagaaaagggatatcctctccaagaagactaaagatctcaccaagctgagggaatgcatggacaagtatggtctaaatctgccgatggtgacctacgtgaaggatgaactcaggtccgctgagaaagtagccaagggaaaatccagacttatagaagcttctagtctcaatgactcagtggccatgaggcagacatttgggaacctatacaagacattccacctcaacccaggcattgtcactggtagtgctgttgggtgcgacccagatgtgttttggagcaaaatacccgtgatgcttgacgggcaccttatagcttttgattactctggctacgacgctagcttgagcccagtgtggtttgcttgtttgaaactcctcctagggaaactagggtatactcataaggaaaccaattacatagactacctctgcaactcccatcacttatacagagataaacactatttcgtgaggggtggtatgccatcaggatgttcaggcaccagtatattcaacaccatgatcaacaacatcattattaggacccttatgctaaaggtctacaaaggtattgacctggatcagtttagaatgatcgcttacggggacgatgtgatagcctcttacccgtggcctattgatgcctcactactagcagaagcgggaaaggattatggtttgatcatgaccccagcagataaaggagagtgttttaatgaggtaacctggacaaatgtaaccttcttgaaaaggtactttagagctgatgaacaatatccattcttggtgcaccccgtgatgcccatgaaagacatacacgaatccattagatggaccaaagacccaaagaacactcaagatcatgtgcgctcgttatgcctattggcttggcacaatggggagcacgaatatgaggaatttatccgaaagatcagaagcgtgcctgttggacgctgtttgaccctcccggtgttctcaacactacgcaggaaatggttagattccttc

SEQ ID NO: 9 - skipped

SEQ ID NO: 10 - DNA, 100 bp, synthetic construct
  source 1..100: mol_type = other DNA
  misc_feature 1..100: note = nucleotide sequence of 3' UTR
aattagagtgcaatcaatgaactatgattggcttaaccctaccgcatgaaccgaactagacaaaagtgcggtaggggtaaattctccgcattcggtgcgg

SEQ ID NO: 11 - protein, 150 aa, synthetic construct
  REGION 1..150: note = 2A protease
GSCGQQSGAVYVGNYRIVNRHLATSHDWQNCVWEDYNRDLLVSTTTAHGCDTIARCQCTAGVYFCASRNKHYPVSFEGPGLVKVQEGEYYPERYQSHVLLAVGFSEPGDCGGILRCEHGVIGLVTMGGEGVVGFADVRDLLWLEDDAMEQ

SEQ ID NO: 12 - protein, 99 aa, synthetic construct
  REGION 1..99: note = 2B
GVRDYVEQLGNAFGSGFTNQICEQVNLLKESLIGQDSILEKSLKALVKIISALVIVVRNHDDLITVTATLALIGCASSPWRWLKQKVCQYYGIPMAERQ

SEQ ID NO: 13 - protein, 329 aa, synthetic construct
  REGION 1..329: note = 2C
NNGWLKKFTEMTNACKGMEWIAVKIQKFIEWLKVKILPEVKEKHEFLTRLKQLPLLESQIATIEQSAPSQSDQEQLFSNVQYFAHYCRKYAPLYAAEAKRVFSLEKKMSNYIQFKSKCRIEPVCLLLHGSPGAGKSVATNLIGRSLAEKLNSSVYSLPPDPDHFDGYKQQAVVIMDDLCQNPDGKDVSLFCQMVSSVDFVPPMAALEEKGILFTSPFVLASTNAGSINAPTVSDSRALARRFHFDMNIEVISMYSQNGKINMPMSVKTCDDECCPVNFKKCCPLVCGKAIQFIDRRNQVRYSLDMLVTEMFREYNHRHSVGATLEALFQ

SEQ ID NO: 14 - protein, 89 aa, synthetic construct
  REGION 1..89: note = 3A
GPPVYREIKISVAPETPPPPAIADLLKSVDSEAIREYCKERGWLVPEVSSTLQIEKHVSRAFICLQALTTFVSVAGIIYIIYKLFAGFQ

SEQ ID NO: 15 - protein, 22 aa, synthetic construct
  REGION 1..22: note = 3B
GAYTGMPNQKPKVPTLRQAKVQ

SEQ ID NO: 16 - protein, 183 aa, synthetic construct
  REGION 1..183: note = 3C
GPAFEFAVAMMKRNASTVKTEYGEFTMLGIYDKWAVLPRHAKPGPTILMNDQEVGVLDAKELVDKDGTNLELTLLKLNRNEKFRDIRGFLAREEVEVSEAVLAINTSKFPSMYIPVGQVTDYGFLNLGGTPTKRMLMYNFPTRAGQCGGVLMSTGKVLGIHVGGNGHQGFSAALLRHYFNEEQ

SEQ ID NO: 17 - protein, 462 aa, synthetic construct
  REGION 1..462: note = 3D
GEIEFIESSKDAGFPVINTPNKTKLEPSVFHQVFEGNKEPAVLRNGDPRLKANFEEAIFSKYIGNVNTHVDEYMIEAVDHYAGQLATLDISTEPMKLEDAVYGTEGLEALDLTTSAGYPYVALGIKKRDILSKKTKDLTKLRECMDKYGLNLPMVTYVKDELRSAEKVAKGKSRLIEASSLNDSVAMRQTFGNLYKTFHLNPGIVTGSAVGCDPDVFWSKIPVMLDGHLIAFDYSGYDASLSPVWFACLKLLLGKLGYTHKETNYIDYLCNSHHLYRDKHYFVRGGMPSGCSGTSIFNTMINNIIIRTLMLKVYKGIDLDQFRMIAYGDDVIASYPWPIDASLLAEAGKDYGLIMTPADKGECFNEVTWTNVTFLKRYFRADEQYPFLVHPVMPMKDIHESIRWTKDPKNTQDHVRSLCLLAWHNGEHEYEEFIRKIRSVPVGRCLTLPVFSTLRRKWLDSF

SEQ ID NO: 18 - skipped

SEQ ID NO: 19 - protein, 5 aa, synthetic construct
  REGION 1..5: note = VP1-5a.a
AMQTT

SEQ ID NO: 20 - protein, 10 aa, synthetic construct
  REGION 1..10: note = VP1-10a.a
RTEITAMQTT

SEQ ID NO: 21 - protein, 15 aa, synthetic construct
  REGION 1..15: note = VP1-15a.a
GVTESRTEITAMQTT

SEQ ID NO: 22 - protein, 20 aa, synthetic construct
  REGION 1..20: note = VP1-20a.a
NFEPTGVTESRTEITAMQTT

SEQ ID NO: 23 - protein, 25 aa, synthetic construct
  REGION 1..25: note = VP1-25a.a
KAGNVNFEPTGVTESRTGITAMQTT

SEQ ID NO: 24 - skipped

SEQ ID NO: 25 - DNA, 15 bp, synthetic construct
  source 1..15: mol_type = other DNA
  misc_feature 1..15: note = nucleotide sequence coding VP1-5a.a
gcaatgcagaccacc

SEQ ID NO: 26 - DNA, 30 bp, synthetic construct
  source 1..30: mol_type = other DNA
  misc_feature 1..30: note = nucleotide sequence coding VP1-10a.a
cgcactgaaattacggcaatgcagaccacc

SEQ ID NO: 27 - DNA, 45 bp, synthetic construct
  source 1..45: mol_type = other DNA
  misc_feature 1..45: note = nucleotide sequence coding VP1-15a.a
ggggtgacggagtcccgcactgaaattacggcaatgcagaccacc

SEQ ID NO: 28 - DNA, 60 bp, synthetic construct
  source 1..60: mol_type = other DNA
  misc_feature 1..60: note = nucleotide sequence coding VP1-20a.a
aactttgagccaacaggggtgacggagtcccgcactgaaattacggcaatgcagaccacc

SEQ ID NO: 29 - DNA, 75 bp, synthetic construct
  source 1..75: mol_type = other DNA
  misc_feature 1..75: note = nucleotide sequence coding VP1-25a.a
aaagcaggaaacgtcaactttgagccaacaggggtgacggagtctcgtactggaattacggcaatgcagaccacc

SEQ ID NO: 30 - RNA, 15 nt, synthetic construct
  source 1..15: mol_type = other RNA
  misc_feature 1..15: note = nucleotide sequence coding VP1-5a.a
gcaatgcagaccacc

SEQ ID NO: 31 - RNA, 30 nt, synthetic construct
  source 1..30: mol_type = other RNA
  misc_feature 1..30: note = nucleotide sequence coding VP1-10a.a
cgcactgaaattacggcaatgcagaccacc

SEQ ID NO: 32 - RNA, 45 nt, synthetic construct
  source 1..45: mol_type = other RNA
  misc_feature 1..45: note = nucleotide sequence coding VP1-15a.a
ggggtgacggagtcccgcactgaaattacggcaatgcagaccacc

SEQ ID NO: 33 - RNA, 60 nt, synthetic construct
  source 1..60: mol_type = other RNA
  misc_feature 1..60: note = nucleotide sequence coding VP1-20a.a
aactttgagccaacaggggtgacggagtcccgcactgaaattacggcaatgcagaccacc

SEQ ID NO: 34 - RNA, 75 nt, synthetic construct
  source 1..75: mol_type = other RNA
  misc_feature 1..75: note = nucleotide sequence coding VP1-25a.a
aaagcaggaaacgtcaactttgagccaacaggggtgacggagtctcgtactggaattacggcaatgcagaccacc

SEQ ID NO: 35-37 - skipped (3 entries)

SEQ ID NO: 38 - DNA, 50 bp, synthetic construct
  source 1..50: mol_type = other DNA
aaaaaaaaaaaaaaaaaaaaaaaaaaaaaaaaaaaaaaaaaaaaaaaaaa

SEQ ID NO: 39 - DNA, 70 bp, synthetic construct
  source 1..70: mol_type = other DNA
  misc_feature 1..70: note = nucleotide sequence of 100X poly(A)
aaaaaaaaaaaaaaaaaaaaaaaaaaaaaaaaaaaaaaaaaaaaaaaaaaaaaaaaaaaaaaaaaaaaaa

SEQ ID NO: 40 - DNA, 120 bp, synthetic construct
  source 1..120: mol_type = other DNA
  misc_feature 1..120: note = nucleotide sequence of 120X poly(A)
aaaaaaaaaaaaaaaaaaaaaaaaaaaaaaaaaaaaaaaaaaaaaaaaaaaaaaaaaaaaaaaaaaaaaaaaaaaaaaaaaaaaaaaaaaaaaaaaaaaaaaaaaaaaaaaaaaaaaaaa

SEQ ID NO: 41 - DNA, 1653 bp, synthetic construct
  source 1..1653: mol_type = other DNA
  misc_feature 1..1653: note = nucleotide sequence coding luciferase
atggaagacgccaaaaacataaagaaaggcccggcgccattctatccgctggaagatggaaccgctggagagcaactgcataaggctatgaagagatacgccctggttcctggaacaattgcttttacagatgcacatatcgaggtggacatcacttacgctgagtacttcgaaatgtccgttcggttggcagaagctatgaaacgatatgggctgaatacaaatcacagaatcgtcgtatgcagtgaaaactctcttcaattctttatgccggtgttgggcgcgttatttatcggagttgcagttgcgcccgcgaacgacatttataatgaacgtgaattgctcaacagtatgggcatttcgcagcctaccgtggtgttcgtttccaaaaaggggttgcaaaaaattttgaacgtgcaaaaaaagctcccaatcatccaaaaaattattatcatggattctaaaacggattaccagggatttcagtcgatgtacacgttcgtcacatctcatctacctcccggttttaatgaatacgattttgtgccagagtccttcgatagggacaagacaattgcactgatcatgaactcctctggatctactggtctgcctaaaggtgtcgctctgcctcatagaactgcctgcgtgagattctcgcatgccagagatcctatttttggcaatcaaatcattccggatactgcgattttaagtgttgttccattccatcacggttttggaatgtttactacactcggatatttgatatgtggatttcgagtcgtcttaatgtatagatttgaagaagagctgtttctgaggagccttcaggattacaagattcaaagtgcgctgctggtgccaaccctattctccttcttcgccaaaagcactctgattgacaaatacgatttatctaatttacacgaaattgcttctggtggcgctcccctctctaaggaagtcggggaagcggttgccaagaggttccatctgccaggtatcaggcaaggatatgggctcactgagactacatcagctattctgattacacccgagggggatgataaaccgggcgcggtcggtaaagttgttccattttttgaagcgaaggttgtggatctggataccgggaaaacgctgggcgttaatcaaagaggcgaactgtgtgtgagaggtcctatgattatgtccggttatgtaaacaatccggaagcgaccaacgccttgattgacaaggatggatggctacattctggagacatagcttactgggacgaagacgaacacttcttcatcgttgaccgcctgaagtctctgattaagtacaaaggctatcaggtggctcccgctgaattggaatccatcttgctccaacaccccaacatcttcgacgcaggtgtcgcaggtcttcccgacgatgacgccggtgaacttcccgccgccgttgttgttttggagcacggaaagacgatgacggaaaaagagatcgtggattacgtcgccagtcaagtaacaaccgcgaaaaagttgcgcggaggagttgtgtttgtggacgaagtaccgaaaggtcttaccggaaaactcgacgcaagaaaaatcagagagatcctcataaaggccaagaagggcggaaagatcgccgtgtaa

SEQ ID NO: 42 - RNA, 1653 nt, synthetic construct
  source 1..1653: mol_type = other RNA
  misc_feature 1..1653: note = nucleotide sequence coding luciferase
atggaagacgccaaaaacataaagaaaggcccggcgccattctatccgctggaagatggaaccgctggagagcaactgcataaggctatgaagagatacgccctggttcctggaacaattgcttttacagatgcacatatcgaggtggacatcacttacgctgagtacttcgaaatgtccgttcggttggcagaagctatgaaacgatatgggctgaatacaaatcacagaatcgtcgtatgcagtgaaaactctcttcaattctttatgccggtgttgggcgcgttatttatcggagttgcagttgcgcccgcgaacgacatttataatgaacgtgaattgctcaacagtatgggcatttcgcagcctaccgtggtgttcgtttccaaaaaggggttgcaaaaaattttgaacgtgcaaaaaaagctcccaatcatccaaaaaattattatcatggattctaaaacggattaccagggatttcagtcgatgtacacgttcgtcacatctcatctacctcccggttttaatgaatacgattttgtgccagagtccttcgatagggacaagacaattgcactgatcatgaactcctctggatctactggtctgcctaaaggtgtcgctctgcctcatagaactgcctgcgtgagattctcgcatgccagagatcctatttttggcaatcaaatcattccggatactgcgattttaagtgttgttccattccatcacggttttggaatgtttactacactcggatatttgatatgtggatttcgagtcgtcttaatgtatagatttgaagaagagctgtttctgaggagccttcaggattacaagattcaaagtgcgctgctggtgccaaccctattctccttcttcgccaaaagcactctgattgacaaatacgatttatctaatttacacgaaattgcttctggtggcgctcccctctctaaggaagtcggggaagcggttgccaagaggttccatctgccaggtatcaggcaaggatatgggctcactgagactacatcagctattctgattacacccgagggggatgataaaccgggcgcggtcggtaaagttgttccattttttgaagcgaaggttgtggatctggataccgggaaaacgctgggcgttaatcaaagaggcgaactgtgtgtgagaggtcctatgattatgtccggttatgtaaacaatccggaagcgaccaacgccttgattgacaaggatggatggctacattctggagacatagcttactgggacgaagacgaacacttcttcatcgttgaccgcctgaagtctctgattaagtacaaaggctatcaggtggctcccgctgaattggaatccatcttgctccaacaccccaacatcttcgacgcaggtgtcgcaggtcttcccgacgatgacgccggtgaacttcccgccgccgttgttgttttggagcacggaaagacgatgacggaaaaagagatcgtggattacgtcgccagtcaagtaacaaccgcgaaaaagttgcgcggaggagttgtgtttgtggacgaagtaccgaaaggtcttaccggaaaactcgacgcaagaaaaatcagagagatcctcataaaggccaagaagggcggaaagatcgccgtgtaa

SEQ ID NO: 43 - DNA, 3200 bp, synthetic construct
  source 1..3200: mol_type = other DNA
  misc_feature 1..3200: note = nucleotide sequence coding SFTS B antigen
atgatgaaggttatctggttctccagcctgatctgtctggtgatccagtgtagcggcgacaccggacctatcatttgtgccggccctatccactccaacaagtccgccgacatcccccacctcctgggatactctgaaaaaatctgccaaatcgatagactgatccacgtgtccagctggctgcgaaaccacagccagttccagggctatgtgggccaaagaggaggcagaagccaggtgagctactaccccgccgagaatagctacagcagatggtccggcctgctgagcccttgcgacgccgattggctgggaatgctggtggtgaagaaggccaagggcagcgacatgatcgtgcccggccctagctacaagggcaaggtctttttcgaacggcccacctttgatggctacgtgggctggggatgcggctctggcaaaagccggacagaatctggagagctgtgcagcagcgacagcggcaccagctctggcctgctgccttcggatagagtgctgtggatcggcgatgtcgcatgccagcctatgacccctatccctgaggagacattcctggagctgaaatctttcagtcaaagcgagttccccgacatctgtaagatcgacggcatcgtgtttaaccagtgtgaaggcgaatccctgcctcagccgttcgacgtggcctggatggacgtcggccacagccacaagatcatcatgagagagcacaaaaccaagtgggtccaggagtctagcagcaaagacttcgtgtgctataaggaaggaacaggcccttgctccgagagcgaggaaaagacatgcaagaccagcgggtcttgcagaggagacatgcagttttgtaaagtggccggatgcgagcacggcgaggaggccagcgaggctaagtgccgctgtagcctcgttcacaagccaggagaggtggttgtgtcctacggcggcatgcgggtgagacccaagtgctacggcttcagcagaatgatggccacactggaggtgaatccacctgaacagcggatcggccagtgcaccggctgccacctggaatgcatcaacggcggcgtgagactgataacactgactagcgaactgaagagcgccacagtgtgcgccagccacttctgctcaagcgccaccagcggcaagaaatctactgagatccagttccactccggcagcctggtcggcaagaccgccatccacgtgaagggcgctctggtggatggcacagagttcacgttcgagggctcatgcatgttccctgatggctgcgacgccgtggactgcaccttctgccgggagttcctgaaaaacccccagtgttatcctgctaaaaagtggctgttcatcatcatcgtgatcctgctcggatacgccggcctgatgctgctgaccaacgtgctgaaggccatcggcgtgtggggcagctgggtgatcgcccccgtgaagctgatgttcgccatcatcaagaaactcatgagaaccgtgtcctgcctgatgggcaagctgatggaccggggcagacaggtgatccatgaggaaattggcgagaacagagagggcaaccaggacgacgtaagaatcgagatggccagacccagacgggtgcggcactggatgtacagccctgtgattttgaccatcctggctatcggactggctgaaggctgcgacgagatggtgcatgctgattctaaactggtatcttgtagacagggcagcggaaacatgaaagaatgcgtgaccaccggtcgggccctcctgcccgctgtgaatcccggccaggaggcctgcctgcacttcaccgcccctggcagccccgatagcaagtgcctgaagattaaggtgaagcggatcaacctgaagtgcaagaaatctagcagctacttcgtgcctgacgctagatccagatgcacctctgttaggagatgtagatgggccggagactgccagagcggctgccctcctcatttcacaagcaacagcttcagcgatgattgggccggaaaaatggacagagccggcctcggattctccgggtgcagcgatggatgcggaggcgccgcctgcggctgcttcaacgccgctcctagctgtatcttctggcggaagtgggtggaaaaccctcacggcatcatctggaaggttagcccatgcgccgcctgggtgccctctgccgtaatcgagctgaccatgccttctggtgaagtgcggacttttcaccccatgtcgggcatccctacccaggtgttcaagggcgtgagcgtgacctacctgggcagcgacatggaagtgagcggcctgacagacctgtgtgaaattgaagagctgaagtctaaaaagctggccctggcgccctgtaaccaagccggcatgggagtggtgggaaaggtcggcgagatccagtgcagctccgaggagagcgccagaacaatcaagaaggacggctgtatctggaacgccgatctggtgggcatcgagcttagagtggacgacgccgtgtgctacagcaagatcacctccgtggaagccgttgctaattacagcgccatccctaccacaatcggcggcctgcggttcgagcggtctcacgacagccaaggcaaaatcagcggcagccctctggacattaccgccatcagaggctcttttagcgtgaactacagaggcctgagattgtctctgtctgagatcaccgcaacctgtacaggcgaggtgacaaacgtgtccggctgctacagctgtatgaccggcgctaaggtgtctatcaagctgcactccagcaagaacagcacagcccacgtgcggtgcaagggcgacgaaaccgccttcagtgtgctggaaggcgtgcacagctacaccgtgagcctgagcttcgaccacgccgtcgtggacgagcagtgccagctgaactgcggcggtcacgagagccaggtgaccctgaagggaaacctgatcttcctggacgtgccaaagttcgtggacggcagctacatgcagacctaccacagcaccgtgcctaccggagccaacatcccatctcctacagattggctgaacgccctgttcggcaatggcctgtccagatggattctgggagtgatcggcgtgctgctgggcggcctggccctgttcttcctgatcatgtccctgtttaagctgggcacaaagcaggtctttag

SEQ ID NO: 44 - RNA, 3200 nt, synthetic construct
  source 1..3200: mol_type = other RNA
  misc_feature 1..3200: note = nucleotide sequence coding SFTS B antigen
atgatgaaggttatctggttctccagcctgatctgtctggtgatccagtgtagcggcgacaccggacctatcatttgtgccggccctatccactccaacaagtccgccgacatcccccacctcctgggatactctgaaaaaatctgccaaatcgatagactgatccacgtgtccagctggctgcgaaaccacagccagttccagggctatgtgggccaaagaggaggcagaagccaggtgagctactaccccgccgagaatagctacagcagatggtccggcctgctgagcccttgcgacgccgattggctgggaatgctggtggtgaagaaggccaagggcagcgacatgatcgtgcccggccctagctacaagggcaaggtctttttcgaacggcccacctttgatggctacgtgggctggggatgcggctctggcaaaagccggacagaatctggagagctgtgcagcagcgacagcggcaccagctctggcctgctgccttcggatagagtgctgtggatcggcgatgtcgcatgccagcctatgacccctatccctgaggagacattcctggagctgaaatctttcagtcaaagcgagttccccgacatctgtaagatcgacggcatcgtgtttaaccagtgtgaaggcgaatccctgcctcagccgttcgacgtggcctggatggacgtcggccacagccacaagatcatcatgagagagcacaaaaccaagtgggtccaggagtctagcagcaaagacttcgtgtgctataaggaaggaacaggcccttgctccgagagcgaggaaaagacatgcaagaccagcgggtcttgcagaggagacatgcagttttgtaaagtggccggatgcgagcacggcgaggaggccagcgaggctaagtgccgctgtagcctcgttcacaagccaggagaggtggttgtgtcctacggcggcatgcgggtgagacccaagtgctacggcttcagcagaatgatggccacactggaggtgaatccacctgaacagcggatcggccagtgcaccggctgccacctggaatgcatcaacggcggcgtgagactgataacactgactagcgaactgaagagcgccacagtgtgcgccagccacttctgctcaagcgccaccagcggcaagaaatctactgagatccagttccactccggcagcctggtcggcaagaccgccatccacgtgaagggcgctctggtggatggcacagagttcacgttcgagggctcatgcatgttccctgatggctgcgacgccgtggactgcaccttctgccgggagttcctgaaaaacccccagtgttatcctgctaaaaagtggctgttcatcatcatcgtgatcctgctcggatacgccggcctgatgctgctgaccaacgtgctgaaggccatcggcgtgtggggcagctgggtgatcgcccccgtgaagctgatgttcgccatcatcaagaaactcatgagaaccgtgtcctgcctgatgggcaagctgatggaccggggcagacaggtgatccatgaggaaattggcgagaacagagagggcaaccaggacgacgtaagaatcgagatggccagacccagacgggtgcggcactggatgtacagccctgtgattttgaccatcctggctatcggactggctgaaggctgcgacgagatggtgcatgctgattctaaactggtatcttgtagacagggcagcggaaacatgaaagaatgcgtgaccaccggtcgggccctcctgcccgctgtgaatcccggccaggaggcctgcctgcacttcaccgcccctggcagccccgatagcaagtgcctgaagattaaggtgaagcggatcaacctgaagtgcaagaaatctagcagctacttcgtgcctgacgctagatccagatgcacctctgttaggagatgtagatgggccggagactgccagagcggctgccctcctcatttcacaagcaacagcttcagcgatgattgggccggaaaaatggacagagccggcctcggattctccgggtgcagcgatggatgcggaggcgccgcctgcggctgcttcaacgccgctcctagctgtatcttctggcggaagtgggtggaaaaccctcacggcatcatctggaaggttagcccatgcgccgcctgggtgccctctgccgtaatcgagctgaccatgccttctggtgaagtgcggacttttcaccccatgtcgggcatccctacccaggtgttcaagggcgtgagcgtgacctacctgggcagcgacatggaagtgagcggcctgacagacctgtgtgaaattgaagagctgaagtctaaaaagctggccctggcgccctgtaaccaagccggcatgggagtggtgggaaaggtcggcgagatccagtgcagctccgaggagagcgccagaacaatcaagaaggacggctgtatctggaacgccgatctggtgggcatcgagcttagagtggacgacgccgtgtgctacagcaagatcacctccgtggaagccgttgctaattacagcgccatccctaccacaatcggcggcctgcggttcgagcggtctcacgacagccaaggcaaaatcagcggcagccctctggacattaccgccatcagaggctcttttagcgtgaactacagaggcctgagattgtctctgtctgagatcaccgcaacctgtacaggcgaggtgacaaacgtgtccggctgctacagctgtatgaccggcgctaaggtgtctatcaagctgcactccagcaagaacagcacagcccacgtgcggtgcaagggcgacgaaaccgccttcagtgtgctggaaggcgtgcacagctacaccgtgagcctgagcttcgaccacgccgtcgtggacgagcagtgccagctgaactgcggcggtcacgagagccaggtgaccctgaagggaaacctgatcttcctggacgtgccaaagttcgtggacggcagctacatgcagacctaccacagcaccgtgcctaccggagccaacatcccatctcctacagattggctgaacgccctgttcggcaatggcctgtccagatggattctgggagtgatcggcgtgctgctgggcggcctggccctgttcttcctgatcatgtccctgtttaagctgggcacaaagcaggtctttag

SEQ ID NO: 45 - protein, 1073 aa, synthetic construct
  REGION 1..1073: note = SFTS B antigen
MMKVIWFSSLICLVIQCSGDTGPIICAGPIHSNKSANIPHLLGYSEKICQIDRLIHVSSWLRNHSQFQGYVGQRGGRSQVSYYPAENSYSRWSGLLSPCDADWLGMLVVKKAKGSDMIVPGPSYKGKVFFERPTFDGYVGWGCGSGKSRTESGELCSSDSGTSSGLLPSDRVLWIGDVACQPMTPIPEETFLELKSFSQSEFPDICKIDGIVFNQCESESLPQPFDVAWMDVGHSHKIIMREHKTKWVQESSSKDFVCYKEGTGPCSESEEKTCKTSGSCRGDMQFCKVAGCEHGEEASEAKCRCSLVHKPGEVVVSYGGMRVRPKCYGFSRMMATLEVNPPEQRIGQCTGCHLECINGGVRLITLTSELKSATVCASHFCSSATSGKKSTEIQFHSGSLVGKTAIHVKGALVDGTEFTFEGSCMFPDGCDAVDCTFCREFLKNPQCYPAKKWLFIIIVILLGYAGLMLLTNVLKAIGVWGSWVIAPVKLMFAIIKKLMRSVSCLMGKLMDRGRQVIHEEIGENREGNQDDVRIEMARPRRVRHWMYSPVILTILAIGLAEGCDEMVHADSKLVSCKQGSGNMKECVTTGRALLPAVNPGQEACLHFTAPGSPDSKCLKIKVKRINLKCKKSSSYFVPDARSRCTSVRRCRWAGDCQSGCPSHFTSNSFSDDWAGKMDRAGLGFSGCSDGCGGAACGCFNAAPSCIFWRKWVENPHGIIWKVSPCAAWVPSAVIELTMPSGEVRTFHPMSGIPTQVFKGVSVTYLGSDMEVSGLTDLCEIEELKSKKLALAPCNQAGMGVVGKVGEIQCSSEESARTIKKDGCIWNADLVGIELRVDDAVCYSKITSVEAVANYSAIPTTIGGLRFERSHDSQGKISGSPLDITAIRGSFSVNYRGLRLSLSEITATCTGEVTNVSGCYSCMTGAKVSIKLHSSKNSTAHVRCKGDETAFSVLEGVHSYTVSLSFDHAVVDEQCQLNCGGHESQVTLKGNLIFLDVPKFVDGSYMQTYHSSVPTGANIPSPTDWLNALFGNGLSRWILGVIGVLLGGLALFFLIMSLFKLGTKQVFRSRTKLA

SEQ ID NO: 46 - DNA, 3849 bp, synthetic construct
  source 1..3849: mol_type = other DNA
  misc_feature 1..3849: note = nucleotide sequence coding SARS antigen
atgtttgtgttcctggtgctgctgccactggtgtccagccagtgtgtgaacctgaccaccaggacccaacttcctcctgcctacaccaactccttcaccaggggagtctactaccctgacaaggtgttcaggtcctctgtgctgcacagcacccaggacctgttcctgccattcttcagcaatgtgacctggttccatgccatccatgtgtctggcaccaatggcaccaagaggtttgacaaccctgtgctgccattcaatgatggagtctactttgccagcacagagaagagcaacatcatcaggggctggatttttggcaccaccctggacagcaagacccagtccctgctgattgtgaacaatgccaccaatgtggtgattaaggtgtgtgagttccagttctgtaatgacccattcctgggagtctactaccacaagaacaacaagtcctggatggagtctgagttcagggtctactcctctgccaacaactgtacctttgaatatgtgagccaaccattcctgatggacttggagggcaagcagggcaacttcaagaacctgagggagtttgtgttcaagaacattgatggctacttcaagatttacagcaaacacacaccaatcaacctggtgagggacctgccacagggcttctctgccttggaaccactggtggacctgccaattggcatcaacatcaccaggttccagaccctgctggctctgcacaggtcctacctgacacctggagactcctcctctggctggacagcaggagcagcagcctactatgtgggctacctccaaccaaggaccttcctgctgaaatacaatgagaatggcaccatcacagatgctgtggactgtgccctggacccactgtctgagaccaagtgtaccctgaaatccttcacagtggagaagggcatctaccagaccagcaacttcagggtccaaccaacagagagcattgtgaggtttccaaacatcaccaacctgtgtccatttggagaggtgttcaatgccaccaggtttgcctctgtctatgcctggaacaggaagaggattagcaactgtgtggctgactactctgtgctctacaactctgcctccttcagcaccttcaagtgttatggagtgagcccaaccaaactgaatgacctgtgtttcaccaatgtctatgctgactcctttgtgattaggggagatgaggtgagacagattgcccctggacaaacaggcaagattgctgactacaactacaaactgcctgatgacttcacaggctgtgtgattgcctggaacagcaacaacctggacagcaaggtgggaggcaactacaactacctctacagactgttcaggaagagcaacctgaaaccatttgagagggacatcagcacagagatttaccaggctggcagcacaccatgtaatggagtggagggcttcaactgttactttccactccaatcctatggcttccaaccaaccaatggagtgggctaccaaccatacagggtggtggtgctgtcctttgaactgctccatgcccctgccacagtgtgtggaccaaagaagagcaccaacctggtgaagaacaagtgtgtgaacttcaacttcaatggactgacaggcacaggagtgctgacagagagcaacaagaagttcctgccattccaacagtttggcagggacattgctgacaccacagatgctgtgagggacccacagaccttggagattctggacatcacaccatgttcctttggaggagtgtctgtgattacacctggcaccaacaccagcaaccaggtggctgtgctctaccaggatgtgaactgtactgaggtgcctgtggctatccatgctgaccaacttacaccaacctggagggtctacagcacaggcagcaatgtgttccagaccagggctggctgtctgattggagcagagcatgtgaacaactcctatgagtgtgacatcccaattggagcaggcatctgtgcctcctaccagacccagaccaacagcccaaggagggcaaggtctgtggcaagccagagcatcattgcctacacaatgagtctgggagcagagaactctgtggcttacagcaacaacagcattgccatcccaaccaacttcaccatctctgtgaccacagagattctgcctgtgagtatgaccaagacctctgtggactgtacaatgtatatctgtggagacagcacagagtgtagcaacctgctgctccaatatggctccttctgtacccaacttaacagggctctgacaggcattgctgtggaacaggacaagaacacccaggaggtgtttgcccaggtgaagcagatttacaagacacctccaatcaaggactttggaggcttcaacttcagccagattctgcctgacccaagcaagccaagcaagaggtccttcattgaggacctgctgttcaacaaggtgaccctggctgatgctggcttcatcaagcaatatggagactgtctgggagacattgctgccagggacctgatttgtgcccagaagttcaatggactgacagtgctgcctccactgctgacagatgagatgattgcccaatacacctctgccctgctggctggcaccatcacctctggctggacctttggagcaggagcagccctccaaatcccatttgctatgcagatggcttacaggttcaatggcattggagtgacccagaatgtgctctatgagaaccagaaactgattgccaaccagttcaactctgccattggcaagattcaggactccctgtccagcacagcctctgccctgggcaaactccaagatgtggtgaaccagaatgcccaggctctgaacaccctggtgaagcaactttccagcaactttggagccatctcctctgtgctgaatgacatcctgagcagactggacaaggtggaggctgaggtccagattgacagactgattacaggcagactccaatccctccaaacctatgtgacccaacaacttatcagggctgctgagattagggcatctgccaacctggctgccaccaagatgagtgagtgtgtgctgggacaaagcaagagggtggacttctgtggcaagggctaccacctgatgagttttccacagtctgcccctcatggagtggtgttcctgcatgtgacctatgtgcctgcccaggagaagaacttcaccacagcccctgccatctgccatgatggcaaggctcactttccaagggagggagtgtttgtgagcaatggcacccactggtttgtgacccagaggaacttctatgaaccacagattatcaccacagacaacacctttgtgtctggcaactgtgatgtggtgattggcattgtgaacaacacagtctatgacccactccaacctgaactggactccttcaaggaggaactggacaaatacttcaagaaccacaccagccctgatgtggacctgggagacatctctggcatcaatgcctctgtggtgaacatccagaaggagattgacagactgaatgaggtggctaagaacctgaatgagtccctgattgacctccaagaactgggcaaatatgaacaatacatcaagtggccatggtacatctggctgggcttcattgctggactgattgccattgtgatggtgaccataatgctgtgttgtatgacctcctgttgttcctgtctgaaaggctgttgttcctgtggctcctgttgtaagtttgatgaggatgactctgaacctgtgctgaaaggagtgaaactgcactacaccaactttgagccaacaggggtgacggagtcc

SEQ ID NO: 47 - RNA, 3849 nt, synthetic construct
  source 1..3849: mol_type = other RNA
  misc_feature 1..3849: note = nucleotide sequence coding SARS antigen
atgtttgtgttcctggtgctgctgccactggtgtccagccagtgtgtgaacctgaccaccaggacccaacttcctcctgcctacaccaactccttcaccaggggagtctactaccctgacaaggtgttcaggtcctctgtgctgcacagcacccaggacctgttcctgccattcttcagcaatgtgacctggttccatgccatccatgtgtctggcaccaatggcaccaagaggtttgacaaccctgtgctgccattcaatgatggagtctactttgccagcacagagaagagcaacatcatcaggggctggatttttggcaccaccctggacagcaagacccagtccctgctgattgtgaacaatgccaccaatgtggtgattaaggtgtgtgagttccagttctgtaatgacccattcctgggagtctactaccacaagaacaacaagtcctggatggagtctgagttcagggtctactcctctgccaacaactgtacctttgaatatgtgagccaaccattcctgatggacttggagggcaagcagggcaacttcaagaacctgagggagtttgtgttcaagaacattgatggctacttcaagatttacagcaaacacacaccaatcaacctggtgagggacctgccacagggcttctctgccttggaaccactggtggacctgccaattggcatcaacatcaccaggttccagaccctgctggctctgcacaggtcctacctgacacctggagactcctcctctggctggacagcaggagcagcagcctactatgtgggctacctccaaccaaggaccttcctgctgaaatacaatgagaatggcaccatcacagatgctgtggactgtgccctggacccactgtctgagaccaagtgtaccctgaaatccttcacagtggagaagggcatctaccagaccagcaacttcagggtccaaccaacagagagcattgtgaggtttccaaacatcaccaacctgtgtccatttggagaggtgttcaatgccaccaggtttgcctctgtctatgcctggaacaggaagaggattagcaactgtgtggctgactactctgtgctctacaactctgcctccttcagcaccttcaagtgttatggagtgagcccaaccaaactgaatgacctgtgtttcaccaatgtctatgctgactcctttgtgattaggggagatgaggtgagacagattgcccctggacaaacaggcaagattgctgactacaactacaaactgcctgatgacttcacaggctgtgtgattgcctggaacagcaacaacctggacagcaaggtgggaggcaactacaactacctctacagactgttcaggaagagcaacctgaaaccatttgagagggacatcagcacagagatttaccaggctggcagcacaccatgtaatggagtggagggcttcaactgttactttccactccaatcctatggcttccaaccaaccaatggagtgggctaccaaccatacagggtggtggtgctgtcctttgaactgctccatgcccctgccacagtgtgtggaccaaagaagagcaccaacctggtgaagaacaagtgtgtgaacttcaacttcaatggactgacaggcacaggagtgctgacagagagcaacaagaagttcctgccattccaacagtttggcagggacattgctgacaccacagatgctgtgagggacccacagaccttggagattctggacatcacaccatgttcctttggaggagtgtctgtgattacacctggcaccaacaccagcaaccaggtggctgtgctctaccaggatgtgaactgtactgaggtgcctgtggctatccatgctgaccaacttacaccaacctggagggtctacagcacaggcagcaatgtgttccagaccagggctggctgtctgattggagcagagcatgtgaacaactcctatgagtgtgacatcccaattggagcaggcatctgtgcctcctaccagacccagaccaacagcccaaggagggcaaggtctgtggcaagccagagcatcattgcctacacaatgagtctgggagcagagaactctgtggcttacagcaacaacagcattgccatcccaaccaacttcaccatctctgtgaccacagagattctgcctgtgagtatgaccaagacctctgtggactgtacaatgtatatctgtggagacagcacagagtgtagcaacctgctgctccaatatggctccttctgtacccaacttaacagggctctgacaggcattgctgtggaacaggacaagaacacccaggaggtgtttgcccaggtgaagcagatttacaagacacctccaatcaaggactttggaggcttcaacttcagccagattctgcctgacccaagcaagccaagcaagaggtccttcattgaggacctgctgttcaacaaggtgaccctggctgatgctggcttcatcaagcaatatggagactgtctgggagacattgctgccagggacctgatttgtgcccagaagttcaatggactgacagtgctgcctccactgctgacagatgagatgattgcccaatacacctctgccctgctggctggcaccatcacctctggctggacctttggagcaggagcagccctccaaatcccatttgctatgcagatggcttacaggttcaatggcattggagtgacccagaatgtgctctatgagaaccagaaactgattgccaaccagttcaactctgccattggcaagattcaggactccctgtccagcacagcctctgccctgggcaaactccaagatgtggtgaaccagaatgcccaggctctgaacaccctggtgaagcaactttccagcaactttggagccatctcctctgtgctgaatgacatcctgagcagactggacaaggtggaggctgaggtccagattgacagactgattacaggcagactccaatccctccaaacctatgtgacccaacaacttatcagggctgctgagattagggcatctgccaacctggctgccaccaagatgagtgagtgtgtgctgggacaaagcaagagggtggacttctgtggcaagggctaccacctgatgagttttccacagtctgcccctcatggagtggtgttcctgcatgtgacctatgtgcctgcccaggagaagaacttcaccacagcccctgccatctgccatgatggcaaggctcactttccaagggagggagtgtttgtgagcaatggcacccactggtttgtgacccagaggaacttctatgaaccacagattatcaccacagacaacacctttgtgtctggcaactgtgatgtggtgattggcattgtgaacaacacagtctatgacccactccaacctgaactggactccttcaaggaggaactggacaaatacttcaagaaccacaccagccctgatgtggacctgggagacatctctggcatcaatgcctctgtggtgaacatccagaaggagattgacagactgaatgaggtggctaagaacctgaatgagtccctgattgacctccaagaactgggcaaatatgaacaatacatcaagtggccatggtacatctggctgggcttcattgctggactgattgccattgtgatggtgaccataatgctgtgttgtatgacctcctgttgttcctgtctgaaaggctgttgttcctgtggctcctgttgtaagtttgatgaggatgactctgaacctgtgctgaaaggagtgaaactgcactacaccaactttgagccaacaggggtgacggagtcc

SEQ ID NO: 48 - protein, 1283 aa, synthetic construct
  REGION 1..1283: note = SARS antigen
MFVFLVLLPLVSSQCVNLTTRTQLPPAYTNSFTRGVYYPDKVFRSSVLHSTQDLFLPFFSNVTWFHAIHVSGTNGTKRFDNPVLPFNDGVYFASTEKSNIIRGWIFGTTLDSKTQSLLIVNNATNVVIKVCEFQFCNDPFLGVYYHKNNKSWMESEFRVYSSANNCTFEYVSQPFLMDLEGKQGNFKNLREFVFKNIDGYFKIYSKHTPINLVRDLPQGFSALEPLVDLPIGINITRFQTLLALHRSYLTPGDSSSGWTAGAAAYYVGYLQPRTFLLKYNENGTITDAVDCALDPLSETKCTLKSFTVEKGIYQTSNFRVQPTESIVRFPNITNLCPFGEVFNATRFASVYAWNRKRISNCVADYSVLYNSASFSTFKCYGVSPTKLNDLCFTNVYADSFVIRGDEVRQIAPGQTGKIADYNYKLPDDFTGCVIAWNSNNLDSKVGGNYNYLYRLFRKSNLKPFERDISTEIYQAGSTPCNGVEGFNCYFPLQSYGFQPTNGVGYQPYRVVVLSFELLHAPATVCGPKKSTNLVKNKCVNFNFNGLTGTGVLTESNKKFLPFQQFGRDIADTTDAVRDPQTLEILDITPCSFGGVSVITPGTNTSNQVAVLYQDVNCTEVPVAIHADQLTPTWRVYSTGSNVFQTRAGCLIGAEHVNNSYECDIPIGAGICASYQTQTNSPRRARSVASQSIIAYTMSLGAENSVAYSNNSIAIPTNFTISVTTEILPVSMTKTSVDCTMYICGDSTECSNLLLQYGSFCTQLNRALTGIAVEQDKNTQEVFAQVKQIYKTPPIKDFGGFNFSQILPDPSKPSKRSFIEDLLFNKVTLADAGFIKQYGDCLGDIAARDLICAQKFNGLTVLPPLLTDEMIAQYTSALLAGTITSGWTFGAGAALQIPFAMQMAYRFNGIGVTQNVLYENQKLIANQFNSAIGKIQDSLSSTASALGKLQDVVNQNAQALNTLVKQLSSNFGAISSVLNDILSRLDKVEAEVQIDRLITGRLQSLQTYVTQQLIRAAEIRASANLAATKMSECVLGQSKRVDFCGKGYHLMSFPQSAPHGVVFLHVTYVPAQEKNFTTAPAICHDGKAHFPREGVFVSNGTHWFVTQRNFYEPQIITTDNTFVSGNCDVVIGIVNNTVYDPLQPELDSFKEELDKYFKNHTSPDVDLGDISGINASVVNIQKEIDRLNEVAKNLNESLIDLQELGKYEQYIKWPWYIWLGFIAGLIAIVMVTIMLCCMTSCCSCLKGCCSCGSCCKFDEDDSEPVLKGVKLHYTNFEPTGVTES

SEQ ID NO: 49 - DNA, 36 bp, synthetic construct
  source 1..36: mol_type = other DNA
  misc_feature 1..36: note = nucleotide sequence coding 3C protease recognition sequence
ctcgaggctttgttccaaggaccaccagtatacagg

SEQ ID NO: 50 - protein, 12 aa, synthetic construct
  REGION 1..12: note = 3C protease recognition sequence
LEALFQGPPVYR

SEQ ID NO: 51 - DNA, 1698 bp, synthetic construct
  source 1..1698: mol_type = other DNA
  misc_feature 1..1698: note = nucleotide sequence coding H3N2 antigen
atgaaaaccgtgatcgccctcagttacatcttctgcctcgcctttggacagaatctcctcggaaacgaaaacaacgctgccacactctgcctgggacaccacgccgtgcccaacggcacaatggtgaagaccatcaccgacgatcagatcgaggtgaccaatgccaccgagctggtgcagaacagctccaccggcaaaatctgcaacaatccccacaagatcctggacggcagggattgcaccctgatcgacgctctgctgggcgaccctcactgcgacgtgttccagaatgagacatgggatctgttcgtggagaggagcaatgccttctccaactgctacccctacgacgtgcctgattacgccagcctgcggtccatcgtggccagctccggcaccctggagttcatcaccgagggcttcacctgggctggagtgacccagaacggaggcagcggagcttgcaagaggggacccgccaatagcttcttctcccggctgaactggctgaccaagtccggcaatacctaccccgtgctgaacgtgaccatgcctaacaataacaatttcgacaagctgtacatctggggcgtgcaccaccctagcaccgatcaggagcagaccagcctgtacatccaggcctccggcagggtgaccgtgagcaccaggcggtcccagcagaccatcatccccaacatcggctccaggcctctggtgcggggacagagcggccggatctccgtgtactggaccatcgtgaagcccggcgacatcctggtcatcaacagcaatggcaacctgatcgcccctcgcggctacttcaagatgcacatcggcaagagcagcatcatgagatccgacgcccccatcgatacctgcatcagcgagtgcatcacccctaatggctccatccccaacgagaagcctttccagaatgtgaacaagatcacctacggcgcctgccccaagtacgtgaagcagaataccctgaagctggccaccggcatgcgcaacgtgcctgagagacagaccgtgggcctgttcggagctatcgctggcttcatcgagaatggctgggagggcatggtggacggctggtacggcttccgccaccagaacagcgagggcaccggacaggctgccgacctgaagtccacccaggccgccatcgatcagatcaatggcaagctgaacagagtgatcgagaagaccaacgagaagttccaccagatcgagaaggagttcagcgaggtggagggacgcatccaggacctggagaggtacgtggaggacaccaagatcgatctgtggagctacaatgccgagctgctggtggccctggagaatcagaacaccatcgacctgaccgattccgagatgaacaagctgttcgagaagacccgcagacagctgcgcgagaatgccgaggacatgggcaacggctgcttcaaaatctaccacaagtgcgataacgcctgcatcgagagcatcagaaatggcacctacgaccacaacatctaccgcgatgaggccgtgaacaatagattccagatcaagggcgtggagctgaagtccggctacaaggactggattctgtggatcagcttcgccatctcctgcttcctgctgtgcgtggtgctgctggggtttattatgtgggcttgtcagagggggaacatcaggtgtaacatttgtatt

SEQ ID NO: 52 - RNA, 1698 nt, synthetic construct
  source 1..1698: mol_type = other RNA
  misc_feature 1..1698: note = nucleotide sequence coding H3N2 antigen
atgaaaaccgtgatcgccctcagttacatcttctgcctcgcctttggacagaatctcctcggaaacgaaaacaacgctgccacactctgcctgggacaccacgccgtgcccaacggcacaatggtgaagaccatcaccgacgatcagatcgaggtgaccaatgccaccgagctggtgcagaacagctccaccggcaaaatctgcaacaatccccacaagatcctggacggcagggattgcaccctgatcgacgctctgctgggcgaccctcactgcgacgtgttccagaatgagacatgggatctgttcgtggagaggagcaatgccttctccaactgctacccctacgacgtgcctgattacgccagcctgcggtccatcgtggccagctccggcaccctggagttcatcaccgagggcttcacctgggctggagtgacccagaacggaggcagcggagcttgcaagaggggacccgccaatagcttcttctcccggctgaactggctgaccaagtccggcaatacctaccccgtgctgaacgtgaccatgcctaacaataacaatttcgacaagctgtacatctggggcgtgcaccaccctagcaccgatcaggagcagaccagcctgtacatccaggcctccggcagggtgaccgtgagcaccaggcggtcccagcagaccatcatccccaacatcggctccaggcctctggtgcggggacagagcggccggatctccgtgtactggaccatcgtgaagcccggcgacatcctggtcatcaacagcaatggcaacctgatcgcccctcgcggctacttcaagatgcacatcggcaagagcagcatcatgagatccgacgcccccatcgatacctgcatcagcgagtgcatcacccctaatggctccatccccaacgagaagcctttccagaatgtgaacaagatcacctacggcgcctgccccaagtacgtgaagcagaataccctgaagctggccaccggcatgcgcaacgtgcctgagagacagaccgtgggcctgttcggagctatcgctggcttcatcgagaatggctgggagggcatggtggacggctggtacggcttccgccaccagaacagcgagggcaccggacaggctgccgacctgaagtccacccaggccgccatcgatcagatcaatggcaagctgaacagagtgatcgagaagaccaacgagaagttccaccagatcgagaaggagttcagcgaggtggagggacgcatccaggacctggagaggtacgtggaggacaccaagatcgatctgtggagctacaatgccgagctgctggtggccctggagaatcagaacaccatcgacctgaccgattccgagatgaacaagctgttcgagaagacccgcagacagctgcgcgagaatgccgaggacatgggcaacggctgcttcaaaatctaccacaagtgcgataacgcctgcatcgagagcatcagaaatggcacctacgaccacaacatctaccgcgatgaggccgtgaacaatagattccagatcaagggcgtggagctgaagtccggctacaaggactggattctgtggatcagcttcgccatctcctgcttcctgctgtgcgtggtgctgctggggtttattatgtgggcttgtcagagggggaacatcaggtgtaacatttgtatt

SEQ ID NO: 53 - protein, 192 aa, synthetic construct
  REGION 1..192: note = H3N2 antigen
EGTGQAADLKSTQAAIDQINGKLNRVIEKTNEKFHQIEKEFSEVEGRIQDLERYVEDTKIDLWSYNAELLVALENQNTIDLTDSEMNKLFEKTRRQLRENAEDMGNGCFKIYHKCDNACIESIRNGTYDHNIYRDEAVNNRFQIKGVELKSGYKDWILWISFAISCFLLCVVLLGFIMWACQRGNIRCNICI

SEQ ID NO: 54 - DNA, 1695 bp, synthetic construct
  source 1..1695: mol_type = other DNA
  misc_feature 1..1695: note = nucleotide sequence coding H3N8 antigen
atgaaaacaaccattattttaatactactgacccattgggcctacagtcaaaacccaatcagtggcaataacacagccacactgtgtctgggacaccatgcagtagcaaatggaacattggtaaagacaatgagtgatgatcaaattgaggtgacaaatgctacagaattagttcagagcatttcaatggggaaaatatgcaacaaatcatatagagttctagatggaagaaattgcacattaatagatgcaatgctaggagacccccagtgtgacgcctttcagtatgagagttgggacctctttatagaaagaagcaacgctttcagcaattgctacccatatgacatccctgactatgcatcgctccgatccattgtagcatcctcaggaacagtggaattcacagcagagggattcacatggacaggtgtcactcaaaacggaagaagtggagcctgcaaaaggggatcagccgatagtttctttagccgactgaattggctaacaaaatctggaagctcttaccccacattgaatgtaacaatgcctaacaataaaaatttcgacaagctatacatctgggggattcatcacccgagctcgaatcaagagcagacaaaattgtacattcaagaatcaggacgagtaacagtctcaacaaaaagaagtcaacaaacaataatccctcacatcggatctagaccgttgatcagaggtcaatcaggcaggataagcatatactggaccattgtaaaacctggagatatcctaatgataaacagtaatggcaacttagttgcaccgcggggatatttcaaattgaacccaggaaaaagctctgtaattagatccgatgtacccatagacatttgtgtgtctgaatgtattacaccaaatggaagcatctccaacgacaagccattccaaaatgtgaacaaagttacatatggaaaatgccccaagtatatcaggcaaaacactttaaagttggccactgggatgaggaatgtgccagaaaagcaaaccagaggaatctttggggcgatagcgggattcatcgaaaacggctgggaaggaatggttgatgggtggtatgggttccgatatcaaaactctgaaggaacagggcaagctgcagatctaaagagcactcaagcagccatcgaccagattaatggaaagttaaacagggtgattgaaagaaccaatgagaaattccatcaaatagagaaggaattctcagaagtagaaggaagaattcaggacttggagaaatatgtagaagacaccaaaatagacctatggtcctacaatgcagaactactggtggctctagaaaatcaacatacaattgacttaacagatgcagaaatgaataaattatttgagaagactagacgccagttaagagaaaatgcagaagacatgggaaatggatgtttcaagatttaccacaagtgtgataatgcatgcattgagtcaataagaactggaacatatgaccattacatatacagagatgaagcaataaacaaccgatttcagatcaaaggtgtagaattgaaatcaggctacaaagattggatactgtggatttcattcgccatatcatgcttcttaatttgcgttgttctattgggtttcattatgtgggcttgccaaaaaggcaacatcagatgcaacatttgcatt

SEQ ID NO: 55 - RNA, 1695 nt, synthetic construct
  source 1..1695: mol_type = other RNA
  misc_feature 1..1695: note = nucleotide sequence coding H3N8 antigen
atgaaaacaaccattattttaatactactgacccattgggcctacagtcaaaacccaatcagtggcaataacacagccacactgtgtctgggacaccatgcagtagcaaatggaacattggtaaagacaatgagtgatgatcaaattgaggtgacaaatgctacagaattagttcagagcatttcaatggggaaaatatgcaacaaatcatatagagttctagatggaagaaattgcacattaatagatgcaatgctaggagacccccagtgtgacgcctttcagtatgagagttgggacctctttatagaaagaagcaacgctttcagcaattgctacccatatgacatccctgactatgcatcgctccgatccattgtagcatcctcaggaacagtggaattcacagcagagggattcacatggacaggtgtcactcaaaacggaagaagtggagcctgcaaaaggggatcagccgatagtttctttagccgactgaattggctaacaaaatctggaagctcttaccccacattgaatgtaacaatgcctaacaataaaaatttcgacaagctatacatctgggggattcatcacccgagctcgaatcaagagcagacaaaattgtacattcaagaatcaggacgagtaacagtctcaacaaaaagaagtcaacaaacaataatccctcacatcggatctagaccgttgatcagaggtcaatcaggcaggataagcatatactggaccattgtaaaacctggagatatcctaatgataaacagtaatggcaacttagttgcaccgcggggatatttcaaattgaacccaggaaaaagctctgtaattagatccgatgtacccatagacatttgtgtgtctgaatgtattacaccaaatggaagcatctccaacgacaagccattccaaaatgtgaacaaagttacatatggaaaatgccccaagtatatcaggcaaaacactttaaagttggccactgggatgaggaatgtgccagaaaagcaaaccagaggaatctttggggcgatagcgggattcatcgaaaacggctgggaaggaatggttgatgggtggtatgggttccgatatcaaaactctgaaggaacagggcaagctgcagatctaaagagcactcaagcagccatcgaccagattaatggaaagttaaacagggtgattgaaagaaccaatgagaaattccatcaaatagagaaggaattctcagaagtagaaggaagaattcaggacttggagaaatatgtagaagacaccaaaatagacctatggtcctacaatgcagaactactggtggctctagaaaatcaacatacaattgacttaacagatgcagaaatgaataaattatttgagaagactagacgccagttaagagaaaatgcagaagacatgggaaatggatgtttcaagatttaccacaagtgtgataatgcatgcattgagtcaataagaactggaacatatgaccattacatatacagagatgaagcaataaacaaccgatttcagatcaaaggtgtagaattgaaatcaggctacaaagattggatactgtggatttcattcgccatatcatgcttcttaatttgcgttgttctattgggtttcattatgtgggcttgccaaaaaggcaacatcagatgcaacatttgcatt

SEQ ID NO: 56 - protein, 565 aa, synthetic construct
  REGION 1..565: note = H3N8 antigen
MKTTIILILLTHWAYSQNPISGNNTATLCLGHHAVANGTLVKTMSDDQIEVTNATELVQSISMGKICNKSYRVLDGRNCTLIDAMLGDPQCDAFQYESWDLFIERSNAFSNCYPYDIPDYASLRSIVASSGTVEFTAEGFTWTGVTQNGRSGACKRGSADSFFSRLNWLTKSGSSYPTLNVTMPNNKNFDKLYIWGIHHPSSNQEQTKLYIQESGRVTVSTKRSQQTIIPHIGSRPLIRGQSGRISIYWTIVKPGDILMINSNGNLVAPRGYFKLNPGKSSVIRSDVPIDICVSECITPNGSISNDKPFQNVNKVTYGKCPKYIRQNTLKLATGMRNVPEKQTRGIFGAIAGFIENGWEGMVDGWYGFRYQNSEGTGQAADLKSTQAAIDQINGKLNRVIERTNEKFHQIEKEFSEVEGRIQDLEKYVEDTKIDLWSYNAELLVALENQHTIDLTDAEMNKLFEKTRRQLRENAEDMGNGCFKIYHKCDNACIESIRTGTYDHYIYRDEAINNRFQIKGVELKSGYKDWILWISFAISCFLICVVLLGFIMWACQKGNIRCNICI

SEQ ID NO: 57 - RNA, 36 nt, synthetic construct
  source 1..36: mol_type = other RNA
  misc_feature 1..36: note = nucleotide sequence coding 3C protease recognition sequence
ctcgaggctttgttccaaggaccaccagtatacagg

SEQ ID NO: 58 - DNA, 623 bp, synthetic construct
  source 1..623: mol_type = other DNA
  misc_feature 1..623: note = nucleotide sequence of IRES
ttaaaacagcctgtgggttgtacccacccacagggcccactgggcgctagcactctggtatcacggtacctttgtgtgcctgttttatatcccctttccccgattgtaacttagaagatgtacacactgatcaatagcgggcatagcacaccagctatgtcttgatcaagcactcctgtatccccggaccaagtatcaatagactgctcacgcggttgaaggagaaaacgttcgtcacccggctaactacttcgagaaacccagtagtatcatgaaagttgcgaggcgtttcgttcagcacacccccagtgtagatcgggtcgatgagtcaccgcatcccccacgggcgaccgtggcggtggctgcgctggcggcctgcctacggggcaacccgtaggacgcttcaatacagacatggtgcgaagagtcgattgagctagttagtagtcctccggcccctgaatgcggctaatcctaactgcggagcacatgccctcaacccagggggtattgtgtcgtaacgggcaactctgcagcggaaccgactactttgggtgtccgtgtttccttttatccttatactggctgcttatggtgacaattgaaagattgttgccatatag

SEQ ID NO: 59 - RNA, 623 nt, synthetic construct
  source 1..623: mol_type = other RNA
  misc_feature 1..623: note = nucleotide sequence of IRES
ttaaaacagcctgtgggttgtacccacccacagggcccactgggcgctagcactctggtatcacggtacctttgtgtgcctgttttatatcccctttccccgattgtaacttagaagatgtacacactgatcaatagcgggcatagcacaccagctatgtcttgatcaagcactcctgtatccccggaccaagtatcaatagactgctcacgcggttgaaggagaaaacgttcgtcacccggctaactacttcgagaaacccagtagtatcatgaaagttgcgaggcgtttcgttcagcacacccccagtgtagatcgggtcgatgagtcaccgcatcccccacgggcgaccgtggcggtggctgcgctggcggcctgcctacggggcaacccgtaggacgcttcaatacagacatggtgcgaagagtcgattgagctagttagtagtcctccggcccctgaatgcggctaatcctaactgcggagcacatgccctcaacccagggggtattgtgtcgtaacgggcaactctgcagcggaaccgactactttgggtgtccgtgtttccttttatccttatactggctgcttatggtgacaattgaaagattgttgccatatag

SEQ ID NO: 60 - RNA, 743 nt, synthetic construct
  source 1..743: mol_type = other RNA
  misc_feature 1..743: map = nucleotide sequence of 5' UTR
ttaaaacagcctgtgggttgtacccacccacagggcccactgggcgctagcactctggtatcacggtacctttgtgtgcctgttttatatcccctttccccgattgtaacttagaagatgtacacactgatcaatagcgggcatagcacaccagctatgtcttgatcaagcactcctgtatccccggaccaagtatcaatagactgctcacgcggttgaaggagaaaacgttcgtcacccggctaactacttcgagaaacccagtagtatcatgaaagttgcgaggcgtttcgttcagcacacccccagtgtagatcgggtcgatgagtcaccgcatcccccacgggcgaccgtggcggtggctgcgctggcggcctgcctacggggcaacccgtaggacgcttcaatacagacatggtgcgaagagtcgattgagctagttagtagtcctccggcccctgaatgcggctaatcctaactgcggagcacatgccctcaacccagggggtattgtgtcgtaacgggcaactctgcagcggaaccgactactttgggtgtccgtgtttccttttatccttatactggctgcttatggtgacaattgaaagattgttgccatatagctattggattggccatccagtgtctaatagagctgttatttacctctttgttggatttataccactcaacctaaaagaagttaaaacactacagctcattttacaactgaatacagcaaa

SEQ ID NO: 61 - RNA, 450 nt, synthetic construct
  source 1..450: mol_type = other RNA
  misc_feature 1..450: note = nucleotide sequence coding 2A protease
ggttcatgtgggcaacaatcaggagctgtgtacgtgggcaattacaggattgtaaacagacacctggcaacgagccacgattggcaaaattgcgtgtgggaggactacaacagggatctcctggtcagcacaacaactgctcatggttgtgatactatagcacggtgccaatgtactgctggcgtgtacttttgtgcatctagaaacaagcactacccagtgagcttcgagggtccaggtctagtgaaagttcaggagggcgagtactaccccgagagataccagtcgcacgtactccttgcagttggattttcagaaccgggtgattgtggaggtattttgaggtgtgaacatggagtcattgggctcgttaccatgggtggtgagggtgtagtaggcttcgctgacgtgcgggatcttttgtggttggaagacgacgccatggagcag

SEQ ID NO: 62 - RNA, 297 nt, synthetic construct
  source 1..297: mol_type = other RNA
  misc_feature 1..297: note = nucleotide sequence coding 2B
ggtgttagagattatgtagagcaactgggaaatgcatttggctcaggtttcactaaccaaatctgtgagcaagttaacctccttaaagaatctctgatagggcaggattccatattggaaaaatccctgaaggccctggttaaaatcatatcagccctggtgatagtggttaggaaccacgacgacctgattacagtgactgccacactagctttaatcggttgcgcatcatctccatggcgatggctcaaacaaaaagtgtgtcaatactacggaatccccatggcagaaaggcag

SEQ ID NO: 63 - RNA, 987 nt, synthetic construct
  source 1..987: mol_type = other RNA
  misc_feature 1..987: note = nucleotide sequence coding 2C
aataacggttggttaaagaaattcactgaaatgaccaacgcctgcaagggcatggagtggattgctgttaaaattcaaaagttcatcgagtggctcaaagtaaagattctgcctgaagtgaaggagaaacatgagttccttaccagattgaagcaattgccactccttgaaagtcaaattgccaccattgagcaaagcgcaccctcacaaagtgatcaagagcagcttttttcgaatgttcagtacttcgcccattactgcaggaagtatgcacctctgtatgctgccgaagcaaaaagagtgttctcattagaaaagaaaatgagtaattacatacagttcaagtccaaatgccgcattgagcctgtatgcttactccttcacggtagtccaggggctggcaagtcagtagctaccaacctgatagggagatcccttgcagagaagctcaatagctctgtgtactctttaccaccagatccagatcattttgatgggtacaaacagcaggcagtggtgatcatggatgatctctgtcaaaaccccgatgggaaggacgtgtccttgttttgccaaatggtgtctagtgtagattttgtgccacccatggcggcgctggaagaaaaaggcattctctttacgtccccgtttgtgttggcatcaaccaacgcggggtccatcaatgcaccaacagtgtcagacagcagagcacttgccagaaggtttcactttgacatgaatattgaggtgatttcgatgtacagccagaatggtaaaattaacatgcccatgtctgttaagacatgtgatgatgaatgctgcccggtcaatttcaaaaagtgttgcccactagtgtgtggcaaggccatccagtttattgacaggagaaaccaagttagatattcactggacatgctggttactgagatgtttagagagtacaaccacagacacagtgtgggtgctaccctcgaggctttgttccaa

SEQ ID NO: 64 - RNA, 267 nt, synthetic construct
  source 1..267: mol_type = other RNA
  misc_feature 1..267: note = nucleotide sequence coding 3A
ggaccaccagtatacagggaaatcaaaatcagtgtggccccggaaacaccccctccaccagcaattgctgaccttctaaaatctgtagacagtgaggcaataagggagtactgcaaggaaaggggttggcttgtgccagaggtcagctccactctacaaattgaaaaacatgttagcagggcatttatttgcttgcaagcgctaactacatttgtttcagtggctggtataatctacatcatttacaagttgtttgccggctttcag

SEQ ID NO: 65 - RNA, 66 nt, synthetic construct
  source 1..66: mol_type = other RNA
  misc_feature 1..66: note = nucleotide sequence coding 3B
ggtgcatacactggaatgcccaaccagaaacccaaggtgcccaccttaagacaagctaaggtgcaa

SEQ ID NO: 66 - RNA, 549 nt, synthetic construct
  source 1..549: mol_type = other RNA
  misc_feature 1..549: note = nucleotide sequence coding 3C
ggtccggcatttgaatttgccgtagcaatgatgaaaaggaacgccagcacagtcaagacagaatacggtgagttcacgatgcttggcatctatgataaatgggcagtgctgccgcgccacgccaagcctggaccaactattttaatgaatgatcaggaggttggtgtgctcgatgccaaagagttagttgataaagacggaaccaacctggagctgacactattgaagcttaaccgcaatgaaaagttcagagacatcagaggttttcttgcaagggaagaagttgaggtaagtgaggctgttttggcaataaacacgagcaagttcccaagcatgtacatccctgtgggccaagtcaccgattacggatttttaaatctaggtggcaccccaacaaagagaatgctcatgtacaacttccctaccagagcgggacagtgtggtggtgtccttatgtcaacaggaaaggtccttggcatacacgtgggaggaaatggtcaccaaggcttctctgctgctctcctcagacactacttcaacgaggaacag

SEQ ID NO: 67 - RNA, 1386 nt, synthetic construct
  source 1..1386: mol_type = other RNA
  misc_feature 1..1386: note = nucleotide sequence coding 3D
ggcgaaatagagtttattgagagctctaaagatgcaggatttcctgtgatcaacacccctaataaaaccaaactggaaccaagtgtgtttcatcaggtttttgagggcaacaaagaaccagcagtcctaagaaacggagacccgcgacttaaagccaactttgaggaagcgatattttccaagtacatcggaaatgtgaacacacatgtggacgagtacatgatagaagctgttgatcactacgctggacagctggcaactctggacatcagtacagaacctatgaagcttgaggatgctgtttatggcactgaaggcttggaagcattggacttgaccactagcgcaggatatccttatgtcgccttgggcatcaagaaaagggatatcctctccaagaagactaaagatctcaccaagctgagggaatgcatggacaagtatggtctaaatctgccgatggtgacctacgtgaaggatgaactcaggtccgctgagaaagtagccaagggaaaatccagacttatagaagcttctagtctcaatgactcagtggccatgaggcagacatttgggaacctatacaagacattccacctcaacccaggcattgtcactggtagtgctgttgggtgcgacccagatgtgttttggagcaaaatacccgtgatgcttgacgggcaccttatagcttttgattactctggctacgacgctagcttgagcccagtgtggtttgcttgtttgaaactcctcctagggaaactagggtatactcataaggaaaccaattacatagactacctctgcaactcccatcacttatacagagataaacactatttcgtgaggggtggtatgccatcaggatgttcaggcaccagtatattcaacaccatgatcaacaacatcattattaggacccttatgctaaaggtctacaaaggtattgacctggatcagtttagaatgatcgcttacggggacgatgtgatagcctcttacccgtggcctattgatgcctcactactagcagaagcgggaaaggattatggtttgatcatgaccccagcagataaaggagagtgttttaatgaggtaacctggacaaatgtaaccttcttgaaaaggtactttagagctgatgaacaatatccattcttggtgcaccccgtgatgcccatgaaagacatacacgaatccattagatggaccaaagacccaaagaacactcaagatcatgtgcgctcgttatgcctattggcttggcacaatggggagcacgaatatgaggaatttatccgaaagatcagaagcgtgcctgttggacgctgtttgaccctcccggtgttctcaacactacgcaggaaatggttagattccttc

SEQ ID NO: 68 - skipped

SEQ ID NO: 69 - RNA, 100 nt, synthetic construct
  source 1..100: mol_type = other RNA
  misc_feature 1..100: note = nucleotide sequence of 3' UTR
aattagagtgcaatcaatgaactatgattggcttaaccctaccgcatgaaccgaactagacaaaagtgcggtaggggtaaattctccgcattcggtgcgg

SEQ ID NO: 70 - protein, 283 aa, synthetic construct
  REGION 1..283: note = VP1
GPPGEAVERAIARVADTISSGPVNSESIPALTAAETGHTSQVVPADTMQTRHVKNYHSRSESTVENFLCRSACVYYTTYKNHGTDGDNFAYWVINTRQVAQLRRKLEMFTYARFDLELTFVITSTQEQSTIQGQDSPVLTHQIMYVPPGGPVPTKINSYSWQTSTNPSVFWTEGSAPPRISIPFISIGNAYSMFYDGWARFDKQGTYGINTLNNMGTLYMRHVNDGSPGPIVSTVRIYFKPKHVKTWVPRPPRLCQYQKAGNVNFEPTGVTESRTGITAMQTT

SEQ ID NO: 71 - DNA, 849 bp, synthetic construct
  source 1..849: mol_type = other DNA
  misc_feature 1..849: note = nucleotide sequence coding VP1
ggaccacccggggaagctgtcgaacgagcgattgctcgcgtggctgatactataagcagtggccctgttaattcagagtcaatcccggcactaacagcagcggagaccgggcacacatcccaggtggttccagcggacaccatgcaaaccaggcacgtgaagaattatcactcgcgatccgaatccacagtagagaacttcctgtgtagatccgcgtgtgtgtattacacaacctacaagaaccatggcactgatggagacaatttcgcctactgggtgatcaacacaagacaggtcgcgcagctgcgccgcaaattagaaatgtttacgtatgccagatttgacttagaactcacatttgtgataacaagcacacaagaacaatccaccatccaaggtcaagattcgcctgtgttaactcatcaaataatgtatgtgcccccaggaggcccggtgcccaccaagattaacagctacagctggcaaacatcaactaacccaagtgtcttttggacagaggggagtgctcctccacgcatatctataccatttattagtattgggaatgcttacagtatgttctatgacgggtgggctaggtttgacaagcaagggacttatggtataaacaccttgaacaacatgggtaccctgtacatgcgtcacgtaaatgatgggagtccaggtcctatcgtgagcactgtacgcatttacttcaaacccaaacacgtgaaaacgtgggttcccagaccaccaaggctatgtcaatatcaaaaagcaggaaacgtcaactttgagccaacaggggtgacggagtctcgtactggaattacggcaatgcagaccacc

SEQ ID NO: 72 - RNA, 849 nt, synthetic construct
  source 1..849: mol_type = other RNA
  misc_feature 1..849: note = nucleotide sequence coding VP1
ggaccacccggggaagctgtcgaacgagcgattgctcgcgtggctgatactataagcagtggccctgttaattcagagtcaatcccggcactaacagcagcggagaccgggcacacatcccaggtggttccagcggacaccatgcaaaccaggcacgtgaagaattatcactcgcgatccgaatccacagtagagaacttcctgtgtagatccgcgtgtgtgtattacacaacctacaagaaccatggcactgatggagacaatttcgcctactgggtgatcaacacaagacaggtcgcgcagctgcgccgcaaattagaaatgtttacgtatgccagatttgacttagaactcacatttgtgataacaagcacacaagaacaatccaccatccaaggtcaagattcgcctgtgttaactcatcaaataatgtatgtgcccccaggaggcccggtgcccaccaagattaacagctacagctggcaaacatcaactaacccaagtgtcttttggacagaggggagtgctcctccacgcatatctataccatttattagtattgggaatgcttacagtatgttctatgacgggtgggctaggtttgacaagcaagggacttatggtataaacaccttgaacaacatgggtaccctgtacatgcgtcacgtaaatgatgggagtccaggtcctatcgtgagcactgtacgcatttacttcaaacccaaacacgtgaaaacgtgggttcccagaccaccaaggctatgtcaatatcaaaaagcaggaaacgtcaactttgagccaacaggggtgacggagtctcgtactggaattacggcaatgcagaccacc

SEQ ID NO: 73 - DNA, 450 bp, synthetic construct
  source 1..450: mol_type = other DNA
  misc_feature 1..450: note = nucleotide sequence coding 2A protease mutant
ggttcatgtgggcaacaatcaggagctgtgtacgtgggcaattacaggattgtaaacagacacctggcaacgagccacgattggcaaaattgcgtgtgggaggactacaacagggatctcctggtcagcacaacaactgctcatggttgtgatactatagcacggtgccaatgtactgctggcgtgtacttttgtgcatctagaaacaagcactacccagtgagcttcgagggtccaggtctagtgaaagttcaggagagcgagtactaccccgagaggtaccagtcgcacgtactccttgcagttggattttcagaaccgggtgattgtggaggtattttgaggtgtgaacatggagtcattgggctcgttaccatgggtggtgagggtgtagtaggcttcgctgacgtgcgggatcttttgtggttggaagacgacgccatggagcag

SEQ ID NO: 74 - RNA, 450 nt, synthetic construct
  source 1..450: mol_type = other RNA
  misc_feature 1..450: note = nucleotide sequence coding 2A protease mutant
ggttcatgtgggcaacaatcaggagctgtgtacgtgggcaattacaggattgtaaacagacacctggcaacgagccacgattggcaaaattgcgtgtgggaggactacaacagggatctcctggtcagcacaacaactgctcatggttgtgatactatagcacggtgccaatgtactgctggcgtgtacttttgtgcatctagaaacaagcactacccagtgagcttcgagggtccaggtctagtgaaagttcaggagagcgagtactaccccgagaggtaccagtcgcacgtactccttgcagttggattttcagaaccgggtgattgtggaggtattttgaggtgtgaacatggagtcattgggctcgttaccatgggtggtgagggtgtagtaggcttcgctgacgtgcgggatcttttgtggttggaagacgacgccatggagcag

SEQ ID NO: 75 - protein, 150 aa, synthetic construct
  REGION 1..150: note = 2A protease mutant
GSCGQQSGAVYVGNYRIVNRHLATSHDWQNCVWEDYNRDLLVSTTTAHGCDTIARCQCTAGVYFCASRNKHYPVSFEGPGLVKVQESEYYPERYQSHVLLAVGFSEPGDCGGILRCEHGVIGLVTMGGEGVVGFADVRDLLWLEDDAMEQ

SEQ ID NO: 76 - DNA, 743 bp, synthetic construct
  source 1..743: mol_type = other DNA
  misc_feature 1..743: note = nucleotide sequence of 5' UTR mutant
ttaaaacagcctgtgggttgtacccacccacagggcccactgggcgctagcactctggtatcacggtacctttgtgtgcctgttttatatcccctttccccgattgtaacttagaagatgtacacactgatcaatagcgggcatagcacaccagctatgtcttgatcaagcactcctgtatccccggaccaagtatcaatagactgctcacgcggttgaaggagaaaacgttcgttacccggctaactacttcgagaaacccagtagtatcatgaaagttgcgaggcgtttcgttcagcacacccccagtgtagatcgggtcgatgagtcaccgcatcccccacgggcgaccgtggcggtggctgcgctggcggcctgcctacggagcaacccgtaggacgcttcaatacagacatggtgcgaagagtcgattgagctagttagtagtcctccggcccctgaatgcggctaatcctaactgcggagcacatgccctcaacccagggggtattgtgtcgtaacgggcaactctgcagcggaaccgactactttgggtgtccgtgtttccttttatccttatactggctgcttatggtgacaattgaaagattgttgccatatagctattggattggccatccagtgtctaatagagctgttatttacctctttgttggatttataccactcaacctaaaagaagttaaaacactacagctcattttacaactgaatacagcaaa

SEQ ID NO: 77 - RNA, 743 nt, synthetic construct
  source 1..743: mol_type = other RNA
  misc_feature 1..624: note = nucleotide sequence of 5' UTR mutant
ttaaaacagcctgtgggttgtacccacccacagggcccactgggcgctagcactctggtatcacggtacctttgtgtgcctgttttatatcccctttccccgattgtaacttagaagatgtacacactgatcaatagcgggcatagcacaccagctatgtcttgatcaagcactcctgtatccccggaccaagtatcaatagactgctcacgcggttgaaggagaaaacgttcgttacccggctaactacttcgagaaacccagtagtatcatgaaagttgcgaggcgtttcgttcagcacacccccagtgtagatcgggtcgatgagtcaccgcatcccccacgggcgaccgtggcggtggctgcgctggcggcctgcctacggagcaacccgtaggacgcttcaatacagacatggtgcgaagagtcgattgagctagttagtagtcctccggcccctgaatgcggctaatcctaactgcggagcacatgccctcaacccagggggtattgtgtcgtaacgggcaactctgcagcggaaccgactactttgggtgtccgtgtttccttttatccttatactggctgcttatggtgacaattgaaagattgttgccatatagctattggattggccatccagtgtctaatagagctgttatttacctctttgttggatttataccactcaacctaaaagaagttaaaacactacagctcattttacaactgaatacagcaaa

SEQ ID NO: 78 - protein, 69 aa, synthetic construct
  REGION 1..69: note = VP4
MGAQVSTQKTGAHETGVSASGNSIIHYTNINYYKDAASNSANRQEFAQDPGKFTEPVKDIMIKSMPALN

SEQ ID NO: 79 - protein, 261 aa, synthetic construct
  REGION 1..261: note = VP2
SPSAEECGYSDRVRSITLGNSTITTQECANVVVGYGTWPTYLKDEEATAEDQPTQPDVATCRFYTLESVMWQQSSPGWWWKFPDALSNMGLFGQNMQYHYLGRAGYTVHVQCNASKFHQGCLLVVCVPEAEMGCATIANKPDQKSLSNGETANTFDSQDTTGQTAVQANVINAGMGVGVGNLTIFPHQWINLRTNNSATIVMPYINSVPMDNMFRHNNFTLMIIPFAPLSYSTGATTYVPITVTVAPMCAEYNGLRLAGRQ

SEQ ID NO: 80 - protein, 238 aa, synthetic construct
  REGION 1..238: note = VP3
GLPTMLTPGSSQFLTSDDFQSPSAMPQFDVTPEMAIPGQVNNLMEIAEVDSVVPVNNTEGKVSSIEAYQIPVQSNSTNGSQVFGFPLIPGASSVLNRTLLGEILNYYTHWSGSIKLTFMFCGSAMATGKFLLAYSPPGAGAPTTRKEAMLGTHVIWDVGLQSSCVLCIPWISQTHYRYVVVDEYTAGGYITCWYQTNIVVPADTQSGCKILCFVSACNDFSVRMLKDTPFIKQDNFFQ

SEQ ID NO: 81 - DNA, 624 bp, synthetic construct
  source 1..624: mol_type = other DNA
  misc_feature 1..624: note = nucleotide sequence of IRES mutant
ttaaaacagcctgtgggttgtacccacccacagggcccactgggcgctagcactctggtatcacggtacctttgtgtgcctgttttatatcccctttccccgattgtaacttagaagatgtacacactgatcaatagcgggcatagcacaccagctatgtcttgatcaagcactcctgtatccccggaccaagtatcaatagactgctcacgcggttgaaggagaaaacgttcgttacccggctaactacttcgagaaacccagtagtatcatgaaagttgcgaggcgtttcgttcagcacacccccagtgtagatcgggtcgatgagtcaccgcatcccccacgggcgaccgtggcggtggctgcgctggcggcctgcctacggagcaacccgtaggacgcttcaatacagacatggtgcgaagagtcgattgagctagttagtagtcctccggcccctgaatgcggctaatcctaactgcggagcacatgccctcaacccagggggtattgtgtcgtaacgggcaactctgcagcggaaccgactactttgggtgtccgtgtttccttttatccttatactggctgcttatggtgacaattgaaagattgttgccatatagc

SEQ ID NO: 82 - RNA, 624 nt, synthetic construct
  source 1..624: mol_type = other RNA
  misc_feature 1..624: note = nucleotide sequence of IRES mutant
ttaaaacagcctgtgggttgtacccacccacagggcccactgggcgctagcactctggtatcacggtacctttgtgtgcctgttttatatcccctttccccgattgtaacttagaagatgtacacactgatcaatagcgggcatagcacaccagctatgtcttgatcaagcactcctgtatccccggaccaagtatcaatagactgctcacgcggttgaaggagaaaacgttcgttacccggctaactacttcgagaaacccagtagtatcatgaaagttgcgaggcgtttcgttcagcacacccccagtgtagatcgggtcgatgagtcaccgcatcccccacgggcgaccgtggcggtggctgcgctggcggcctgcctacggagcaacccgtaggacgcttcaatacagacatggtgcgaagagtcgattgagctagttagtagtcctccggcccctgaatgcggctaatcctaactgcggagcacatgccctcaacccagggggtattgtgtcgtaacgggcaactctgcagcggaaccgactactttgggtgtccgtgtttccttttatccttatactggctgcttatggtgacaattgaaagattgttgccatatagc

SEQ ID NO: 83 - DNA, 3200 bp, synthetic construct; identical to SEQ ID NO: 43
  source 1..3200: mol_type = other DNA
  misc_feature 1..3200: note = nucleotide sequence coding SFTS ABDEF antigen

SEQ ID NO: 84 - RNA, 3200 nt, synthetic construct; identical to SEQ ID NO: 44
  source 1..3200: mol_type = other RNA
  misc_feature 1..3200: note = nucleotide sequence coding SFTS ABDEF antigen

SEQ ID NO: 85 - protein, 1073 aa, synthetic construct; identical to SEQ ID NO: 45
  REGION 1..1073: note = SFTS ABDEF antigen

SEQ ID NO: 86 - DNA, 743 bp, synthetic construct; identical to SEQ ID NO: 76
  source 1..743: mol_type = other DNA
  misc_feature 1..743: note = nucleotide sequence of 5' UTR mutant

SEQ ID NO: 87 - RNA, 743 nt, synthetic construct; identical to SEQ ID NO: 77
  source 1..743: mol_type = other RNA
  misc_feature 1..743: note = nucleotide sequence of 5' UTR mutant

SEQ ID NO: 88 - DNA, 207 bp, synthetic construct
  source 1..207: mol_type = other DNA
  misc_feature 1..207: note = nucleotide sequence coding VP4
atgggagctcaggtttcaacgcaaaaaactggagcacacgagaccggagtgagtgctagcggcaattccatcattcattacacaaatattaactactataaggatgctgcgtctaattcagctaaccggcaagaatttgctcaggatccaggtaagttcacagaaccagtaaaggatattatgattaagtcaatgccagccctcaat

SEQ ID NO: 89 - DNA, 783 bp, synthetic construct
  source 1..783: mol_type = other DNA
  misc_feature 1..783: note = nucleotide sequence coding VP2
tcgccatctgccgaggagtgtgggtacagtgacagggtgagatctattacgttgggaaactcaacaatcaccacgcaggagtgtgctaatgtggtggttggatatggcacatggcccacgtatctcaaagatgaagaggctacggcagaggatcaaccaactcaaccagacgtggcaacatgtagattctacaccttagagtccgtgatgtggcagcagagctcacctggatggtggtggaaattcccggacgccctttcaaacatgggtttgttcgggcaaaacatgcagtaccattatttagggagagctggatacactgtgcatgtacagtgcaacgcctccaaattccaccaaggatgcttgttggttgtgtgtgtgccagaggctgagatgggctgtgcaaccatagctaataagccagatcaaaagagcctgagtaatggagaaacagccaacacgtttgattcacaagacacgaccggacaaacagctgtgcaggctaacgtcattaacgcaggtatgggggtgggtgttggtaacctaaccatttttccacatcagtggatcaacctgcgaactaacaacagtgccacaattgttatgccatatataaatagtgtgccaatggataatatgttcagacacaacaacttcaccctaatgattataccttttgcaccattgagttatagcacgggcgcaaccacctacgtgcctattacggtgactgtggcgccaatgtgcgcagaatacaatggtttgcgattggcagggagacaa

SEQ ID NO: 90 - DNA, 714 bp, synthetic construct
  source 1..714: mol_type = other DNA
  misc_feature 1..714: note = nucleotide sequence coding VP3
gggttacccacaatgctaacacctggtagcagccaatttttgacctctgatgacttccagtcgccttccgccatgccacagttcgacgtgacgccagaaatggcaattcctgggcaggtgaataacttgatggagatcgcggaagttgattccgtggttccagttaacaatactgagggcaaagtatcatcaattgaagcgtaccaaatacctgtacaatcaaactcaactaatggctcacaagtatttgggtttcctctcatccccggcgccagtagtgtgctaaatagaacactcctgggtgagatccttaattattatacacattggtcaggaagcatcaaattgacatttatgttttgcgggtctgcaatggctaccggtaagtttctattggcttattcaccccctggtgctggtgcaccaacaaccaggaaagaagcaatgcttggaacacacgtcatctgggacgttgggttgcagtccagctgtgtgttatgcattccatggatcagtcaaacacattacagatatgtggtggtggacgagtacaccgctggagggtacatcacttgttggtaccagacaaatattgtggtacctgctgacacacaaagtggctgcaagatcttgtgttttgtatcagcatgcaacgacttttccgtgaggatgctaaaggacacaccttttataaagcaggacaactttttccaa

SEQ ID NO: 91 - RNA, 207 nt, synthetic construct
  source 1..207: mol_type = other RNA
  misc_feature 1..207: note = nucleotide sequence coding VP4
atgggagctcaggtttcaacgcaaaaaactggagcacacgagaccggagtgagtgctagcggcaattccatcattcattacacaaatattaactactataaggatgctgcgtctaattcagctaaccggcaagaatttgctcaggatccaggtaagttcacagaaccagtaaaggatattatgattaagtcaatgccagccctcaat

SEQ ID NO: 92 - RNA, 783 nt, synthetic construct
  source 1..783: mol_type = other RNA
  misc_feature 1..783: note = nucleotide sequence coding VP2
tcgccatctgccgaggagtgtgggtacagtgacagggtgagatctattacgttgggaaactcaacaatcaccacgcaggagtgtgctaatgtggtggttggatatggcacatggcccacgtatctcaaagatgaagaggctacggcagaggatcaaccaactcaaccagacgtggcaacatgtagattctacaccttagagtccgtgatgtggcagcagagctcacctggatggtggtggaaattcccggacgccctttcaaacatgggtttgttcgggcaaaacatgcagtaccattatttagggagagctggatacactgtgcatgtacagtgcaacgcctccaaattccaccaaggatgcttgttggttgtgtgtgtgccagaggctgagatgggctgtgcaaccatagctaataagccagatcaaaagagcctgagtaatggagaaacagccaacacgtttgattcacaagacacgaccggacaaacagctgtgcaggctaacgtcattaacgcaggtatgggggtgggtgttggtaacctaaccatttttccacatcagtggatcaacctgcgaactaacaacagtgccacaattgttatgccatatataaatagtgtgccaatggataatatgttcagacacaacaacttcaccctaatgattataccttttgcaccattgagttatagcacgggcgcaaccacctacgtgcctattacggtgactgtggcgccaatgtgcgcagaatacaatggtttgcgattggcagggagacaa

SEQ ID NO: 93 - RNA, 714 nt, synthetic construct
  source 1..714: mol_type = other RNA
  misc_feature 1..714: note = nucleotide sequence coding VP3
gggttacccacaatgctaacacctggtagcagccaatttttgacctctgatgacttccagtcgccttccgccatgccacagttcgacgtgacgccagaaatggcaattcctgggcaggtgaataacttgatggagatcgcggaagttgattccgtggttccagttaacaatactgagggcaaagtatcatcaattgaagcgtaccaaatacctgtacaatcaaactcaactaatggctcacaagtatttgggtttcctctcatccccggcgccagtagtgtgctaaatagaacactcctgggtgagatccttaattattatacacattggtcaggaagcatcaaattgacatttatgttttgcgggtctgcaatggctaccggtaagtttctattggcttattcaccccctggtgctggtgcaccaacaaccaggaaagaagcaatgcttggaacacacgtcatctgggacgttgggttgcagtccagctgtgtgttatgcattccatggatcagtcaaacacattacagatatgtggtggtggacgagtacaccgctggagggtacatcacttgttggtaccagacaaatattgtggtacctgctgacacacaaagtggctgcaagatcttgtgttttgtatcagcatgcaacgacttttccgtgaggatgctaaaggacacaccttttataaagcaggacaactttttccaa

SEQ ID NO: 94 - DNA, 20 bp, synthetic construct
  source 1..20: mol_type = other DNA
  misc_feature 1..20: note = nucleotide sequence of T7 promoter
taatacgactcactataggg

SEQ ID NO: 95 - DNA, 38 bp, synthetic construct
  source 1..38: mol_type = other DNA
  misc_feature 1..38: note = nucleotide sequence of human globulin 5' UTR
gagaataaactagtattcttctggtccccacagactca

SEQ ID NO: 96 - RNA, 38 nt, synthetic construct
  source 1..38: mol_type = other RNA
  misc_feature 1..38: note = nucleotide sequence of human globulin 5' UTR
gagaataaactagtattcttctggtccccacagactca

SEQ ID NO: 97 - DNA, 295 bp, synthetic construct
  source 1..295: mol_type = other DNA
  misc_feature 1..295: note = nucleotide sequence of human globulin 3' UTR
ctcgagctggtactgcatgcacgcaatgctagctgcccctttcccgtcctgggtaccccgagtctcccccgacctcgggtcccaggtatgctcccacctccacctgccccactcaccacctctgctagttccagacacctcccaagcacgcagcaatgcagctcaaaacgcttagcctagccacacccccacgggaaacagcagtgattaacctttagcaataaacgaaagtttaactaagctatactaaccccagggttggtcaatttcgtgccagccacaccctggagctagc

SEQ ID NO: 98 - RNA, 295 nt, synthetic construct
  source 1..295: mol_type = other RNA
  misc_feature 1..295: note = nucleotide sequence of human globulin 3' UTR
ctcgagctggtactgcatgcacgcaatgctagctgcccctttcccgtcctgggtaccccgagtctcccccgacctcgggtcccaggtatgctcccacctccacctgccccactcaccacctctgctagttccagacacctcccaagcacgcagcaatgcagctcaaaacgcttagcctagccacacccccacgggaaacagcagtgattaacctttagcaataaacgaaagtttaactaagctatactaaccccagggttggtcaatttcgtgccagccacaccctggagctagc

SEQ ID NO: 99 - DNA, 7101 bp, synthetic construct
  source 1..7101: mol_type = other DNA
  misc_feature 1..7101: note = nucleotide sequence coding coxsachievirus B5
ttaaaacagcctgtgggttgtacccacccacagggcccactgggcgctagcactctggtatcacggtacctttgtgtgcctgttttatatcccctttccccgattgtaacttagaagatgtacacactgatcaatagcgggcatagcacaccagctatgtcttgatcaagcactcctgtatccccggaccaagtatcaatagactgctcacgcggttgaaggagaaaacgttcgttacccggctaactacttcgagaaacccagtagtatcatgaaagttgcgaggcgtttcgttcagcacacccccagtgtagatcgggtcgatgagtcaccgcatcccccacgggcgaccgtggcggtggctgcgctggcggcctgcctacggagcaacccgtaggacgcttcaatacagacatggtgcgaagagtcgattgagctagttagtagtcctccggcccctgaatgcggctaatcctaactgcggagcacatgccctcaacccagggggtattgtgtcgtaacgggcaactctgcagcggaaccgactactttgggtgtccgtgtttccttttatccttatactggctgcttatggtgacaattgaaagattgttgccatatagctattggattggccatccagtgtctaatagagctgttatttacctctttgttggatttataccactcaacctaaaagaagttaaaacactacagctcattttacaactgaatacagcaaaatgggagctcaggtttcaacgcaaaaaactggagcacacgagaccggagtgagtgctagcggcaattccatcattcattacacaaatattaactactataaggatgctgcgtctaattcagctaaccggcaagaatttgctcaggatccaggtaagttcacagaaccagtaaaggatattatgattaagtcaatgccagccctcaattcgccatctgccgaggagtgtgggtacagtgacagggtgagatctattacgttgggaaactcaacaatcaccacgcaggagtgtgctaatgtggtggttggatatggcacatggcccacgtatctcaaagatgaagaggctacggcagaggatcaaccaactcaaccagacgtggcaacatgtagattctacaccttagagtccgtgatgtggcagcagagctcacctggatggtggtggaaattcccggacgccctttcaaacatgggtttgttcgggcaaaacatgcagtaccattatttagggagagctggatacactgtgcatgtacagtgcaacgcctccaaattccaccaaggatgcttgttggttgtgtgtgtgccagaggctgagatgggctgtgcaaccatagctaataagccagatcaaaagagcctgagtaatggagaaacagccaacacgtttgattcacaagacacgaccggacaaacagctgtgcaggctaacgtcattaacgcaggtatgggggtgggtgttggtaacctaaccatttttccacatcagtggatcaacctgcgaactaacaacagtgccacaattgttatgccatatataaatagtgtgccaatggataatatgttcagacacaacaacttcaccctaatgattataccttttgcaccattgagttatagcacgggcgcaaccacctacgtgcctattacggtgactgtggcgccaatgtgcgcagaatacaatggtttgcgattggcagggagacaagggttacccacaatgctaacacctggtagcagccaatttttgacctctgatgacttccagtcgccttccgccatgccacagttcgacgtgacgccagaaatggcaattcctgggcaggtgaataacttgatggagatcgcggaagttgattccgtggttccagttaacaatactgagggcaaagtatcatcaattgaagcgtaccaaatacctgtacaatcaaactcaactaatggctcacaagtatttgggtttcctctcatccccggcgccagtagtgtgctaaatagaacactcctgggtgagatccttaattattatacacattggtcaggaagcatcaaattgacatttatgttttgcgggtctgcaatggctaccggtaagtttctattggcttattcaccccctggtgctggtgcaccaacaaccaggaaagaagcaatgcttggaacacacgtcatctgggacgttgggttgcagtccagctgtgtgttatgcattccatggatcagtcaaacacattacagatatgtggtggtggacgagtacaccgctggagggtacatcacttgttggtaccagacaaatattgtggtacctgctgacacacaaagtggctgcaagatcttgtgttttgtatcagcatgcaacgacttttccgtgaggatgctaaaggacacaccttttataaagcaggacaactttttccaaggaccacccggggaagctgtcgaacgagcgattgctcgcgtggctgatactataagcagtggccctgttaattcagagtcaatcccggcactaacagcagcggagaccgggcacacatcccaggtggttccagcggacaccatgcaaaccaggcacgtgaagaattatcactcgcgatccgaatccacagtagagaacttcctgtgtagatccgcgtgtgtgtattacacaacctacaagaaccatggcactgatggagacaatttcgcctactgggtgatcaacacaagacaggtcgcgcagctgcgccgcaaattagaaatgtttacgtatgccagatttgacttagaactcacatttgtgataacaagcacacaagaacaatccaccatccaaggtcaagattcgcctgtgttaactcatcaaataatgtatgtgcccccaggaggcccggtgcccaccaagattaacagctacagctggcaaacatcaactaacccaagtgtcttttggacagaggggagtgctcctccacgcatatctataccatttattagtattgggaatgcttacagtatgttctatgacgggtgggctaggtttgacaagcaagggacttatggtataaacaccttgaacaacatgggtaccctgtacatgcgtcacgtaaatgatgggagtccaggtcctatcgtgagcactgtacgcatttacttcaaacccaaacacgtgaaaacgtgggttcccagaccaccaaggctatgtcaatatcaaaaagcaggaaacgtcaactttgagccaacaggggtgacggagtctcgtactggaattacggcaatgcagaccaccggtttatgtgggcaacaatcaggagccgtgtatgtgggcaattacaggatcataaacagacacctggcaacgagccacgattggcaaaattgcgtgtgggaggactataacagggatctcctggttagcacaacaactgctcatggttgtgatactatagcacggtgccaatgtaccactggcgtgtacttttgtgcatctagaaacaagcactacccagtgagcttcaagggtccaggtctagtgaaggttcaggagagcgagtactaccctgagagataccagtcgcacgtactccttgcagctggattttcagaaccgggtgactgtggaggtattttgaggtgtgaacatggagtcattgggcttgttaccatgggtggtgagggtgtggtaggcttcgctgacgtgcgggaccttttgtggttggaagatgacgccatggagcagaataacggctggttaaagaaattcactgaaatgaccaacgcctgcaagggcatggagtggattgctgttaagattcaaaagtttatcgagtggctcaaagtaaagattctgcctgaagtgaaggagaaacatgagttcctcaccagattgaagcaattgccactccttgaaagtcaaattgccaccattgagcagagcgcaccctcacaaagtgatcaagagcagcttttttcgaatgtccagtacttcgcccattactgcaggaagtatgcacctctgtatgctgccgaagcaaaaagagtgttctcattagaaaagaaaatgagtaattacatacagttcaagtccaaatgccgtattgagcctgtatgcttactccttcacggtagtccaggggctggtaagtcagtagctaccaacctgatagggagatcccttgcagagaagcttaacagctctgtgtactctttaccaccagatccagatcactttgatgggtacaaacagcaggcagtggtgattatggatgatctctgtcaaaaccccgatgggaaggacgtgtccttgttttgccaaatggtgtctagtgtagattttgtgccacccatggcggcgttggaagaaaaaggcattctctttacgtccccgtttgtgttggcatcaaccaacgcggggtccatcaacgcaccaacagtgtcagacagcagggcgcttgccagaaggtttcactttgacatgaatattgaggtgatttcgatgtacagccagaatggtaaaattaacatgcccatgtctgttaagacatgtgatgatgagtgctgcccggtcaatttcaaaaagtgttgcccactagtgtgtggcaaggctatccagttcattgacaggagaaaccaagttagatattcactggacatgttggttactgagatgtttagagagtacaaccacagacacagtgtgggtgctaccctcgaggctttgttccaaggaccaccagtgtacagggaaatcaaaatcagtgtggccccggaaacgccccctccaccagcaattgctgaccttctaaaatctgtagacagtgaggcagtaagggagtactgtaaggaaaagggttggcttgtgccagaggtcaactccactctacaaattgaaaaacatgtaagcagggcattcatttgcttgcaagcgctaactacatttgtttcggtggctggtataatttacatcatttacaagttgtttgccggctttcaaggtgcatacaccggtatacccagtcaaaaacccaaagtaccgactctgagacaagccaaggttcaaggtccagcatttgaatttgccgtagcaatgatgaagaggaacgccagcacagtcaagacagaatacggtgagtttacgatgcttggcatctatgacaagtgggcagtgctgccgcgccacgccaagcctggaccaactattttaatgaatgatcaggaggttggtgtgcttgatgccaaggagctagttgataaagacggaaccaacctggagctaacactattaaagctcaaccgcaatgaaaagttcagagatatcagaggtttccttgcaagggaagaagttgaggtaagtgaggctgttttggcaataaacacgagcaagttcccaagcatgtacatccctgtgggccaagtcaccgactacggatttttaaatctaggtggcaccccaacaaagagaatgctcatgtacaacttccctaccagagcaggacagtgtggtggtgtccttatgtcaacaggaaaggtccttggcatacacgtaggaggaaatggccaccaaggcttctctgctgctctcctcagacactacttcaatgaggaacagggcgagatagagttcattgagagctctaaagatgcaggatttcctgtgatcaacacccctagtaaaaccaaactggaaccaagtgtgtttcatcaggtttttgagggcaacaaagaaccggcggtcttaagaaacggagatccgcgacttaaagccaactttgaggaagcgatattttccaagtacatcggaaatgtgaacacacatgtggacgagtacatgatagaagctgttgatcactacgctgggcagctggcaactctggacatcagtacagaacctatgaagcttgaggatgctgtttatggcactgaaggcttggaagcattggacttgaccactagcgcaggatacccttatgtcgccttaggcatcaagaaaagggatatcctctccaagaagactaaagatctcactaagctgagggaatgcatggacaagtatggtctaaatctaccgatggtgacctacgtgaaggatgaactcaggtccgctgagaaagtagccaagggaaaatccagactcatagaagcttctagtctcaatgactcagtggccatgaggcaaacgtttgggaatctatataagacattccaccttaacccaggcattgtcactggtagtgctgttgggtgcgacccagatgtgttttggagcaaaatacccgtgatgctcgacgggcaccttatagcttttgattactctggctacgacgctagcttgagcccagtgtggtttgcttgtttgaaacttctcctagggaaactagggtatacccataaggaaaccaactacatagactacctctgcaactcccatcatttgtacagagataagcactatttcgtgaggggtggtatgccatcaggatgttcaggcaccagcatatttaactccatgatcaacaacatcattatcaggacccttatgctaaaggtctacaaaggtattgacctggatcagtttagaatgatcgcttacggcgacgatgtgatagcctcttacccgtggcctattgatgcctcactactagcagaagcaggaaaggattatggtttgatcatgaccccagcagataaaggagagtgttttaatgaggtaacctggacaaatgtaaccttcttgaaaaggtattttagggctgatgaacaatatccattcttggtgcaccctgtgatgcccatgaaagacatacatgaatccattagatggaccaaagacccaaagaacactcaagatcatgtgcgctcgctgtgcctattggcttggcacaatggagagcacgaatatgaggaatttatccgaaagatcagaagcgtgcctgttggacgctgtttgaccctcccagcgttttcaacactacgcaggaaatggttagactccttcaattagagtgcaatcaatgaactatgattggcttaaccctaccgcatgaaccgaactagacaaaagtgcggtaggggtaaattctccgcattcggtgcgg

SEQ ID NO: 100 - RNA, 7101 nt, synthetic construct
  source 1..7101: mol_type = other RNA
  misc_feature 1..7101: note = nucleotide sequence coding coxsachievirus B5
ttaaaacagcctgtgggttgtacccacccacagggcccactgggcgctagcactctggtatcacggtacctttgtgtgcctgttttatatcccctttccccgattgtaacttagaagatgtacacactgatcaatagcgggcatagcacaccagctatgtcttgatcaagcactcctgtatccccggaccaagtatcaatagactgctcacgcggttgaaggagaaaacgttcgttacccggctaactacttcgagaaacccagtagtatcatgaaagttgcgaggcgtttcgttcagcacacccccagtgtagatcgggtcgatgagtcaccgcatcccccacgggcgaccgtggcggtggctgcgctggcggcctgcctacggagcaacccgtaggacgcttcaatacagacatggtgcgaagagtcgattgagctagttagtagtcctccggcccctgaatgcggctaatcctaactgcggagcacatgccctcaacccagggggtattgtgtcgtaacgggcaactctgcagcggaaccgactactttgggtgtccgtgtttccttttatccttatactggctgcttatggtgacaattgaaagattgttgccatatagctattggattggccatccagtgtctaatagagctgttatttacctctttgttggatttataccactcaacctaaaagaagttaaaacactacagctcattttacaactgaatacagcaaaatgggagctcaggtttcaacgcaaaaaactggagcacacgagaccggagtgagtgctagcggcaattccatcattcattacacaaatattaactactataaggatgctgcgtctaattcagctaaccggcaagaatttgctcaggatccaggtaagttcacagaaccagtaaaggatattatgattaagtcaatgccagccctcaattcgccatctgccgaggagtgtgggtacagtgacagggtgagatctattacgttgggaaactcaacaatcaccacgcaggagtgtgctaatgtggtggttggatatggcacatggcccacgtatctcaaagatgaagaggctacggcagaggatcaaccaactcaaccagacgtggcaacatgtagattctacaccttagagtccgtgatgtggcagcagagctcacctggatggtggtggaaattcccggacgccctttcaaacatgggtttgttcgggcaaaacatgcagtaccattatttagggagagctggatacactgtgcatgtacagtgcaacgcctccaaattccaccaaggatgcttgttggttgtgtgtgtgccagaggctgagatgggctgtgcaaccatagctaataagccagatcaaaagagcctgagtaatggagaaacagccaacacgtttgattcacaagacacgaccggacaaacagctgtgcaggctaacgtcattaacgcaggtatgggggtgggtgttggtaacctaaccatttttccacatcagtggatcaacctgcgaactaacaacagtgccacaattgttatgccatatataaatagtgtgccaatggataatatgttcagacacaacaacttcaccctaatgattataccttttgcaccattgagttatagcacgggcgcaaccacctacgtgcctattacggtgactgtggcgccaatgtgcgcagaatacaatggtttgcgattggcagggagacaagggttacccacaatgctaacacctggtagcagccaatttttgacctctgatgacttccagtcgccttccgccatgccacagttcgacgtgacgccagaaatggcaattcctgggcaggtgaataacttgatggagatcgcggaagttgattccgtggttccagttaacaatactgagggcaaagtatcatcaattgaagcgtaccaaatacctgtacaatcaaactcaactaatggctcacaagtatttgggtttcctctcatccccggcgccagtagtgtgctaaatagaacactcctgggtgagatccttaattattatacacattggtcaggaagcatcaaattgacatttatgttttgcgggtctgcaatggctaccggtaagtttctattggcttattcaccccctggtgctggtgcaccaacaaccaggaaagaagcaatgcttggaacacacgtcatctgggacgttgggttgcagtccagctgtgtgttatgcattccatggatcagtcaaacacattacagatatgtggtggtggacgagtacaccgctggagggtacatcacttgttggtaccagacaaatattgtggtacctgctgacacacaaagtggctgcaagatcttgtgttttgtatcagcatgcaacgacttttccgtgaggatgctaaaggacacaccttttataaagcaggacaactttttccaaggaccacccggggaagctgtcgaacgagcgattgctcgcgtggctgatactataagcagtggccctgttaattcagagtcaatcccggcactaacagcagcggagaccgggcacacatcccaggtggttccagcggacaccatgcaaaccaggcacgtgaagaattatcactcgcgatccgaatccacagtagagaacttcctgtgtagatccgcgtgtgtgtattacacaacctacaagaaccatggcactgatggagacaatttcgcctactgggtgatcaacacaagacaggtcgcgcagctgcgccgcaaattagaaatgtttacgtatgccagatttgacttagaactcacatttgtgataacaagcacacaagaacaatccaccatccaaggtcaagattcgcctgtgttaactcatcaaataatgtatgtgcccccaggaggcccggtgcccaccaagattaacagctacagctggcaaacatcaactaacccaagtgtcttttggacagaggggagtgctcctccacgcatatctataccatttattagtattgggaatgcttacagtatgttctatgacgggtgggctaggtttgacaagcaagggacttatggtataaacaccttgaacaacatgggtaccctgtacatgcgtcacgtaaatgatgggagtccaggtcctatcgtgagcactgtacgcatttacttcaaacccaaacacgtgaaaacgtgggttcccagaccaccaaggctatgtcaatatcaaaaagcaggaaacgtcaactttgagccaacaggggtgacggagtctcgtactggaattacggcaatgcagaccaccggtttatgtgggcaacaatcaggagccgtgtatgtgggcaattacaggatcataaacagacacctggcaacgagccacgattggcaaaattgcgtgtgggaggactataacagggatctcctggttagcacaacaactgctcatggttgtgatactatagcacggtgccaatgtaccactggcgtgtacttttgtgcatctagaaacaagcactacccagtgagcttcaagggtccaggtctagtgaaggttcaggagagcgagtactaccctgagagataccagtcgcacgtactccttgcagctggattttcagaaccgggtgactgtggaggtattttgaggtgtgaacatggagtcattgggcttgttaccatgggtggtgagggtgtggtaggcttcgctgacgtgcgggaccttttgtggttggaagatgacgccatggagcagaataacggctggttaaagaaattcactgaaatgaccaacgcctgcaagggcatggagtggattgctgttaagattcaaaagtttatcgagtggctcaaagtaaagattctgcctgaagtgaaggagaaacatgagttcctcaccagattgaagcaattgccactccttgaaagtcaaattgccaccattgagcagagcgcaccctcacaaagtgatcaagagcagcttttttcgaatgtccagtacttcgcccattactgcaggaagtatgcacctctgtatgctgccgaagcaaaaagagtgttctcattagaaaagaaaatgagtaattacatacagttcaagtccaaatgccgtattgagcctgtatgcttactccttcacggtagtccaggggctggtaagtcagtagctaccaacctgatagggagatcccttgcagagaagcttaacagctctgtgtactctttaccaccagatccagatcactttgatgggtacaaacagcaggcagtggtgattatggatgatctctgtcaaaaccccgatgggaaggacgtgtccttgttttgccaaatggtgtctagtgtagattttgtgccacccatggcggcgttggaagaaaaaggcattctctttacgtccccgtttgtgttggcatcaaccaacgcggggtccatcaacgcaccaacagtgtcagacagcagggcgcttgccagaaggtttcactttgacatgaatattgaggtgatttcgatgtacagccagaatggtaaaattaacatgcccatgtctgttaagacatgtgatgatgagtgctgcccggtcaatttcaaaaagtgttgcccactagtgtgtggcaaggctatccagttcattgacaggagaaaccaagttagatattcactggacatgttggttactgagatgtttagagagtacaaccacagacacagtgtgggtgctaccctcgaggctttgttccaaggaccaccagtgtacagggaaatcaaaatcagtgtggccccggaaacgccccctccaccagcaattgctgaccttctaaaatctgtagacagtgaggcagtaagggagtactgtaaggaaaagggttggcttgtgccagaggtcaactccactctacaaattgaaaaacatgtaagcagggcattcatttgcttgcaagcgctaactacatttgtttcggtggctggtataatttacatcatttacaagttgtttgccggctttcaaggtgcatacaccggtatacccagtcaaaaacccaaagtaccgactctgagacaagccaaggttcaaggtccagcatttgaatttgccgtagcaatgatgaagaggaacgccagcacagtcaagacagaatacggtgagtttacgatgcttggcatctatgacaagtgggcagtgctgccgcgccacgccaagcctggaccaactattttaatgaatgatcaggaggttggtgtgcttgatgccaaggagctagttgataaagacggaaccaacctggagctaacactattaaagctcaaccgcaatgaaaagttcagagatatcagaggtttccttgcaagggaagaagttgaggtaagtgaggctgttttggcaataaacacgagcaagttcccaagcatgtacatccctgtgggccaagtcaccgactacggatttttaaatctaggtggcaccccaacaaagagaatgctcatgtacaacttccctaccagagcaggacagtgtggtggtgtccttatgtcaacaggaaaggtccttggcatacacgtaggaggaaatggccaccaaggcttctctgctgctctcctcagacactacttcaatgaggaacagggcgagatagagttcattgagagctctaaagatgcaggatttcctgtgatcaacacccctagtaaaaccaaactggaaccaagtgtgtttcatcaggtttttgagggcaacaaagaaccggcggtcttaagaaacggagatccgcgacttaaagccaactttgaggaagcgatattttccaagtacatcggaaatgtgaacacacatgtggacgagtacatgatagaagctgttgatcactacgctgggcagctggcaactctggacatcagtacagaacctatgaagcttgaggatgctgtttatggcactgaaggcttggaagcattggacttgaccactagcgcaggatacccttatgtcgccttaggcatcaagaaaagggatatcctctccaagaagactaaagatctcactaagctgagggaatgcatggacaagtatggtctaaatctaccgatggtgacctacgtgaaggatgaactcaggtccgctgagaaagtagccaagggaaaatccagactcatagaagcttctagtctcaatgactcagtggccatgaggcaaacgtttgggaatctatataagacattccaccttaacccaggcattgtcactggtagtgctgttgggtgcgacccagatgtgttttggagcaaaatacccgtgatgctcgacgggcaccttatagcttttgattactctggctacgacgctagcttgagcccagtgtggtttgcttgtttgaaacttctcctagggaaactagggtatacccataaggaaaccaactacatagactacctctgcaactcccatcatttgtacagagataagcactatttcgtgaggggtggtatgccatcaggatgttcaggcaccagcatatttaactccatgatcaacaacatcattatcaggacccttatgctaaaggtctacaaaggtattgacctggatcagtttagaatgatcgcttacggcgacgatgtgatagcctcttacccgtggcctattgatgcctcactactagcagaagcaggaaaggattatggtttgatcatgaccccagcagataaaggagagtgttttaatgaggtaacctggacaaatgtaaccttcttgaaaaggtattttagggctgatgaacaatatccattcttggtgcaccctgtgatgcccatgaaagacatacatgaatccattagatggaccaaagacccaaagaacactcaagatcatgtgcgctcgctgtgcctattggcttggcacaatggagagcacgaatatgaggaatttatccgaaagatcagaagcgtgcctgttggacgctgtttgaccctcccagcgttttcaacactacgcaggaaatggttagactccttcaattagagtgcaatcaatgaactatgattggcttaaccctaccgcatgaaccgaactagacaaaagtgcggtaggggtaaattctccgcattcggtgcgg

SEQ ID NO: 101 - protein, 2087 aa, synthetic construct
  REGION 1..2087: note = coxsachievirus B5
MGAQVSTQKTGAHETGVSASGNSIIHYTNINYYKDAASNSANRQEFAQDPGKFTEPVKDIMIKSMPALNSPSAEECGYSDRVRSITLGNSTITTQECANVVVGYGTWPTYLKDEEATAEDQPTQPDVATCRFYTLESVMWQQSSPGWWWKFPDALSNMGLFGQNMQYHYLGRAGYTVHVQCNASKFHQGCLLVVCVPEAEMGCATIANKPDQKSLSNGETANTFDSQDTTGQTAVQANVINAGMGVGVGNLTIFPHQWINLRTNNSATIVMPYINSVPMDNMFRHNNFTLMIIPFAPLSYSTGATTYVPITVTVAPMCAEYNGLRLAGRQGLPTMLTPGSSQFLTSDDFQSPSAMPQFDVTPEMAIPGQVNNLMEIAEVDSVVPVNNTEGKVSSIEAYQIPVQSNSTNGSQVFGFPLIPGASSVLNRTLLGEILNYYTHWSGSIKLTFMFCGSAMATGKFLLAYSPPGAGAPTTRKEAMLGTHVIWDVGLQSSCVLCIPWISQTHYRYVVVDEYTAGGYITCWYQTNIVVPADTQSGCKILCFVSACNDFSVRMLKDTPFIKQDNFFQGPPGEAVERAIARVADTISSGPVNSESIPALTAAETGHTSQVVPADTMQTRHVKNYHSRSESTVENFLCRSACVYYTTYKNHGTDGDNFAYWVINTRQVAQLRRKLEMFTYARFDLELTFVITSTQEQSTIQGQDSPVLTHQIMYVPPGGPVPTKINSYSWQTSTNPSVFWTEGSAPPRISIPFISIGNAYSMFYDGWARFDKQGTYGINTLNNMGTLYMRHVNDGSPGPIVSTVRIYFKPKHVKTWVPRPPRLCQYQKAGNVNFEPTGVTESRTGITAMQTTGLCGQQSGAVYVGNYRIINRHLATSHDWQNCVWEDYNRDLLVSTTTAHGCDTIARCQCTTGVYFCASRNKHYPVSFKGPGLVKVQESEYYPERYQSHVLLAAGFSEPGDCGGILRCEHGVIGLVTMGGEGVVGFADVRDLLWLEDDAMEQNNGWLKKFTEMTNACKGMEWIAVKIQKFIEWLKVKILPEVKEKHEFLTRLKQLPLLESQIATIEQSAPSQSDQEQLFSNVQYFAHYCRKYAPLYAAEAKRVFSLEKKMSNYIQFKSKCRIEPVCLLLHGSPGAGKSVATNLIGRSLAEKLNSSVYSLPPDPDHFDGYKQQAVVIMDDLCQNPDGKDVSLFCQMVSSVDFVPPMAALEEKGILFTSPFVLASTNAGSINAPTVSDSRALARRFHFDMNIEVISMYSQNGKINMPMSVKTCDDECCPVNFKKCCPLVCGKAIQFIDRRNQVRYSLDMLVTEMFREYNHRHSVGATLEALFQGPPVYREIKISVAPETPPPPAIADLLKSVDSEAVREYCKEKGWLVPEVNSTLQIEKHVSRAFICLQALTTFVSVAGIIYIIYKLFAGFQGAYTGIPSQKPKVPTLRQAKVQGPAFEFAVAMMKRNASTVKTEYGEFTMLGIYDKWAVLPRHAKPGPTILMNDQEVGVLDAKELVDKDGTNLELTLLKLNRNEKFRDIRGFLAREEVEVSEAVLAINTSKFPSMYIPVGQVTDYGFLNLGGTPTKRMLMYNFPTRAGQCGGVLMSTGKVLGIHVGGNGHQGFSAALLRHYFNEEQGEIEFIESSKDAGFPVINTPSKTKLEPSVFHQVFEGNKEPAVLRNGDPRLKANFEEAIFSKYIGNVNTHVDEYMIEAVDHYAGQLATLDISTEPMKLEDAVYGTEGLEALDLTTSAGYPYVALGIKKRDILSKKTKDLTKLRECMDKYGLNLPMVTYVKDELRSAEKVAKGKSRLIEASSLNDSVAMRQTFGNLYKTFHLNPGIVTGSAVGCDPDVFWSKIPVMLDGHLIAFDYSGYDASLSPVWFACLKLLLGKLGYTHKETNYIDYLCNSHHLYRDKHYFVRGGMPSGCSGTSIFNSMINNIIIRTLMLKVYKGIDLDQFRMIAYGDDVIASYPWPIDASLLAEAGKDYGLIMTPADKGECFNEVTWTNVTFLKRYFRADEQYPFLVHPVMPMKDIHESIRWTKDPKNTQDHVRSLCLLAWHNGEHEYEEFIRKIRSVPVGRCLTLPAFSTLRRKWLDSFN

SEQ ID NO: 102 - DNA, 7101 bp, synthetic construct
  source 1..7101: mol_type = other DNA
  misc_feature 1..7101: note = nucleotide sequence coding modified coxachievirus B5
ttaaaacagcctgtgggttgtacccacccacagggcccactgggcgctagcactctggtatcacggtacctttgtgtgcctgttttatatcccctttccccgattgtaacttagaagatgtacacactgatcaatagcgggcatagcacaccagctatgtcttgatcaagcactcctgtatccccggaccaagtatcaatagactgctcacgcggttgaaggagaaaacgttcgtcacccggctaactacttcgagaaacccagtagtatcatgaaagttgcgaggcgtttcgttcagcacacccccagtgtagatcgggtcgatgagtcaccgcatcccccacgggcgaccgtggcggtggctgcgctggcggcctgcctacggggcaacccgtaggacgcttcaatacagacatggtgcgaagagtcgattgagctagttagtagtcctccggcccctgaatgcggctaatcctaactgcggagcacatgccctcaacccagggggtattgtgtcgtaacgggcaactctgcagcggaaccgactactttgggtgtccgtgtttccttttatccttatactggctgcttatggtgacaattgaaagattgttgccatatagctattggattggccatccagtgtctaatagagctgttatttacctctttgttggatttataccactcaacctaaaagaagttaaaacactacagctcattttacaactgaatacagcaaaatgggagctcaggtttcaacgcaaaaaactggagcacacgagaccggagtgagtgctagcggcaattccatcattcattacacaaatattaactactataaggatgctgcgtctaattcagctaaccggcaagaatttgctcaggatccaggtaagttcacagaaccagtaaaggatattatgattaagtcaatgccagccctcaattcgccatctgccgaggagtgtgggtacagtgacagggtgagatctattacgttgggaaactcaacaatcaccacgcaggagtgtgctaatgtggtggttggatatggcacatggcccacgtatctcaaagatgaagaggctacggcagaggatcaaccaactcaaccagacgtggcaacatgtagattctacaccttagagtccgtgatgtggcagcagagctcacctggatggtggtggaaattcccggacgccctttcaaacatgggtttgttcgggcaaaacatgcagtaccattatttagggagagctggatacactgtgcatgtacagtgcaacgcctccaaattccaccaaggatgcttgttggttgtgtgtgtgccagaggctgagatgggctgtgcaaccatagctaataagccagatcaaaagagcctgagtaatggagaaacagccaacacgtttgattcacaagacacgaccggacaaacagctgtgcaggctaacgtcattaacgcaggtatgggggtgggtgttggtaacctaaccatttttccacatcagtggatcaacctgcgaactaacaacagtgccacaattgttatgccatatataaatagtgtgccaatggataatatgttcagacacaacaacttcaccctaatgattataccttttgcaccattgagttatagcacgggcgcaaccacctacgtgcctattacggtgactgtggcgccaatgtgcgcagaatacaatggtttgcgattggcagggagacaagggttacccacaatgctaacacctggtagcagccaatttttgacctctgatgacttccagtcgccttccgccatgccacagttcgacgtgacgccagaaatggcaattcctgggcaggtgaataacttgatggagatcgcggaagttgattccgtggttccagttaacaatactgagggcaaagtatcatcaattgaagcgtaccaaatacctgtacaatcaaactcaactaatggctcacaagtatttgggtttcctctcatccccggcgccagtagtgtgctaaatagaacactcctgggtgagatccttaattattatacacattggtcaggaagcatcaaattgacatttatgttttgcgggtctgcaatggctaccggtaagtttctattggcttattcaccccctggtgctggtgcaccaacaaccaggaaagaagcaatgcttggaacacacgtcatctgggacgttgggttgcagtccagctgtgtgttatgcattccatggatcagtcaaacacattacagatatgtggtggtggacgagtacaccgctggagggtacatcacttgttggtaccagacaaatattgtggtacctgctgacacacaaagtggctgcaagatcttgtgttttgtatcagcatgcaacgacttttccgtgaggatgctaaaggacacaccttttataaagcaggacaactttttccaaggaccacccggggaagctgtcgaacgagcgattgctcgcgtggctgatactataagcagtggccctgttaattcagagtcaatcccgacactaacagcagcggagaccgggcacacatcccaggtggttccagcggacaccatgcaaaccaggcacgtgaagaattatcactcgcgatccgaatccacagtagagaacttcctgtgtagatccgcgtgtgtgtattacacaacctacaagaaccatggcactgatggagacaatttcgcctactgggtgatcaacacaagacaggtcgcgcagctgcgccgcaaattagaaatgtttacgtatgccagatttgacttagaactcacatttgtgataacaagcacacaagaacaatccaccatcaaaggtcaagattcgcctgtgttaactcatcaaataatgtatgtgcccccaggaggcccggtgcccaccaagattaacagctacagctggcaaacatcaactaacccaagtgtcttttggacagaggggagtgctcctccacgcatatctataccatttattagtattgggaatgcttacagtatgttctatgacgggtgggctaggtttgacaagcaagggacttatggtataaacaccttgaacaacatgggtaccctgtacatgcgtcacgtaaatgatgggagtccaggtcctatcgcgagcactgtacgcatttacttcaaacccaaacacgtgaaaacgtgggttcccagaccaccaaggctatgtcaatatcaaaaagcgggaaacgtcaactttgagccaacaggggtgacggagtctcgtactggaattacggcaatgcagaccaccggttcatgtgggcaacaatcaggagctgtgtacgtgggcaattacaggattgtaaacagacacctggcaacgagccacgattggcaaaattgcgtgtgggaggactacaacagggatctcctggtcagcacaacaactgctcatggttgtgatactatagcacggtgccaatgtactgctggcgtgtacttttgtgcatctagaaacaagcactacccagtgagcttcgagggtccaggtctagtgaaagttcaggagggcgagtactaccccgagagataccagtcgcacgtactccttgcagttggattttcagaaccgggtgattgtggaggtattttgaggtgtgaacatggagtcattgggctcgttaccatgggtggtgagggtgtagtaggcttcgctgacgtgcgggatcttttgtggttggaagacgacgccatggagcagaataacggttggttaaagaaattcactgaaatgaccaacgcctgcaagggcatggagtggattgctgttaaaattcaaaagttcatcgagtggctcaaagtaaagattctgcctgaagtgaaggagaaacatgagttccttaccagattgaagcaattgccactccttgaaagtcaaattgccaccattgagcaaagcgcaccctcacaaagtgatcaagagcagcttttttcgaatgttcagtacttcgcccattactgcaggaagtatgcacctctgtatgctgccgaagcaaaaagagtgttctcattagaaaagaaaatgagtaattacatacagttcaagtccaaatgccgcattgagcctgtatgcttactccttcacggtagtccaggggctggcaagtcagtagctaccaacctgatagggagatcccttgcagagaagctcaatagctctgtgtactctttaccaccagatccagatcattttgatgggtacaaacagcaggcagtggtgatcatggatgatctctgtcaaaaccccgatgggaaggacgtgtccttgttttgccaaatggtgtctagtgtagattttgtgccacccatggcggcgctggaagaaaaaggcattctctttacgtccccgtttgtgttggcatcaaccaacgcggggtccatcaatgcaccaacagtgtcagacagcagagcacttgccagaaggtttcactttgacatgaatattgaggtgatttcgatgtacagccagaatggtaaaattaacatgcccatgtctgttaagacatgtgatgatgaatgctgcccggtcaatttcaaaaagtgttgcccactagtgtgtggcaaggccatccagtttattgacaggagaaaccaagttagatattcactggacatgctggttactgagatgtttagagagtacaaccacagacacagtgtgggtgctaccctcgaggctttgttccaaggaccaccagtatacagggaaatcaaaatcagtgtggccccggaaacaccccctccaccagcaattgctgaccttctaaaatctgtagacagtgaggcaataagggagtactgcaaggaaaggggttggcttgtgccagaggtcagctccactctacaaattgaaaaacatgttagcagggcatttatttgcttgcaagcgctaactacatttgtttcagtggctggtataatctacatcatttacaagttgtttgccggctttcagggtgcatacactggaatgcccaaccagaaacccaaggtgcccaccttaagacaagctaaggtgcaaggtccggcatttgaatttgccgtagcaatgatgaaaaggaacgccagcacagtcaagacagaatacggtgagttcacgatgcttggcatctatgataaatgggcagtgctgccgcgccacgccaagcctggaccaactattttaatgaatgatcaggaggttggtgtgctcgatgccaaagagttagttgataaagacggaaccaacctggagctgacactattgaagcttaaccgcaatgaaaagttcagagacatcagaggttttcttgcaagggaagaagttgaggtaagtgaggctgttttggcaataaacacgagcaagttcccaagcatgtacatccctgtgggccaagtcaccgattacggatttttaaatctaggtggcaccccaacaaagagaatgctcatgtacaacttccctaccagagcgggacagtgtggtggtgtccttatgtcaacaggaaaggtccttggcatacacgtgggaggaaatggtcaccaaggcttctctgctgctctcctcagacactacttcaacgaggaacagggcgaaatagagtttattgagagctctaaagatgcaggatttcctgtgatcaacacccctaataaaaccaaactggaaccaagtgtgtttcatcaggtttttgagggcaacaaagaaccagcagtcctaagaaacggagacccgcgacttaaagccaactttgaggaagcgatattttccaagtacatcggaaatgtgaacacacatgtggacgagtacatgatagaagctgttgatcactacgctggacagctggcaactctggacatcagtacagaacctatgaagcttgaggatgctgtttatggcactgaaggcttggaagcattggacttgaccactagcgcaggatatccttatgtcgccttgggcatcaagaaaagggatatcctctccaagaagactaaagatctcaccaagctgagggaatgcatggacaagtatggtctaaatctgccgatggtgacctacgtgaaggatgaactcaggtccgctgagaaagtagccaagggaaaatccagacttatagaagcttctagtctcaatgactcagtggccatgaggcagacatttgggaacctatacaagacattccacctcaacccaggcattgtcactggtagtgctgttgggtgcgacccagatgtgttttggagcaaaatacccgtgatgcttgacgggcaccttatagcttttgattactctggctacgacgctagcttgagcccagtgtggtttgcttgtttgaaactcctcctagggaaactagggtatactcataaggaaaccaattacatagactacctctgcaactcccatcacttatacagagataaacactatttcgtgaggggtggtatgccatcaggatgttcaggcaccagtatattcaacaccatgatcaacaacatcattattaggacccttatgctaaaggtctacaaaggtattgacctggatcagtttagaatgatcgcttacggggacgatgtgatagcctcttacccgtggcctattgatgcctcactactagcagaagcgggaaaggattatggtttgatcatgaccccagcagataaaggagagtgttttaatgaggtaacctggacaaatgtaaccttcttgaaaaggtactttagagctgatgaacaatatccattcttggtgcaccccgtgatgcccatgaaagacatacacgaatccattagatggaccaaagacccaaagaacactcaagatcatgtgcgctcgttatgcctattggcttggcacaatggggagcacgaatatgaggaatttatccgaaagatcagaagcgtgcctgttggacgctgtttgaccctcccggtgttctcaacactacgcaggaaatggttagattccttcaattagagtgcaatcaatgaactatgattggcttaaccctaccgcatgaaccgaactagacaaaagtgcggtaggggtaaattctccgcattcggtgcgg

SEQ ID NO: 103 - RNA, 7101 nt, synthetic construct
  source 1..7101: mol_type = other RNA
  misc_feature 1..7101: note = nucleotide sequence coding modified coxachievirus B5
ttaaaacagcctgtgggttgtacccacccacagggcccactgggcgctagcactctggtatcacggtacctttgtgtgcctgttttatatcccctttccccgattgtaacttagaagatgtacacactgatcaatagcgggcatagcacaccagctatgtcttgatcaagcactcctgtatccccggaccaagtatcaatagactgctcacgcggttgaaggagaaaacgttcgtcacccggctaactacttcgagaaacccagtagtatcatgaaagttgcgaggcgtttcgttcagcacacccccagtgtagatcgggtcgatgagtcaccgcatcccccacgggcgaccgtggcggtggctgcgctggcggcctgcctacggggcaacccgtaggacgcttcaatacagacatggtgcgaagagtcgattgagctagttagtagtcctccggcccctgaatgcggctaatcctaactgcggagcacatgccctcaacccagggggtattgtgtcgtaacgggcaactctgcagcggaaccgactactttgggtgtccgtgtttccttttatccttatactggctgcttatggtgacaattgaaagattgttgccatatagctattggattggccatccagtgtctaatagagctgttatttacctctttgttggatttataccactcaacctaaaagaagttaaaacactacagctcattttacaactgaatacagcaaaatgggagctcaggtttcaacgcaaaaaactggagcacacgagaccggagtgagtgctagcggcaattccatcattcattacacaaatattaactactataaggatgctgcgtctaattcagctaaccggcaagaatttgctcaggatccaggtaagttcacagaaccagtaaaggatattatgattaagtcaatgccagccctcaattcgccatctgccgaggagtgtgggtacagtgacagggtgagatctattacgttgggaaactcaacaatcaccacgcaggagtgtgctaatgtggtggttggatatggcacatggcccacgtatctcaaagatgaagaggctacggcagaggatcaaccaactcaaccagacgtggcaacatgtagattctacaccttagagtccgtgatgtggcagcagagctcacctggatggtggtggaaattcccggacgccctttcaaacatgggtttgttcgggcaaaacatgcagtaccattatttagggagagctggatacactgtgcatgtacagtgcaacgcctccaaattccaccaaggatgcttgttggttgtgtgtgtgccagaggctgagatgggctgtgcaaccatagctaataagccagatcaaaagagcctgagtaatggagaaacagccaacacgtttgattcacaagacacgaccggacaaacagctgtgcaggctaacgtcattaacgcaggtatgggggtgggtgttggtaacctaaccatttttccacatcagtggatcaacctgcgaactaacaacagtgccacaattgttatgccatatataaatagtgtgccaatggataatatgttcagacacaacaacttcaccctaatgattataccttttgcaccattgagttatagcacgggcgcaaccacctacgtgcctattacggtgactgtggcgccaatgtgcgcagaatacaatggtttgcgattggcagggagacaagggttacccacaatgctaacacctggtagcagccaatttttgacctctgatgacttccagtcgccttccgccatgccacagttcgacgtgacgccagaaatggcaattcctgggcaggtgaataacttgatggagatcgcggaagttgattccgtggttccagttaacaatactgagggcaaagtatcatcaattgaagcgtaccaaatacctgtacaatcaaactcaactaatggctcacaagtatttgggtttcctctcatccccggcgccagtagtgtgctaaatagaacactcctgggtgagatccttaattattatacacattggtcaggaagcatcaaattgacatttatgttttgcgggtctgcaatggctaccggtaagtttctattggcttattcaccccctggtgctggtgcaccaacaaccaggaaagaagcaatgcttggaacacacgtcatctgggacgttgggttgcagtccagctgtgtgttatgcattccatggatcagtcaaacacattacagatatgtggtggtggacgagtacaccgctggagggtacatcacttgttggtaccagacaaatattgtggtacctgctgacacacaaagtggctgcaagatcttgtgttttgtatcagcatgcaacgacttttccgtgaggatgctaaaggacacaccttttataaagcaggacaactttttccaaggaccacccggggaagctgtcgaacgagcgattgctcgcgtggctgatactataagcagtggccctgttaattcagagtcaatcccgacactaacagcagcggagaccgggcacacatcccaggtggttccagcggacaccatgcaaaccaggcacgtgaagaattatcactcgcgatccgaatccacagtagagaacttcctgtgtagatccgcgtgtgtgtattacacaacctacaagaaccatggcactgatggagacaatttcgcctactgggtgatcaacacaagacaggtcgcgcagctgcgccgcaaattagaaatgtttacgtatgccagatttgacttagaactcacatttgtgataacaagcacacaagaacaatccaccatcaaaggtcaagattcgcctgtgttaactcatcaaataatgtatgtgcccccaggaggcccggtgcccaccaagattaacagctacagctggcaaacatcaactaacccaagtgtcttttggacagaggggagtgctcctccacgcatatctataccatttattagtattgggaatgcttacagtatgttctatgacgggtgggctaggtttgacaagcaagggacttatggtataaacaccttgaacaacatgggtaccctgtacatgcgtcacgtaaatgatgggagtccaggtcctatcgcgagcactgtacgcatttacttcaaacccaaacacgtgaaaacgtgggttcccagaccaccaaggctatgtcaatatcaaaaagcgggaaacgtcaactttgagccaacaggggtgacggagtctcgtactggaattacggcaatgcagaccaccggttcatgtgggcaacaatcaggagctgtgtacgtgggcaattacaggattgtaaacagacacctggcaacgagccacgattggcaaaattgcgtgtgggaggactacaacagggatctcctggtcagcacaacaactgctcatggttgtgatactatagcacggtgccaatgtactgctggcgtgtacttttgtgcatctagaaacaagcactacccagtgagcttcgagggtccaggtctagtgaaagttcaggagggcgagtactaccccgagagataccagtcgcacgtactccttgcagttggattttcagaaccgggtgattgtggaggtattttgaggtgtgaacatggagtcattgggctcgttaccatgggtggtgagggtgtagtaggcttcgctgacgtgcgggatcttttgtggttggaagacgacgccatggagcagaataacggttggttaaagaaattcactgaaatgaccaacgcctgcaagggcatggagtggattgctgttaaaattcaaaagttcatcgagtggctcaaagtaaagattctgcctgaagtgaaggagaaacatgagttccttaccagattgaagcaattgccactccttgaaagtcaaattgccaccattgagcaaagcgcaccctcacaaagtgatcaagagcagcttttttcgaatgttcagtacttcgcccattactgcaggaagtatgcacctctgtatgctgccgaagcaaaaagagtgttctcattagaaaagaaaatgagtaattacatacagttcaagtccaaatgccgcattgagcctgtatgcttactccttcacggtagtccaggggctggcaagtcagtagctaccaacctgatagggagatcccttgcagagaagctcaatagctctgtgtactctttaccaccagatccagatcattttgatgggtacaaacagcaggcagtggtgatcatggatgatctctgtcaaaaccccgatgggaaggacgtgtccttgttttgccaaatggtgtctagtgtagattttgtgccacccatggcggcgctggaagaaaaaggcattctctttacgtccccgtttgtgttggcatcaaccaacgcggggtccatcaatgcaccaacagtgtcagacagcagagcacttgccagaaggtttcactttgacatgaatattgaggtgatttcgatgtacagccagaatggtaaaattaacatgcccatgtctgttaagacatgtgatgatgaatgctgcccggtcaatttcaaaaagtgttgcccactagtgtgtggcaaggccatccagtttattgacaggagaaaccaagttagatattcactggacatgctggttactgagatgtttagagagtacaaccacagacacagtgtgggtgctaccctcgaggctttgttccaaggaccaccagtatacagggaaatcaaaatcagtgtggccccggaaacaccccctccaccagcaattgctgaccttctaaaatctgtagacagtgaggcaataagggagtactgcaaggaaaggggttggcttgtgccagaggtcagctccactctacaaattgaaaaacatgttagcagggcatttatttgcttgcaagcgctaactacatttgtttcagtggctggtataatctacatcatttacaagttgtttgccggctttcagggtgcatacactggaatgcccaaccagaaacccaaggtgcccaccttaagacaagctaaggtgcaaggtccggcatttgaatttgccgtagcaatgatgaaaaggaacgccagcacagtcaagacagaatacggtgagttcacgatgcttggcatctatgataaatgggcagtgctgccgcgccacgccaagcctggaccaactattttaatgaatgatcaggaggttggtgtgctcgatgccaaagagttagttgataaagacggaaccaacctggagctgacactattgaagcttaaccgcaatgaaaagttcagagacatcagaggttttcttgcaagggaagaagttgaggtaagtgaggctgttttggcaataaacacgagcaagttcccaagcatgtacatccctgtgggccaagtcaccgattacggatttttaaatctaggtggcaccccaacaaagagaatgctcatgtacaacttccctaccagagcgggacagtgtggtggtgtccttatgtcaacaggaaaggtccttggcatacacgtgggaggaaatggtcaccaaggcttctctgctgctctcctcagacactacttcaacgaggaacagggcgaaatagagtttattgagagctctaaagatgcaggatttcctgtgatcaacacccctaataaaaccaaactggaaccaagtgtgtttcatcaggtttttgagggcaacaaagaaccagcagtcctaagaaacggagacccgcgacttaaagccaactttgaggaagcgatattttccaagtacatcggaaatgtgaacacacatgtggacgagtacatgatagaagctgttgatcactacgctggacagctggcaactctggacatcagtacagaacctatgaagcttgaggatgctgtttatggcactgaaggcttggaagcattggacttgaccactagcgcaggatatccttatgtcgccttgggcatcaagaaaagggatatcctctccaagaagactaaagatctcaccaagctgagggaatgcatggacaagtatggtctaaatctgccgatggtgacctacgtgaaggatgaactcaggtccgctgagaaagtagccaagggaaaatccagacttatagaagcttctagtctcaatgactcagtggccatgaggcagacatttgggaacctatacaagacattccacctcaacccaggcattgtcactggtagtgctgttgggtgcgacccagatgtgttttggagcaaaatacccgtgatgcttgacgggcaccttatagcttttgattactctggctacgacgctagcttgagcccagtgtggtttgcttgtttgaaactcctcctagggaaactagggtatactcataaggaaaccaattacatagactacctctgcaactcccatcacttatacagagataaacactatttcgtgaggggtggtatgccatcaggatgttcaggcaccagtatattcaacaccatgatcaacaacatcattattaggacccttatgctaaaggtctacaaaggtattgacctggatcagtttagaatgatcgcttacggggacgatgtgatagcctcttacccgtggcctattgatgcctcactactagcagaagcgggaaaggattatggtttgatcatgaccccagcagataaaggagagtgttttaatgaggtaacctggacaaatgtaaccttcttgaaaaggtactttagagctgatgaacaatatccattcttggtgcaccccgtgatgcccatgaaagacatacacgaatccattagatggaccaaagacccaaagaacactcaagatcatgtgcgctcgttatgcctattggcttggcacaatggggagcacgaatatgaggaatttatccgaaagatcagaagcgtgcctgttggacgctgtttgaccctcccggtgttctcaacactacgcaggaaatggttagattccttcaattagagtgcaatcaatgaactatgattggcttaaccctaccgcatgaaccgaactagacaaaagtgcggtaggggtaaattctccgcattcggtgcgg

SEQ ID NO: 104 - protein, 2087 aa, synthetic construct
  REGION 1..2087: note = modified coxachievirus B5
MGAQVSTQKTGAHETGVSASGNSIIHYTNINYYKDAASNSANRQEFAQDPGKFTEPVKDIMIKSMPALNSPSAEECGYSDRVRSITLGNSTITTQECANVVVGYGTWPTYLKDEEATAEDQPTQPDVATCRFYTLESVMWQQSSPGWWWKFPDALSNMGLFGQNMQYHYLGRAGYTVHVQCNASKFHQGCLLVVCVPEAEMGCATIANKPDQKSLSNGETANTFDSQDTTGQTAVQANVINAGMGVGVGNLTIFPHQWINLRTNNSATIVMPYINSVPMDNMFRHNNFTLMIIPFAPLSYSTGATTYVPITVTVAPMCAEYNGLRLAGRQGLPTMLTPGSSQFLTSDDFQSPSAMPQFDVTPEMAIPGQVNNLMEIAEVDSVVPVNNTEGKVSSIEAYQIPVQSNSTNGSQVFGFPLIPGASSVLNRTLLGEILNYYTHWSGSIKLTFMFCGSAMATGKFLLAYSPPGAGAPTTRKEAMLGTHVIWDVGLQSSCVLCIPWISQTHYRYVVVDEYTAGGYITCWYQTNIVVPADTQSGCKILCFVSACNDFSVRMLKDTPFIKQDNFFQGPPGEAVERAIARVADTISSGPVNSESIPTLTAAETGHTSQVVPADTMQTRHVKNYHSRSESTVENFLCRSACVYYTTYKNHGTDGDNFAYWVINTRQVAQLRRKLEMFTYARFDLELTFVITSTQEQSTIKGQDSPVLTHQIMYVPPGGPVPTKINSYSWQTSTNPSVFWTEGSAPPRISIPFISIGNAYSMFYDGWARFDKQGTYGINTLNNMGTLYMRHVNDGSPGPIASTVRIYFKPKHVKTWVPRPPRLCQYQKAGNVNFEPTGVTESRTGITAMQTTGSCGQQSGAVYVGNYRIVNRHLATSHDWQNCVWEDYNRDLLVSTTTAHGCDTIARCQCTAGVYFCASRNKHYPVSFEGPGLVKVQEGEYYPERYQSHVLLAVGFSEPGDCGGILRCEHGVIGLVTMGGEGVVGFADVRDLLWLEDDAMEQNNGWLKKFTEMTNACKGMEWIAVKIQKFIEWLKVKILPEVKEKHEFLTRLKQLPLLESQIATIEQSAPSQSDQEQLFSNVQYFAHYCRKYAPLYAAEAKRVFSLEKKMSNYIQFKSKCRIEPVCLLLHGSPGAGKSVATNLIGRSLAEKLNSSVYSLPPDPDHFDGYKQQAVVIMDDLCQNPDGKDVSLFCQMVSSVDFVPPMAALEEKGILFTSPFVLASTNAGSINAPTVSDSRALARRFHFDMNIEVISMYSQNGKINMPMSVKTCDDECCPVNFKKCCPLVCGKAIQFIDRRNQVRYSLDMLVTEMFREYNHRHSVGATLEALFQGPPVYREIKISVAPETPPPPAIADLLKSVDSEAIREYCKERGWLVPEVSSTLQIEKHVSRAFICLQALTTFVSVAGIIYIIYKLFAGFQGAYTGMPNQKPKVPTLRQAKVQGPAFEFAVAMMKRNASTVKTEYGEFTMLGIYDKWAVLPRHAKPGPTILMNDQEVGVLDAKELVDKDGTNLELTLLKLNRNEKFRDIRGFLAREEVEVSEAVLAINTSKFPSMYIPVGQVTDYGFLNLGGTPTKRMLMYNFPTRAGQCGGVLMSTGKVLGIHVGGNGHQGFSAALLRHYFNEEQGEIEFIESSKDAGFPVINTPNKTKLEPSVFHQVFEGNKEPAVLRNGDPRLKANFEEAIFSKYIGNVNTHVDEYMIEAVDHYAGQLATLDISTEPMKLEDAVYGTEGLEALDLTTSAGYPYVALGIKKRDILSKKTKDLTKLRECMDKYGLNLPMVTYVKDELRSAEKVAKGKSRLIEASSLNDSVAMRQTFGNLYKTFHLNPGIVTGSAVGCDPDVFWSKIPVMLDGHLIAFDYSGYDASLSPVWFACLKLLLGKLGYTHKETNYIDYLCNSHHLYRDKHYFVRGGMPSGCSGTSIFNTMINNIIIRTLMLKVYKGIDLDQFRMIAYGDDVIASYPWPIDASLLAEAGKDYGLIMTPADKGECFNEVTWTNVTFLKRYFRADEQYPFLVHPVMPMKDIHESIRWTKDPKNTQDHVRSLCLLAWHNGEHEYEEFIRKIRSVPVGRCLTLPVFSTLRRKWLDSFN

SEQ ID NO: 105 - protein, 564 aa, synthetic construct
  REGION 1..564: note = H5N8 antigen
MEKIVLLLAVVSLVKSDQICIGYHANNSTKQVDTIMEKNVTVTHAQDILEKTHNGKLCDLNGVKPLILKDCSVAGWLLGNPMCDEFIRVPEWSYIVERANPANDLCYPGTLNDYEELKHLLSRINHFEKTLIIPKSSWPNHETSLGVSAACPYQGAPSFFRNVVWLIKKNDAYPTIKISYNNTNREDLLILWGIHHSNNAAEQTNLYKNPDTYVSVGTSTLNQRLVPKIATRSQVNGQRGRMDFFWTILKPNDAIHFESNGNFIAPEYAYKIVKKGDSTIMKSEMEYGHCNTKCQTPIGAINSSMPFHNIHPLTIGECPKYVKSNKLVLATGLRNSPLRETVGLFGAIAGFIEGGWQGMVDGWYGYHHSNEQGSGYAADKESTQKAIDGVTNKVNSIIDKMNTQFEAVGREFNNLERRIENLNKKMEDGFLDVWTYNAELLVLMENERTLDFHDSNVKNLYDKVRLQLRDNAKELGNGCFEFYHKCDNECMESVRNGTYDYPKYSEEARLKREEISGVKLESIGTYQILSIYSTVASSLALAIIVAGLSLWMCSNGSLQCRICI

SEQ ID NO: 106 - DNA, 1692 bp, synthetic construct
  source 1..1692: mol_type = other DNA
  misc_feature 1..1692: note = nucleotide sequence coding H5N8 antigen
atggaaaagatcgtgctgctgctggccgtggtgtccctggtcaaaagcgaccagatctgcatcggctaccacgccaacaacagcaccaaacaggtggacaccatcatggaaaaaaacgtgaccgtgacacacgcccaggacatcctggaaaagacccacaacggcaagctgtgcgacctgaacggcgtgaagcctctgatcctgaaggactgttctgtggccggatggctgctgggcaaccctatgtgtgacgagttcatcagagtgcccgagtggtcctacatcgtggaaagagctaaccccgccaacgacctgtgctaccctggcacactgaacgactacgaggaactgaagcacctcctgagcagaatcaaccacttcgagaaaaccctgatcatccccaagagcagctggcccaaccacgagacatctctgggagtgtctgccgcatgtccataccagggcgctcccagcttcttcagaaacgtcgtgtggctgatcaagaagaacgacgcttaccccaccatcaagatcagctacaacaacaccaaccgcgaggacctgctgatcctgtggggaatccaccactctaacaacgccgccgagcagaccaacctgtacaagaaccctgacacctacgtgtccgtgggcacaagcaccctgaaccagagactggtgcccaagatcgccaccagatctcaagtgaacggccagaggggcagaatggacttcttctggaccatcctgaagcctaacgacgccatccactttgagagcaacggcaactttatcgcccctgagtacgcctacaagatcgtgaagaagggcgacagcacaatcatgaagtccgagatggaatacggccactgcaacaccaagtgtcagacccctatcggcgccatcaactccagcatgcccttccacaacatccatcctctgaccatcggcgagtgccccaaatacgtgaagtccaacaagctggtgctggccaccggcctgagaaactctccactgagagagacggtaggcctgtttggcgctatcgccggctttattgaaggcggctggcaaggcatggtggacggatggtacggctatcaccacagcaacgagcaaggctctggctacgccgctgacaaagagagcacccagaaagccatcgacggcgtgaccaacaaagtgaacagcatcatcgacaagatgaacacccagttcgaggccgtgggcagagagttcaacaacctggaaagaaggatcgagaacctcaacaagaaaatggaagatggcttcctggacgtgtggacctacaacgctgagctgctggtcctgatggaaaacgagagaaccctggacttccacgacagcaacgtgaagaacctgtacgacaaagtgcggctgcagctgagagacaacgccaaagaactcggcaacggctgcttcgagttctaccacaagtgcgacaacgagtgcatggaaagcgtgcggaacggcacctacgactaccccaagtacagcgaggaagccagactgaagagagaagagatcagcggagtgaagctggaatccatcggcacataccagatcctgagcatctacagcaccgtggcctcttctctggccctggctatcattgtggctggcctgagcctgtggatgtgcagcaatggcagcctgcagtgcagaatctgcatc

SEQ ID NO: 107 - RNA, 1692 nt, synthetic construct
  source 1..1692: mol_type = other RNA
  misc_feature 1..1692: note = nucleotide sequence coding H5N8 antigen
atggaaaagatcgtgctgctgctggccgtggtgtccctggtcaaaagcgaccagatctgcatcggctaccacgccaacaacagcaccaaacaggtggacaccatcatggaaaaaaacgtgaccgtgacacacgcccaggacatcctggaaaagacccacaacggcaagctgtgcgacctgaacggcgtgaagcctctgatcctgaaggactgttctgtggccggatggctgctgggcaaccctatgtgtgacgagttcatcagagtgcccgagtggtcctacatcgtggaaagagctaaccccgccaacgacctgtgctaccctggcacactgaacgactacgaggaactgaagcacctcctgagcagaatcaaccacttcgagaaaaccctgatcatccccaagagcagctggcccaaccacgagacatctctgggagtgtctgccgcatgtccataccagggcgctcccagcttcttcagaaacgtcgtgtggctgatcaagaagaacgacgcttaccccaccatcaagatcagctacaacaacaccaaccgcgaggacctgctgatcctgtggggaatccaccactctaacaacgccgccgagcagaccaacctgtacaagaaccctgacacctacgtgtccgtgggcacaagcaccctgaaccagagactggtgcccaagatcgccaccagatctcaagtgaacggccagaggggcagaatggacttcttctggaccatcctgaagcctaacgacgccatccactttgagagcaacggcaactttatcgcccctgagtacgcctacaagatcgtgaagaagggcgacagcacaatcatgaagtccgagatggaatacggccactgcaacaccaagtgtcagacccctatcggcgccatcaactccagcatgcccttccacaacatccatcctctgaccatcggcgagtgccccaaatacgtgaagtccaacaagctggtgctggccaccggcctgagaaactctccactgagagagacggtaggcctgtttggcgctatcgccggctttattgaaggcggctggcaaggcatggtggacggatggtacggctatcaccacagcaacgagcaaggctctggctacgccgctgacaaagagagcacccagaaagccatcgacggcgtgaccaacaaagtgaacagcatcatcgacaagatgaacacccagttcgaggccgtgggcagagagttcaacaacctggaaagaaggatcgagaacctcaacaagaaaatggaagatggcttcctggacgtgtggacctacaacgctgagctgctggtcctgatggaaaacgagagaaccctggacttccacgacagcaacgtgaagaacctgtacgacaaagtgcggctgcagctgagagacaacgccaaagaactcggcaacggctgcttcgagttctaccacaagtgcgacaacgagtgcatggaaagcgtgcggaacggcacctacgactaccccaagtacagcgaggaagccagactgaagagagaagagatcagcggagtgaagctggaatccatcggcacataccagatcctgagcatctacagcaccgtggcctcttctctggccctggctatcattgtggctggcctgagcctgtggatgtgcagcaatggcagcctgcagtgcagaatctgcatc

SEQ ID NO: 108 - DNA, 34 bp, synthetic construct
  source 1..34: mol_type = other DNA
  misc_feature 1..34: note = universal primer F
agtctagactccgtcttaaaacagcctgtgggtt

SEQ ID NO: 109 - DNA, 23 bp, synthetic construct
  source 1..23: mol_type = other DNA
  misc_feature 1..23: note = universal primer R
gctgggaccatgccggccttttt

SEQ ID NO: 110 - RNA, 6146 nt, synthetic construct
  source 1..6146: mol_type = other RNA
  misc_feature 1..6146: note = H5N8 mRNA construct
gagaataaactagtattcttctggtccccacagactcaatggaaaagatcgtgctgctgctggccgtggtgtccctggtcaaaagcgaccagatctgcatcggctaccacgccaacaacagcaccaaacaggtggacaccatcatggaaaaaaacgtgaccgtgacacacgcccaggacatcctggaaaagacccacaacggcaagctgtgcgacctgaacggcgtgaagcctctgatcctgaaggactgttctgtggccggatggctgctgggcaaccctatgtgtgacgagttcatcagagtgcccgagtggtcctacatcgtggaaagagctaaccccgccaacgacctgtgctaccctggcacactgaacgactacgaggaactgaagcacctcctgagcagaatcaaccacttcgagaaaaccctgatcatccccaagagcagctggcccaaccacgagacatctctgggagtgtctgccgcatgtccataccagggcgctcccagcttcttcagaaacgtcgtgtggctgatcaagaagaacgacgcttaccccaccatcaagatcagctacaacaacaccaaccgcgaggacctgctgatcctgtggggaatccaccactctaacaacgccgccgagcagaccaacctgtacaagaaccctgacacctacgtgtccgtgggcacaagcaccctgaaccagagactggtgcccaagatcgccaccagatctcaagtgaacggccagaggggcagaatggacttcttctggaccatcctgaagcctaacgacgccatccactttgagagcaacggcaactttatcgcccctgagtacgcctacaagatcgtgaagaagggcgacagcacaatcatgaagtccgagatggaatacggccactgcaacaccaagtgtcagacccctatcggcgccatcaactccagcatgcccttccacaacatccatcctctgaccatcggcgagtgccccaaatacgtgaagtccaacaagctggtgctggccaccggcctgagaaactctccactgagagagacggtaggcctgtttggcgctatcgccggctttattgaaggcggctggcaaggcatggtggacggatggtacggctatcaccacagcaacgagcaaggctctggctacgccgctgacaaagagagcacccagaaagccatcgacggcgtgaccaacaaagtgaacagcatcatcgacaagatgaacacccagttcgaggccgtgggcagagagttcaacaacctggaaagaaggatcgagaacctcaacaagaaaatggaagatggcttcctggacgtgtggacctacaacgctgagctgctggtcctgatggaaaacgagagaaccctggacttccacgacagcaacgtgaagaacctgtacgacaaagtgcggctgcagctgagagacaacgccaaagaactcggcaacggctgcttcgagttctaccacaagtgcgacaacgagtgcatggaaagcgtgcggaacggcacctacgactaccccaagtacagcgaggaagccagactgaagagagaagagatcagcggagtgaagctggaatccatcggcacataccagatcctgagcatctacagcaccgtggcctcttctctggccctggctatcattgtggctggcctgagcctgtggatgtgcagcaatggcagcctgcagtgcagaatctgcatcaactttgagccaacaggggtgacggagtcccgcactgaaattacggcaatgcagaccaccggttcatgtgggcaacaatcaggagctgtgtacgtgggcaattacaggattgtaaacagacacctggcaacgagccacgattggcaaaattgcgtgtgggaggactacaacagggatctcctggtcagcacaacaactgctcatggttgtgatactatagcacggtgccaatgtactgctggcgtgtacttttgtgcatctagaaacaagcactacccagtgagcttcgagggtccaggtctagtgaaagttcaggagggcgagtactaccccgagagataccagtcgcacgtactccttgcagttggattttcagaaccgggtgattgtggaggtattttgaggtgtgaacatggagtcattgggctcgttaccatgggtggtgagggtgtagtaggcttcgctgacgtgcgggatcttttgtggttggaagacgacgccatggagcagggtgttagagattatgtagagcaactgggaaatgcatttggctcaggtttcactaaccaaatctgtgagcaagttaacctccttaaagaatctctgatagggcaggattccatattggaaaaatccctgaaggccctggttaaaatcatatcagccctggtgatagtggttaggaaccacgacgacctgattacagtgactgccacactagctttaatcggttgcgcatcatctccatggcgatggctcaaacaaaaagtgtgtcaatactacggaatccccatggcagaaaggcagaataacggttggttaaagaaattcactgaaatgaccaacgcctgcaagggcatggagtggattgctgttaaaattcaaaagttcatcgagtggctcaaagtaaagattctgcctgaagtgaaggagaaacatgagttccttaccagattgaagcaattgccactccttgaaagtcaaattgccaccattgagcaaagcgcaccctcacaaagtgatcaagagcagcttttttcgaatgttcagtacttcgcccattactgcaggaagtatgcacctctgtatgctgccgaagcaaaaagagtgttctcattagaaaagaaaatgagtaattacatacagttcaagtccaaatgccgcattgagcctgtatgcttactccttcacggtagtccaggggctggcaagtcagtagctaccaacctgatagggagatcccttgcagagaagctcaatagctctgtgtactctttaccaccagatccagatcattttgatgggtacaaacagcaggcagtggtgatcatggatgatctctgtcaaaaccccgatgggaaggacgtgtccttgttttgccaaatggtgtctagtgtagattttgtgccacccatggcggcgctggaagaaaaaggcattctctttacgtccccgtttgtgttggcatcaaccaacgcggggtccatcaatgcaccaacagtgtcagacagcagagcacttgccagaaggtttcactttgacatgaatattgaggtgatttcgatgtacagccagaatggtaaaattaacatgcccatgtctgttaagacatgtgatgatgaatgctgcccggtcaatttcaaaaagtgttgcccactagtgtgtggcaaggccatccagtttattgacaggagaaaccaagttagatattcactggacatgctggttactgagatgtttagagagtacaaccacagacacagtgtgggtgctaccctcgaggctttgttccaaggaccaccagtatacagggaaatcaaaatcagtgtggccccggaaacaccccctccaccagcaattgctgaccttctaaaatctgtagacagtgaggcaataagggagtactgcaaggaaaggggttggcttgtgccagaggtcagctccactctacaaattgaaaaacatgttagcagggcatttatttgcttgcaagcgctaactacatttgtttcagtggctggtataatctacatcatttacaagttgtttgccggctttcagggtgcatacactggaatgcccaaccagaaacccaaggtgcccaccttaagacaagctaaggtgcaaggtccggcatttgaatttgccgtagcaatgatgaaaaggaacgccagcacagtcaagacagaatacggtgagttcacgatgcttggcatctatgataaatgggcagtgctgccgcgccacgccaagcctggaccaactattttaatgaatgatcaggaggttggtgtgctcgatgccaaagagttagttgataaagacggaaccaacctggagctgacactattgaagcttaaccgcaatgaaaagttcagagacatcagaggttttcttgcaagggaagaagttgaggtaagtgaggctgttttggcaataaacacgagcaagttcccaagcatgtacatccctgtgggccaagtcaccgattacggatttttaaatctaggtggcaccccaacaaagagaatgctcatgtacaacttccctaccagagcgggacagtgtggtggtgtccttatgtcaacaggaaaggtccttggcatacacgtgggaggaaatggtcaccaaggcttctctgctgctctcctcagacactacttcaacgaggaacagggcgaaatagagtttattgagagctctaaagatgcaggatttcctgtgatcaacacccctaataaaaccaaactggaaccaagtgtgtttcatcaggtttttgagggcaacaaagaaccagcagtcctaagaaacggagacccgcgacttaaagccaactttgaggaagcgatattttccaagtacatcggaaatgtgaacacacatgtggacgagtacatgatagaagctgttgatcactacgctggacagctggcaactctggacatcagtacagaacctatgaagcttgaggatgctgtttatggcactgaaggcttggaagcattggacttgaccactagcgcaggatatccttatgtcgccttgggcatcaagaaaagggatatcctctccaagaagactaaagatctcaccaagctgagggaatgcatggacaagtatggtctaaatctgccgatggtgacctacgtgaaggatgaactcaggtccgctgagaaagtagccaagggaaaatccagacttatagaagcttctagtctcaatgactcagtggccatgaggcagacatttgggaacctatacaagacattccacctcaacccaggcattgtcactggtagtgctgttgggtgcgacccagatgtgttttggagcaaaatacccgtgatgcttgacgggcaccttatagcttttgattactctggctacgacgctagcttgagcccagtgtggtttgcttgtttgaaactcctcctagggaaactagggtatactcataaggaaaccaattacatagactacctctgcaactcccatcacttatacagagataaacactatttcgtgaggggtggtatgccatcaggatgttcaggcaccagtatattcaacaccatgatcaacaacatcattattaggacccttatgctaaaggtctacaaaggtattgacctggatcagtttagaatgatcgcttacggggacgatgtgatagcctcttacccgtggcctattgatgcctcactactagcagaagcgggaaaggattatggtttgatcatgaccccagcagataaaggagagtgttttaatgaggtaacctggacaaatgtaaccttcttgaaaaggtactttagagctgatgaacaatatccattcttggtgcaccccgtgatgcccatgaaagacatacacgaatccattagatggaccaaagacccaaagaacactcaagatcatgtgcgctcgttatgcctattggcttggcacaatggggagcacgaatatgaggaatttatccgaaagatcagaagcgtgcctgttggacgctgtttgaccctcccggtgttctcaacactacgcaggaaatggttagattccttctgataatagctcgagctggtactgcatgcacgcaatgctagctgcccctttcccgtcctgggtaccccgagtctcccccgacctcgggtcccaggtatgctcccacctccacctgccccactcaccacctctgctagttccagacacctcccaagcacgcagcaatgcagctcaaaacgcttagcctagccacacccccacgggaaacagcagtgattaacctttagcaataaacgaaagtttaactaagctatactaaccccagggttggtcaatttcgtgccagccacaccctggagctagcaaaaaaaaaaaaaaaaaaaaaaaaaaaaaaaaaaaaaaaaaaaaaaaaaa

SEQ ID NO: 111 - RNA, 6731 nt, synthetic construct
  source 1..6731: mol_type = other RNA
  misc_feature 1..6713: note = H5N8 saRNA construct
ttaaaacagcctgtgggttgtacccacccacagggcccactgggcgctagcactctggtatcacggtacctttgtgtgcctgttttatatcccctttccccgattgtaacttagaagatgtacacactgatcaatagcgggcatagcacaccagctatgtcttgatcaagcactcctgtatccccggaccaagtatcaatagactgctcacgcggttgaaggagaaaacgttcgttacccggctaactacttcgagaaacccagtagtatcatgaaagttgcgaggcgtttcgttcagcacacccccagtgtagatcgggtcgatgagtcaccgcatcccccacgggcgaccgtggcggtggctgcgctggcggcctgcctacggggcaacccgtaggacgcttcaatacagacatggtgcgaagagtcgattgagctagttagtagtcctccggcccctgaatgcggctaatcctaactgcggagcacatgccctcaacccagggggtattgtgtcgtaacgggcaactctgcagcggaaccgactactttgggtgtccgtgtttccttttatccttatactggctgcttatggtgacaattgaaagattgttgccatatagctattggattggccatccagtgtctaatagagctgttatttacctctttgttggatttataccactcaacctaaaagaagttaaaacactacagctcattttacaactgaatacagcaaaccaccatggaaaagatcgtgctgctgctggccgtggtgtccctggtcaaaagcgaccagatctgcatcggctaccacgccaacaacagcaccaaacaggtggacaccatcatggaaaaaaacgtgaccgtgacacacgcccaggacatcctggaaaagacccacaacggcaagctgtgcgacctgaacggcgtgaagcctctgatcctgaaggactgttctgtggccggatggctgctgggcaaccctatgtgtgacgagttcatcagagtgcccgagtggtcctacatcgtggaaagagctaaccccgccaacgacctgtgctaccctggcacactgaacgactacgaggaactgaagcacctcctgagcagaatcaaccacttcgagaaaaccctgatcatccccaagagcagctggcccaaccacgagacatctctgggagtgtctgccgcatgtccataccagggcgctcccagcttcttcagaaacgtcgtgtggctgatcaagaagaacgacgcttaccccaccatcaagatcagctacaacaacaccaaccgcgaggacctgctgatcctgtggggaatccaccactctaacaacgccgccgagcagaccaacctgtacaagaaccctgacacctacgtgtccgtgggcacaagcaccctgaaccagagactggtgcccaagatcgccaccagatctcaagtgaacggccagaggggcagaatggacttcttctggaccatcctgaagcctaacgacgccatccactttgagagcaacggcaactttatcgcccctgagtacgcctacaagatcgtgaagaagggcgacagcacaatcatgaagtccgagatggaatacggccactgcaacaccaagtgtcagacccctatcggcgccatcaactccagcatgcccttccacaacatccatcctctgaccatcggcgagtgccccaaatacgtgaagtccaacaagctggtgctggccaccggcctgagaaactctccactgagagagacggtaggcctgtttggcgctatcgccggctttattgaaggcggctggcaaggcatggtggacggatggtacggctatcaccacagcaacgagcaaggctctggctacgccgctgacaaagagagcacccagaaagccatcgacggcgtgaccaacaaagtgaacagcatcatcgacaagatgaacacccagttcgaggccgtgggcagagagttcaacaacctggaaagaaggatcgagaacctcaacaagaaaatggaagatggcttcctggacgtgtggacctacaacgctgagctgctggtcctgatggaaaacgagagaaccctggacttccacgacagcaacgtgaagaacctgtacgacaaagtgcggctgcagctgagagacaacgccaaagaactcggcaacggctgcttcgagttctaccacaagtgcgacaacgagtgcatggaaagcgtgcggaacggcacctacgactaccccaagtacagcgaggaagccagactgaagagagaagagatcagcggagtgaagctggaatccatcggcacataccagatcctgagcatctacagcaccgtggcctcttctctggccctggctatcattgtggctggcctgagcctgtggatgtgcagcaatggcagcctgcagtgcagaatctgcatcaactttgagccaacaggggtgacggagtcccgcactgaaattacggcaatgcagaccaccggttcatgtgggcaacaatcaggagctgtgtacgtgggcaattacaggattgtaaacagacacctggcaacgagccacgattggcaaaattgcgtgtgggaggactacaacagggatctcctggtcagcacaacaactgctcatggttgtgatactatagcacggtgccaatgtactgctggcgtgtacttttgtgcatctagaaacaagcactacccagtgagcttcgagggtccaggtctagtgaaagttcaggagagcgagtactaccccgagagataccagtcgcacgtactccttgcagttggattttcagaaccgggtgattgtggaggtattttgaggtgtgaacatggagtcattgggctcgttaccatgggtggtgagggtgtagtaggcttcgctgacgtgcgggatcttttgtggttggaagacgacgccatggagcagggtgttagagattatgtagagcaactgggaaatgcatttggctcaggtttcactaaccaaatctgtgagcaagttaacctccttaaagaatctctgatagggcaggattccatattggaaaaatccctgaaggccctggttaaaatcatatcagccctggtgatagtggttaggaaccacgacgacctgattacagtgactgccacactagctttaatcggttgcgcatcatctccatggcgatggctcaaacaaaaagtgtgtcaatactacggaatccccatggcagaaaggcagaataacggttggttaaagaaattcactgaaatgaccaacgcctgcaagggcatggagtggattgctgttaaaattcaaaagttcatcgagtggctcaaagtaaagattctgcctgaagtgaaggagaaacatgagttccttaccagattgaagcaattgccactccttgaaagtcaaattgccaccattgagcaaagcgcaccctcacaaagtgatcaagagcagcttttttcgaatgttcagtacttcgcccattactgcaggaagtatgcacctctgtatgctgccgaagcaaaaagagtgttctcattagaaaagaaaatgagtaattacatacagttcaagtccaaatgccgcattgagcctgtatgcttactccttcacggtagtccaggggctggcaagtcagtagctaccaacctgatagggagatcccttgcagagaagctcaatagctctgtgtactctttaccaccagatccagatcattttgatgggtacaaacagcaggcagtggtgatcatggatgatctctgtcaaaaccccgatgggaaggacgtgtccttgttttgccaaatggtgtctagtgtagattttgtgccacccatggcggcgctggaagaaaaaggcattctctttacgtccccgtttgtgttggcatcaaccaacgcggggtccatcaatgcaccaacagtgtcagacagcagagcacttgccagaaggtttcactttgacatgaatattgaggtgatttcgatgtacagccagaatggtaaaattaacatgcccatgtctgttaagacatgtgatgatgaatgctgcccggtcaatttcaaaaagtgttgcccactagtgtgtggcaaggccatccagtttattgacaggagaaaccaagttagatattcactggacatgctggttactgagatgtttagagagtacaaccacagacacagtgtgggtgctaccctcgaggctttgttccaaggaccaccagtatacagggaaatcaaaatcagtgtggccccggaaacaccccctccaccagcaattgctgaccttctaaaatctgtagacagtgaggcaataagggagtactgcaaggaaaggggttggcttgtgccagaggtcagctccactctacaaattgaaaaacatgttagcagggcatttatttgcttgcaagcgctaactacatttgtttcagtggctggtataatctacatcatttacaagttgtttgccggctttcagggtgcatacactggaatgcccaaccagaaacccaaggtgcccaccttaagacaagctaaggtgcaaggtccggcatttgaatttgccgtagcaatgatgaaaaggaacgccagcacagtcaagacagaatacggtgagttcacgatgcttggcatctatgataaatgggcagtgctgccgcgccacgccaagcctggaccaactattttaatgaatgatcaggaggttggtgtgctcgatgccaaagagttagttgataaagacggaaccaacctggagctgacactattgaagcttaaccgcaatgaaaagttcagagacatcagaggttttcttgcaagggaagaagttgaggtaagtgaggctgttttggcaataaacacgagcaagttcccaagcatgtacatccctgtgggccaagtcaccgattacggatttttaaatctaggtggcaccccaacaaagagaatgctcatgtacaacttccctaccagagcgggacagtgtggtggtgtccttatgtcaacaggaaaggtccttggcatacacgtgggaggaaatggtcaccaaggcttctctgctgctctcctcagacactacttcaacgaggaacagggcgaaatagagtttattgagagctctaaagatgcaggatttcctgtgatcaacacccctaataaaaccaaactggaaccaagtgtgtttcatcaggtttttgagggcaacaaagaaccagcagtcctaagaaacggagacccgcgacttaaagccaactttgaggaagcgatattttccaagtacatcggaaatgtgaacacacatgtggacgagtacatgatagaagctgttgatcactacgctggacagctggcaactctggacatcagtacagaacctatgaagcttgaggatgctgtttatggcactgaaggcttggaagcattggacttgaccactagcgcaggatatccttatgtcgccttgggcatcaagaaaagggatatcctctccaagaagactaaagatctcaccaagctgagggaatgcatggacaagtatggtctaaatctgccgatggtgacctacgtgaaggatgaactcaggtccgctgagaaagtagccaagggaaaatccagacttatagaagcttctagtctcaatgactcagtggccatgaggcagacatttgggaacctatacaagacattccacctcaacccaggcattgtcactggtagtgctgttgggtgcgacccagatgtgttttggagcaaaatacccgtgatgcttgacgggcaccttatagcttttgattactctggctacgacgctagcttgagcccagtgtggtttgcttgtttgaaactcctcctagggaaactagggtatactcataaggaaaccaattacatagactacctctgcaactcccatcacttatacagagataaacactatttcgtgaggggtggtatgccatcaggatgttcaggcaccagtatattcaacaccatgatcaacaacatcattattaggacccttatgctaaaggtctacaaaggtattgacctggatcagtttagaatgatcgcttacggggacgatgtgatagcctcttacccgtggcctattgatgcctcactactagcagaagcgggaaaggattatggtttgatcatgaccccagcagataaaggagagtgttttaatgaggtaacctggacaaatgtaaccttcttgaaaaggtactttagagctgatgaacaatatccattcttggtgcaccccgtgatgcccatgaaagacatacacgaatccattagatggaccaaagacccaaagaacactcaagatcatgtgcgctcgttatgcctattggcttggcacaatggggagcacgaatatgaggaatttatccgaaagatcagaagcgtgcctgttggacgctgtttgaccctcccggtgttctcaacactacgcaggaaatggttagattccttctgataatagaattagagtgcaatcaatgaactatgattggcttaaccctaccgcatgaaccgaactagacaaaagtgcggtaggggtaaattctccgcattcggtgcggaaaaaaaaaaaaaaaaaaaaaaaaaaaaaaaaaaaaaaaaaaaaaaaaaaaaaaaaaaaaaaaaaaaaaaaaaaaaaaaaaaaaaaaaaaaaaaaaaaaaaaaaaaaaaaaaaaaaaaaa

SEQ ID NO: 112 - RNA, 8255 nt, synthetic construct
  source 1..8255: mol_type = other RNA
  misc_feature 1..8255: note = SFTS A saRNA construct
ttaaaacagcctgtgggttgtacccacccacagggcccactgggcgctagcactctggtatcacggtacctttgtgtgcctgttttatatcccctttccccgattgtaacttagaagatgtacacactgatcaatagcgggcatagcacaccagctatgtcttgatcaagcactcctgtatccccggaccaagtatcaatagactgctcacgcggttgaaggagaaaacgttcgtcacccggctaactacttcgagaaacccagtagtatcatgaaagttgcgaggcgtttcgttcagcacacccccagtgtagatcgggtcgatgagtcaccgcatcccccacgggcgaccgtggcggtggctgcgctggcggcctgcctacggggcaacccgtaggacgcttcaatacagacatggtgcgaagagtcgattgagctagttagtagtcctccggcccctgaatgcggctaatcctaactgcggagcacatgccctcaacccagggggtattgtgtcgtaacgggcaactctgcagcggaaccgactactttgggtgtccgtgtttccttttatccttatactggctgcttatggtgacaattgaaagattgttgccatatagctattggattggccatccagtgtctaatagagctgttatttacctctttgttggatttataccactcaacctaaaagaagttaaaacactacagctcattttacaactgaatacagcaaaccaccatgatgaaagtcatctggttcagtagcctgatctgcctggtcatccagtgcggaggcgacaccggccctatcatttgcgccggacccatccactccaacaagtccgctgatattcctcacctgctgggctattctgaaaaaatctgccagatcgacagactgatccatgtgtccagctggctgagaaaccactcccagttccagggatatgtgggccagagaggcggccggtcccaggtgagctactaccctgctgaaaactcctacagcagatggagcgggctgctgtctccttgcgacgccgactggctgggcatgctggtggtgaagaaggccaagggtagtgacatgatcgtgcccggccctagctacaagggcaaggtgttctttgaacggcctacatttgacggttacgtgggatggggatgtggcagcggcaagagcagaacagaatctggagagctgtgctctagcgatagcggaaccagcagcggtctgctgcctagcgacagagtgctgtggatcggcgacgtggcttgtcagcctatgacccctatccccgaggaaaccttcctggaactgaagtcttttagccaaagcgagttccccgacatctgcaaaattgacggcatcgtgtttaatcagtgcgagggcgagagccttcctcaacccttcgacgtggcctggatggacgtgggccactcccacaagatcattatgagagaacacaagaccaagtgggtgcaagagtcctcttcgaaggacttcgtgtgctacaaggagggcaccggcccctgtagcgaaagcgaagagaagacctgtaaaaccagcggcagctgtagaggcgacatgcagttctgcaaggtggccggatgcgagcacggcgaagaggcctctgaagccaagtgcagatgcagcctggttcataagccaggagaagtggtcgtatcctacggcggcatgagagtgcggcccaagtgctacggttttagcagaatgatggccaccctggaagtcaaccagcctgagcaaagaatcggccaatgcaccggctgccacctggaatgcatcaacggcggcgttcggctgatcaccctgaccagcgagctgaagagcgctacagtgtgcgccagccacttctgcagcagcgccaccagcggcaagaagtccaccgaaatccagttccacagcggctccctggtcggcaaaacagctatccacgtgaagggcgccctggtggacggcaccgagttcaccttcgagggcagctgtatgttccctgacggatgtgatgccgtggattgcacattttgtcgggagttcctgaaaaacccccagtgctaccccgccaagaaatggctgtttatcattatcgtgatcctgctgggatacgccggcctgatgctgctgactaatgtgctgaaggctataggcgtgtggggcagctgggtcatcgcccctgtgaagctagtgttcgccatcatcaagaaactgatgcgggccgtgagctgtctgatgggcaagctgatggaccggggccggcaggtgattcacgaagaaatcggagagaacagagagggcaaccaggacgatgtgcgcatcgaaatggccagacccagacgggtgcgccactggatgtacagccctgtgatcctgacaatccttgctatcggcctggccgagggctgcgacgagatggtgcatgccgacagcaagctggtgagctgcagacagggtagcggaaacatgaaggagtgcgtcaccaccggcagagccctgctgcccgctgtaaaccctggccaggaggcctgcctccacttcaccgcccctggatcacctgatagcaagtgtctgaagatcaaggtgaaaagaatcaatctgaaatgcaaaaagtccagcagctacttcgtgcctgatgccagaagcagatgcacatctgtgcggcggtgcagatgggccggcgactgccagagcggctgtcctcctcacttcaccagcaacagcttctctgacgactgggccggaaagatggatagagccggcctgggcttcagcggatgtagcgatggctgcggcggcgccgcttgcggctgcttcaacgccgctcctagctgcatcttctggcggaagtgggttgagaacccacacggcatcatctggaaggtgtccccatgcgcggcctgggtgccaagcgccgtgatcgagctgaccatgcctagcggagaagtgcggacattccaccctatgagcggcatcccaacacaggtgttcaagggcgtctccgtgacatacctgggtagcgacatggaagtgtccggcttgacagacctgtgcgagatcgaggaactgaagtctaagaagctggccctggccccttgcaaccaggccggaatgggcgtggtgggcaaagtgggcgagatccaatgtagctctgaggaaagcgctagaaccataaagaaagacggctgcatctggaacgctgatctggtgggcatcgagctgcgtgtggatgacgccgtttgttacagcaagatcactagcgtggaggccgtggccaattactctgctatcccaacaacaatcggcggcctgagattcgagcggagccacgactctcagggcaaaatcagcggcagtcccctggacatcaccgccatcagaggctcatttagcgtgaactacagaggtctgcgtctgagcctctccgagatcaccgccacatgcaccggcgaggtgaccaacgtgtctggctgttactcatgcatgacaggagcgaaggtgtctatcaagctgcacagctctaagaacagcaccgcccacgtgcggtgcaagggcgatgaaaccgccttcagcgttctggagggcgtgcactcttatagtgtgagcctgagctttgatcacgccgtggtggacgagcagtgtcagctgaactgtggcgggcacgagagccaggtcaccctgcggggcaatctgattttcctggacgttcctaagttcgtggacggcagctacatgcagacctaccacagcaccgtgcccacaggcgccaatatcccttctccaaccgactggctgaacgcccttttcggcaacggcttgtctaggtggattctgggagtgatcggagtcctgctgggtggactggccctgttcttcctgatcatgagccttttcaagttgggcacaaagcaggtgttcagatcaagaaccaagttggcatgaaactttgagccaacaggggtgacggagtcccgcactgaaattacggcaatgcagaccaccggttcatgtgggcaacaatcaggagctgtgtacgtgggcaattacaggattgtaaacagacacctggcaacgagccacgattggcaaaattgcgtgtgggaggactacaacagggatctcctggtcagcacaacaactgctcatggttgtgatactatagcacggtgccaatgtactgctggcgtgtacttttgtgcatctagaaacaagcactacccagtgagcttcgagggtccaggtctagtgaaagttcaggagggcgagtactaccccgagagataccagtcgcacgtactccttgcagttggattttcagaaccgggtgattgtggaggtattttgaggtgtgaacatggagtcattgggctcgttaccatgggtggtgagggtgtagtaggcttcgctgacgtgcgggatcttttgtggttggaagacgacgccatggagcagggtgttagagattatgtagagcaactgggaaatgcatttggctcaggtttcactaaccaaatctgtgagcaagttaacctccttaaagaatctctgatagggcaggattccatattggaaaaatccctgaaggccctggttaaaatcatatcagccctggtgatagtggttaggaaccacgacgacctgattacagtgactgccacactagctttaatcggttgcgcatcatctccatggcgatggctcaaacaaaaagtgtgtcaatactacggaatccccatggcagaaaggcagaataacggttggttaaagaaattcactgaaatgaccaacgcctgcaagggcatggagtggattgctgttaaaattcaaaagttcatcgagtggctcaaagtaaagattctgcctgaagtgaaggagaaacatgagttccttaccagattgaagcaattgccactccttgaaagtcaaattgccaccattgagcaaagcgcaccctcacaaagtgatcaagagcagcttttttcgaatgttcagtacttcgcccattactgcaggaagtatgcacctctgtatgctgccgaagcaaaaagagtgttctcattagaaaagaaaatgagtaattacatacagttcaagtccaaatgccgcattgagcctgtatgcttactccttcacggtagtccaggggctggcaagtcagtagctaccaacctgatagggagatcccttgcagagaagctcaatagctctgtgtactctttaccaccagatccagatcattttgatgggtacaaacagcaggcagtggtgatcatggatgatctctgtcaaaaccccgatgggaaggacgtgtccttgttttgccaaatggtgtctagtgtagattttgtgccacccatggcggcgctggaagaaaaaggcattctctttacgtccccgtttgtgttggcatcaaccaacgcggggtccatcaatgcaccaacagtgtcagacagcagagcacttgccagaaggtttcactttgacatgaatattgaggtgatttcgatgtacagccagaatggtaaaattaacatgcccatgtctgttaagacatgtgatgatgaatgctgcccggtcaatttcaaaaagtgttgcccactagtgtgtggcaaggccatccagtttattgacaggagaaaccaagttagatattcactggacatgctggttactgagatgtttagagagtacaaccacagacacagtgtgggtgctaccctcgaggctttgttccaaggaccaccagtatacagggaaatcaaaatcagtgtggccccggaaacaccccctccaccagcaattgctgaccttctaaaatctgtagacagtgaggcaataagggagtactgcaaggaaaggggttggcttgtgccagaggtcagctccactctacaaattgaaaaacatgttagcagggcatttatttgcttgcaagcgctaactacatttgtttcagtggctggtataatctacatcatttacaagttgtttgccggctttcagggtgcatacactggaatgcccaaccagaaacccaaggtgcccaccttaagacaagctaaggtgcaaggtccggcatttgaatttgccgtagcaatgatgaaaaggaacgccagcacagtcaagacagaatacggtgagttcacgatgcttggcatctatgataaatgggcagtgctgccgcgccacgccaagcctggaccaactattttaatgaatgatcaggaggttggtgtgctcgatgccaaagagttagttgataaagacggaaccaacctggagctgacactattgaagcttaaccgcaatgaaaagttcagagacatcagaggttttcttgcaagggaagaagttgaggtaagtgaggctgttttggcaataaacacgagcaagttcccaagcatgtacatccctgtgggccaagtcaccgattacggatttttaaatctaggtggcaccccaacaaagagaatgctcatgtacaacttccctaccagagcgggacagtgtggtggtgtccttatgtcaacaggaaaggtccttggcatacacgtgggaggaaatggtcaccaaggcttctctgctgctctcctcagacactacttcaacgaggaacagggcgaaatagagtttattgagagctctaaagatgcaggatttcctgtgatcaacacccctaataaaaccaaactggaaccaagtgtgtttcatcaggtttttgagggcaacaaagaaccagcagtcctaagaaacggagacccgcgacttaaagccaactttgaggaagcgatattttccaagtacatcggaaatgtgaacacacatgtggacgagtacatgatagaagctgttgatcactacgctggacagctggcaactctggacatcagtacagaacctatgaagcttgaggatgctgtttatggcactgaaggcttggaagcattggacttgaccactagcgcaggatatccttatgtcgccttgggcatcaagaaaagggatatcctctccaagaagactaaagatctcaccaagctgagggaatgcatggacaagtatggtctaaatctgccgatggtgacctacgtgaaggatgaactcaggtccgctgagaaagtagccaagggaaaatccagacttatagaagcttctagtctcaatgactcagtggccatgaggcagacatttgggaacctatacaagacattccacctcaacccaggcattgtcactggtagtgctgttgggtgcgacccagatgtgttttggagcaaaatacccgtgatgcttgacgggcaccttatagcttttgattactctggctacgacgctagcttgagcccagtgtggtttgcttgtttgaaactcctcctagggaaactagggtatactcataaggaaaccaattacatagactacctctgcaactcccatcacttatacagagataaacactatttcgtgaggggtggtatgccatcaggatgttcaggcaccagtatattcaacaccatgatcaacaacatcattattaggacccttatgctaaaggtctacaaaggtattgacctggatcagtttagaatgatcgcttacggggacgatgtgatagcctcttacccgtggcctattgatgcctcactactagcagaagcgggaaaggattatggtttgatcatgaccccagcagataaaggagagtgttttaatgaggtaacctggacaaatgtaaccttcttgaaaaggtactttagagctgatgaacaatatccattcttggtgcaccccgtgatgcccatgaaagacatacacgaatccattagatggaccaaagacccaaagaacactcaagatcatgtgcgctcgttatgcctattggcttggcacaatggggagcacgaatatgaggaatttatccgaaagatcagaagcgtgcctgttggacgctgtttgaccctcccggtgttctcaacactacgcaggaaatggttagattccttctaaaattagagtgcaatcaatgaactatgattggcttaaccctaccgcatgaaccgaactagacaaaagtgcggtaggggtaaattctccgcattcggtgcggaaaaaaaaaaaaaaaaaaaaaaaaaaaaaaaaaaaaaaaaaaaaaaaaaaaaaaaaaaaaaaaaaaaaaaaaaaaaaaaaaaaaaaaaaaaaaaaaaaaaaaaaaaaaaaaaaaaaaaaa

SEQ ID NO: 113 - RNA, 8252 nt, synthetic construct
  source 1..8252: mol_type = other RNA
  misc_feature 1..8252: note = SFTS B saRNA construct
ttaaaacagcctgtgggttgtacccacccacagggcccactgggcgctagcactctggtatcacggtacctttgtgtgcctgttttatatcccctttccccgattgtaacttagaagatgtacacactgatcaatagcgggcatagcacaccagctatgtcttgatcaagcactcctgtatccccggaccaagtatcaatagactgctcacgcggttgaaggagaaaacgttcgtcacccggctaactacttcgagaaacccagtagtatcatgaaagttgcgaggcgtttcgttcagcacacccccagtgtagatcgggtcgatgagtcaccgcatcccccacgggcgaccgtggcggtggctgcgctggcggcctgcctacggggcaacccgtaggacgcttcaatacagacatggtgcgaagagtcgattgagctagttagtagtcctccggcccctgaatgcggctaatcctaactgcggagcacatgccctcaacccagggggtattgtgtcgtaacgggcaactctgcagcggaaccgactactttgggtgtccgtgtttccttttatccttatactggctgcttatggtgacaattgaaagattgttgccatatagctattggattggccatccagtgtctaatagagctgttatttacctctttgttggatttataccactcaacctaaaagaagttaaaacactacagctcattttacaactgaatacagcaaaccaccatgatgaaggtgatctggttcagctcccttatctgtctggtgattcagtgttctggcgacaccggccctatcatctgtgccggacccatccatagcaacaagagcgccaatatcccccacctgctgggctacagtgagaaaatctgccagatcgacagactgatccacgtgagcagctggctgagaaaccactctcaatttcagggctacgtaggtcagagaggcggtcggagccaggtgagctactaccctgccgagaactcttatagccggtggtctggattgctgtcgccttgcgacgccgattggctggggatgctggtcgtgaaaaaggccaagggcagcgatatgatcgtgccaggcccttcttataaaggcaaggtgttcttcgaaagacctacatttgacggatatgtgggatggggctgcggctccggcaagagcagaacagaatccggcgagctgtgcagctctgattctggaaccagcagcggactgctgccttctgatagagtgctgtggatcggcgatgtggcctgccagcctatgacccctatacccgaggaaacattcctggaactgaaaagttttagccagagcgagtttcctgacatctgcaagatcgacggaatcgtgtttaaccagtgcgagtctgagagccttcctcagcctttcgacgtggcctggatggatgtgggccacagccacaagatcatcatgagagagcacaagaccaagtgggtgcaggagagcagcagcaaagacttcgtctgctacaaggaaggcaccggcccatgctctgagagcgaggaaaagacctgtaaaaccagtggctcttgcaggggcgacatgcagttctgtaaggttgccgggtgcgaacacggcgaggaggcctctgaggccaagtgcagatgctccctggtgcacaaacctggggaggtggtggtgagctacggcggcatgcgggtgcggcccaagtgctacggcttctccagaatgatggccaccctggaagtgaatcctccagagcagcggatcggccagtgtacaggctgccacctggaatgcattaacggcggagtcaggctgattacactaacctccgagctgaagtctgccacagtgtgcgcgagccacttctgcagcagcgccacaagcggcaagaagtctacagagatccagttccacagcggcagcctggtgggcaagaccgccatccatgtgaagggcgccctggtggacggcacagagttcacctttgagggctcctgcatgttccccgatggctgtgatgccgtggactgcaccttctgcagagagttcctgaagaacccacagtgttaccctgccaagaagtggctgttcatcatcatcgtgatcctgctcggctacgccggactgatgttgctgaccaacgtgctgaaggccatcggcgtgtggggctcctgggtcatcgcccccgtcaagctgatgttcgccatcatcaagaagctgatgcgcagcgtgtcgtgcctgatgggcaagctcatggatagaggcagacaggtgattcacgaggagatcggcgagaacagagagggaaaccaagacgatgtgcggatcgaaatggccagacctcggagagtgcggcactggatgtacagccctgtgatccttacaatcctggccatcggcctggccgaaggctgtgacgagatggtgcacgccgactccaagctggtctcttgcaaacagggctccggaaatatgaaggagtgtgtgaccaccggaagagccctgctgcctgccgtgaaccctggacaggaggcttgcctgcatttcaccgcccctggtagccctgacagcaaatgtctgaaaatcaaagtgaaacgaatcaacctgaagtgcaaaaagtcaagctcttacttcgtgcccgacgcacgatctcggtgtaccagcgttcggcggtgcagatgggccggcgattgccagagcggctgtccttcccatttcacaagcaacagcttcagtgacgactgggccggcaagatggatagagccggcctggggttctccggctgttccgacggctgcggaggagctgcttgtggctgcttcaacgccgctccaagctgcatcttctggagaaagtgggtggaaaatcctcacggcatcatctggaaggtgagcccatgcgctgcctgggtgccctcggctgtcatcgagctgacaatgccttctggcgaagtgcggacatttcaccccatgagcggcatccccacccaggttttcaagggggtgagcgtgacctacctgggcagcgacatggaagtgagcggcctgacagacctgtgcgagatcgaggaactgaaaagcaagaagctggccctggctccttgcaaccaggccggaatgggcgtggtgggaaaggtgggagaaatccaatgtagctccgaagaaagcgccagaaccattaagaaggacgggtgcatctggaacgctgatctggtcggtattgaactgcgagtggacgacgccgtgtgctactccaaaatcaccagtgttgaggccgtcgccaattacagcgccattcccaccactatcggcggactgaggttcgagagaagccacgactctcagggcaagatcagcggcagcccactggacatcacagccatcagaggctcattctccgtgaactaccggggcttgagactgtctctgagcgaaatcaccgccacctgcaccggcgaggtgacaaacgtgtccggctgctacagctgtatgaccggcgccaaggtgtctatcaagctgcactccagcaagaacagcaccgcccacgtgagatgtaaaggcgacgagacagctttcagcgtgctggagggcgtacacagctacaccgtgtccctgagcttcgaccacgccgtggtggacgagcagtgccagctaaactgcggaggccacgaaagccaagtgaccctgaagggcaacctgatcttcctggatgtgcctaagttcgtggacggcagctacatgcaaacataccacagctcagtgcctacgggcgccaacatcccttctccaaccgactggctgaacgctctgtttggcaatggactgagcaggtggattctgggcgtgatcggggtgctgctgggcggcctggccctgttcttcctgataatgagcctgtttaagctgggcaccaagcaggtgttcagatccagaaccaagctggctaactttgagccaacaggggtgacggagtcccgcactgaaattacggcaatgcagaccaccggttcatgtgggcaacaatcaggagctgtgtacgtgggcaattacaggattgtaaacagacacctggcaacgagccacgattggcaaaattgcgtgtgggaggactacaacagggatctcctggtcagcacaacaactgctcatggttgtgatactatagcacggtgccaatgtactgctggcgtgtacttttgtgcatctagaaacaagcactacccagtgagcttcgagggtccaggtctagtgaaagttcaggagggcgagtactaccccgagagataccagtcgcacgtactccttgcagttggattttcagaaccgggtgattgtggaggtattttgaggtgtgaacatggagtcattgggctcgttaccatgggtggtgagggtgtagtaggcttcgctgacgtgcgggatcttttgtggttggaagacgacgccatggagcagggtgttagagattatgtagagcaactgggaaatgcatttggctcaggtttcactaaccaaatctgtgagcaagttaacctccttaaagaatctctgatagggcaggattccatattggaaaaatccctgaaggccctggttaaaatcatatcagccctggtgatagtggttaggaaccacgacgacctgattacagtgactgccacactagctttaatcggttgcgcatcatctccatggcgatggctcaaacaaaaagtgtgtcaatactacggaatccccatggcagaaaggcagaataacggttggttaaagaaattcactgaaatgaccaacgcctgcaagggcatggagtggattgctgttaaaattcaaaagttcatcgagtggctcaaagtaaagattctgcctgaagtgaaggagaaacatgagttccttaccagattgaagcaattgccactccttgaaagtcaaattgccaccattgagcaaagcgcaccctcacaaagtgatcaagagcagcttttttcgaatgttcagtacttcgcccattactgcaggaagtatgcacctctgtatgctgccgaagcaaaaagagtgttctcattagaaaagaaaatgagtaattacatacagttcaagtccaaatgccgcattgagcctgtatgcttactccttcacggtagtccaggggctggcaagtcagtagctaccaacctgatagggagatcccttgcagagaagctcaatagctctgtgtactctttaccaccagatccagatcattttgatgggtacaaacagcaggcagtggtgatcatggatgatctctgtcaaaaccccgatgggaaggacgtgtccttgttttgccaaatggtgtctagtgtagattttgtgccacccatggcggcgctggaagaaaaaggcattctctttacgtccccgtttgtgttggcatcaaccaacgcggggtccatcaatgcaccaacagtgtcagacagcagagcacttgccagaaggtttcactttgacatgaatattgaggtgatttcgatgtacagccagaatggtaaaattaacatgcccatgtctgttaagacatgtgatgatgaatgctgcccggtcaatttcaaaaagtgttgcccactagtgtgtggcaaggccatccagtttattgacaggagaaaccaagttagatattcactggacatgctggttactgagatgtttagagagtacaaccacagacacagtgtgggtgctaccctcgaggctttgttccaaggaccaccagtatacagggaaatcaaaatcagtgtggccccggaaacaccccctccaccagcaattgctgaccttctaaaatctgtagacagtgaggcaataagggagtactgcaaggaaaggggttggcttgtgccagaggtcagctccactctacaaattgaaaaacatgttagcagggcatttatttgcttgcaagcgctaactacatttgtttcagtggctggtataatctacatcatttacaagttgtttgccggctttcagggtgcatacactggaatgcccaaccagaaacccaaggtgcccaccttaagacaagctaaggtgcaaggtccggcatttgaatttgccgtagcaatgatgaaaaggaacgccagcacagtcaagacagaatacggtgagttcacgatgcttggcatctatgataaatgggcagtgctgccgcgccacgccaagcctggaccaactattttaatgaatgatcaggaggttggtgtgctcgatgccaaagagttagttgataaagacggaaccaacctggagctgacactattgaagcttaaccgcaatgaaaagttcagagacatcagaggttttcttgcaagggaagaagttgaggtaagtgaggctgttttggcaataaacacgagcaagttcccaagcatgtacatccctgtgggccaagtcaccgattacggatttttaaatctaggtggcaccccaacaaagagaatgctcatgtacaacttccctaccagagcgggacagtgtggtggtgtccttatgtcaacaggaaaggtccttggcatacacgtgggaggaaatggtcaccaaggcttctctgctgctctcctcagacactacttcaacgaggaacagggcgaaatagagtttattgagagctctaaagatgcaggatttcctgtgatcaacacccctaataaaaccaaactggaaccaagtgtgtttcatcaggtttttgagggcaacaaagaaccagcagtcctaagaaacggagacccgcgacttaaagccaactttgaggaagcgatattttccaagtacatcggaaatgtgaacacacatgtggacgagtacatgatagaagctgttgatcactacgctggacagctggcaactctggacatcagtacagaacctatgaagcttgaggatgctgtttatggcactgaaggcttggaagcattggacttgaccactagcgcaggatatccttatgtcgccttgggcatcaagaaaagggatatcctctccaagaagactaaagatctcaccaagctgagggaatgcatggacaagtatggtctaaatctgccgatggtgacctacgtgaaggatgaactcaggtccgctgagaaagtagccaagggaaaatccagacttatagaagcttctagtctcaatgactcagtggccatgaggcagacatttgggaacctatacaagacattccacctcaacccaggcattgtcactggtagtgctgttgggtgcgacccagatgtgttttggagcaaaatacccgtgatgcttgacgggcaccttatagcttttgattactctggctacgacgctagcttgagcccagtgtggtttgcttgtttgaaactcctcctagggaaactagggtatactcataaggaaaccaattacatagactacctctgcaactcccatcacttatacagagataaacactatttcgtgaggggtggtatgccatcaggatgttcaggcaccagtatattcaacaccatgatcaacaacatcattattaggacccttatgctaaaggtctacaaaggtattgacctggatcagtttagaatgatcgcttacggggacgatgtgatagcctcttacccgtggcctattgatgcctcactactagcagaagcgggaaaggattatggtttgatcatgaccccagcagataaaggagagtgttttaatgaggtaacctggacaaatgtaaccttcttgaaaaggtactttagagctgatgaacaatatccattcttggtgcaccccgtgatgcccatgaaagacatacacgaatccattagatggaccaaagacccaaagaacactcaagatcatgtgcgctcgttatgcctattggcttggcacaatggggagcacgaatatgaggaatttatccgaaagatcagaagcgtgcctgttggacgctgtttgaccctcccggtgttctcaacactacgcaggaaatggttagattccttctaaaattagagtgcaatcaatgaactatgattggcttaaccctaccgcatgaaccgaactagacaaaagtgcggtaggggtaaattctccgcattcggtgcggaaaaaaaaaaaaaaaaaaaaaaaaaaaaaaaaaaaaaaaaaaaaaaaaaaaaaaaaaaaaaaaaaaaaaaaaaaaaaaaaaaaaaaaaaaaaaaaaaaaaaaaaaaaaaaaaaaaaaaaa

SEQ ID NO: 114 - RNA, 8252 nt, synthetic construct
  source 1..8252: mol_type = other RNA
  misc_feature 1..8252: note = SFTS DEF saRNA construct
ttaaaacagcctgtgggttgtacccacccacagggcccactgggcgctagcactctggtatcacggtacctttgtgtgcctgttttatatcccctttccccgattgtaacttagaagatgtacacactgatcaatagcgggcatagcacaccagctatgtcttgatcaagcactcctgtatccccggaccaagtatcaatagactgctcacgcggttgaaggagaaaacgttcgtcacccggctaactacttcgagaaacccagtagtatcatgaaagttgcgaggcgtttcgttcagcacacccccagtgtagatcgggtcgatgagtcaccgcatcccccacgggcgaccgtggcggtggctgcgctggcggcctgcctacggggcaacccgtaggacgcttcaatacagacatggtgcgaagagtcgattgagctagttagtagtcctccggcccctgaatgcggctaatcctaactgcggagcacatgccctcaacccagggggtattgtgtcgtaacgggcaactctgcagcggaaccgactactttgggtgtccgtgtttccttttatccttatactggctgcttatggtgacaattgaaagattgttgccatatagctattggattggccatccagtgtctaatagagctgttatttacctctttgttggatttataccactcaacctaaaagaagttaaaacactacagctcattttacaactgaatacagcaaaccaccatgatgaaggtgatctggttctcttctctgatctgctttgtgatccagtgcagcggcgatagcgggccaatcatctgcgccggaccaatccacagcaacaagagcgccgacatcccccacctgcttggctactcagaaaaaatctgccagatcgacagactaatacacgtgagcagctggctgcggaaccacagccagtttcagggctatgtgggccagagaggaggcagaagccaagtgagctactaccctgctgaaaacagctacagcagatggtccggcctgctctccccatgtgatgccgattggctgggcatgctcgtggtgaagaaagccaagggctccgatatgatcgtgcccggccctagctacaaggggaaggtgtttttcgagagacctacattcgacggctacgtgggctggggctgcggcagcggcaaaagccggaccgagagcggcgaactgtgtagcagcgacagcggaacaagcagcggtctgctccccagcgaccgggtgctgtggatcggcgacgttgcctgtcagcccatgacccctatccccgaggagacatttctggaactgaagtcgttctcccagagcgagttccctgacatctgcaagattgacggcattgtgttcaatcagtgcgagggcgagagcctgcctcagcctttcgacgtggcttggatggatgtgggccacagccacaagatcatcatgagagagcacaaaaccaagtgggtccaggagtcgtccagcaaggacttcgtgtgttataaggaaggcacaggcccctgcagcgagtccgaagagaagacctgcaagaccagcggcagctgtagaggcgacatgcagttctgcaaagtggccggctgtgaacacggagaagaggccagcgaggctaagtgccggtgcagcctggtgcacaagcctggcgaggtggtcgtatcttacggcggcatgcgggtgcggcctaagtgctacggcttcagccggatgatggccaccctggaggtgaatccgcccgagcagcggatcggccagtgtaccggatgccacctggagtgcattaacggcggcgtgcggctgatcaccctgaccagcgaactgaagtctgctaccgtgtgcgcgagccatttctgcagctcagccaccagtggaaaaaagagcaccgagatccagttccacagcggctctctggtcggcaagacagccatccacgtgaagggcgccctggtggacggcaccgagttcacctttgagggcagctgcatgttccctgacggctgtgacgccgtggactgcaccttctgcagagagttcctgaaaaacccccagtgttaccccgctaagaaatggctgttcatcatcattgtcatcctgctgggctacgccggactcatgctgctgacaaacgtgctgaaggccatcggagtttggggaagttgggtgatcgcccctgtgaaactgatgttcgccatcatcaagaaactgatgcgaaccgtgagctgcctgatgggcaagttgatggatagaggcagacaggtgatccacgaggagatcggcgaaaacagagaaggcaaccaggacgacgtgcggatcgagatggccagacccagaagagtgcggcactggatgtactcccctgtgatcctgaccatcctggccatcggcctagctgaaggctgcgacgaaatggtgcacgccgactctaagctcgtatcatgccggcagggcagcggcaatatgaaggagtgtgtgacaaccggcagagccctgctgcctgccgtgaaccccggccaggaggcctgcctgcactttacggcccctggttctcccgacagcaagtgcctgaagatcaaggtcaagagaatcaacctgaaatgcaagaagagcagcagctacttcgtgcctgacgccagaagtagatgtacaagcgtgcgccgctgccgctgggcaggcgattgccagagcggatgtcctcctcacttcacctctaatagtttcagcgacgattgggctggcaaaatggaccgcgccggcctgggattttctggatgcagtgatggctgcggcggcgccgcctgcggatgttttaacgccgctcctagttgcatcttctggcggaagtgggtggaaaaccctcatggcatcatctggaaggtgagcccatgcgctgcttgggtgccttctgccgtgatcgagctgaccatgccttctggagaggtgcggacatttcaccctatgtccggcatccctacgcaggtgttcaagggcgtgtctgtgacatatctgggctccgacatggaagtgtccggtctgacagacctgtgcgaaatcgaggaactgaagtctaagaagctggccctggccccctgtaatcaagccggcatgggcgtggtgggcaaggtgggtgagatccaatgttcgagcgaggaaagcgcccggaccatcaaaaaagacggctgtatctggaacgctgatctggtgggcatcgagctgagagttgatgacgctgtttgctacagcaagatcacctccgtggaagccgtggccaattacagcgccatccccaccaccatcggcggcctgagattcgagagaagccacgatagccagggcaagatcagcggctcccctctggacattactgccatcagaggcagcttcagcgtgaactacagaggcctgaggctgtctctgagcgaaatcaccgctacatgcaccggagaagtgaccaacgtgtctggctgttacagctgtatgaccggcgcaaaagtgtctatcaagctgcactctagcaagaacagtacagcccacgtcagatgcaagggagatgagacagccttcagcgtgctggagggggttcacagctacaccgtgagcctgagctttgaccatgccgtggtggacgagcagtgccagctgaactgcggcggccacgagagccaggtaacactgaagggcaacctgatcttcctggatgtgccaaaattcgtggatggcagctacatgcaaacctaccacagtaccgttccaaccggcgccaacatccctagccctacagattggcttaacgccctgttcggcaacggcctgagcagatggattctgggcgtgattggagtgctgctgggtggactggcactgttcttcctgattatgtctctgttcaagctgggcacaaagcaggtgttcagatccagaaccaagctggccaactttgagccaacaggggtgacggagtcccgcactgaaattacggcaatgcagaccaccggttcatgtgggcaacaatcaggagctgtgtacgtgggcaattacaggattgtaaacagacacctggcaacgagccacgattggcaaaattgcgtgtgggaggactacaacagggatctcctggtcagcacaacaactgctcatggttgtgatactatagcacggtgccaatgtactgctggcgtgtacttttgtgcatctagaaacaagcactacccagtgagcttcgagggtccaggtctagtgaaagttcaggagggcgagtactaccccgagagataccagtcgcacgtactccttgcagttggattttcagaaccgggtgattgtggaggtattttgaggtgtgaacatggagtcattgggctcgttaccatgggtggtgagggtgtagtaggcttcgctgacgtgcgggatcttttgtggttggaagacgacgccatggagcagggtgttagagattatgtagagcaactgggaaatgcatttggctcaggtttcactaaccaaatctgtgagcaagttaacctccttaaagaatctctgatagggcaggattccatattggaaaaatccctgaaggccctggttaaaatcatatcagccctggtgatagtggttaggaaccacgacgacctgattacagtgactgccacactagctttaatcggttgcgcatcatctccatggcgatggctcaaacaaaaagtgtgtcaatactacggaatccccatggcagaaaggcagaataacggttggttaaagaaattcactgaaatgaccaacgcctgcaagggcatggagtggattgctgttaaaattcaaaagttcatcgagtggctcaaagtaaagattctgcctgaagtgaaggagaaacatgagttccttaccagattgaagcaattgccactccttgaaagtcaaattgccaccattgagcaaagcgcaccctcacaaagtgatcaagagcagcttttttcgaatgttcagtacttcgcccattactgcaggaagtatgcacctctgtatgctgccgaagcaaaaagagtgttctcattagaaaagaaaatgagtaattacatacagttcaagtccaaatgccgcattgagcctgtatgcttactccttcacggtagtccaggggctggcaagtcagtagctaccaacctgatagggagatcccttgcagagaagctcaatagctctgtgtactctttaccaccagatccagatcattttgatgggtacaaacagcaggcagtggtgatcatggatgatctctgtcaaaaccccgatgggaaggacgtgtccttgttttgccaaatggtgtctagtgtagattttgtgccacccatggcggcgctggaagaaaaaggcattctctttacgtccccgtttgtgttggcatcaaccaacgcggggtccatcaatgcaccaacagtgtcagacagcagagcacttgccagaaggtttcactttgacatgaatattgaggtgatttcgatgtacagccagaatggtaaaattaacatgcccatgtctgttaagacatgtgatgatgaatgctgcccggtcaatttcaaaaagtgttgcccactagtgtgtggcaaggccatccagtttattgacaggagaaaccaagttagatattcactggacatgctggttactgagatgtttagagagtacaaccacagacacagtgtgggtgctaccctcgaggctttgttccaaggaccaccagtatacagggaaatcaaaatcagtgtggccccggaaacaccccctccaccagcaattgctgaccttctaaaatctgtagacagtgaggcaataagggagtactgcaaggaaaggggttggcttgtgccagaggtcagctccactctacaaattgaaaaacatgttagcagggcatttatttgcttgcaagcgctaactacatttgtttcagtggctggtataatctacatcatttacaagttgtttgccggctttcagggtgcatacactggaatgcccaaccagaaacccaaggtgcccaccttaagacaagctaaggtgcaaggtccggcatttgaatttgccgtagcaatgatgaaaaggaacgccagcacagtcaagacagaatacggtgagttcacgatgcttggcatctatgataaatgggcagtgctgccgcgccacgccaagcctggaccaactattttaatgaatgatcaggaggttggtgtgctcgatgccaaagagttagttgataaagacggaaccaacctggagctgacactattgaagcttaaccgcaatgaaaagttcagagacatcagaggttttcttgcaagggaagaagttgaggtaagtgaggctgttttggcaataaacacgagcaagttcccaagcatgtacatccctgtgggccaagtcaccgattacggatttttaaatctaggtggcaccccaacaaagagaatgctcatgtacaacttccctaccagagcgggacagtgtggtggtgtccttatgtcaacaggaaaggtccttggcatacacgtgggaggaaatggtcaccaaggcttctctgctgctctcctcagacactacttcaacgaggaacagggcgaaatagagtttattgagagctctaaagatgcaggatttcctgtgatcaacacccctaataaaaccaaactggaaccaagtgtgtttcatcaggtttttgagggcaacaaagaaccagcagtcctaagaaacggagacccgcgacttaaagccaactttgaggaagcgatattttccaagtacatcggaaatgtgaacacacatgtggacgagtacatgatagaagctgttgatcactacgctggacagctggcaactctggacatcagtacagaacctatgaagcttgaggatgctgtttatggcactgaaggcttggaagcattggacttgaccactagcgcaggatatccttatgtcgccttgggcatcaagaaaagggatatcctctccaagaagactaaagatctcaccaagctgagggaatgcatggacaagtatggtctaaatctgccgatggtgacctacgtgaaggatgaactcaggtccgctgagaaagtagccaagggaaaatccagacttatagaagcttctagtctcaatgactcagtggccatgaggcagacatttgggaacctatacaagacattccacctcaacccaggcattgtcactggtagtgctgttgggtgcgacccagatgtgttttggagcaaaatacccgtgatgcttgacgggcaccttatagcttttgattactctggctacgacgctagcttgagcccagtgtggtttgcttgtttgaaactcctcctagggaaactagggtatactcataaggaaaccaattacatagactacctctgcaactcccatcacttatacagagataaacactatttcgtgaggggtggtatgccatcaggatgttcaggcaccagtatattcaacaccatgatcaacaacatcattattaggacccttatgctaaaggtctacaaaggtattgacctggatcagtttagaatgatcgcttacggggacgatgtgatagcctcttacccgtggcctattgatgcctcactactagcagaagcgggaaaggattatggtttgatcatgaccccagcagataaaggagagtgttttaatgaggtaacctggacaaatgtaaccttcttgaaaaggtactttagagctgatgaacaatatccattcttggtgcaccccgtgatgcccatgaaagacatacacgaatccattagatggaccaaagacccaaagaacactcaagatcatgtgcgctcgttatgcctattggcttggcacaatggggagcacgaatatgaggaatttatccgaaagatcagaagcgtgcctgttggacgctgtttgaccctcccggtgttctcaacactacgcaggaaatggttagattccttctaaaattagagtgcaatcaatgaactatgattggcttaaccctaccgcatgaaccgaactagacaaaagtgcggtaggggtaaattctccgcattcggtgcggaaaaaaaaaaaaaaaaaaaaaaaaaaaaaaaaaaaaaaaaaaaaaaaaaaaaaaaaaaaaaaaaaaaaaaaaaaaaaaaaaaaaaaaaaaaaaaaaaaaaaaaaaaaaaaaaaaaaaaaa

SEQ ID NO: 115 - RNA, 8255 nt, synthetic construct
  source 1..8255: mol_type = other RNA
  misc_feature 1..8255: note = SFTS ABDEF saRNA construct
ttaaaacagcctgtgggttgtacccacccacagggcccactgggcgctagcactctggtatcacggtacctttgtgtgcctgttttatatcccctttccccgattgtaacttagaagatgtacacactgatcaatagcgggcatagcacaccagctatgtcttgatcaagcactcctgtatccccggaccaagtatcaatagactgctcacgcggttgaaggagaaaacgttcgtcacccggctaactacttcgagaaacccagtagtatcatgaaagttgcgaggcgtttcgttcagcacacccccagtgtagatcgggtcgatgagtcaccgcatcccccacgggcgaccgtggcggtggctgcgctggcggcctgcctacggggcaacccgtaggacgcttcaatacagacatggtgcgaagagtcgattgagctagttagtagtcctccggcccctgaatgcggctaatcctaactgcggagcacatgccctcaacccagggggtattgtgtcgtaacgggcaactctgcagcggaaccgactactttgggtgtccgtgtttccttttatccttatactggctgcttatggtgacaattgaaagattgttgccatatagctattggattggccatccagtgtctaatagagctgttatttacctctttgttggatttataccactcaacctaaaagaagttaaaacactacagctcattttacaactgaatacagcaaaccaccatgatgaaggttatctggttctccagcctgatctgtctggtgatccagtgtagcggcgacaccggacctatcatttgtgccggccctatccactccaacaagtccgccgacatcccccacctcctgggatactctgaaaaaatctgccaaatcgatagactgatccacgtgtccagctggctgcgaaaccacagccagttccagggctatgtgggccaaagaggaggcagaagccaggtgagctactaccccgccgagaatagctacagcagatggtccggcctgctgagcccttgcgacgccgattggctgggaatgctggtggtgaagaaggccaagggcagcgacatgatcgtgcccggccctagctacaagggcaaggtctttttcgaacggcccacctttgatggctacgtgggctggggatgcggctctggcaaaagccggacagaatctggagagctgtgcagcagcgacagcggcaccagctctggcctgctgccttcggatagagtgctgtggatcggcgatgtcgcatgccagcctatgacccctatccctgaggagacattcctggagctgaaatctttcagtcaaagcgagttccccgacatctgtaagatcgacggcatcgtgtttaaccagtgtgaaggcgaatccctgcctcagccgttcgacgtggcctggatggacgtcggccacagccacaagatcatcatgagagagcacaaaaccaagtgggtccaggagtctagcagcaaagacttcgtgtgctataaggaaggaacaggcccttgctccgagagcgaggaaaagacatgcaagaccagcgggtcttgcagaggagacatgcagttttgtaaagtggccggatgcgagcacggcgaggaggccagcgaggctaagtgccgctgtagcctcgttcacaagccaggagaggtggttgtgtcctacggcggcatgcgggtgagacccaagtgctacggcttcagcagaatgatggccacactggaggtgaatccacctgaacagcggatcggccagtgcaccggctgccacctggaatgcatcaacggcggcgtgagactgataacactgactagcgaactgaagagcgccacagtgtgcgccagccacttctgctcaagcgccaccagcggcaagaaatctactgagatccagttccactccggcagcctggtcggcaagaccgccatccacgtgaagggcgctctggtggatggcacagagttcacgttcgagggctcatgcatgttccctgatggctgcgacgccgtggactgcaccttctgccgggagttcctgaaaaacccccagtgttatcctgctaaaaagtggctgttcatcatcatcgtgatcctgctcggatacgccggcctgatgctgctgaccaacgtgctgaaggccatcggcgtgtggggcagctgggtgatcgcccccgtgaagctgatgttcgccatcatcaagaaactcatgagaaccgtgtcctgcctgatgggcaagctgatggaccggggcagacaggtgatccatgaggaaattggcgagaacagagagggcaaccaggacgacgtaagaatcgagatggccagacccagacgggtgcggcactggatgtacagccctgtgattttgaccatcctggctatcggactggctgaaggctgcgacgagatggtgcatgctgattctaaactggtatcttgtagacagggcagcggaaacatgaaagaatgcgtgaccaccggtcgggccctcctgcccgctgtgaatcccggccaggaggcctgcctgcacttcaccgcccctggcagccccgatagcaagtgcctgaagattaaggtgaagcggatcaacctgaagtgcaagaaatctagcagctacttcgtgcctgacgctagatccagatgcacctctgttaggagatgtagatgggccggagactgccagagcggctgccctcctcatttcacaagcaacagcttcagcgatgattgggccggaaaaatggacagagccggcctcggattctccgggtgcagcgatggatgcggaggcgccgcctgcggctgcttcaacgccgctcctagctgtatcttctggcggaagtgggtggaaaaccctcacggcatcatctggaaggttagcccatgcgccgcctgggtgccctctgccgtaatcgagctgaccatgccttctggtgaagtgcggacttttcaccccatgtcgggcatccctacccaggtgttcaagggcgtgagcgtgacctacctgggcagcgacatggaagtgagcggcctgacagacctgtgtgaaattgaagagctgaagtctaaaaagctggccctggcgccctgtaaccaagccggcatgggagtggtgggaaaggtcggcgagatccagtgcagctccgaggagagcgccagaacaatcaagaaagacggctgtatctggaacgccgatctggtgggcatcgagcttagagtggacgacgccgtgtgctacagcaagatcacctccgtggaagccgttgctaattacagcgccatccctaccacaatcggcggcctgcggttcgagcggtctcacgacagccaaggcaaaatcagcggcagccctctggacattaccgccatcagaggctcttttagcgtgaactacagaggcctgagattgtctctgtctgagatcaccgcaacctgtacaggcgaggtgacaaacgtgtccggctgctacagctgtatgaccggcgctaaggtgtctatcaagctgcactccagcaagaacagcacagcccacgtgcggtgcaagggcgacgaaaccgccttcagtgtgctggaaggcgtgcacagctacaccgtgagcctgagcttcgaccacgccgtcgtggacgagcagtgccagctgaactgcggcggtcacgagagccaggtgaccctgaagggaaacctgatcttcctggacgtgccaaagttcgtggacggcagctacatgcagacctaccacagcaccgtgcctaccggagccaacatcccatctcctacagattggctgaacgccctgttcggcaatggcctgtccagatggattctgggagtgatcggcgtgctgctgggcggcctggccctgttcttcctgatcatgtccctgtttaagctgggcacaaagcaggtctttagaagtcgcaccaagctcgcttgaaactttgagccaacaggggtgacggagtcccgcactgaaattacggcaatgcagaccaccggttcatgtgggcaacaatcaggagctgtgtacgtgggcaattacaggattgtaaacagacacctggcaacgagccacgattggcaaaattgcgtgtgggaggactacaacagggatctcctggtcagcacaacaactgctcatggttgtgatactatagcacggtgccaatgtactgctggcgtgtacttttgtgcatctagaaacaagcactacccagtgagcttcgagggtccaggtctagtgaaagttcaggagggcgagtactaccccgagagataccagtcgcacgtactccttgcagttggattttcagaaccgggtgattgtggaggtattttgaggtgtgaacatggagtcattgggctcgttaccatgggtggtgagggtgtagtaggcttcgctgacgtgcgggatcttttgtggttggaagacgacgccatggagcagggtgttagagattatgtagagcaactgggaaatgcatttggctcaggtttcactaaccaaatctgtgagcaagttaacctccttaaagaatctctgatagggcaggattccatattggaaaaatccctgaaggccctggttaaaatcatatcagccctggtgatagtggttaggaaccacgacgacctgattacagtgactgccacactagctttaatcggttgcgcatcatctccatggcgatggctcaaacaaaaagtgtgtcaatactacggaatccccatggcagaaaggcagaataacggttggttaaagaaattcactgaaatgaccaacgcctgcaagggcatggagtggattgctgttaaaattcaaaagttcatcgagtggctcaaagtaaagattctgcctgaagtgaaggagaaacatgagttccttaccagattgaagcaattgccactccttgaaagtcaaattgccaccattgagcaaagcgcaccctcacaaagtgatcaagagcagcttttttcgaatgttcagtacttcgcccattactgcaggaagtatgcacctctgtatgctgccgaagcaaaaagagtgttctcattagaaaagaaaatgagtaattacatacagttcaagtccaaatgccgcattgagcctgtatgcttactccttcacggtagtccaggggctggcaagtcagtagctaccaacctgatagggagatcccttgcagagaagctcaatagctctgtgtactctttaccaccagatccagatcattttgatgggtacaaacagcaggcagtggtgatcatggatgatctctgtcaaaaccccgatgggaaggacgtgtccttgttttgccaaatggtgtctagtgtagattttgtgccacccatggcggcgctggaagaaaaaggcattctctttacgtccccgtttgtgttggcatcaaccaacgcggggtccatcaatgcaccaacagtgtcagacagcagagcacttgccagaaggtttcactttgacatgaatattgaggtgatttcgatgtacagccagaatggtaaaattaacatgcccatgtctgttaagacatgtgatgatgaatgctgcccggtcaatttcaaaaagtgttgcccactagtgtgtggcaaggccatccagtttattgacaggagaaaccaagttagatattcactggacatgctggttactgagatgtttagagagtacaaccacagacacagtgtgggtgctaccctcgaggctttgttccaaggaccaccagtatacagggaaatcaaaatcagtgtggccccggaaacaccccctccaccagcaattgctgaccttctaaaatctgtagacagtgaggcaataagggagtactgcaaggaaaggggttggcttgtgccagaggtcagctccactctacaaattgaaaaacatgttagcagggcatttatttgcttgcaagcgctaactacatttgtttcagtggctggtataatctacatcatttacaagttgtttgccggctttcagggtgcatacactggaatgcccaaccagaaacccaaggtgcccaccttaagacaagctaaggtgcaaggtccggcatttgaatttgccgtagcaatgatgaaaaggaacgccagcacagtcaagacagaatacggtgagttcacgatgcttggcatctatgataaatgggcagtgctgccgcgccacgccaagcctggaccaactattttaatgaatgatcaggaggttggtgtgctcgatgccaaagagttagttgataaagacggaaccaacctggagctgacactattgaagcttaaccgcaatgaaaagttcagagacatcagaggttttcttgcaagggaagaagttgaggtaagtgaggctgttttggcaataaacacgagcaagttcccaagcatgtacatccctgtgggccaagtcaccgattacggatttttaaatctaggtggcaccccaacaaagagaatgctcatgtacaacttccctaccagagcgggacagtgtggtggtgtccttatgtcaacaggaaaggtccttggcatacacgtgggaggaaatggtcaccaaggcttctctgctgctctcctcagacactacttcaacgaggaacagggcgaaatagagtttattgagagctctaaagatgcaggatttcctgtgatcaacacccctaataaaaccaaactggaaccaagtgtgtttcatcaggtttttgagggcaacaaagaaccagcagtcctaagaaacggagacccgcgacttaaagccaactttgaggaagcgatattttccaagtacatcggaaatgtgaacacacatgtggacgagtacatgatagaagctgttgatcactacgctggacagctggcaactctggacatcagtacagaacctatgaagcttgaggatgctgtttatggcactgaaggcttggaagcattggacttgaccactagcgcaggatatccttatgtcgccttgggcatcaagaaaagggatatcctctccaagaagactaaagatctcaccaagctgagggaatgcatggacaagtatggtctaaatctgccgatggtgacctacgtgaaggatgaactcaggtccgctgagaaagtagccaagggaaaatccagacttatagaagcttctagtctcaatgactcagtggccatgaggcagacatttgggaacctatacaagacattccacctcaacccaggcattgtcactggtagtgctgttgggtgcgacccagatgtgttttggagcaaaatacccgtgatgcttgacgggcaccttatagcttttgattactctggctacgacgctagcttgagcccagtgtggtttgcttgtttgaaactcctcctagggaaactagggtatactcataaggaaaccaattacatagactacctctgcaactcccatcacttatacagagataaacactatttcgtgaggggtggtatgccatcaggatgttcaggcaccagtatattcaacaccatgatcaacaacatcattattaggacccttatgctaaaggtctacaaaggtattgacctggatcagtttagaatgatcgcttacggggacgatgtgatagcctcttacccgtggcctattgatgcctcactactagcagaagcgggaaaggattatggtttgatcatgaccccagcagataaaggagagtgttttaatgaggtaacctggacaaatgtaaccttcttgaaaaggtactttagagctgatgaacaatatccattcttggtgcaccccgtgatgcccatgaaagacatacacgaatccattagatggaccaaagacccaaagaacactcaagatcatgtgcgctcgttatgcctattggcttggcacaatggggagcacgaatatgaggaatttatccgaaagatcagaagcgtgcctgttggacgctgtttgaccctcccggtgttctcaacactacgcaggaaatggttagattccttctaaaattagagtgcaatcaatgaactatgattggcttaaccctaccgcatgaaccgaactagacaaaagtgcggtaggggtaaattctccgcattcggtgcggaaaaaaaaaaaaaaaaaaaaaaaaaaaaaaaaaaaaaaaaaaaaaaaaaaaaaaaaaaaaaaaaaaaaaaaaaaaaaaaaaaaaaaaaaaaaaaaaaaaaaaaaaaaaaaaaaaaaaaaa

SEQ ID NO: 116 - protein, 1073 aa, synthetic construct
  REGION 1..1073: note = SFTS A antigen
MMKVIWFSSLICLVIQCSGDTGPIICAGPIHSNKSADIPHLLGYSEKICQIDRLIHVSSWLRNHSQFQGYVGQRGGRSQVSYYPAENSYSRWSGLLSPCDADWLGMLVVKKAKGSDMIVPGPSYKGKVFFERPTFDGYVGWGCGSGKSRTESGELCSSDSGTSSGLLPSDRVLWIGDVACQPMTPIPEETFLELKSFSQSEFPDICKIDGIVFNQCEGESLPQPFDVAWMDVGHSHKIIMREHKTKWVQESSSKDFVCYKEGTGPCSESEEKTCKTSGSCRGDMQFCKVAGCEHGEEASEAKCRCSLVHKPGEVVVSYGGMRVRPKCYGFSRMMATLEVNPPEQRIGQCTGCHLECINGGVRLITLTSELKSATVCASHFCSSATSGKKSTEIQFHSGSLVGKTAIHVKGALVDGTEFTFEGSCMFPDGCDAVDCTFCREFLKNPQCYPAKKWLFIIIVILLGYAGLMLLTNVLKAIGVWGSWVIAPVKLMFAIIKKLMRTVSCLMGKLMDRGRQVIHEEIGENREGNQDDVRIEMARPRRVRHWMYSPVILTILAIGLAEGCDEMVHADSKLVSCRQGSGNMKECVTTGRALLPAVNPGQEACLHFTAPGSPDSKCLKIKVKRINLKCKKSSSYFVPDARSRCTSVRRCRWAGDCQSGCPPHFTSNSFSDDWAGKMDRAGLGFSGCSDGCGGAACGCFNAAPSCIFWRKWVENPHGIIWKVSPCAAWVPSAVIELTMPSGEVRTFHPMSGIPTQVFKGVSVTYLGSDMEVSGLTDLCEIEELKSKKLALAPCNQAGMGVVGKVGEIQCSSEESARTIKKDGCIWNADLVGIELRVDDAVCYSKITSVEAVANYSAIPTTIGGLRFERSHDSQGKISGSPLDITAIRGSFSVNYRGLRLSLSEITATCTGEVTNVSGCYSCMTGAKVSIKLHSSKNSTAHVRCKGDETAFSVLEGVHSYTVSLSFDHAVVDEQCQLNCGGHESQVTLKGNLIFLDVPKFVDGSYMQTYHSTVPTGANIPSPTDWLNALFGNGLSRWILGVIGVLLGGLALFFLIMSLFKLGTKQVFRSRTKLA

SEQ ID NO: 117 - RNA, 3222 nt, synthetic construct
  source 1..3222: mol_type = other RNA
  misc_feature 1..3222: note = nucleotide sequence coding SFTS A antigen
atgatgaaagtcatctggttcagtagcctgatctgcctggtcatccagtgcggaggcgacaccggccctatcatttgcgccggacccatccactccaacaagtccgctgatattcctcacctgctgggctattctgaaaaaatctgccagatcgacagactgatccatgtgtccagctggctgagaaaccactcccagttccagggatatgtgggccagagaggcggccggtcccaggtgagctactaccctgctgaaaactcctacagcagatggagcgggctgctgtctccttgcgacgccgactggctgggcatgctggtggtgaagaaggccaagggtagtgacatgatcgtgcccggccctagctacaagggcaaggtgttctttgaacggcctacatttgacggttacgtgggatggggatgtggcagcggcaagagcagaacagaatctggagagctgtgctctagcgatagcggaaccagcagcggtctgctgcctagcgacagagtgctgtggatcggcgacgtggcttgtcagcctatgacccctatccccgaggaaaccttcctggaactgaagtcttttagccaaagcgagttccccgacatctgcaaaattgacggcatcgtgtttaatcagtgcgagggcgagagccttcctcaacccttcgacgtggcctggatggacgtgggccactcccacaagatcattatgagagaacacaagaccaagtgggtgcaagagtcctcttcgaaggacttcgtgtgctacaaggagggcaccggcccctgtagcgaaagcgaagagaagacctgtaaaaccagcggcagctgtagaggcgacatgcagttctgcaaggtggccggatgcgagcacggcgaagaggcctctgaagccaagtgcagatgcagcctggttcataagccaggagaagtggtcgtatcctacggcggcatgagagtgcggcccaagtgctacggttttagcagaatgatggccaccctggaagtcaaccagcctgagcaaagaatcggccaatgcaccggctgccacctggaatgcatcaacggcggcgttcggctgatcaccctgaccagcgagctgaagagcgctacagtgtgcgccagccacttctgcagcagcgccaccagcggcaagaagtccaccgaaatccagttccacagcggctccctggtcggcaaaacagctatccacgtgaagggcgccctggtggacggcaccgagttcaccttcgagggcagctgtatgttccctgacggatgtgatgccgtggattgcacattttgtcgggagttcctgaaaaacccccagtgctaccccgccaagaaatggctgtttatcattatcgtgatcctgctgggatacgccggcctgatgctgctgactaatgtgctgaaggctataggcgtgtggggcagctgggtcatcgcccctgtgaagctagtgttcgccatcatcaagaaactgatgcgggccgtgagctgtctgatgggcaagctgatggaccggggccggcaggtgattcacgaagaaatcggagagaacagagagggcaaccaggacgatgtgcgcatcgaaatggccagacccagacgggtgcgccactggatgtacagccctgtgatcctgacaatccttgctatcggcctggccgagggctgcgacgagatggtgcatgccgacagcaagctggtgagctgcagacagggtagcggaaacatgaaggagtgcgtcaccaccggcagagccctgctgcccgctgtaaaccctggccaggaggcctgcctccacttcaccgcccctggatcacctgatagcaagtgtctgaagatcaaggtgaaaagaatcaatctgaaatgcaaaaagtccagcagctacttcgtgcctgatgccagaagcagatgcacatctgtgcggcggtgcagatgggccggcgactgccagagcggctgtcctcctcacttcaccagcaacagcttctctgacgactgggccggaaagatggatagagccggcctgggcttcagcggatgtagcgatggctgcggcggcgccgcttgcggctgcttcaacgccgctcctagctgcatcttctggcggaagtgggttgagaacccacacggcatcatctggaaggtgtccccatgcgcggcctgggtgccaagcgccgtgatcgagctgaccatgcctagcggagaagtgcggacattccaccctatgagcggcatcccaacacaggtgttcaagggcgtctccgtgacatacctgggtagcgacatggaagtgtccggcttgacagacctgtgcgagatcgaggaactgaagtctaagaagctggccctggccccttgcaaccaggccggaatgggcgtggtgggcaaagtgggcgagatccaatgtagctctgaggaaagcgctagaaccataaagaaagacggctgcatctggaacgctgatctggtgggcatcgagctgcgtgtggatgacgccgtttgttacagcaagatcactagcgtggaggccgtggccaattactctgctatcccaacaacaatcggcggcctgagattcgagcggagccacgactctcagggcaaaatcagcggcagtcccctggacatcaccgccatcagaggctcatttagcgtgaactacagaggtctgcgtctgagcctctccgagatcaccgccacatgcaccggcgaggtgaccaacgtgtctggctgttactcatgcatgacaggagcgaaggtgtctatcaagctgcacagctctaagaacagcaccgcccacgtgcggtgcaagggcgatgaaaccgccttcagcgttctggagggcgtgcactcttatagtgtgagcctgagctttgatcacgccgtggtggacgagcagtgtcagctgaactgtggcgggcacgagagccaggtcaccctgcggggcaatctgattttcctggacgttcctaagttcgtggacggcagctacatgcagacctaccacagcaccgtgcccacaggcgccaatatcccttctccaaccgactggctgaacgcccttttcggcaacggcttgtctaggtggattctgggagtgatcggagtcctgctgggtggactggccctgttcttcctgatcatgagccttttcaagttgggcacaaagcaggtgttcagatcaagaaccaagttggcatga

SEQ ID NO: 118 - DNA, 3222 bp, synthetic construct
  source 1..3222: mol_type = other DNA
  misc_feature 1..3222: note = nucleotide sequence coding SFTS A antigen
atgatgaaagtcatctggttcagtagcctgatctgcctggtcatccagtgcggaggcgacaccggccctatcatttgcgccggacccatccactccaacaagtccgctgatattcctcacctgctgggctattctgaaaaaatctgccagatcgacagactgatccatgtgtccagctggctgagaaaccactcccagttccagggatatgtgggccagagaggcggccggtcccaggtgagctactaccctgctgaaaactcctacagcagatggagcgggctgctgtctccttgcgacgccgactggctgggcatgctggtggtgaagaaggccaagggtagtgacatgatcgtgcccggccctagctacaagggcaaggtgttctttgaacggcctacatttgacggttacgtgggatggggatgtggcagcggcaagagcagaacagaatctggagagctgtgctctagcgatagcggaaccagcagcggtctgctgcctagcgacagagtgctgtggatcggcgacgtggcttgtcagcctatgacccctatccccgaggaaaccttcctggaactgaagtcttttagccaaagcgagttccccgacatctgcaaaattgacggcatcgtgtttaatcagtgcgagggcgagagccttcctcaacccttcgacgtggcctggatggacgtgggccactcccacaagatcattatgagagaacacaagaccaagtgggtgcaagagtcctcttcgaaggacttcgtgtgctacaaggagggcaccggcccctgtagcgaaagcgaagagaagacctgtaaaaccagcggcagctgtagaggcgacatgcagttctgcaaggtggccggatgcgagcacggcgaagaggcctctgaagccaagtgcagatgcagcctggttcataagccaggagaagtggtcgtatcctacggcggcatgagagtgcggcccaagtgctacggttttagcagaatgatggccaccctggaagtcaaccagcctgagcaaagaatcggccaatgcaccggctgccacctggaatgcatcaacggcggcgttcggctgatcaccctgaccagcgagctgaagagcgctacagtgtgcgccagccacttctgcagcagcgccaccagcggcaagaagtccaccgaaatccagttccacagcggctccctggtcggcaaaacagctatccacgtgaagggcgccctggtggacggcaccgagttcaccttcgagggcagctgtatgttccctgacggatgtgatgccgtggattgcacattttgtcgggagttcctgaaaaacccccagtgctaccccgccaagaaatggctgtttatcattatcgtgatcctgctgggatacgccggcctgatgctgctgactaatgtgctgaaggctataggcgtgtggggcagctgggtcatcgcccctgtgaagctagtgttcgccatcatcaagaaactgatgcgggccgtgagctgtctgatgggcaagctgatggaccggggccggcaggtgattcacgaagaaatcggagagaacagagagggcaaccaggacgatgtgcgcatcgaaatggccagacccagacgggtgcgccactggatgtacagccctgtgatcctgacaatccttgctatcggcctggccgagggctgcgacgagatggtgcatgccgacagcaagctggtgagctgcagacagggtagcggaaacatgaaggagtgcgtcaccaccggcagagccctgctgcccgctgtaaaccctggccaggaggcctgcctccacttcaccgcccctggatcacctgatagcaagtgtctgaagatcaaggtgaaaagaatcaatctgaaatgcaaaaagtccagcagctacttcgtgcctgatgccagaagcagatgcacatctgtgcggcggtgcagatgggccggcgactgccagagcggctgtcctcctcacttcaccagcaacagcttctctgacgactgggccggaaagatggatagagccggcctgggcttcagcggatgtagcgatggctgcggcggcgccgcttgcggctgcttcaacgccgctcctagctgcatcttctggcggaagtgggttgagaacccacacggcatcatctggaaggtgtccccatgcgcggcctgggtgccaagcgccgtgatcgagctgaccatgcctagcggagaagtgcggacattccaccctatgagcggcatcccaacacaggtgttcaagggcgtctccgtgacatacctgggtagcgacatggaagtgtccggcttgacagacctgtgcgagatcgaggaactgaagtctaagaagctggccctggccccttgcaaccaggccggaatgggcgtggtgggcaaagtgggcgagatccaatgtagctctgaggaaagcgctagaaccataaagaaagacggctgcatctggaacgctgatctggtgggcatcgagctgcgtgtggatgacgccgtttgttacagcaagatcactagcgtggaggccgtggccaattactctgctatcccaacaacaatcggcggcctgagattcgagcggagccacgactctcagggcaaaatcagcggcagtcccctggacatcaccgccatcagaggctcatttagcgtgaactacagaggtctgcgtctgagcctctccgagatcaccgccacatgcaccggcgaggtgaccaacgtgtctggctgttactcatgcatgacaggagcgaaggtgtctatcaagctgcacagctctaagaacagcaccgcccacgtgcggtgcaagggcgatgaaaccgccttcagcgttctggagggcgtgcactcttatagtgtgagcctgagctttgatcacgccgtggtggacgagcagtgtcagctgaactgtggcgggcacgagagccaggtcaccctgcggggcaatctgattttcctggacgttcctaagttcgtggacggcagctacatgcagacctaccacagcaccgtgcccacaggcgccaatatcccttctccaaccgactggctgaacgcccttttcggcaacggcttgtctaggtggattctgggagtgatcggagtcctgctgggtggactggccctgttcttcctgatcatgagccttttcaagttgggcacaaagcaggtgttcagatcaagaaccaagttggcatga

SEQ ID NO: 119 - protein, 1073 aa, synthetic construct
  REGION 1..1073: note = SFTS DEF antigen
MMKVIWFSSLICFVIQCSGDSGPIICAGPIHSNKSADIPHLLGYSEKICQIDRLIHVSSWLRNHSQFQGYVGQRGGRSQVSYYPAENSYSRWSGLLSPCDADWLGMLVVKKAKGSDMIVPGPSYKGKVFFERPTFDGYVGWGCGSGKSRTESGELCSSDSGTSSGLLPSDRVLWIGDVACQPMTPIPEETFLELKSFSQSEFPDICKIDGIVFNQCEGESLPQPFDVAWMDVGHSHKIIMREHKTKWVQESSSKDFVCYKEGTGPCSESEEKTCKTSGSCRGDMQFCKVAGCEHGEEASEAKCRCSLVHKPGEVVVSYGGMRVRPKCYGFSRMMATLEVNPPEQRIGQCTGCHLECINGGVRLITLTSELKSATVCASHFCSSATSGKKSTEIQFHSGSLVGKTAIHVKGALVDGTEFTFEGSCMFPDGCDAVDCTFCREFLKNPQCYPAKKWLFIIIVILLGYAGLMLLTNVLKAIGVWGSWVIAPVKLMFAIIKKLMRTVSCLMGKLMDRGRQVIHEEIGENREGNQDDVRIEMARPRRVRHWMYSPVILTILAIGLAEGCDEMVHADSKLVSCRQGSGNMKECVTTGRALLPAVNPGQEACLHFTAPGSPDSKCLKIKVKRINLKCKKSSSYFVPDARSRCTSVRRCRWAGDCQSGCPPHFTSNSFSDDWAGKMDRAGLGFSGCSDGCGGAACGCFNAAPSCIFWRKWVENPHGIIWKVSPCAAWVPSAVIELTMPSGEVRTFHPMSGIPTQVFKGVSVTYLGSDMEVSGLTDLCEIEELKSKKLALAPCNQAGMGVVGKVGEIQCSSEESARTIKKDGCIWNADLVGIELRVDDAVCYSKITSVEAVANYSAIPTTIGGLRFERSHDSQGKISGSPLDITAIRGSFSVNYRGLRLSLSEITATCTGEVTNVSGCYSCMTGAKVSIKLHSSKNSTAHVRCKGDETAFSVLEGVHSYTVSLSFDHAVVDEQCQLNCGGHESQVTLKGNLIFLDVPKFVDGSYMQTYHSTVPTGANIPSPTDWLNALFGNGLSRWILGVIGVLLGGLALFFLIMSLFKLGTKQVFRSRTKLA

SEQ ID NO: 120 - RNA, 3222 nt, synthetic construct
  source 1..3222: mol_type = other RNA
  misc_feature 1..3222: note = nucleotide sequence coding SFTS DEF antigen
atgatgaaggtgatctggttctcttctctgatctgctttgtgatccagtgcagcggcgatagcgggccaatcatctgcgccggaccaatccacagcaacaagagcgccgacatcccccacctgcttggctactcagaaaaaatctgccagatcgacagactaatacacgtgagcagctggctgcggaaccacagccagtttcagggctatgtgggccagagaggaggcagaagccaagtgagctactaccctgctgaaaacagctacagcagatggtccggcctgctctccccatgtgatgccgattggctgggcatgctcgtggtgaagaaagccaagggctccgatatgatcgtgcccggccctagctacaaggggaaggtgtttttcgagagacctacattcgacggctacgtgggctggggctgcggcagcggcaaaagccggaccgagagcggcgaactgtgtagcagcgacagcggaacaagcagcggtctgctccccagcgaccgggtgctgtggatcggcgacgttgcctgtcagcccatgacccctatccccgaggagacatttctggaactgaagtcgttctcccagagcgagttccctgacatctgcaagattgacggcattgtgttcaatcagtgcgagggcgagagcctgcctcagcctttcgacgtggcttggatggatgtgggccacagccacaagatcatcatgagagagcacaaaaccaagtgggtccaggagtcgtccagcaaggacttcgtgtgttataaggaaggcacaggcccctgcagcgagtccgaagagaagacctgcaagaccagcggcagctgtagaggcgacatgcagttctgcaaagtggccggctgtgaacacggagaagaggccagcgaggctaagtgccggtgcagcctggtgcacaagcctggcgaggtggtcgtctcttacggcggcatgcgggtgcggcctaagtgctacggcttcagccggatgatggccaccctggaggtgaatccgcccgagcagcggatcggccagtgtaccggatgccacctggagtgcattaacggcggcgtgcggctgatcaccctgaccagcgaactgaagtctgctaccgtgtgcgcgagccatttctgcagctcagccaccagtggaaaaaagagcaccgagatccagttccacagcggctctctggtcggcaagacagccatccacgtgaagggcgccctggtggacggcaccgagttcacctttgagggcagctgcatgttccctgacggctgtgacgccgtggactgcaccttctgcagagagttcctgaaaaacccccagtgttaccccgctaagaaatggctgttcatcatcattgtcatcctgctgggctacgccggactcatgctgctgacaaacgtgctgaaggccatcggagtttggggaagttgggtgatcgcccctgtgaaactgatgttcgccatcatcaagaaactgatgcgaaccgtgagctgcctgatgggcaagttgatggatagaggcagacaggtgatccacgaggagatcggcgaaaacagagaaggcaaccaggacgacgtgcggatcgagatggccagacccagaagagtgcggcactggatgtactcccctgtgatcctgaccatcctggccatcggcctagctgaaggctgcgacgaaatggtgcacgccgactctaagctcgtctcatgccggcagggcagcggcaatatgaaggagtgtgtgacaaccggcagagccctgctgcctgccgtgaaccccggccaggaggcctgcctgcactttacggcccctggttctcccgacagcaagtgcctgaagatcaaggtcaagagaatcaacctgaaatgcaagaagagcagcagctacttcgtgcctgacgccagaagtagatgtacaagcgtgcgccgctgccgctgggcaggcgattgccagagcggatgtcctcctcacttcacctctaatagtttcagcgacgattgggctggcaaaatggaccgcgccggcctgggattttctggatgcagtgatggctgcggcggcgccgcctgcggatgttttaacgccgctcctagttgcatcttctggcggaagtgggtggaaaaccctcatggcatcatctggaaggtgagcccatgcgctgcttgggtgccttctgccgtgatcgagctgaccatgccttctggagaggtgcggacatttcaccctatgtccggcatccctacgcaggtgttcaagggcgtgtctgtgacatatctgggctccgacatggaagtgtccggtctgacagacctgtgcgaaatcgaggaactgaagtctaagaagctggccctggccccctgtaatcaagccggcatgggcgtggtgggcaaggtgggtgagatccaatgttcgagcgaggaaagcgcccggaccatcaaaaaagacggctgtatctggaacgctgatctggtgggcatcgagctgagagttgatgacgctgtttgctacagcaagatcacctccgtggaagccgtggccaattacagcgccatccccaccaccatcggcggcctgagattcgagagaagccacgatagccagggcaagatcagcggctcccctctggacattactgccatcagaggcagcttcagcgtgaactacagaggcctgaggctgtctctgagcgaaatcaccgctacatgcaccggagaagtgaccaacgtgtctggctgttacagctgtatgaccggcgcaaaagtgtctatcaagctgcactctagcaagaacagtacagcccacgtcagatgcaagggagatgagacagccttcagcgtgctggagggggttcacagctacaccgtgagcctgagctttgaccatgccgtggtggacgagcagtgccagctgaactgcggcggccacgagagccaggtaacactgaagggcaacctgatcttcctggatgtgccaaaattcgtggatggcagctacatgcaaacctaccacagtaccgttccaaccggcgccaacatccctagccctacagattggcttaacgccctgttcggcaacggcctgagcagatggattctgggcgtgattggagtgctgctgggtggactggcactgttcttcctgattatgtctctgttcaagctgggcacaaagcaggtgttcagatccagaaccaagctggcctga

SEQ ID NO: 121 - DNA, 3222 bp, synthetic construct
  source 1..3222: mol_type = other DNA
  misc_feature 1..3222: note = nucleotide sequence coding SFTS DEF antigen
atgatgaaggtgatctggttctcttctctgatctgctttgtgatccagtgcagcggcgatagcgggccaatcatctgcgccggaccaatccacagcaacaagagcgccgacatcccccacctgcttggctactcagaaaaaatctgccagatcgacagactaatacacgtgagcagctggctgcggaaccacagccagtttcagggctatgtgggccagagaggaggcagaagccaagtgagctactaccctgctgaaaacagctacagcagatggtccggcctgctctccccatgtgatgccgattggctgggcatgctcgtggtgaagaaagccaagggctccgatatgatcgtgcccggccctagctacaaggggaaggtgtttttcgagagacctacattcgacggctacgtgggctggggctgcggcagcggcaaaagccggaccgagagcggcgaactgtgtagcagcgacagcggaacaagcagcggtctgctccccagcgaccgggtgctgtggatcggcgacgttgcctgtcagcccatgacccctatccccgaggagacatttctggaactgaagtcgttctcccagagcgagttccctgacatctgcaagattgacggcattgtgttcaatcagtgcgagggcgagagcctgcctcagcctttcgacgtggcttggatggatgtgggccacagccacaagatcatcatgagagagcacaaaaccaagtgggtccaggagtcgtccagcaaggacttcgtgtgttataaggaaggcacaggcccctgcagcgagtccgaagagaagacctgcaagaccagcggcagctgtagaggcgacatgcagttctgcaaagtggccggctgtgaacacggagaagaggccagcgaggctaagtgccggtgcagcctggtgcacaagcctggcgaggtggtcgtctcttacggcggcatgcgggtgcggcctaagtgctacggcttcagccggatgatggccaccctggaggtgaatccgcccgagcagcggatcggccagtgtaccggatgccacctggagtgcattaacggcggcgtgcggctgatcaccctgaccagcgaactgaagtctgctaccgtgtgcgcgagccatttctgcagctcagccaccagtggaaaaaagagcaccgagatccagttccacagcggctctctggtcggcaagacagccatccacgtgaagggcgccctggtggacggcaccgagttcacctttgagggcagctgcatgttccctgacggctgtgacgccgtggactgcaccttctgcagagagttcctgaaaaacccccagtgttaccccgctaagaaatggctgttcatcatcattgtcatcctgctgggctacgccggactcatgctgctgacaaacgtgctgaaggccatcggagtttggggaagttgggtgatcgcccctgtgaaactgatgttcgccatcatcaagaaactgatgcgaaccgtgagctgcctgatgggcaagttgatggatagaggcagacaggtgatccacgaggagatcggcgaaaacagagaaggcaaccaggacgacgtgcggatcgagatggccagacccagaagagtgcggcactggatgtactcccctgtgatcctgaccatcctggccatcggcctagctgaaggctgcgacgaaatggtgcacgccgactctaagctcgtctcatgccggcagggcagcggcaatatgaaggagtgtgtgacaaccggcagagccctgctgcctgccgtgaaccccggccaggaggcctgcctgcactttacggcccctggttctcccgacagcaagtgcctgaagatcaaggtcaagagaatcaacctgaaatgcaagaagagcagcagctacttcgtgcctgacgccagaagtagatgtacaagcgtgcgccgctgccgctgggcaggcgattgccagagcggatgtcctcctcacttcacctctaatagtttcagcgacgattgggctggcaaaatggaccgcgccggcctgggattttctggatgcagtgatggctgcggcggcgccgcctgcggatgttttaacgccgctcctagttgcatcttctggcggaagtgggtggaaaaccctcatggcatcatctggaaggtgagcccatgcgctgcttgggtgccttctgccgtgatcgagctgaccatgccttctggagaggtgcggacatttcaccctatgtccggcatccctacgcaggtgttcaagggcgtgtctgtgacatatctgggctccgacatggaagtgtccggtctgacagacctgtgcgaaatcgaggaactgaagtctaagaagctggccctggccccctgtaatcaagccggcatgggcgtggtgggcaaggtgggtgagatccaatgttcgagcgaggaaagcgcccggaccatcaaaaaagacggctgtatctggaacgctgatctggtgggcatcgagctgagagttgatgacgctgtttgctacagcaagatcacctccgtggaagccgtggccaattacagcgccatccccaccaccatcggcggcctgagattcgagagaagccacgatagccagggcaagatcagcggctcccctctggacattactgccatcagaggcagcttcagcgtgaactacagaggcctgaggctgtctctgagcgaaatcaccgctacatgcaccggagaagtgaccaacgtgtctggctgttacagctgtatgaccggcgcaaaagtgtctatcaagctgcactctagcaagaacagtacagcccacgtcagatgcaagggagatgagacagccttcagcgtgctggagggggttcacagctacaccgtgagcctgagctttgaccatgccgtggtggacgagcagtgccagctgaactgcggcggccacgagagccaggtaacactgaagggcaacctgatcttcctggatgtgccaaaattcgtggatggcagctacatgcaaacctaccacagtaccgttccaaccggcgccaacatccctagccctacagattggcttaacgccctgttcggcaacggcctgagcagatggattctgggcgtgattggagtgctgctgggtggactggcactgttcttcctgattatgtctctgttcaagctgggcacaaagcaggtgttcagatccagaaccaagctggcctga

SEQ ID NO: 122 - RNA, 3605 nt, synthetic construct
  source 1..3605: mol_type = other RNA
  misc_feature 1..3605: note = SFTS A mRNA construct
gagaataaactagtattcttctggtccccacagactcaatgatgaaagtcatctggttcagtagcctgatctgcctggtcatccagtgcggaggcgacaccggccctatcatttgcgccggacccatccactccaacaagtccgctgatattcctcacctgctgggctattctgaaaaaatctgccagatcgacagactgatccatgtgtccagctggctgagaaaccactcccagttccagggatatgtgggccagagaggcggccggtcccaggtgagctactaccctgctgaaaactcctacagcagatggagcgggctgctgtctccttgcgacgccgactggctgggcatgctggtggtgaagaaggccaagggtagtgacatgatcgtgcccggccctagctacaagggcaaggtgttctttgaacggcctacatttgacggttacgtgggatggggatgtggcagcggcaagagcagaacagaatctggagagctgtgctctagcgatagcggaaccagcagcggtctgctgcctagcgacagagtgctgtggatcggcgacgtggcttgtcagcctatgacccctatccccgaggaaaccttcctggaactgaagtcttttagccaaagcgagttccccgacatctgcaaaattgacggcatcgtgtttaatcagtgcgagggcgagagccttcctcaacccttcgacgtggcctggatggacgtgggccactcccacaagatcattatgagagaacacaagaccaagtgggtgcaagagtcctcttcgaaggacttcgtgtgctacaaggagggcaccggcccctgtagcgaaagcgaagagaagacctgtaaaaccagcggcagctgtagaggcgacatgcagttctgcaaggtggccggatgcgagcacggcgaagaggcctctgaagccaagtgcagatgcagcctggttcataagccaggagaagtggtcgtatcctacggcggcatgagagtgcggcccaagtgctacggttttagcagaatgatggccaccctggaagtcaaccagcctgagcaaagaatcggccaatgcaccggctgccacctggaatgcatcaacggcggcgttcggctgatcaccctgaccagcgagctgaagagcgctacagtgtgcgccagccacttctgcagcagcgccaccagcggcaagaagtccaccgaaatccagttccacagcggctccctggtcggcaaaacagctatccacgtgaagggcgccctggtggacggcaccgagttcaccttcgagggcagctgtatgttccctgacggatgtgatgccgtggattgcacattttgtcgggagttcctgaaaaacccccagtgctaccccgccaagaaatggctgtttatcattatcgtgatcctgctgggatacgccggcctgatgctgctgactaatgtgctgaaggctataggcgtgtggggcagctgggtcatcgcccctgtgaagctagtgttcgccatcatcaagaaactgatgcgggccgtgagctgtctgatgggcaagctgatggaccggggccggcaggtgattcacgaagaaatcggagagaacagagagggcaaccaggacgatgtgcgcatcgaaatggccagacccagacgggtgcgccactggatgtacagccctgtgatcctgacaatccttgctatcggcctggccgagggctgcgacgagatggtgcatgccgacagcaagctggtgagctgcagacagggtagcggaaacatgaaggagtgcgtcaccaccggcagagccctgctgcccgctgtaaaccctggccaggaggcctgcctccacttcaccgcccctggatcacctgatagcaagtgtctgaagatcaaggtgaaaagaatcaatctgaaatgcaaaaagtccagcagctacttcgtgcctgatgccagaagcagatgcacatctgtgcggcggtgcagatgggccggcgactgccagagcggctgtcctcctcacttcaccagcaacagcttctctgacgactgggccggaaagatggatagagccggcctgggcttcagcggatgtagcgatggctgcggcggcgccgcttgcggctgcttcaacgccgctcctagctgcatcttctggcggaagtgggttgagaacccacacggcatcatctggaaggtgtccccatgcgcggcctgggtgccaagcgccgtgatcgagctgaccatgcctagcggagaagtgcggacattccaccctatgagcggcatcccaacacaggtgttcaagggcgtctccgtgacatacctgggtagcgacatggaagtgtccggcttgacagacctgtgcgagatcgaggaactgaagtctaagaagctggccctggccccttgcaaccaggccggaatgggcgtggtgggcaaagtgggcgagatccaatgtagctctgaggaaagcgctagaaccataaagaaagacggctgcatctggaacgctgatctggtgggcatcgagctgcgtgtggatgacgccgtttgttacagcaagatcactagcgtggaggccgtggccaattactctgctatcccaacaacaatcggcggcctgagattcgagcggagccacgactctcagggcaaaatcagcggcagtcccctggacatcaccgccatcagaggctcatttagcgtgaactacagaggtctgcgtctgagcctctccgagatcaccgccacatgcaccggcgaggtgaccaacgtgtctggctgttactcatgcatgacaggagcgaaggtgtctatcaagctgcacagctctaagaacagcaccgcccacgtgcggtgcaagggcgatgaaaccgccttcagcgttctggagggcgtgcactcttatagtgtgagcctgagctttgatcacgccgtggtggacgagcagtgtcagctgaactgtggcgggcacgagagccaggtcaccctgcggggcaatctgattttcctggacgttcctaagttcgtggacggcagctacatgcagacctaccacagcaccgtgcccacaggcgccaatatcccttctccaaccgactggctgaacgcccttttcggcaacggcttgtctaggtggattctgggagtgatcggagtcctgctgggtggactggccctgttcttcctgatcatgagccttttcaagttgggcacaaagcaggtgttcagatcaagaaccaagttggcatgactcgagctggtactgcatgcacgcaatgctagctgcccctttcccgtcctgggtaccccgagtctcccccgacctcgggtcccaggtatgctcccacctccacctgccccactcaccacctctgctagttccagacacctcccaagcacgcagcaatgcagctcaaaacgcttagcctagccacacccccacgggaaacagcagtgattaacctttagcaataaacgaaagtttaactaagctatactaaccccagggttggtcaatttcgtgccagccacaccctggagctagcaaaaaaaaaaaaaaaaaaaaaaaaaaaaaaaaaaaaaaaaaaaaaaaaaa

SEQ ID NO: 123 - RNA, 3605 nt, synthetic construct
  source 1..3605: mol_type = other RNA
  misc_feature 1..3605: note = SFTS B mRNA construct
gagaataaactagtattcttctggtccccacagactcaatgatgaaggtgatctggttcagctcccttatctgtctggtgattcagtgttctggcgacaccggccctatcatctgtgccggacccatccatagcaacaagagcgccaatatcccccacctgctgggctacagtgagaaaatctgccagatcgacagactgatccacgtgagcagctggctgagaaaccactctcaatttcagggctacgtaggtcagagaggcggtcggagccaggtgagctactaccctgccgagaactcttatagccggtggtctggattgctgtcgccttgcgacgccgattggctggggatgctggtcgtgaaaaaggccaagggcagcgatatgatcgtgccaggcccttcttataaaggcaaggtgttcttcgaaagacctacatttgacggatatgtgggatggggctgcggctccggcaagagcagaacagaatccggcgagctgtgcagctctgattctggaaccagcagcggactgctgccttctgatagagtgctgtggatcggcgatgtggcctgccagcctatgacccctatacccgaggaaacattcctggaactgaaaagttttagccagagcgagtttcctgacatctgcaagatcgacggaatcgtgtttaaccagtgcgagtctgagagccttcctcagcctttcgacgtggcctggatggatgtgggccacagccacaagatcatcatgagagagcacaagaccaagtgggtgcaggagagcagcagcaaagacttcgtctgctacaaggaaggcaccggcccatgctctgagagcgaggaaaagacctgtaaaaccagtggctcttgcaggggcgacatgcagttctgtaaggttgccgggtgcgaacacggcgaggaggcctctgaggccaagtgcagatgctccctggtgcacaaacctggggaggtggtggtgagctacggcggcatgcgggtgcggcccaagtgctacggcttctccagaatgatggccaccctggaagtgaatcctccagagcagcggatcggccagtgtacaggctgccacctggaatgcattaacggcggagtcaggctgattacactaacctccgagctgaagtctgccacagtgtgcgcgagccacttctgcagcagcgccacaagcggcaagaagtctacagagatccagttccacagcggcagcctggtgggcaagaccgccatccatgtgaagggcgccctggtggacggcacagagttcacctttgagggctcctgcatgttccccgatggctgtgatgccgtggactgcaccttctgcagagagttcctgaagaacccacagtgttaccctgccaagaagtggctgttcatcatcatcgtgatcctgctcggctacgccggactgatgttgctgaccaacgtgctgaaggccatcggcgtgtggggctcctgggtcatcgcccccgtcaagctgatgttcgccatcatcaagaagctgatgcgcagcgtgtcgtgcctgatgggcaagctcatggatagaggcagacaggtgattcacgaggagatcggcgagaacagagagggaaaccaagacgatgtgcggatcgaaatggccagacctcggagagtgcggcactggatgtacagccctgtgatccttacaatcctggccatcggcctggccgaaggctgtgacgagatggtgcacgccgactccaagctggtctcttgcaaacagggctccggaaatatgaaggagtgtgtgaccaccggaagagccctgctgcctgccgtgaaccctggacaggaggcttgcctgcatttcaccgcccctggtagccctgacagcaaatgtctgaaaatcaaagtgaaacgaatcaacctgaagtgcaaaaagtcaagctcttacttcgtgcccgacgcacgatctcggtgtaccagcgttcggcggtgcagatgggccggcgattgccagagcggctgtccttcccatttcacaagcaacagcttcagtgacgactgggccggcaagatggatagagccggcctggggttctccggctgttccgacggctgcggaggagctgcttgtggctgcttcaacgccgctccaagctgcatcttctggagaaagtgggtggaaaatcctcacggcatcatctggaaggtgagcccatgcgctgcctgggtgccctcggctgtcatcgagctgacaatgccttctggcgaagtgcggacatttcaccccatgagcggcatccccacccaggttttcaagggggtgagcgtgacctacctgggcagcgacatggaagtgagcggcctgacagacctgtgcgagatcgaggaactgaaaagcaagaagctggccctggctccttgcaaccaggccggaatgggcgtggtgggaaaggtgggagaaatccaatgtagctccgaagaaagcgccagaaccattaagaaggacgggtgcatctggaacgctgatctggtcggtattgaactgcgagtggacgacgccgtgtgctactccaaaatcaccagtgttgaggccgtcgccaattacagcgccattcccaccactatcggcggactgaggttcgagagaagccacgactctcagggcaagatcagcggcagcccactggacatcacagccatcagaggctcattctccgtgaactaccggggcttgagactgtctctgagcgaaatcaccgccacctgcaccggcgaggtgacaaacgtgtccggctgctacagctgtatgaccggcgccaaggtgtctatcaagctgcactccagcaagaacagcaccgcccacgtgagatgtaaaggcgacgagacagctttcagcgtgctggagggcgtacacagctacaccgtgtccctgagcttcgaccacgccgtggtggacgagcagtgccagctaaactgcggaggccacgaaagccaagtgaccctgaagggcaacctgatcttcctggatgtgcctaagttcgtggacggcagctacatgcaaacataccacagctcagtgcctacgggcgccaacatcccttctccaaccgactggctgaacgctctgtttggcaatggactgagcaggtggattctgggcgtgatcggggtgctgctgggcggcctggccctgttcttcctgataatgagcctgtttaagctgggcaccaagcaggtgttcagatccagaaccaagctggcttgactcgagctggtactgcatgcacgcaatgctagctgcccctttcccgtcctgggtaccccgagtctcccccgacctcgggtcccaggtatgctcccacctccacctgccccactcaccacctctgctagttccagacacctcccaagcacgcagcaatgcagctcaaaacgcttagcctagccacacccccacgggaaacagcagtgattaacctttagcaataaacgaaagtttaactaagctatactaaccccagggttggtcaatttcgtgccagccacaccctggagctagcaaaaaaaaaaaaaaaaaaaaaaaaaaaaaaaaaaaaaaaaaaaaaaaaaa

SEQ ID NO: 124 - RNA, 3605 nt, synthetic construct
  source 1..3605: mol_type = other RNA
  misc_feature 1..3605: note = SFTS DEF mRNA construct
gagaataaactagtattcttctggtccccacagactcaatgatgaaggtgatctggttctcttctctgatctgctttgtgatccagtgcagcggcgatagcgggccaatcatctgcgccggaccaatccacagcaacaagagcgccgacatcccccacctgcttggctactcagaaaaaatctgccagatcgacagactaatacacgtgagcagctggctgcggaaccacagccagtttcagggctatgtgggccagagaggaggcagaagccaagtgagctactaccctgctgaaaacagctacagcagatggtccggcctgctctccccatgtgatgccgattggctgggcatgctcgtggtgaagaaagccaagggctccgatatgatcgtgcccggccctagctacaaggggaaggtgtttttcgagagacctacattcgacggctacgtgggctggggctgcggcagcggcaaaagccggaccgagagcggcgaactgtgtagcagcgacagcggaacaagcagcggtctgctccccagcgaccgggtgctgtggatcggcgacgttgcctgtcagcccatgacccctatccccgaggagacatttctggaactgaagtcgttctcccagagcgagttccctgacatctgcaagattgacggcattgtgttcaatcagtgcgagggcgagagcctgcctcagcctttcgacgtggcttggatggatgtgggccacagccacaagatcatcatgagagagcacaaaaccaagtgggtccaggagtcgtccagcaaggacttcgtgtgttataaggaaggcacaggcccctgcagcgagtccgaagagaagacctgcaagaccagcggcagctgtagaggcgacatgcagttctgcaaagtggccggctgtgaacacggagaagaggccagcgaggctaagtgccggtgcagcctggtgcacaagcctggcgaggtggtcgtctcttacggcggcatgcgggtgcggcctaagtgctacggcttcagccggatgatggccaccctggaggtgaatccgcccgagcagcggatcggccagtgtaccggatgccacctggagtgcattaacggcggcgtgcggctgatcaccctgaccagcgaactgaagtctgctaccgtgtgcgcgagccatttctgcagctcagccaccagtggaaaaaagagcaccgagatccagttccacagcggctctctggtcggcaagacagccatccacgtgaagggcgccctggtggacggcaccgagttcacctttgagggcagctgcatgttccctgacggctgtgacgccgtggactgcaccttctgcagagagttcctgaaaaacccccagtgttaccccgctaagaaatggctgttcatcatcattgtcatcctgctgggctacgccggactcatgctgctgacaaacgtgctgaaggccatcggagtttggggaagttgggtgatcgcccctgtgaaactgatgttcgccatcatcaagaaactgatgcgaaccgtgagctgcctgatgggcaagttgatggatagaggcagacaggtgatccacgaggagatcggcgaaaacagagaaggcaaccaggacgacgtgcggatcgagatggccagacccagaagagtgcggcactggatgtactcccctgtgatcctgaccatcctggccatcggcctagctgaaggctgcgacgaaatggtgcacgccgactctaagctcgtctcatgccggcagggcagcggcaatatgaaggagtgtgtgacaaccggcagagccctgctgcctgccgtgaaccccggccaggaggcctgcctgcactttacggcccctggttctcccgacagcaagtgcctgaagatcaaggtcaagagaatcaacctgaaatgcaagaagagcagcagctacttcgtgcctgacgccagaagtagatgtacaagcgtgcgccgctgccgctgggcaggcgattgccagagcggatgtcctcctcacttcacctctaatagtttcagcgacgattgggctggcaaaatggaccgcgccggcctgggattttctggatgcagtgatggctgcggcggcgccgcctgcggatgttttaacgccgctcctagttgcatcttctggcggaagtgggtggaaaaccctcatggcatcatctggaaggtgagcccatgcgctgcttgggtgccttctgccgtgatcgagctgaccatgccttctggagaggtgcggacatttcaccctatgtccggcatccctacgcaggtgttcaagggcgtgtctgtgacatatctgggctccgacatggaagtgtccggtctgacagacctgtgcgaaatcgaggaactgaagtctaagaagctggccctggccccctgtaatcaagccggcatgggcgtggtgggcaaggtgggtgagatccaatgttcgagcgaggaaagcgcccggaccatcaaaaaagacggctgtatctggaacgctgatctggtgggcatcgagctgagagttgatgacgctgtttgctacagcaagatcacctccgtggaagccgtggccaattacagcgccatccccaccaccatcggcggcctgagattcgagagaagccacgatagccagggcaagatcagcggctcccctctggacattactgccatcagaggcagcttcagcgtgaactacagaggcctgaggctgtctctgagcgaaatcaccgctacatgcaccggagaagtgaccaacgtgtctggctgttacagctgtatgaccggcgcaaaagtgtctatcaagctgcactctagcaagaacagtacagcccacgtcagatgcaagggagatgagacagccttcagcgtgctggagggggttcacagctacaccgtgagcctgagctttgaccatgccgtggtggacgagcagtgccagctgaactgcggcggccacgagagccaggtaacactgaagggcaacctgatcttcctggatgtgccaaaattcgtggatggcagctacatgcaaacctaccacagtaccgttccaaccggcgccaacatccctagccctacagattggcttaacgccctgttcggcaacggcctgagcagatggattctgggcgtgattggagtgctgctgggtggactggcactgttcttcctgattatgtctctgttcaagctgggcacaaagcaggtgttcagatccagaaccaagctggcctgactcgagctggtactgcatgcacgcaatgctagctgcccctttcccgtcctgggtaccccgagtctcccccgacctcgggtcccaggtatgctcccacctccacctgccccactcaccacctctgctagttccagacacctcccaagcacgcagcaatgcagctcaaaacgcttagcctagccacacccccacgggaaacagcagtgattaacctttagcaataaacgaaagtttaactaagctatactaaccccagggttggtcaatttcgtgccagccacaccctggagctagcaaaaaaaaaaaaaaaaaaaaaaaaaaaaaaaaaaaaaaaaaaaaaaaaaa

SEQ ID NO: 125 - RNA, 3605 nt, synthetic construct
  source 1..3605: mol_type = other RNA
  misc_feature 1..3605: note = SFTS ABDEF mRNA construct
gagaataaactagtattcttctggtccccacagactcaatgatgaaggttatctggttctccagcctgatctgtctggtgatccagtgtagcggcgacaccggacctatcatttgtgccggccctatccactccaacaagtccgccgacatcccccacctcctgggatactctgaaaaaatctgccaaatcgatagactgatccacgtgtccagctggctgcgaaaccacagccagttccagggctatgtgggccaaagaggaggcagaagccaggtgagctactaccccgccgagaatagctacagcagatggtccggcctgctgagcccttgcgacgccgattggctgggaatgctggtggtgaagaaggccaagggcagcgacatgatcgtgcccggccctagctacaagggcaaggtctttttcgaacggcccacctttgatggctacgtgggctggggatgcggctctggcaaaagccggacagaatctggagagctgtgcagcagcgacagcggcaccagctctggcctgctgccttcggatagagtgctgtggatcggcgatgtcgcatgccagcctatgacccctatccctgaggagacattcctggagctgaaatctttcagtcaaagcgagttccccgacatctgtaagatcgacggcatcgtgtttaaccagtgtgaaggcgaatccctgcctcagccgttcgacgtggcctggatggacgtcggccacagccacaagatcatcatgagagagcacaaaaccaagtgggtccaggagtctagcagcaaagacttcgtgtgctataaggaaggaacaggcccttgctccgagagcgaggaaaagacatgcaagaccagcgggtcttgcagaggagacatgcagttttgtaaagtggccggatgcgagcacggcgaggaggccagcgaggctaagtgccgctgtagcctcgttcacaagccaggagaggtggttgtgtcctacggcggcatgcgggtgagacccaagtgctacggcttcagcagaatgatggccacactggaggtgaatccacctgaacagcggatcggccagtgcaccggctgccacctggaatgcatcaacggcggcgtgagactgataacactgactagcgaactgaagagcgccacagtgtgcgccagccacttctgctcaagcgccaccagcggcaagaaatctactgagatccagttccactccggcagcctggtcggcaagaccgccatccacgtgaagggcgctctggtggatggcacagagttcacgttcgagggctcatgcatgttccctgatggctgcgacgccgtggactgcaccttctgccgggagttcctgaaaaacccccagtgttatcctgctaaaaagtggctgttcatcatcatcgtgatcctgctcggatacgccggcctgatgctgctgaccaacgtgctgaaggccatcggcgtgtggggcagctgggtgatcgcccccgtgaagctgatgttcgccatcatcaagaaactcatgagaaccgtgtcctgcctgatgggcaagctgatggaccggggcagacaggtgatccatgaggaaattggcgagaacagagagggcaaccaggacgacgtaagaatcgagatggccagacccagacgggtgcggcactggatgtacagccctgtgattttgaccatcctggctatcggactggctgaaggctgcgacgagatggtgcatgctgattctaaactggtatcttgtagacagggcagcggaaacatgaaagaatgcgtgaccaccggtcgggccctcctgcccgctgtgaatcccggccaggaggcctgcctgcacttcaccgcccctggcagccccgatagcaagtgcctgaagattaaggtgaagcggatcaacctgaagtgcaagaaatctagcagctacttcgtgcctgacgctagatccagatgcacctctgttaggagatgtagatgggccggagactgccagagcggctgccctcctcatttcacaagcaacagcttcagcgatgattgggccggaaaaatggacagagccggcctcggattctccgggtgcagcgatggatgcggaggcgccgcctgcggctgcttcaacgccgctcctagctgtatcttctggcggaagtgggtggaaaaccctcacggcatcatctggaaggttagcccatgcgccgcctgggtgccctctgccgtaatcgagctgaccatgccttctggtgaagtgcggacttttcaccccatgtcgggcatccctacccaggtgttcaagggcgtgagcgtgacctacctgggcagcgacatggaagtgagcggcctgacagacctgtgtgaaattgaagagctgaagtctaaaaagctggccctggcgccctgtaaccaagccggcatgggagtggtgggaaaggtcggcgagatccagtgcagctccgaggagagcgccagaacaatcaagaaagacggctgtatctggaacgccgatctggtgggcatcgagcttagagtggacgacgccgtgtgctacagcaagatcacctccgtggaagccgttgctaattacagcgccatccctaccacaatcggcggcctgcggttcgagcggtctcacgacagccaaggcaaaatcagcggcagccctctggacattaccgccatcagaggctcttttagcgtgaactacagaggcctgagattgtctctgtctgagatcaccgcaacctgtacaggcgaggtgacaaacgtgtccggctgctacagctgtatgaccggcgctaaggtgtctatcaagctgcactccagcaagaacagcacagcccacgtgcggtgcaagggcgacgaaaccgccttcagtgtgctggaaggcgtgcacagctacaccgtgagcctgagcttcgaccacgccgtcgtggacgagcagtgccagctgaactgcggcggtcacgagagccaggtgaccctgaagggaaacctgatcttcctggacgtgccaaagttcgtggacggcagctacatgcagacctaccacagcaccgtgcctaccggagccaacatcccatctcctacagattggctgaacgccctgttcggcaatggcctgtccagatggattctgggagtgatcggcgtgctgctgggcggcctggccctgttcttcctgatcatgtccctgtttaagctgggcacaaagcaggtctttagaagtcgcaccaagctcgcttgactcgagctggtactgcatgcacgcaatgctagctgcccctttcccgtcctgggtaccccgagtctcccccgacctcgggtcccaggtatgctcccacctccacctgccccactcaccacctctgctagttccagacacctcccaagcacgcagcaatgcagctcaaaacgcttagcctagccacacccccacgggaaacagcagtgattaacctttagcaataaacgaaagtttaactaagctatactaaccccagggttggtcaatttcgtgccagccacaccctggagctagcaaaaaaaaaaaaaaaaaaaaaaaaaaaaaaaaaaaaaaaaaaaaaaaaaa

SEQ ID NO: 126 - DNA, 8255 bp, synthetic construct
  source 1..8255: mol_type = other DNA
  misc_feature 1..8255: note = SFTS A DNA vector construct
ttaaaacagcctgtgggttgtacccacccacagggcccactgggcgctagcactctggtatcacggtacctttgtgtgcctgttttatatcccctttccccgattgtaacttagaagatgtacacactgatcaatagcgggcatagcacaccagctatgtcttgatcaagcactcctgtatccccggaccaagtatcaatagactgctcacgcggttgaaggagaaaacgttcgtcacccggctaactacttcgagaaacccagtagtatcatgaaagttgcgaggcgtttcgttcagcacacccccagtgtagatcgggtcgatgagtcaccgcatcccccacgggcgaccgtggcggtggctgcgctggcggcctgcctacggggcaacccgtaggacgcttcaatacagacatggtgcgaagagtcgattgagctagttagtagtcctccggcccctgaatgcggctaatcctaactgcggagcacatgccctcaacccagggggtattgtgtcgtaacgggcaactctgcagcggaaccgactactttgggtgtccgtgtttccttttatccttatactggctgcttatggtgacaattgaaagattgttgccatatagctattggattggccatccagtgtctaatagagctgttatttacctctttgttggatttataccactcaacctaaaagaagttaaaacactacagctcattttacaactgaatacagcaaaccaccatgatgaaagtcatctggttcagtagcctgatctgcctggtcatccagtgcggaggcgacaccggccctatcatttgcgccggacccatccactccaacaagtccgctgatattcctcacctgctgggctattctgaaaaaatctgccagatcgacagactgatccatgtgtccagctggctgagaaaccactcccagttccagggatatgtgggccagagaggcggccggtcccaggtgagctactaccctgctgaaaactcctacagcagatggagcgggctgctgtctccttgcgacgccgactggctgggcatgctggtggtgaagaaggccaagggtagtgacatgatcgtgcccggccctagctacaagggcaaggtgttctttgaacggcctacatttgacggttacgtgggatggggatgtggcagcggcaagagcagaacagaatctggagagctgtgctctagcgatagcggaaccagcagcggtctgctgcctagcgacagagtgctgtggatcggcgacgtggcttgtcagcctatgacccctatccccgaggaaaccttcctggaactgaagtcttttagccaaagcgagttccccgacatctgcaaaattgacggcatcgtgtttaatcagtgcgagggcgagagccttcctcaacccttcgacgtggcctggatggacgtgggccactcccacaagatcattatgagagaacacaagaccaagtgggtgcaagagtcctcttcgaaggacttcgtgtgctacaaggagggcaccggcccctgtagcgaaagcgaagagaagacctgtaaaaccagcggcagctgtagaggcgacatgcagttctgcaaggtggccggatgcgagcacggcgaagaggcctctgaagccaagtgcagatgcagcctggttcataagccaggagaagtggtcgtatcctacggcggcatgagagtgcggcccaagtgctacggttttagcagaatgatggccaccctggaagtcaaccagcctgagcaaagaatcggccaatgcaccggctgccacctggaatgcatcaacggcggcgttcggctgatcaccctgaccagcgagctgaagagcgctacagtgtgcgccagccacttctgcagcagcgccaccagcggcaagaagtccaccgaaatccagttccacagcggctccctggtcggcaaaacagctatccacgtgaagggcgccctggtggacggcaccgagttcaccttcgagggcagctgtatgttccctgacggatgtgatgccgtggattgcacattttgtcgggagttcctgaaaaacccccagtgctaccccgccaagaaatggctgtttatcattatcgtgatcctgctgggatacgccggcctgatgctgctgactaatgtgctgaaggctataggcgtgtggggcagctgggtcatcgcccctgtgaagctagtgttcgccatcatcaagaaactgatgcgggccgtgagctgtctgatgggcaagctgatggaccggggccggcaggtgattcacgaagaaatcggagagaacagagagggcaaccaggacgatgtgcgcatcgaaatggccagacccagacgggtgcgccactggatgtacagccctgtgatcctgacaatccttgctatcggcctggccgagggctgcgacgagatggtgcatgccgacagcaagctggtgagctgcagacagggtagcggaaacatgaaggagtgcgtcaccaccggcagagccctgctgcccgctgtaaaccctggccaggaggcctgcctccacttcaccgcccctggatcacctgatagcaagtgtctgaagatcaaggtgaaaagaatcaatctgaaatgcaaaaagtccagcagctacttcgtgcctgatgccagaagcagatgcacatctgtgcggcggtgcagatgggccggcgactgccagagcggctgtcctcctcacttcaccagcaacagcttctctgacgactgggccggaaagatggatagagccggcctgggcttcagcggatgtagcgatggctgcggcggcgccgcttgcggctgcttcaacgccgctcctagctgcatcttctggcggaagtgggttgagaacccacacggcatcatctggaaggtgtccccatgcgcggcctgggtgccaagcgccgtgatcgagctgaccatgcctagcggagaagtgcggacattccaccctatgagcggcatcccaacacaggtgttcaagggcgtctccgtgacatacctgggtagcgacatggaagtgtccggcttgacagacctgtgcgagatcgaggaactgaagtctaagaagctggccctggccccttgcaaccaggccggaatgggcgtggtgggcaaagtgggcgagatccaatgtagctctgaggaaagcgctagaaccataaagaaagacggctgcatctggaacgctgatctggtgggcatcgagctgcgtgtggatgacgccgtttgttacagcaagatcactagcgtggaggccgtggccaattactctgctatcccaacaacaatcggcggcctgagattcgagcggagccacgactctcagggcaaaatcagcggcagtcccctggacatcaccgccatcagaggctcatttagcgtgaactacagaggtctgcgtctgagcctctccgagatcaccgccacatgcaccggcgaggtgaccaacgtgtctggctgttactcatgcatgacaggagcgaaggtgtctatcaagctgcacagctctaagaacagcaccgcccacgtgcggtgcaagggcgatgaaaccgccttcagcgttctggagggcgtgcactcttatagtgtgagcctgagctttgatcacgccgtggtggacgagcagtgtcagctgaactgtggcgggcacgagagccaggtcaccctgcggggcaatctgattttcctggacgttcctaagttcgtggacggcagctacatgcagacctaccacagcaccgtgcccacaggcgccaatatcccttctccaaccgactggctgaacgcccttttcggcaacggcttgtctaggtggattctgggagtgatcggagtcctgctgggtggactggccctgttcttcctgatcatgagccttttcaagttgggcacaaagcaggtgttcagatcaagaaccaagttggcatgaaactttgagccaacaggggtgacggagtcccgcactgaaattacggcaatgcagaccaccggttcatgtgggcaacaatcaggagctgtgtacgtgggcaattacaggattgtaaacagacacctggcaacgagccacgattggcaaaattgcgtgtgggaggactacaacagggatctcctggtcagcacaacaactgctcatggttgtgatactatagcacggtgccaatgtactgctggcgtgtacttttgtgcatctagaaacaagcactacccagtgagcttcgagggtccaggtctagtgaaagttcaggagggcgagtactaccccgagagataccagtcgcacgtactccttgcagttggattttcagaaccgggtgattgtggaggtattttgaggtgtgaacatggagtcattgggctcgttaccatgggtggtgagggtgtagtaggcttcgctgacgtgcgggatcttttgtggttggaagacgacgccatggagcagggtgttagagattatgtagagcaactgggaaatgcatttggctcaggtttcactaaccaaatctgtgagcaagttaacctccttaaagaatctctgatagggcaggattccatattggaaaaatccctgaaggccctggttaaaatcatatcagccctggtgatagtggttaggaaccacgacgacctgattacagtgactgccacactagctttaatcggttgcgcatcatctccatggcgatggctcaaacaaaaagtgtgtcaatactacggaatccccatggcagaaaggcagaataacggttggttaaagaaattcactgaaatgaccaacgcctgcaagggcatggagtggattgctgttaaaattcaaaagttcatcgagtggctcaaagtaaagattctgcctgaagtgaaggagaaacatgagttccttaccagattgaagcaattgccactccttgaaagtcaaattgccaccattgagcaaagcgcaccctcacaaagtgatcaagagcagcttttttcgaatgttcagtacttcgcccattactgcaggaagtatgcacctctgtatgctgccgaagcaaaaagagtgttctcattagaaaagaaaatgagtaattacatacagttcaagtccaaatgccgcattgagcctgtatgcttactccttcacggtagtccaggggctggcaagtcagtagctaccaacctgatagggagatcccttgcagagaagctcaatagctctgtgtactctttaccaccagatccagatcattttgatgggtacaaacagcaggcagtggtgatcatggatgatctctgtcaaaaccccgatgggaaggacgtgtccttgttttgccaaatggtgtctagtgtagattttgtgccacccatggcggcgctggaagaaaaaggcattctctttacgtccccgtttgtgttggcatcaaccaacgcggggtccatcaatgcaccaacagtgtcagacagcagagcacttgccagaaggtttcactttgacatgaatattgaggtgatttcgatgtacagccagaatggtaaaattaacatgcccatgtctgttaagacatgtgatgatgaatgctgcccggtcaatttcaaaaagtgttgcccactagtgtgtggcaaggccatccagtttattgacaggagaaaccaagttagatattcactggacatgctggttactgagatgtttagagagtacaaccacagacacagtgtgggtgctaccctcgaggctttgttccaaggaccaccagtatacagggaaatcaaaatcagtgtggccccggaaacaccccctccaccagcaattgctgaccttctaaaatctgtagacagtgaggcaataagggagtactgcaaggaaaggggttggcttgtgccagaggtcagctccactctacaaattgaaaaacatgttagcagggcatttatttgcttgcaagcgctaactacatttgtttcagtggctggtataatctacatcatttacaagttgtttgccggctttcagggtgcatacactggaatgcccaaccagaaacccaaggtgcccaccttaagacaagctaaggtgcaaggtccggcatttgaatttgccgtagcaatgatgaaaaggaacgccagcacagtcaagacagaatacggtgagttcacgatgcttggcatctatgataaatgggcagtgctgccgcgccacgccaagcctggaccaactattttaatgaatgatcaggaggttggtgtgctcgatgccaaagagttagttgataaagacggaaccaacctggagctgacactattgaagcttaaccgcaatgaaaagttcagagacatcagaggttttcttgcaagggaagaagttgaggtaagtgaggctgttttggcaataaacacgagcaagttcccaagcatgtacatccctgtgggccaagtcaccgattacggatttttaaatctaggtggcaccccaacaaagagaatgctcatgtacaacttccctaccagagcgggacagtgtggtggtgtccttatgtcaacaggaaaggtccttggcatacacgtgggaggaaatggtcaccaaggcttctctgctgctctcctcagacactacttcaacgaggaacagggcgaaatagagtttattgagagctctaaagatgcaggatttcctgtgatcaacacccctaataaaaccaaactggaaccaagtgtgtttcatcaggtttttgagggcaacaaagaaccagcagtcctaagaaacggagacccgcgacttaaagccaactttgaggaagcgatattttccaagtacatcggaaatgtgaacacacatgtggacgagtacatgatagaagctgttgatcactacgctggacagctggcaactctggacatcagtacagaacctatgaagcttgaggatgctgtttatggcactgaaggcttggaagcattggacttgaccactagcgcaggatatccttatgtcgccttgggcatcaagaaaagggatatcctctccaagaagactaaagatctcaccaagctgagggaatgcatggacaagtatggtctaaatctgccgatggtgacctacgtgaaggatgaactcaggtccgctgagaaagtagccaagggaaaatccagacttatagaagcttctagtctcaatgactcagtggccatgaggcagacatttgggaacctatacaagacattccacctcaacccaggcattgtcactggtagtgctgttgggtgcgacccagatgtgttttggagcaaaatacccgtgatgcttgacgggcaccttatagcttttgattactctggctacgacgctagcttgagcccagtgtggtttgcttgtttgaaactcctcctagggaaactagggtatactcataaggaaaccaattacatagactacctctgcaactcccatcacttatacagagataaacactatttcgtgaggggtggtatgccatcaggatgttcaggcaccagtatattcaacaccatgatcaacaacatcattattaggacccttatgctaaaggtctacaaaggtattgacctggatcagtttagaatgatcgcttacggggacgatgtgatagcctcttacccgtggcctattgatgcctcactactagcagaagcgggaaaggattatggtttgatcatgaccccagcagataaaggagagtgttttaatgaggtaacctggacaaatgtaaccttcttgaaaaggtactttagagctgatgaacaatatccattcttggtgcaccccgtgatgcccatgaaagacatacacgaatccattagatggaccaaagacccaaagaacactcaagatcatgtgcgctcgttatgcctattggcttggcacaatggggagcacgaatatgaggaatttatccgaaagatcagaagcgtgcctgttggacgctgtttgaccctcccggtgttctcaacactacgcaggaaatggttagattccttctaaaattagagtgcaatcaatgaactatgattggcttaaccctaccgcatgaaccgaactagacaaaagtgcggtaggggtaaattctccgcattcggtgcggaaaaaaaaaaaaaaaaaaaaaaaaaaaaaaaaaaaaaaaaaaaaaaaaaaaaaaaaaaaaaaaaaaaaaaaaaaaaaaaaaaaaaaaaaaaaaaaaaaaaaaaaaaaaaaaaaaaaaaaa

SEQ ID NO: 127 - DNA, 8252 bp, synthetic construct
  source 1..8252: mol_type = other DNA
  misc_feature 1..8252: note = SFTS B DNA vector construct
ttaaaacagcctgtgggttgtacccacccacagggcccactgggcgctagcactctggtatcacggtacctttgtgtgcctgttttatatcccctttccccgattgtaacttagaagatgtacacactgatcaatagcgggcatagcacaccagctatgtcttgatcaagcactcctgtatccccggaccaagtatcaatagactgctcacgcggttgaaggagaaaacgttcgtcacccggctaactacttcgagaaacccagtagtatcatgaaagttgcgaggcgtttcgttcagcacacccccagtgtagatcgggtcgatgagtcaccgcatcccccacgggcgaccgtggcggtggctgcgctggcggcctgcctacggggcaacccgtaggacgcttcaatacagacatggtgcgaagagtcgattgagctagttagtagtcctccggcccctgaatgcggctaatcctaactgcggagcacatgccctcaacccagggggtattgtgtcgtaacgggcaactctgcagcggaaccgactactttgggtgtccgtgtttccttttatccttatactggctgcttatggtgacaattgaaagattgttgccatatagctattggattggccatccagtgtctaatagagctgttatttacctctttgttggatttataccactcaacctaaaagaagttaaaacactacagctcattttacaactgaatacagcaaaccaccatgatgaaggtgatctggttcagctcccttatctgtctggtgattcagtgttctggcgacaccggccctatcatctgtgccggacccatccatagcaacaagagcgccaatatcccccacctgctgggctacagtgagaaaatctgccagatcgacagactgatccacgtgagcagctggctgagaaaccactctcaatttcagggctacgtaggtcagagaggcggtcggagccaggtgagctactaccctgccgagaactcttatagccggtggtctggattgctgtcgccttgcgacgccgattggctggggatgctggtcgtgaaaaaggccaagggcagcgatatgatcgtgccaggcccttcttataaaggcaaggtgttcttcgaaagacctacatttgacggatatgtgggatggggctgcggctccggcaagagcagaacagaatccggcgagctgtgcagctctgattctggaaccagcagcggactgctgccttctgatagagtgctgtggatcggcgatgtggcctgccagcctatgacccctatacccgaggaaacattcctggaactgaaaagttttagccagagcgagtttcctgacatctgcaagatcgacggaatcgtgtttaaccagtgcgagtctgagagccttcctcagcctttcgacgtggcctggatggatgtgggccacagccacaagatcatcatgagagagcacaagaccaagtgggtgcaggagagcagcagcaaagacttcgtctgctacaaggaaggcaccggcccatgctctgagagcgaggaaaagacctgtaaaaccagtggctcttgcaggggcgacatgcagttctgtaaggttgccgggtgcgaacacggcgaggaggcctctgaggccaagtgcagatgctccctggtgcacaaacctggggaggtggtggtgagctacggcggcatgcgggtgcggcccaagtgctacggcttctccagaatgatggccaccctggaagtgaatcctccagagcagcggatcggccagtgtacaggctgccacctggaatgcattaacggcggagtcaggctgattacactaacctccgagctgaagtctgccacagtgtgcgcgagccacttctgcagcagcgccacaagcggcaagaagtctacagagatccagttccacagcggcagcctggtgggcaagaccgccatccatgtgaagggcgccctggtggacggcacagagttcacctttgagggctcctgcatgttccccgatggctgtgatgccgtggactgcaccttctgcagagagttcctgaagaacccacagtgttaccctgccaagaagtggctgttcatcatcatcgtgatcctgctcggctacgccggactgatgttgctgaccaacgtgctgaaggccatcggcgtgtggggctcctgggtcatcgcccccgtcaagctgatgttcgccatcatcaagaagctgatgcgcagcgtgtcgtgcctgatgggcaagctcatggatagaggcagacaggtgattcacgaggagatcggcgagaacagagagggaaaccaagacgatgtgcggatcgaaatggccagacctcggagagtgcggcactggatgtacagccctgtgatccttacaatcctggccatcggcctggccgaaggctgtgacgagatggtgcacgccgactccaagctggtctcttgcaaacagggctccggaaatatgaaggagtgtgtgaccaccggaagagccctgctgcctgccgtgaaccctggacaggaggcttgcctgcatttcaccgcccctggtagccctgacagcaaatgtctgaaaatcaaagtgaaacgaatcaacctgaagtgcaaaaagtcaagctcttacttcgtgcccgacgcacgatctcggtgtaccagcgttcggcggtgcagatgggccggcgattgccagagcggctgtccttcccatttcacaagcaacagcttcagtgacgactgggccggcaagatggatagagccggcctggggttctccggctgttccgacggctgcggaggagctgcttgtggctgcttcaacgccgctccaagctgcatcttctggagaaagtgggtggaaaatcctcacggcatcatctggaaggtgagcccatgcgctgcctgggtgccctcggctgtcatcgagctgacaatgccttctggcgaagtgcggacatttcaccccatgagcggcatccccacccaggttttcaagggggtgagcgtgacctacctgggcagcgacatggaagtgagcggcctgacagacctgtgcgagatcgaggaactgaaaagcaagaagctggccctggctccttgcaaccaggccggaatgggcgtggtgggaaaggtgggagaaatccaatgtagctccgaagaaagcgccagaaccattaagaaggacgggtgcatctggaacgctgatctggtcggtattgaactgcgagtggacgacgccgtgtgctactccaaaatcaccagtgttgaggccgtcgccaattacagcgccattcccaccactatcggcggactgaggttcgagagaagccacgactctcagggcaagatcagcggcagcccactggacatcacagccatcagaggctcattctccgtgaactaccggggcttgagactgtctctgagcgaaatcaccgccacctgcaccggcgaggtgacaaacgtgtccggctgctacagctgtatgaccggcgccaaggtgtctatcaagctgcactccagcaagaacagcaccgcccacgtgagatgtaaaggcgacgagacagctttcagcgtgctggagggcgtacacagctacaccgtgtccctgagcttcgaccacgccgtggtggacgagcagtgccagctaaactgcggaggccacgaaagccaagtgaccctgaagggcaacctgatcttcctggatgtgcctaagttcgtggacggcagctacatgcaaacataccacagctcagtgcctacgggcgccaacatcccttctccaaccgactggctgaacgctctgtttggcaatggactgagcaggtggattctgggcgtgatcggggtgctgctgggcggcctggccctgttcttcctgataatgagcctgtttaagctgggcaccaagcaggtgttcagatccagaaccaagctggctaactttgagccaacaggggtgacggagtcccgcactgaaattacggcaatgcagaccaccggttcatgtgggcaacaatcaggagctgtgtacgtgggcaattacaggattgtaaacagacacctggcaacgagccacgattggcaaaattgcgtgtgggaggactacaacagggatctcctggtcagcacaacaactgctcatggttgtgatactatagcacggtgccaatgtactgctggcgtgtacttttgtgcatctagaaacaagcactacccagtgagcttcgagggtccaggtctagtgaaagttcaggagggcgagtactaccccgagagataccagtcgcacgtactccttgcagttggattttcagaaccgggtgattgtggaggtattttgaggtgtgaacatggagtcattgggctcgttaccatgggtggtgagggtgtagtaggcttcgctgacgtgcgggatcttttgtggttggaagacgacgccatggagcagggtgttagagattatgtagagcaactgggaaatgcatttggctcaggtttcactaaccaaatctgtgagcaagttaacctccttaaagaatctctgatagggcaggattccatattggaaaaatccctgaaggccctggttaaaatcatatcagccctggtgatagtggttaggaaccacgacgacctgattacagtgactgccacactagctttaatcggttgcgcatcatctccatggcgatggctcaaacaaaaagtgtgtcaatactacggaatccccatggcagaaaggcagaataacggttggttaaagaaattcactgaaatgaccaacgcctgcaagggcatggagtggattgctgttaaaattcaaaagttcatcgagtggctcaaagtaaagattctgcctgaagtgaaggagaaacatgagttccttaccagattgaagcaattgccactccttgaaagtcaaattgccaccattgagcaaagcgcaccctcacaaagtgatcaagagcagcttttttcgaatgttcagtacttcgcccattactgcaggaagtatgcacctctgtatgctgccgaagcaaaaagagtgttctcattagaaaagaaaatgagtaattacatacagttcaagtccaaatgccgcattgagcctgtatgcttactccttcacggtagtccaggggctggcaagtcagtagctaccaacctgatagggagatcccttgcagagaagctcaatagctctgtgtactctttaccaccagatccagatcattttgatgggtacaaacagcaggcagtggtgatcatggatgatctctgtcaaaaccccgatgggaaggacgtgtccttgttttgccaaatggtgtctagtgtagattttgtgccacccatggcggcgctggaagaaaaaggcattctctttacgtccccgtttgtgttggcatcaaccaacgcggggtccatcaatgcaccaacagtgtcagacagcagagcacttgccagaaggtttcactttgacatgaatattgaggtgatttcgatgtacagccagaatggtaaaattaacatgcccatgtctgttaagacatgtgatgatgaatgctgcccggtcaatttcaaaaagtgttgcccactagtgtgtggcaaggccatccagtttattgacaggagaaaccaagttagatattcactggacatgctggttactgagatgtttagagagtacaaccacagacacagtgtgggtgctaccctcgaggctttgttccaaggaccaccagtatacagggaaatcaaaatcagtgtggccccggaaacaccccctccaccagcaattgctgaccttctaaaatctgtagacagtgaggcaataagggagtactgcaaggaaaggggttggcttgtgccagaggtcagctccactctacaaattgaaaaacatgttagcagggcatttatttgcttgcaagcgctaactacatttgtttcagtggctggtataatctacatcatttacaagttgtttgccggctttcagggtgcatacactggaatgcccaaccagaaacccaaggtgcccaccttaagacaagctaaggtgcaaggtccggcatttgaatttgccgtagcaatgatgaaaaggaacgccagcacagtcaagacagaatacggtgagttcacgatgcttggcatctatgataaatgggcagtgctgccgcgccacgccaagcctggaccaactattttaatgaatgatcaggaggttggtgtgctcgatgccaaagagttagttgataaagacggaaccaacctggagctgacactattgaagcttaaccgcaatgaaaagttcagagacatcagaggttttcttgcaagggaagaagttgaggtaagtgaggctgttttggcaataaacacgagcaagttcccaagcatgtacatccctgtgggccaagtcaccgattacggatttttaaatctaggtggcaccccaacaaagagaatgctcatgtacaacttccctaccagagcgggacagtgtggtggtgtccttatgtcaacaggaaaggtccttggcatacacgtgggaggaaatggtcaccaaggcttctctgctgctctcctcagacactacttcaacgaggaacagggcgaaatagagtttattgagagctctaaagatgcaggatttcctgtgatcaacacccctaataaaaccaaactggaaccaagtgtgtttcatcaggtttttgagggcaacaaagaaccagcagtcctaagaaacggagacccgcgacttaaagccaactttgaggaagcgatattttccaagtacatcggaaatgtgaacacacatgtggacgagtacatgatagaagctgttgatcactacgctggacagctggcaactctggacatcagtacagaacctatgaagcttgaggatgctgtttatggcactgaaggcttggaagcattggacttgaccactagcgcaggatatccttatgtcgccttgggcatcaagaaaagggatatcctctccaagaagactaaagatctcaccaagctgagggaatgcatggacaagtatggtctaaatctgccgatggtgacctacgtgaaggatgaactcaggtccgctgagaaagtagccaagggaaaatccagacttatagaagcttctagtctcaatgactcagtggccatgaggcagacatttgggaacctatacaagacattccacctcaacccaggcattgtcactggtagtgctgttgggtgcgacccagatgtgttttggagcaaaatacccgtgatgcttgacgggcaccttatagcttttgattactctggctacgacgctagcttgagcccagtgtggtttgcttgtttgaaactcctcctagggaaactagggtatactcataaggaaaccaattacatagactacctctgcaactcccatcacttatacagagataaacactatttcgtgaggggtggtatgccatcaggatgttcaggcaccagtatattcaacaccatgatcaacaacatcattattaggacccttatgctaaaggtctacaaaggtattgacctggatcagtttagaatgatcgcttacggggacgatgtgatagcctcttacccgtggcctattgatgcctcactactagcagaagcgggaaaggattatggtttgatcatgaccccagcagataaaggagagtgttttaatgaggtaacctggacaaatgtaaccttcttgaaaaggtactttagagctgatgaacaatatccattcttggtgcaccccgtgatgcccatgaaagacatacacgaatccattagatggaccaaagacccaaagaacactcaagatcatgtgcgctcgttatgcctattggcttggcacaatggggagcacgaatatgaggaatttatccgaaagatcagaagcgtgcctgttggacgctgtttgaccctcccggtgttctcaacactacgcaggaaatggttagattccttctaaaattagagtgcaatcaatgaactatgattggcttaaccctaccgcatgaaccgaactagacaaaagtgcggtaggggtaaattctccgcattcggtgcggaaaaaaaaaaaaaaaaaaaaaaaaaaaaaaaaaaaaaaaaaaaaaaaaaaaaaaaaaaaaaaaaaaaaaaaaaaaaaaaaaaaaaaaaaaaaaaaaaaaaaaaaaaaaaaaaaaaaaaaa

SEQ ID NO: 128 - DNA, 8252 bp, synthetic construct
  source 1..8252: mol_type = other DNA
  misc_feature 1..8252: note = SFTS DEF DNA vector construct
ttaaaacagcctgtgggttgtacccacccacagggcccactgggcgctagcactctggtatcacggtacctttgtgtgcctgttttatatcccctttccccgattgtaacttagaagatgtacacactgatcaatagcgggcatagcacaccagctatgtcttgatcaagcactcctgtatccccggaccaagtatcaatagactgctcacgcggttgaaggagaaaacgttcgtcacccggctaactacttcgagaaacccagtagtatcatgaaagttgcgaggcgtttcgttcagcacacccccagtgtagatcgggtcgatgagtcaccgcatcccccacgggcgaccgtggcggtggctgcgctggcggcctgcctacggggcaacccgtaggacgcttcaatacagacatggtgcgaagagtcgattgagctagttagtagtcctccggcccctgaatgcggctaatcctaactgcggagcacatgccctcaacccagggggtattgtgtcgtaacgggcaactctgcagcggaaccgactactttgggtgtccgtgtttccttttatccttatactggctgcttatggtgacaattgaaagattgttgccatatagctattggattggccatccagtgtctaatagagctgttatttacctctttgttggatttataccactcaacctaaaagaagttaaaacactacagctcattttacaactgaatacagcaaaccaccatgatgaaggtgatctggttctcttctctgatctgctttgtgatccagtgcagcggcgatagcgggccaatcatctgcgccggaccaatccacagcaacaagagcgccgacatcccccacctgcttggctactcagaaaaaatctgccagatcgacagactaatacacgtgagcagctggctgcggaaccacagccagtttcagggctatgtgggccagagaggaggcagaagccaagtgagctactaccctgctgaaaacagctacagcagatggtccggcctgctctccccatgtgatgccgattggctgggcatgctcgtggtgaagaaagccaagggctccgatatgatcgtgcccggccctagctacaaggggaaggtgtttttcgagagacctacattcgacggctacgtgggctggggctgcggcagcggcaaaagccggaccgagagcggcgaactgtgtagcagcgacagcggaacaagcagcggtctgctccccagcgaccgggtgctgtggatcggcgacgttgcctgtcagcccatgacccctatccccgaggagacatttctggaactgaagtcgttctcccagagcgagttccctgacatctgcaagattgacggcattgtgttcaatcagtgcgagggcgagagcctgcctcagcctttcgacgtggcttggatggatgtgggccacagccacaagatcatcatgagagagcacaaaaccaagtgggtccaggagtcgtccagcaaggacttcgtgtgttataaggaaggcacaggcccctgcagcgagtccgaagagaagacctgcaagaccagcggcagctgtagaggcgacatgcagttctgcaaagtggccggctgtgaacacggagaagaggccagcgaggctaagtgccggtgcagcctggtgcacaagcctggcgaggtggtcgtatcttacggcggcatgcgggtgcggcctaagtgctacggcttcagccggatgatggccaccctggaggtgaatccgcccgagcagcggatcggccagtgtaccggatgccacctggagtgcattaacggcggcgtgcggctgatcaccctgaccagcgaactgaagtctgctaccgtgtgcgcgagccatttctgcagctcagccaccagtggaaaaaagagcaccgagatccagttccacagcggctctctggtcggcaagacagccatccacgtgaagggcgccctggtggacggcaccgagttcacctttgagggcagctgcatgttccctgacggctgtgacgccgtggactgcaccttctgcagagagttcctgaaaaacccccagtgttaccccgctaagaaatggctgttcatcatcattgtcatcctgctgggctacgccggactcatgctgctgacaaacgtgctgaaggccatcggagtttggggaagttgggtgatcgcccctgtgaaactgatgttcgccatcatcaagaaactgatgcgaaccgtgagctgcctgatgggcaagttgatggatagaggcagacaggtgatccacgaggagatcggcgaaaacagagaaggcaaccaggacgacgtgcggatcgagatggccagacccagaagagtgcggcactggatgtactcccctgtgatcctgaccatcctggccatcggcctagctgaaggctgcgacgaaatggtgcacgccgactctaagctcgtatcatgccggcagggcagcggcaatatgaaggagtgtgtgacaaccggcagagccctgctgcctgccgtgaaccccggccaggaggcctgcctgcactttacggcccctggttctcccgacagcaagtgcctgaagatcaaggtcaagagaatcaacctgaaatgcaagaagagcagcagctacttcgtgcctgacgccagaagtagatgtacaagcgtgcgccgctgccgctgggcaggcgattgccagagcggatgtcctcctcacttcacctctaatagtttcagcgacgattgggctggcaaaatggaccgcgccggcctgggattttctggatgcagtgatggctgcggcggcgccgcctgcggatgttttaacgccgctcctagttgcatcttctggcggaagtgggtggaaaaccctcatggcatcatctggaaggtgagcccatgcgctgcttgggtgccttctgccgtgatcgagctgaccatgccttctggagaggtgcggacatttcaccctatgtccggcatccctacgcaggtgttcaagggcgtgtctgtgacatatctgggctccgacatggaagtgtccggtctgacagacctgtgcgaaatcgaggaactgaagtctaagaagctggccctggccccctgtaatcaagccggcatgggcgtggtgggcaaggtgggtgagatccaatgttcgagcgaggaaagcgcccggaccatcaaaaaagacggctgtatctggaacgctgatctggtgggcatcgagctgagagttgatgacgctgtttgctacagcaagatcacctccgtggaagccgtggccaattacagcgccatccccaccaccatcggcggcctgagattcgagagaagccacgatagccagggcaagatcagcggctcccctctggacattactgccatcagaggcagcttcagcgtgaactacagaggcctgaggctgtctctgagcgaaatcaccgctacatgcaccggagaagtgaccaacgtgtctggctgttacagctgtatgaccggcgcaaaagtgtctatcaagctgcactctagcaagaacagtacagcccacgtcagatgcaagggagatgagacagccttcagcgtgctggagggggttcacagctacaccgtgagcctgagctttgaccatgccgtggtggacgagcagtgccagctgaactgcggcggccacgagagccaggtaacactgaagggcaacctgatcttcctggatgtgccaaaattcgtggatggcagctacatgcaaacctaccacagtaccgttccaaccggcgccaacatccctagccctacagattggcttaacgccctgttcggcaacggcctgagcagatggattctgggcgtgattggagtgctgctgggtggactggcactgttcttcctgattatgtctctgttcaagctgggcacaaagcaggtgttcagatccagaaccaagctggccaactttgagccaacaggggtgacggagtcccgcactgaaattacggcaatgcagaccaccggttcatgtgggcaacaatcaggagctgtgtacgtgggcaattacaggattgtaaacagacacctggcaacgagccacgattggcaaaattgcgtgtgggaggactacaacagggatctcctggtcagcacaacaactgctcatggttgtgatactatagcacggtgccaatgtactgctggcgtgtacttttgtgcatctagaaacaagcactacccagtgagcttcgagggtccaggtctagtgaaagttcaggagggcgagtactaccccgagagataccagtcgcacgtactccttgcagttggattttcagaaccgggtgattgtggaggtattttgaggtgtgaacatggagtcattgggctcgttaccatgggtggtgagggtgtagtaggcttcgctgacgtgcgggatcttttgtggttggaagacgacgccatggagcagggtgttagagattatgtagagcaactgggaaatgcatttggctcaggtttcactaaccaaatctgtgagcaagttaacctccttaaagaatctctgatagggcaggattccatattggaaaaatccctgaaggccctggttaaaatcatatcagccctggtgatagtggttaggaaccacgacgacctgattacagtgactgccacactagctttaatcggttgcgcatcatctccatggcgatggctcaaacaaaaagtgtgtcaatactacggaatccccatggcagaaaggcagaataacggttggttaaagaaattcactgaaatgaccaacgcctgcaagggcatggagtggattgctgttaaaattcaaaagttcatcgagtggctcaaagtaaagattctgcctgaagtgaaggagaaacatgagttccttaccagattgaagcaattgccactccttgaaagtcaaattgccaccattgagcaaagcgcaccctcacaaagtgatcaagagcagcttttttcgaatgttcagtacttcgcccattactgcaggaagtatgcacctctgtatgctgccgaagcaaaaagagtgttctcattagaaaagaaaatgagtaattacatacagttcaagtccaaatgccgcattgagcctgtatgcttactccttcacggtagtccaggggctggcaagtcagtagctaccaacctgatagggagatcccttgcagagaagctcaatagctctgtgtactctttaccaccagatccagatcattttgatgggtacaaacagcaggcagtggtgatcatggatgatctctgtcaaaaccccgatgggaaggacgtgtccttgttttgccaaatggtgtctagtgtagattttgtgccacccatggcggcgctggaagaaaaaggcattctctttacgtccccgtttgtgttggcatcaaccaacgcggggtccatcaatgcaccaacagtgtcagacagcagagcacttgccagaaggtttcactttgacatgaatattgaggtgatttcgatgtacagccagaatggtaaaattaacatgcccatgtctgttaagacatgtgatgatgaatgctgcccggtcaatttcaaaaagtgttgcccactagtgtgtggcaaggccatccagtttattgacaggagaaaccaagttagatattcactggacatgctggttactgagatgtttagagagtacaaccacagacacagtgtgggtgctaccctcgaggctttgttccaaggaccaccagtatacagggaaatcaaaatcagtgtggccccggaaacaccccctccaccagcaattgctgaccttctaaaatctgtagacagtgaggcaataagggagtactgcaaggaaaggggttggcttgtgccagaggtcagctccactctacaaattgaaaaacatgttagcagggcatttatttgcttgcaagcgctaactacatttgtttcagtggctggtataatctacatcatttacaagttgtttgccggctttcagggtgcatacactggaatgcccaaccagaaacccaaggtgcccaccttaagacaagctaaggtgcaaggtccggcatttgaatttgccgtagcaatgatgaaaaggaacgccagcacagtcaagacagaatacggtgagttcacgatgcttggcatctatgataaatgggcagtgctgccgcgccacgccaagcctggaccaactattttaatgaatgatcaggaggttggtgtgctcgatgccaaagagttagttgataaagacggaaccaacctggagctgacactattgaagcttaaccgcaatgaaaagttcagagacatcagaggttttcttgcaagggaagaagttgaggtaagtgaggctgttttggcaataaacacgagcaagttcccaagcatgtacatccctgtgggccaagtcaccgattacggatttttaaatctaggtggcaccccaacaaagagaatgctcatgtacaacttccctaccagagcgggacagtgtggtggtgtccttatgtcaacaggaaaggtccttggcatacacgtgggaggaaatggtcaccaaggcttctctgctgctctcctcagacactacttcaacgaggaacagggcgaaatagagtttattgagagctctaaagatgcaggatttcctgtgatcaacacccctaataaaaccaaactggaaccaagtgtgtttcatcaggtttttgagggcaacaaagaaccagcagtcctaagaaacggagacccgcgacttaaagccaactttgaggaagcgatattttccaagtacatcggaaatgtgaacacacatgtggacgagtacatgatagaagctgttgatcactacgctggacagctggcaactctggacatcagtacagaacctatgaagcttgaggatgctgtttatggcactgaaggcttggaagcattggacttgaccactagcgcaggatatccttatgtcgccttgggcatcaagaaaagggatatcctctccaagaagactaaagatctcaccaagctgagggaatgcatggacaagtatggtctaaatctgccgatggtgacctacgtgaaggatgaactcaggtccgctgagaaagtagccaagggaaaatccagacttatagaagcttctagtctcaatgactcagtggccatgaggcagacatttgggaacctatacaagacattccacctcaacccaggcattgtcactggtagtgctgttgggtgcgacccagatgtgttttggagcaaaatacccgtgatgcttgacgggcaccttatagcttttgattactctggctacgacgctagcttgagcccagtgtggtttgcttgtttgaaactcctcctagggaaactagggtatactcataaggaaaccaattacatagactacctctgcaactcccatcacttatacagagataaacactatttcgtgaggggtggtatgccatcaggatgttcaggcaccagtatattcaacaccatgatcaacaacatcattattaggacccttatgctaaaggtctacaaaggtattgacctggatcagtttagaatgatcgcttacggggacgatgtgatagcctcttacccgtggcctattgatgcctcactactagcagaagcgggaaaggattatggtttgatcatgaccccagcagataaaggagagtgttttaatgaggtaacctggacaaatgtaaccttcttgaaaaggtactttagagctgatgaacaatatccattcttggtgcaccccgtgatgcccatgaaagacatacacgaatccattagatggaccaaagacccaaagaacactcaagatcatgtgcgctcgttatgcctattggcttggcacaatggggagcacgaatatgaggaatttatccgaaagatcagaagcgtgcctgttggacgctgtttgaccctcccggtgttctcaacactacgcaggaaatggttagattccttctaaaattagagtgcaatcaatgaactatgattggcttaaccctaccgcatgaaccgaactagacaaaagtgcggtaggggtaaattctccgcattcggtgcggaaaaaaaaaaaaaaaaaaaaaaaaaaaaaaaaaaaaaaaaaaaaaaaaaaaaaaaaaaaaaaaaaaaaaaaaaaaaaaaaaaaaaaaaaaaaaaaaaaaaaaaaaaaaaaaaaaaaaaaa

SEQ ID NO: 129 - DNA, 8255 bp, synthetic construct
  source 1..8255: mol_type = other DNA
  misc_feature 1..8255: note = SFTS ABDEF DNA vector construct
ttaaaacagcctgtgggttgtacccacccacagggcccactgggcgctagcactctggtatcacggtacctttgtgtgcctgttttatatcccctttccccgattgtaacttagaagatgtacacactgatcaatagcgggcatagcacaccagctatgtcttgatcaagcactcctgtatccccggaccaagtatcaatagactgctcacgcggttgaaggagaaaacgttcgtcacccggctaactacttcgagaaacccagtagtatcatgaaagttgcgaggcgtttcgttcagcacacccccagtgtagatcgggtcgatgagtcaccgcatcccccacgggcgaccgtggcggtggctgcgctggcggcctgcctacggggcaacccgtaggacgcttcaatacagacatggtgcgaagagtcgattgagctagttagtagtcctccggcccctgaatgcggctaatcctaactgcggagcacatgccctcaacccagggggtattgtgtcgtaacgggcaactctgcagcggaaccgactactttgggtgtccgtgtttccttttatccttatactggctgcttatggtgacaattgaaagattgttgccatatagctattggattggccatccagtgtctaatagagctgttatttacctctttgttggatttataccactcaacctaaaagaagttaaaacactacagctcattttacaactgaatacagcaaaccaccatgatgaaggttatctggttctccagcctgatctgtctggtgatccagtgtagcggcgacaccggacctatcatttgtgccggccctatccactccaacaagtccgccgacatcccccacctcctgggatactctgaaaaaatctgccaaatcgatagactgatccacgtgtccagctggctgcgaaaccacagccagttccagggctatgtgggccaaagaggaggcagaagccaggtgagctactaccccgccgagaatagctacagcagatggtccggcctgctgagcccttgcgacgccgattggctgggaatgctggtggtgaagaaggccaagggcagcgacatgatcgtgcccggccctagctacaagggcaaggtctttttcgaacggcccacctttgatggctacgtgggctggggatgcggctctggcaaaagccggacagaatctggagagctgtgcagcagcgacagcggcaccagctctggcctgctgccttcggatagagtgctgtggatcggcgatgtcgcatgccagcctatgacccctatccctgaggagacattcctggagctgaaatctttcagtcaaagcgagttccccgacatctgtaagatcgacggcatcgtgtttaaccagtgtgaaggcgaatccctgcctcagccgttcgacgtggcctggatggacgtcggccacagccacaagatcatcatgagagagcacaaaaccaagtgggtccaggagtctagcagcaaagacttcgtgtgctataaggaaggaacaggcccttgctccgagagcgaggaaaagacatgcaagaccagcgggtcttgcagaggagacatgcagttttgtaaagtggccggatgcgagcacggcgaggaggccagcgaggctaagtgccgctgtagcctcgttcacaagccaggagaggtggttgtgtcctacggcggcatgcgggtgagacccaagtgctacggcttcagcagaatgatggccacactggaggtgaatccacctgaacagcggatcggccagtgcaccggctgccacctggaatgcatcaacggcggcgtgagactgataacactgactagcgaactgaagagcgccacagtgtgcgccagccacttctgctcaagcgccaccagcggcaagaaatctactgagatccagttccactccggcagcctggtcggcaagaccgccatccacgtgaagggcgctctggtggatggcacagagttcacgttcgagggctcatgcatgttccctgatggctgcgacgccgtggactgcaccttctgccgggagttcctgaaaaacccccagtgttatcctgctaaaaagtggctgttcatcatcatcgtgatcctgctcggatacgccggcctgatgctgctgaccaacgtgctgaaggccatcggcgtgtggggcagctgggtgatcgcccccgtgaagctgatgttcgccatcatcaagaaactcatgagaaccgtgtcctgcctgatgggcaagctgatggaccggggcagacaggtgatccatgaggaaattggcgagaacagagagggcaaccaggacgacgtaagaatcgagatggccagacccagacgggtgcggcactggatgtacagccctgtgattttgaccatcctggctatcggactggctgaaggctgcgacgagatggtgcatgctgattctaaactggtatcttgtagacagggcagcggaaacatgaaagaatgcgtgaccaccggtcgggccctcctgcccgctgtgaatcccggccaggaggcctgcctgcacttcaccgcccctggcagccccgatagcaagtgcctgaagattaaggtgaagcggatcaacctgaagtgcaagaaatctagcagctacttcgtgcctgacgctagatccagatgcacctctgttaggagatgtagatgggccggagactgccagagcggctgccctcctcatttcacaagcaacagcttcagcgatgattgggccggaaaaatggacagagccggcctcggattctccgggtgcagcgatggatgcggaggcgccgcctgcggctgcttcaacgccgctcctagctgtatcttctggcggaagtgggtggaaaaccctcacggcatcatctggaaggttagcccatgcgccgcctgggtgccctctgccgtaatcgagctgaccatgccttctggtgaagtgcggacttttcaccccatgtcgggcatccctacccaggtgttcaagggcgtgagcgtgacctacctgggcagcgacatggaagtgagcggcctgacagacctgtgtgaaattgaagagctgaagtctaaaaagctggccctggcgccctgtaaccaagccggcatgggagtggtgggaaaggtcggcgagatccagtgcagctccgaggagagcgccagaacaatcaagaaagacggctgtatctggaacgccgatctggtgggcatcgagcttagagtggacgacgccgtgtgctacagcaagatcacctccgtggaagccgttgctaattacagcgccatccctaccacaatcggcggcctgcggttcgagcggtctcacgacagccaaggcaaaatcagcggcagccctctggacattaccgccatcagaggctcttttagcgtgaactacagaggcctgagattgtctctgtctgagatcaccgcaacctgtacaggcgaggtgacaaacgtgtccggctgctacagctgtatgaccggcgctaaggtgtctatcaagctgcactccagcaagaacagcacagcccacgtgcggtgcaagggcgacgaaaccgccttcagtgtgctggaaggcgtgcacagctacaccgtgagcctgagcttcgaccacgccgtcgtggacgagcagtgccagctgaactgcggcggtcacgagagccaggtgaccctgaagggaaacctgatcttcctggacgtgccaaagttcgtggacggcagctacatgcagacctaccacagcaccgtgcctaccggagccaacatcccatctcctacagattggctgaacgccctgttcggcaatggcctgtccagatggattctgggagtgatcggcgtgctgctgggcggcctggccctgttcttcctgatcatgtccctgtttaagctgggcacaaagcaggtctttagaagtcgcaccaagctcgcttgaaactttgagccaacaggggtgacggagtcccgcactgaaattacggcaatgcagaccaccggttcatgtgggcaacaatcaggagctgtgtacgtgggcaattacaggattgtaaacagacacctggcaacgagccacgattggcaaaattgcgtgtgggaggactacaacagggatctcctggtcagcacaacaactgctcatggttgtgatactatagcacggtgccaatgtactgctggcgtgtacttttgtgcatctagaaacaagcactacccagtgagcttcgagggtccaggtctagtgaaagttcaggagggcgagtactaccccgagagataccagtcgcacgtactccttgcagttggattttcagaaccgggtgattgtggaggtattttgaggtgtgaacatggagtcattgggctcgttaccatgggtggtgagggtgtagtaggcttcgctgacgtgcgggatcttttgtggttggaagacgacgccatggagcagggtgttagagattatgtagagcaactgggaaatgcatttggctcaggtttcactaaccaaatctgtgagcaagttaacctccttaaagaatctctgatagggcaggattccatattggaaaaatccctgaaggccctggttaaaatcatatcagccctggtgatagtggttaggaaccacgacgacctgattacagtgactgccacactagctttaatcggttgcgcatcatctccatggcgatggctcaaacaaaaagtgtgtcaatactacggaatccccatggcagaaaggcagaataacggttggttaaagaaattcactgaaatgaccaacgcctgcaagggcatggagtggattgctgttaaaattcaaaagttcatcgagtggctcaaagtaaagattctgcctgaagtgaaggagaaacatgagttccttaccagattgaagcaattgccactccttgaaagtcaaattgccaccattgagcaaagcgcaccctcacaaagtgatcaagagcagcttttttcgaatgttcagtacttcgcccattactgcaggaagtatgcacctctgtatgctgccgaagcaaaaagagtgttctcattagaaaagaaaatgagtaattacatacagttcaagtccaaatgccgcattgagcctgtatgcttactccttcacggtagtccaggggctggcaagtcagtagctaccaacctgatagggagatcccttgcagagaagctcaatagctctgtgtactctttaccaccagatccagatcattttgatgggtacaaacagcaggcagtggtgatcatggatgatctctgtcaaaaccccgatgggaaggacgtgtccttgttttgccaaatggtgtctagtgtagattttgtgccacccatggcggcgctggaagaaaaaggcattctctttacgtccccgtttgtgttggcatcaaccaacgcggggtccatcaatgcaccaacagtgtcagacagcagagcacttgccagaaggtttcactttgacatgaatattgaggtgatttcgatgtacagccagaatggtaaaattaacatgcccatgtctgttaagacatgtgatgatgaatgctgcccggtcaatttcaaaaagtgttgcccactagtgtgtggcaaggccatccagtttattgacaggagaaaccaagttagatattcactggacatgctggttactgagatgtttagagagtacaaccacagacacagtgtgggtgctaccctcgaggctttgttccaaggaccaccagtatacagggaaatcaaaatcagtgtggccccggaaacaccccctccaccagcaattgctgaccttctaaaatctgtagacagtgaggcaataagggagtactgcaaggaaaggggttggcttgtgccagaggtcagctccactctacaaattgaaaaacatgttagcagggcatttatttgcttgcaagcgctaactacatttgtttcagtggctggtataatctacatcatttacaagttgtttgccggctttcagggtgcatacactggaatgcccaaccagaaacccaaggtgcccaccttaagacaagctaaggtgcaaggtccggcatttgaatttgccgtagcaatgatgaaaaggaacgccagcacagtcaagacagaatacggtgagttcacgatgcttggcatctatgataaatgggcagtgctgccgcgccacgccaagcctggaccaactattttaatgaatgatcaggaggttggtgtgctcgatgccaaagagttagttgataaagacggaaccaacctggagctgacactattgaagcttaaccgcaatgaaaagttcagagacatcagaggttttcttgcaagggaagaagttgaggtaagtgaggctgttttggcaataaacacgagcaagttcccaagcatgtacatccctgtgggccaagtcaccgattacggatttttaaatctaggtggcaccccaacaaagagaatgctcatgtacaacttccctaccagagcgggacagtgtggtggtgtccttatgtcaacaggaaaggtccttggcatacacgtgggaggaaatggtcaccaaggcttctctgctgctctcctcagacactacttcaacgaggaacagggcgaaatagagtttattgagagctctaaagatgcaggatttcctgtgatcaacacccctaataaaaccaaactggaaccaagtgtgtttcatcaggtttttgagggcaacaaagaaccagcagtcctaagaaacggagacccgcgacttaaagccaactttgaggaagcgatattttccaagtacatcggaaatgtgaacacacatgtggacgagtacatgatagaagctgttgatcactacgctggacagctggcaactctggacatcagtacagaacctatgaagcttgaggatgctgtttatggcactgaaggcttggaagcattggacttgaccactagcgcaggatatccttatgtcgccttgggcatcaagaaaagggatatcctctccaagaagactaaagatctcaccaagctgagggaatgcatggacaagtatggtctaaatctgccgatggtgacctacgtgaaggatgaactcaggtccgctgagaaagtagccaagggaaaatccagacttatagaagcttctagtctcaatgactcagtggccatgaggcagacatttgggaacctatacaagacattccacctcaacccaggcattgtcactggtagtgctgttgggtgcgacccagatgtgttttggagcaaaatacccgtgatgcttgacgggcaccttatagcttttgattactctggctacgacgctagcttgagcccagtgtggtttgcttgtttgaaactcctcctagggaaactagggtatactcataaggaaaccaattacatagactacctctgcaactcccatcacttatacagagataaacactatttcgtgaggggtggtatgccatcaggatgttcaggcaccagtatattcaacaccatgatcaacaacatcattattaggacccttatgctaaaggtctacaaaggtattgacctggatcagtttagaatgatcgcttacggggacgatgtgatagcctcttacccgtggcctattgatgcctcactactagcagaagcgggaaaggattatggtttgatcatgaccccagcagataaaggagagtgttttaatgaggtaacctggacaaatgtaaccttcttgaaaaggtactttagagctgatgaacaatatccattcttggtgcaccccgtgatgcccatgaaagacatacacgaatccattagatggaccaaagacccaaagaacactcaagatcatgtgcgctcgttatgcctattggcttggcacaatggggagcacgaatatgaggaatttatccgaaagatcagaagcgtgcctgttggacgctgtttgaccctcccggtgttctcaacactacgcaggaaatggttagattccttctaaaattagagtgcaatcaatgaactatgattggcttaaccctaccgcatgaaccgaactagacaaaagtgcggtaggggtaaattctccgcattcggtgcggaaaaaaaaaaaaaaaaaaaaaaaaaaaaaaaaaaaaaaaaaaaaaaaaaaaaaaaaaaaaaaaaaaaaaaaaaaaaaaaaaaaaaaaaaaaaaaaaaaaaaaaaaaaaaaaaaaaaaaaa

SEQ ID NO: 130 - RNA, 1698 nt, synthetic construct; identical to SEQ ID NO: 52
  source 1..1698: mol_type = other RNA
  misc_feature 1..1698: note = H3N2 mRNA construct

SEQ ID NO: 131 - RNA, 6658 nt, synthetic construct
  source 1..6658: mol_type = other RNA
  misc_feature 1..6658: note = H3N2 saRNA construct
ttaaaacagcctgtgggttgtacccacccacagggcccactgggcgctagcactctggtatcacggtacctttgtgtgcctgttttatatcccctttccccgattgtaacttagaagatgtacacactgatcaatagcgggcatagcacaccagctatgtcttgatcaagcactcctgtatccccggaccaagtatcaatagactgctcacgcggttgaaggagaaaacgttcgtcacccggctaactacttcgagaaacccagtagtatcatgaaagttgcgaggcgtttcgttcagcacacccccagtgtagatcgggtcgatgagtcaccgcatcccccacgggcgaccgtggcggtggctgcgctggcggcctgcctacggggcaacccgtaggacgcttcaatacagacatggtgcgaagagtcgattgagctagttagtagtcctccggcccctgaatgcggctaatcctaactgcggagcacatgccctcaacccagggggtattgtgtcgtaacgggcaactctgcagcggaaccgactactttgggtgtccgtgtttccttttatccttatactggctgcttatggtgacaattgaaagattgttgccatatagctattggattggccatccagtgtctaatagagctgttatttacctctttgttggatttataccactcaacctaaaagaagttaaaacactacagctcattttacaactgaatacagcaaaccaccatgaaaaccgtgatcgccctcagttacatcttctgcctcgcctttggacagaatctcctcggaaacgaaaacaacgctgccacactctgcctgggacaccacgccgtgcccaacggcacaatggtgaagaccatcaccgacgatcagatcgaggtgaccaatgccaccgagctggtgcagaacagctccaccggcaaaatctgcaacaatccccacaagatcctggacggcagggattgcaccctgatcgacgctctgctgggcgaccctcactgcgacgtgttccagaatgagacatgggatctgttcgtggagaggagcaatgccttctccaactgctacccctacgacgtgcctgattacgccagcctgcggtccatcgtggccagctccggcaccctggagttcatcaccgagggcttcacctgggctggagtgacccagaacggaggcagcggagcttgcaagaggggacccgccaatagcttcttctcccggctgaactggctgaccaagtccggcaatacctaccccgtgctgaacgtgaccatgcctaacaataacaatttcgacaagctgtacatctggggcgtgcaccaccctagcaccgatcaggagcagaccagcctgtacatccaggcctccggcagggtgaccgtgagcaccaggcggtcccagcagaccatcatccccaacatcggctccaggcctctggtgcggggacagagcggccggatctccgtgtactggaccatcgtgaagcccggcgacatcctggtcatcaacagcaatggcaacctgatcgcccctcgcggctacttcaagatgcacatcggcaagagcagcatcatgagatccgacgcccccatcgatacctgcatcagcgagtgcatcacccctaatggctccatccccaacgagaagcctttccagaatgtgaacaagatcacctacggcgcctgccccaagtacgtgaagcagaataccctgaagctggccaccggcatgcgcaacgtgcctgagagacagaccgtgggcctgttcggagctatcgctggcttcatcgagaatggctgggagggcatggtggacggctggtacggcttccgccaccagaacagcgagggcaccggacaggctgccgacctgaagtccacccaggccgccatcgatcagatcaatggcaagctgaacagagtgatcgagaagaccaacgagaagttccaccagatcgagaaggagttcagcgaggtggagggacgcatccaggacctggagaggtacgtggaggacaccaagatcgatctgtggagctacaatgccgagctgctggtggccctggagaatcagaacaccatcgacctgaccgattccgagatgaacaagctgttcgagaagacccgcagacagctgcgcgagaatgccgaggacatgggcaacggctgcttcaaaatctaccacaagtgcgataacgcctgcatcgagagcatcagaaatggcacctacgaccacaacatctaccgcgatgaggccgtgaacaatagattccagatcaagggcgtggagctgaagtccggctacaaggactggattctgtggatcagcttcgccatctcctgcttcctgctgtgcgtggtgctgctggggtttattatgtgggcttgtcagagggggaacatcaggtgtaacatttgtaactttgagccaacaggggtgacggagtcccgcactgaaattacggcaatgcagaccaccggttcatgtgggcaacaatcaggagctgtgtacgtgggcaattacaggattgtaaacagacacctggcaacgagccacgattggcaaaattgcgtgtgggaggactacaacagggatctcctggtcagcacaacaactgctcatggttgtgatactatagcacggtgccaatgtactgctggcgtgtacttttgtgcatctagaaacaagcactacccagtgagcttcgagggtccaggtctagtgaaagttcaggagggcgagtactaccccgagagataccagtcgcacgtactccttgcagttggattttcagaaccgggtgattgtggaggtattttgaggtgtgaacatggagtcattgggctcgttaccatgggtggtgagggtgtagtaggcttcgctgacgtgcgggatcttttgtggttggaagacgacgccatggagcagggtgttagagattatgtagagcaactgggaaatgcatttggctcaggtttcactaaccaaatctgtgagcaagttaacctccttaaagaatctctgatagggcaggattccatattggaaaaatccctgaaggccctggttaaaatcatatcagccctggtgatagtggttaggaaccacgacgacctgattacagtgactgccacactagctttaatcggttgcgcatcatctccatggcgatggctcaaacaaaaagtgtgtcaatactacggaatccccatggcagaaaggcagaataacggttggttaaagaaattcactgaaatgaccaacgcctgcaagggcatggagtggattgctgttaaaattcaaaagttcatcgagtggctcaaagtaaagattctgcctgaagtgaaggagaaacatgagttccttaccagattgaagcaattgccactccttgaaagtcaaattgccaccattgagcaaagcgcaccctcacaaagtgatcaagagcagcttttttcgaatgttcagtacttcgcccattactgcaggaagtatgcacctctgtatgctgccgaagcaaaaagagtgttctcattagaaaagaaaatgagtaattacatacagttcaagtccaaatgccgcattgagcctgtatgcttactccttcacggtagtccaggggctggcaagtcagtagctaccaacctgatagggagatcccttgcagagaagctcaatagctctgtgtactctttaccaccagatccagatcattttgatgggtacaaacagcaggcagtggtgatcatggatgatctctgtcaaaaccccgatgggaaggacgtgtccttgttttgccaaatggtgtctagtgtagattttgtgccacccatggcggcgctggaagaaaaaggcattctctttacgtccccgtttgtgttggcatcaaccaacgcggggtccatcaatgcaccaacagtgtcagacagcagagcacttgccagaaggtttcactttgacatgaatattgaggtgatttcgatgtacagccagaatggtaaaattaacatgcccatgtctgttaagacatgtgatgatgaatgctgcccggtcaatttcaaaaagtgttgcccactagtgtgtggcaaggccatccagtttattgacaggagaaaccaagttagatattcactggacatgctggttactgagatgtttagagagtacaaccacagacacagtgtgggtgctaccctcgaggctttgttccaaggaccaccagtatacagggaaatcaaaatcagtgtggccccggaaacaccccctccaccagcaattgctgaccttctaaaatctgtagacagtgaggcaataagggagtactgcaaggaaaggggttggcttgtgccagaggtcagctccactctacaaattgaaaaacatgttagcagggcatttatttgcttgcaagcgctaactacatttgtttcagtggctggtataatctacatcatttacaagttgtttgccggctttcagggtgcatacactggaatgcccaaccagaaacccaaggtgcccaccttaagacaagctaaggtgcaaggtccggcatttgaatttgccgtagcaatgatgaaaaggaacgccagcacagtcaagacagaatacggtgagttcacgatgcttggcatctatgataaatgggcagtgctgccgcgccacgccaagcctggaccaactattttaatgaatgatcaggaggttggtgtgctcgatgccaaagagttagttgataaagacggaaccaacctggagctgacactattgaagcttaaccgcaatgaaaagttcagagacatcagaggttttcttgcaagggaagaagttgaggtaagtgaggctgttttggcaataaacacgagcaagttcccaagcatgtacatccctgtgggccaagtcaccgattacggatttttaaatctaggtggcaccccaacaaagagaatgctcatgtacaacttccctaccagagcgggacagtgtggtggtgtccttatgtcaacaggaaaggtccttggcatacacgtgggaggaaatggtcaccaaggcttctctgctgctctcctcagacactacttcaacgaggaacagggcgaaatagagtttattgagagctctaaagatgcaggatttcctgtgatcaacacccctaataaaaccaaactggaaccaagtgtgtttcatcaggtttttgagggcaacaaagaaccagcagtcctaagaaacggagacccgcgacttaaagccaactttgaggaagcgatattttccaagtacatcggaaatgtgaacacacatgtggacgagtacatgatagaagctgttgatcactacgctggacagctggcaactctggacatcagtacagaacctatgaagcttgaggatgctgtttatggcactgaaggcttggaagcattggacttgaccactagcgcaggatatccttatgtcgccttgggcatcaagaaaagggatatcctctccaagaagactaaagatctcaccaagctgagggaatgcatggacaagtatggtctaaatctgccgatggtgacctacgtgaaggatgaactcaggtccgctgagaaagtagccaagggaaaatccagacttatagaagcttctagtctcaatgactcagtggccatgaggcagacatttgggaacctatacaagacattccacctcaacccaggcattgtcactggtagtgctgttgggtgcgacccagatgtgttttggagcaaaatacccgtgatgcttgacgggcaccttatagcttttgattactctggctacgacgctagcttgagcccagtgtggtttgcttgtttgaaactcctcctagggaaactagggtatactcataaggaaaccaattacatagactacctctgcaactcccatcacttatacagagataaacactatttcgtgaggggtggtatgccatcaggatgttcaggcaccagtatattcaacaccatgatcaacaacatcattattaggacccttatgctaaaggtctacaaaggtattgacctggatcagtttagaatgatcgcttacggggacgatgtgatagcctcttacccgtggcctattgatgcctcactactagcagaagcgggaaaggattatggtttgatcatgaccccagcagataaaggagagtgttttaatgaggtaacctggacaaatgtaaccttcttgaaaaggtactttagagctgatgaacaatatccattcttggtgcaccccgtgatgcccatgaaagacatacacgaatccattagatggaccaaagacccaaagaacactcaagatcatgtgcgctcgttatgcctattggcttggcacaatggggagcacgaatatgaggaatttatccgaaagatcagaagcgtgcctgttggacgctgtttgaccctcccggtgttctcaacactacgcaggaaatggttagattccttctaaaattagagtgcaatcaatgaactatgattggcttaaccctaccgcatgaaccgaactagacaaaagtgcggtaggggtaaattctccgcattcggtgcggaaaaaaaaaaaaaaaaaaaaaaaaaaaaaaaaaaaaaaaaaaaaaaaaaa

SEQ ID NO: 132 - DNA, 6658 bp, synthetic construct
  source 1..6658: mol_type = other DNA
  misc_feature 1..6658: note = H3N2 DNA vector construct
ttaaaacagcctgtgggttgtacccacccacagggcccactgggcgctagcactctggtatcacggtacctttgtgtgcctgttttatatcccctttccccgattgtaacttagaagatgtacacactgatcaatagcgggcatagcacaccagctatgtcttgatcaagcactcctgtatccccggaccaagtatcaatagactgctcacgcggttgaaggagaaaacgttcgtcacccggctaactacttcgagaaacccagtagtatcatgaaagttgcgaggcgtttcgttcagcacacccccagtgtagatcgggtcgatgagtcaccgcatcccccacgggcgaccgtggcggtggctgcgctggcggcctgcctacggggcaacccgtaggacgcttcaatacagacatggtgcgaagagtcgattgagctagttagtagtcctccggcccctgaatgcggctaatcctaactgcggagcacatgccctcaacccagggggtattgtgtcgtaacgggcaactctgcagcggaaccgactactttgggtgtccgtgtttccttttatccttatactggctgcttatggtgacaattgaaagattgttgccatatagctattggattggccatccagtgtctaatagagctgttatttacctctttgttggatttataccactcaacctaaaagaagttaaaacactacagctcattttacaactgaatacagcaaaccaccatgaaaaccgtgatcgccctcagttacatcttctgcctcgcctttggacagaatctcctcggaaacgaaaacaacgctgccacactctgcctgggacaccacgccgtgcccaacggcacaatggtgaagaccatcaccgacgatcagatcgaggtgaccaatgccaccgagctggtgcagaacagctccaccggcaaaatctgcaacaatccccacaagatcctggacggcagggattgcaccctgatcgacgctctgctgggcgaccctcactgcgacgtgttccagaatgagacatgggatctgttcgtggagaggagcaatgccttctccaactgctacccctacgacgtgcctgattacgccagcctgcggtccatcgtggccagctccggcaccctggagttcatcaccgagggcttcacctgggctggagtgacccagaacggaggcagcggagcttgcaagaggggacccgccaatagcttcttctcccggctgaactggctgaccaagtccggcaatacctaccccgtgctgaacgtgaccatgcctaacaataacaatttcgacaagctgtacatctggggcgtgcaccaccctagcaccgatcaggagcagaccagcctgtacatccaggcctccggcagggtgaccgtgagcaccaggcggtcccagcagaccatcatccccaacatcggctccaggcctctggtgcggggacagagcggccggatctccgtgtactggaccatcgtgaagcccggcgacatcctggtcatcaacagcaatggcaacctgatcgcccctcgcggctacttcaagatgcacatcggcaagagcagcatcatgagatccgacgcccccatcgatacctgcatcagcgagtgcatcacccctaatggctccatccccaacgagaagcctttccagaatgtgaacaagatcacctacggcgcctgccccaagtacgtgaagcagaataccctgaagctggccaccggcatgcgcaacgtgcctgagagacagaccgtgggcctgttcggagctatcgctggcttcatcgagaatggctgggagggcatggtggacggctggtacggcttccgccaccagaacagcgagggcaccggacaggctgccgacctgaagtccacccaggccgccatcgatcagatcaatggcaagctgaacagagtgatcgagaagaccaacgagaagttccaccagatcgagaaggagttcagcgaggtggagggacgcatccaggacctggagaggtacgtggaggacaccaagatcgatctgtggagctacaatgccgagctgctggtggccctggagaatcagaacaccatcgacctgaccgattccgagatgaacaagctgttcgagaagacccgcagacagctgcgcgagaatgccgaggacatgggcaacggctgcttcaaaatctaccacaagtgcgataacgcctgcatcgagagcatcagaaatggcacctacgaccacaacatctaccgcgatgaggccgtgaacaatagattccagatcaagggcgtggagctgaagtccggctacaaggactggattctgtggatcagcttcgccatctcctgcttcctgctgtgcgtggtgctgctggggtttattatgtgggcttgtcagagggggaacatcaggtgtaacatttgtaactttgagccaacaggggtgacggagtcccgcactgaaattacggcaatgcagaccaccggttcatgtgggcaacaatcaggagctgtgtacgtgggcaattacaggattgtaaacagacacctggcaacgagccacgattggcaaaattgcgtgtgggaggactacaacagggatctcctggtcagcacaacaactgctcatggttgtgatactatagcacggtgccaatgtactgctggcgtgtacttttgtgcatctagaaacaagcactacccagtgagcttcgagggtccaggtctagtgaaagttcaggagggcgagtactaccccgagagataccagtcgcacgtactccttgcagttggattttcagaaccgggtgattgtggaggtattttgaggtgtgaacatggagtcattgggctcgttaccatgggtggtgagggtgtagtaggcttcgctgacgtgcgggatcttttgtggttggaagacgacgccatggagcagggtgttagagattatgtagagcaactgggaaatgcatttggctcaggtttcactaaccaaatctgtgagcaagttaacctccttaaagaatctctgatagggcaggattccatattggaaaaatccctgaaggccctggttaaaatcatatcagccctggtgatagtggttaggaaccacgacgacctgattacagtgactgccacactagctttaatcggttgcgcatcatctccatggcgatggctcaaacaaaaagtgtgtcaatactacggaatccccatggcagaaaggcagaataacggttggttaaagaaattcactgaaatgaccaacgcctgcaagggcatggagtggattgctgttaaaattcaaaagttcatcgagtggctcaaagtaaagattctgcctgaagtgaaggagaaacatgagttccttaccagattgaagcaattgccactccttgaaagtcaaattgccaccattgagcaaagcgcaccctcacaaagtgatcaagagcagcttttttcgaatgttcagtacttcgcccattactgcaggaagtatgcacctctgtatgctgccgaagcaaaaagagtgttctcattagaaaagaaaatgagtaattacatacagttcaagtccaaatgccgcattgagcctgtatgcttactccttcacggtagtccaggggctggcaagtcagtagctaccaacctgatagggagatcccttgcagagaagctcaatagctctgtgtactctttaccaccagatccagatcattttgatgggtacaaacagcaggcagtggtgatcatggatgatctctgtcaaaaccccgatgggaaggacgtgtccttgttttgccaaatggtgtctagtgtagattttgtgccacccatggcggcgctggaagaaaaaggcattctctttacgtccccgtttgtgttggcatcaaccaacgcggggtccatcaatgcaccaacagtgtcagacagcagagcacttgccagaaggtttcactttgacatgaatattgaggtgatttcgatgtacagccagaatggtaaaattaacatgcccatgtctgttaagacatgtgatgatgaatgctgcccggtcaatttcaaaaagtgttgcccactagtgtgtggcaaggccatccagtttattgacaggagaaaccaagttagatattcactggacatgctggttactgagatgtttagagagtacaaccacagacacagtgtgggtgctaccctcgaggctttgttccaaggaccaccagtatacagggaaatcaaaatcagtgtggccccggaaacaccccctccaccagcaattgctgaccttctaaaatctgtagacagtgaggcaataagggagtactgcaaggaaaggggttggcttgtgccagaggtcagctccactctacaaattgaaaaacatgttagcagggcatttatttgcttgcaagcgctaactacatttgtttcagtggctggtataatctacatcatttacaagttgtttgccggctttcagggtgcatacactggaatgcccaaccagaaacccaaggtgcccaccttaagacaagctaaggtgcaaggtccggcatttgaatttgccgtagcaatgatgaaaaggaacgccagcacagtcaagacagaatacggtgagttcacgatgcttggcatctatgataaatgggcagtgctgccgcgccacgccaagcctggaccaactattttaatgaatgatcaggaggttggtgtgctcgatgccaaagagttagttgataaagacggaaccaacctggagctgacactattgaagcttaaccgcaatgaaaagttcagagacatcagaggttttcttgcaagggaagaagttgaggtaagtgaggctgttttggcaataaacacgagcaagttcccaagcatgtacatccctgtgggccaagtcaccgattacggatttttaaatctaggtggcaccccaacaaagagaatgctcatgtacaacttccctaccagagcgggacagtgtggtggtgtccttatgtcaacaggaaaggtccttggcatacacgtgggaggaaatggtcaccaaggcttctctgctgctctcctcagacactacttcaacgaggaacagggcgaaatagagtttattgagagctctaaagatgcaggatttcctgtgatcaacacccctaataaaaccaaactggaaccaagtgtgtttcatcaggtttttgagggcaacaaagaaccagcagtcctaagaaacggagacccgcgacttaaagccaactttgaggaagcgatattttccaagtacatcggaaatgtgaacacacatgtggacgagtacatgatagaagctgttgatcactacgctggacagctggcaactctggacatcagtacagaacctatgaagcttgaggatgctgtttatggcactgaaggcttggaagcattggacttgaccactagcgcaggatatccttatgtcgccttgggcatcaagaaaagggatatcctctccaagaagactaaagatctcaccaagctgagggaatgcatggacaagtatggtctaaatctgccgatggtgacctacgtgaaggatgaactcaggtccgctgagaaagtagccaagggaaaatccagacttatagaagcttctagtctcaatgactcagtggccatgaggcagacatttgggaacctatacaagacattccacctcaacccaggcattgtcactggtagtgctgttgggtgcgacccagatgtgttttggagcaaaatacccgtgatgcttgacgggcaccttatagcttttgattactctggctacgacgctagcttgagcccagtgtggtttgcttgtttgaaactcctcctagggaaactagggtatactcataaggaaaccaattacatagactacctctgcaactcccatcacttatacagagataaacactatttcgtgaggggtggtatgccatcaggatgttcaggcaccagtatattcaacaccatgatcaacaacatcattattaggacccttatgctaaaggtctacaaaggtattgacctggatcagtttagaatgatcgcttacggggacgatgtgatagcctcttacccgtggcctattgatgcctcactactagcagaagcgggaaaggattatggtttgatcatgaccccagcagataaaggagagtgttttaatgaggtaacctggacaaatgtaaccttcttgaaaaggtactttagagctgatgaacaatatccattcttggtgcaccccgtgatgcccatgaaagacatacacgaatccattagatggaccaaagacccaaagaacactcaagatcatgtgcgctcgttatgcctattggcttggcacaatggggagcacgaatatgaggaatttatccgaaagatcagaagcgtgcctgttggacgctgtttgaccctcccggtgttctcaacactacgcaggaaatggttagattccttctaaaattagagtgcaatcaatgaactatgattggcttaaccctaccgcatgaaccgaactagacaaaagtgcggtaggggtaaattctccgcattcggtgcggaaaaaaaaaaaaaaaaaaaaaaaaaaaaaaaaaaaaaaaaaaaaaaaaaa

SEQ ID NO: 133 - RNA, 2081 nt, synthetic construct
  source 1..2081: mol_type = other RNA
  misc_feature 1..2081: note = H3N8 mRNA construct
gagaataaactagtattcttctggtccccacagactcaatgaaaacaactattatcctcatcctgctcactcactgggcttactctcagaaccctatctccggcaacaacaccgctacactgtgcctgggacaccacgctgtggctaatggcaccctggtgaagaccatgtccgacgatcagatcgaggtgaccaacgccaccgagctggtgcagagcatcagcatgggcaaaatctgcaataagagctaccgcgtgctggacggcagaaactgcaccctgatcgatgctatgctgggcgacccccagtgcgatgctttccagtacgagtcctgggacctgttcatcgagaggagcaatgccttcagcaactgctacccctacgacatccctgattacgccagcctgagatccatcgtggccagctccggcaccgtggagttcaccgctgagggcttcacctggaccggagtgacccagaatggcaggtccggagcttgcaagaggggcagcgccgactccttcttcagcaggctgaactggctgaccaagagcggcagctcctaccccaccctgaatgtgaccatgcctaacaataagaacttcgataagctgtacatctggggcatccaccaccccagctccaaccaggagcagaccaagctgtacatccaggagtccggccgcgtgaccgtgtccaccaagagaagccagcagaccatcatcccccacatcggcagccgccctctgatcagaggacagtccggccggatcagcatctactggaccatcgtgaagcccggcgacatcctgatgatcaacagcaatggcaacctggtggcccccaggggctacttcaagctgaaccctggcaagagcagcgtgatccggtccgacgtgcctatcgacatctgcgtgagcgagtgcatcacccccaatggcagcatctccaacgataagcctttccagaatgtgaacaaggtgacctacggcaagtgccccaagtacatccgccagaataccctgaagctggccaccggcatgagaaacgtgcctgagaagcagaccgtgggaatcttcggagctatcgctggcttcatcgagaatggctgggagggcatggtggacggctggtacggcttccgctaccagaactccgagggcaccggacaggctgccgacctgaagagcacccaggccgccatcgatcagatcaatggcaagctgaaccgcgtgatcgagcggaccaacgagaagttccaccagatcgagaaggagttctccgaggtggagggcagaatccaggatctggagaagtacgtggaggacaccaagatcgatctgtggagctacaatgccgagctgctggtggccctggagaaccagcacaccatcgacctgaccgatgccgagatgaataagctgttcgagaagaccaggcggcagctgagggagaatgccgaggacatgggcaacggctgcttcaaaatctaccacaagtgcgataacgcctgcatcgagtccatccggaccggcacctacgaccactacatctacagggatgaggccatcaacaatcggttccagatcaagggcgtggagctgaagagcggctacaaggactggattctgtggatctccttcgccatcagctgcttcctgatctgcgtggtgctcctcgggttcattatgtgggcttgccagaagggaaacattcgctgtaacatttgtatctaactcgagctggtactgcatgcacgcaatgctagctgcccctttcccgtcctgggtaccccgagtctcccccgacctcgggtcccaggtatgctcccacctccacctgccccactcaccacctctgctagttccagacacctcccaagcacgcagcaatgcagctcaaaacgcttagcctagccacacccccacgggaaacagcagtgattaacctttagcaataaacgaaagtttaactaagctatactaaccccagggttggtcaatttcgtgccagccacaccctggagctagcaaaaaaaaaaaaaaaaaaaaaaaaaaaaaaaaaaaaaaaaaaaaaaaaaa

SEQ ID NO: 134 - RNA, 6658 nt, synthetic construct
  source 1..6658: mol_type = other RNA
  misc_feature 1..6658: note = H3N8 saRNA construct
ttaaaacagcctgtgggttgtacccacccacagggcccactgggcgctagcactctggtatcacggtacctttgtgtgcctgttttatatcccctttccccgattgtaacttagaagatgtacacactgatcaatagcgggcatagcacaccagctatgtcttgatcaagcactcctgtatccccggaccaagtatcaatagactgctcacgcggttgaaggagaaaacgttcgtcacccggctaactacttcgagaaacccagtagtatcatgaaagttgcgaggcgtttcgttcagcacacccccagtgtagatcgggtcgatgagtcaccgcatcccccacgggcgaccgtggcggtggctgcgctggcggcctgcctacggggcaacccgtaggacgcttcaatacagacatggtgcgaagagtcgattgagctagttagtagtcctccggcccctgaatgcggctaatcctaactgcggagcacatgccctcaacccagggggtattgtgtcgtaacgggcaactctgcagcggaaccgactactttgggtgtccgtgtttccttttatccttatactggctgcttatggtgacaattgaaagattgttgccatatagctattggattggccatccagtgtctaatagagctgttatttacctctttgttggatttataccactcaacctaaaagaagttaaaacactacagctcattttacaactgaatacagcaaaccaccatgaaaacaactattatcctcatcctgctcactcactgggcttactctcagaaccctatctccggcaacaacaccgctacactgtgcctgggacaccacgctgtggctaatggcaccctggtgaagaccatgtccgacgatcagatcgaggtgaccaacgccaccgagctggtgcagagcatcagcatgggcaaaatctgcaataagagctaccgcgtgctggacggcagaaactgcaccctgatcgatgctatgctgggcgacccccagtgcgatgctttccagtacgagtcctgggacctgttcatcgagaggagcaatgccttcagcaactgctacccctacgacatccctgattacgccagcctgagatccatcgtggccagctccggcaccgtggagttcaccgctgagggcttcacctggaccggagtgacccagaatggcaggtccggagcttgcaagaggggcagcgccgactccttcttcagcaggctgaactggctgaccaagagcggcagctcctaccccaccctgaatgtgaccatgcctaacaataagaacttcgataagctgtacatctggggcatccaccaccccagctccaaccaggagcagaccaagctgtacatccaggagtccggccgcgtgaccgtgtccaccaagagaagccagcagaccatcatcccccacatcggcagccgccctctgatcagaggacagtccggccggatcagcatctactggaccatcgtgaagcccggcgacatcctgatgatcaacagcaatggcaacctggtggcccccaggggctacttcaagctgaaccctggcaagagcagcgtgatccggtccgacgtgcctatcgacatctgcgtgagcgagtgcatcacccccaatggcagcatctccaacgataagcctttccagaatgtgaacaaggtgacctacggcaagtgccccaagtacatccgccagaataccctgaagctggccaccggcatgagaaacgtgcctgagaagcagaccgtgggaatcttcggagctatcgctggcttcatcgagaatggctgggagggcatggtggacggctggtacggcttccgctaccagaactccgagggcaccggacaggctgccgacctgaagagcacccaggccgccatcgatcagatcaatggcaagctgaaccgcgtgatcgagcggaccaacgagaagttccaccagatcgagaaggagttctccgaggtggagggcagaatccaggatctggagaagtacgtggaggacaccaagatcgatctgtggagctacaatgccgagctgctggtggccctggagaaccagcacaccatcgacctgaccgatgccgagatgaataagctgttcgagaagaccaggcggcagctgagggagaatgccgaggacatgggcaacggctgcttcaaaatctaccacaagtgcgataacgcctgcatcgagtccatccggaccggcacctacgaccactacatctacagggatgaggccatcaacaatcggttccagatcaagggcgtggagctgaagagcggctacaaggactggattctgtggatctccttcgccatcagctgcttcctgatctgcgtggtgctcctcgggttcattatgtgggcttgccagaagggaaacattcgctgtaacatttgtatcaactttgagccaacaggggtgacggagtcccgcactgaaattacggcaatgcagaccaccggttcatgtgggcaacaatcaggagctgtgtacgtgggcaattacaggattgtaaacagacacctggcaacgagccacgattggcaaaattgcgtgtgggaggactacaacagggatctcctggtcagcacaacaactgctcatggttgtgatactatagcacggtgccaatgtactgctggcgtgtacttttgtgcatctagaaacaagcactacccagtgagcttcgagggtccaggtctagtgaaagttcaggagggcgagtactaccccgagagataccagtcgcacgtactccttgcagttggattttcagaaccgggtgattgtggaggtattttgaggtgtgaacatggagtcattgggctcgttaccatgggtggtgagggtgtagtaggcttcgctgacgtgcgggatcttttgtggttggaagacgacgccatggagcagggtgttagagattatgtagagcaactgggaaatgcatttggctcaggtttcactaaccaaatctgtgagcaagttaacctccttaaagaatctctgatagggcaggattccatattggaaaaatccctgaaggccctggttaaaatcatatcagccctggtgatagtggttaggaaccacgacgacctgattacagtgactgccacactagctttaatcggttgcgcatcatctccatggcgatggctcaaacaaaaagtgtgtcaatactacggaatccccatggcagaaaggcagaataacggttggttaaagaaattcactgaaatgaccaacgcctgcaagggcatggagtggattgctgttaaaattcaaaagttcatcgagtggctcaaagtaaagattctgcctgaagtgaaggagaaacatgagttccttaccagattgaagcaattgccactccttgaaagtcaaattgccaccattgagcaaagcgcaccctcacaaagtgatcaagagcagcttttttcgaatgttcagtacttcgcccattactgcaggaagtatgcacctctgtatgctgccgaagcaaaaagagtgttctcattagaaaagaaaatgagtaattacatacagttcaagtccaaatgccgcattgagcctgtatgcttactccttcacggtagtccaggggctggcaagtcagtagctaccaacctgatagggagatcccttgcagagaagctcaatagctctgtgtactctttaccaccagatccagatcattttgatgggtacaaacagcaggcagtggtgatcatggatgatctctgtcaaaaccccgatgggaaggacgtgtccttgttttgccaaatggtgtctagtgtagattttgtgccacccatggcggcgctggaagaaaaaggcattctctttacgtccccgtttgtgttggcatcaaccaacgcggggtccatcaatgcaccaacagtgtcagacagcagagcacttgccagaaggtttcactttgacatgaatattgaggtgatttcgatgtacagccagaatggtaaaattaacatgcccatgtctgttaagacatgtgatgatgaatgctgcccggtcaatttcaaaaagtgttgcccactagtgtgtggcaaggccatccagtttattgacaggagaaaccaagttagatattcactggacatgctggttactgagatgtttagagagtacaaccacagacacagtgtgggtgctaccctcgaggctttgttccaaggaccaccagtatacagggaaatcaaaatcagtgtggccccggaaacaccccctccaccagcaattgctgaccttctaaaatctgtagacagtgaggcaataagggagtactgcaaggaaaggggttggcttgtgccagaggtcagctccactctacaaattgaaaaacatgttagcagggcatttatttgcttgcaagcgctaactacatttgtttcagtggctggtataatctacatcatttacaagttgtttgccggctttcagggtgcatacactggaatgcccaaccagaaacccaaggtgcccaccttaagacaagctaaggtgcaaggtccggcatttgaatttgccgtagcaatgatgaaaaggaacgccagcacagtcaagacagaatacggtgagttcacgatgcttggcatctatgataaatgggcagtgctgccgcgccacgccaagcctggaccaactattttaatgaatgatcaggaggttggtgtgctcgatgccaaagagttagttgataaagacggaaccaacctggagctgacactattgaagcttaaccgcaatgaaaagttcagagacatcagaggttttcttgcaagggaagaagttgaggtaagtgaggctgttttggcaataaacacgagcaagttcccaagcatgtacatccctgtgggccaagtcaccgattacggatttttaaatctaggtggcaccccaacaaagagaatgctcatgtacaacttccctaccagagcgggacagtgtggtggtgtccttatgtcaacaggaaaggtccttggcatacacgtgggaggaaatggtcaccaaggcttctctgctgctctcctcagacactacttcaacgaggaacagggcgaaatagagtttattgagagctctaaagatgcaggatttcctgtgatcaacacccctaataaaaccaaactggaaccaagtgtgtttcatcaggtttttgagggcaacaaagaaccagcagtcctaagaaacggagacccgcgacttaaagccaactttgaggaagcgatattttccaagtacatcggaaatgtgaacacacatgtggacgagtacatgatagaagctgttgatcactacgctggacagctggcaactctggacatcagtacagaacctatgaagcttgaggatgctgtttatggcactgaaggcttggaagcattggacttgaccactagcgcaggatatccttatgtcgccttgggcatcaagaaaagggatatcctctccaagaagactaaagatctcaccaagctgagggaatgcatggacaagtatggtctaaatctgccgatggtgacctacgtgaaggatgaactcaggtccgctgagaaagtagccaagggaaaatccagacttatagaagcttctagtctcaatgactcagtggccatgaggcagacatttgggaacctatacaagacattccacctcaacccaggcattgtcactggtagtgctgttgggtgcgacccagatgtgttttggagcaaaatacccgtgatgcttgacgggcaccttatagcttttgattactctggctacgacgctagcttgagcccagtgtggtttgcttgtttgaaactcctcctagggaaactagggtatactcataaggaaaccaattacatagactacctctgcaactcccatcacttatacagagataaacactatttcgtgaggggtggtatgccatcaggatgttcaggcaccagtatattcaacaccatgatcaacaacatcattattaggacccttatgctaaaggtctacaaaggtattgacctggatcagtttagaatgatcgcttacggggacgatgtgatagcctcttacccgtggcctattgatgcctcactactagcagaagcgggaaaggattatggtttgatcatgaccccagcagataaaggagagtgttttaatgaggtaacctggacaaatgtaaccttcttgaaaaggtactttagagctgatgaacaatatccattcttggtgcaccccgtgatgcccatgaaagacatacacgaatccattagatggaccaaagacccaaagaacactcaagatcatgtgcgctcgttatgcctattggcttggcacaatggggagcacgaatatgaggaatttatccgaaagatcagaagcgtgcctgttggacgctgtttgaccctcccggtgttctcaacactacgcaggaaatggttagattccttctaaaattagagtgcaatcaatgaactatgattggcttaaccctaccgcatgaaccgaactagacaaaagtgcggtaggggtaaattctccgcattcggtgcggaaaaaaaaaaaaaaaaaaaaaaaaaaaaaaaaaaaaaaaaaaaaaaaaaa

SEQ ID NO: 135 - DNA, 6658 bp, synthetic construct
  source 1..6658: mol_type = other DNA
  misc_feature 1..6658: note = H3N8 DNA vector construct
ttaaaacagcctgtgggttgtacccacccacagggcccactgggcgctagcactctggtatcacggtacctttgtgtgcctgttttatatcccctttccccgattgtaacttagaagatgtacacactgatcaatagcgggcatagcacaccagctatgtcttgatcaagcactcctgtatccccggaccaagtatcaatagactgctcacgcggttgaaggagaaaacgttcgtcacccggctaactacttcgagaaacccagtagtatcatgaaagttgcgaggcgtttcgttcagcacacccccagtgtagatcgggtcgatgagtcaccgcatcccccacgggcgaccgtggcggtggctgcgctggcggcctgcctacggggcaacccgtaggacgcttcaatacagacatggtgcgaagagtcgattgagctagttagtagtcctccggcccctgaatgcggctaatcctaactgcggagcacatgccctcaacccagggggtattgtgtcgtaacgggcaactctgcagcggaaccgactactttgggtgtccgtgtttccttttatccttatactggctgcttatggtgacaattgaaagattgttgccatatagctattggattggccatccagtgtctaatagagctgttatttacctctttgttggatttataccactcaacctaaaagaagttaaaacactacagctcattttacaactgaatacagcaaaccaccatgaaaacaactattatcctcatcctgctcactcactgggcttactctcagaaccctatctccggcaacaacaccgctacactgtgcctgggacaccacgctgtggctaatggcaccctggtgaagaccatgtccgacgatcagatcgaggtgaccaacgccaccgagctggtgcagagcatcagcatgggcaaaatctgcaataagagctaccgcgtgctggacggcagaaactgcaccctgatcgatgctatgctgggcgacccccagtgcgatgctttccagtacgagtcctgggacctgttcatcgagaggagcaatgccttcagcaactgctacccctacgacatccctgattacgccagcctgagatccatcgtggccagctccggcaccgtggagttcaccgctgagggcttcacctggaccggagtgacccagaatggcaggtccggagcttgcaagaggggcagcgccgactccttcttcagcaggctgaactggctgaccaagagcggcagctcctaccccaccctgaatgtgaccatgcctaacaataagaacttcgataagctgtacatctggggcatccaccaccccagctccaaccaggagcagaccaagctgtacatccaggagtccggccgcgtgaccgtgtccaccaagagaagccagcagaccatcatcccccacatcggcagccgccctctgatcagaggacagtccggccggatcagcatctactggaccatcgtgaagcccggcgacatcctgatgatcaacagcaatggcaacctggtggcccccaggggctacttcaagctgaaccctggcaagagcagcgtgatccggtccgacgtgcctatcgacatctgcgtgagcgagtgcatcacccccaatggcagcatctccaacgataagcctttccagaatgtgaacaaggtgacctacggcaagtgccccaagtacatccgccagaataccctgaagctggccaccggcatgagaaacgtgcctgagaagcagaccgtgggaatcttcggagctatcgctggcttcatcgagaatggctgggagggcatggtggacggctggtacggcttccgctaccagaactccgagggcaccggacaggctgccgacctgaagagcacccaggccgccatcgatcagatcaatggcaagctgaaccgcgtgatcgagcggaccaacgagaagttccaccagatcgagaaggagttctccgaggtggagggcagaatccaggatctggagaagtacgtggaggacaccaagatcgatctgtggagctacaatgccgagctgctggtggccctggagaaccagcacaccatcgacctgaccgatgccgagatgaataagctgttcgagaagaccaggcggcagctgagggagaatgccgaggacatgggcaacggctgcttcaaaatctaccacaagtgcgataacgcctgcatcgagtccatccggaccggcacctacgaccactacatctacagggatgaggccatcaacaatcggttccagatcaagggcgtggagctgaagagcggctacaaggactggattctgtggatctccttcgccatcagctgcttcctgatctgcgtggtgctcctcgggttcattatgtgggcttgccagaagggaaacattcgctgtaacatttgtatcaactttgagccaacaggggtgacggagtcccgcactgaaattacggcaatgcagaccaccggttcatgtgggcaacaatcaggagctgtgtacgtgggcaattacaggattgtaaacagacacctggcaacgagccacgattggcaaaattgcgtgtgggaggactacaacagggatctcctggtcagcacaacaactgctcatggttgtgatactatagcacggtgccaatgtactgctggcgtgtacttttgtgcatctagaaacaagcactacccagtgagcttcgagggtccaggtctagtgaaagttcaggagggcgagtactaccccgagagataccagtcgcacgtactccttgcagttggattttcagaaccgggtgattgtggaggtattttgaggtgtgaacatggagtcattgggctcgttaccatgggtggtgagggtgtagtaggcttcgctgacgtgcgggatcttttgtggttggaagacgacgccatggagcagggtgttagagattatgtagagcaactgggaaatgcatttggctcaggtttcactaaccaaatctgtgagcaagttaacctccttaaagaatctctgatagggcaggattccatattggaaaaatccctgaaggccctggttaaaatcatatcagccctggtgatagtggttaggaaccacgacgacctgattacagtgactgccacactagctttaatcggttgcgcatcatctccatggcgatggctcaaacaaaaagtgtgtcaatactacggaatccccatggcagaaaggcagaataacggttggttaaagaaattcactgaaatgaccaacgcctgcaagggcatggagtggattgctgttaaaattcaaaagttcatcgagtggctcaaagtaaagattctgcctgaagtgaaggagaaacatgagttccttaccagattgaagcaattgccactccttgaaagtcaaattgccaccattgagcaaagcgcaccctcacaaagtgatcaagagcagcttttttcgaatgttcagtacttcgcccattactgcaggaagtatgcacctctgtatgctgccgaagcaaaaagagtgttctcattagaaaagaaaatgagtaattacatacagttcaagtccaaatgccgcattgagcctgtatgcttactccttcacggtagtccaggggctggcaagtcagtagctaccaacctgatagggagatcccttgcagagaagctcaatagctctgtgtactctttaccaccagatccagatcattttgatgggtacaaacagcaggcagtggtgatcatggatgatctctgtcaaaaccccgatgggaaggacgtgtccttgttttgccaaatggtgtctagtgtagattttgtgccacccatggcggcgctggaagaaaaaggcattctctttacgtccccgtttgtgttggcatcaaccaacgcggggtccatcaatgcaccaacagtgtcagacagcagagcacttgccagaaggtttcactttgacatgaatattgaggtgatttcgatgtacagccagaatggtaaaattaacatgcccatgtctgttaagacatgtgatgatgaatgctgcccggtcaatttcaaaaagtgttgcccactagtgtgtggcaaggccatccagtttattgacaggagaaaccaagttagatattcactggacatgctggttactgagatgtttagagagtacaaccacagacacagtgtgggtgctaccctcgaggctttgttccaaggaccaccagtatacagggaaatcaaaatcagtgtggccccggaaacaccccctccaccagcaattgctgaccttctaaaatctgtagacagtgaggcaataagggagtactgcaaggaaaggggttggcttgtgccagaggtcagctccactctacaaattgaaaaacatgttagcagggcatttatttgcttgcaagcgctaactacatttgtttcagtggctggtataatctacatcatttacaagttgtttgccggctttcagggtgcatacactggaatgcccaaccagaaacccaaggtgcccaccttaagacaagctaaggtgcaaggtccggcatttgaatttgccgtagcaatgatgaaaaggaacgccagcacagtcaagacagaatacggtgagttcacgatgcttggcatctatgataaatgggcagtgctgccgcgccacgccaagcctggaccaactattttaatgaatgatcaggaggttggtgtgctcgatgccaaagagttagttgataaagacggaaccaacctggagctgacactattgaagcttaaccgcaatgaaaagttcagagacatcagaggttttcttgcaagggaagaagttgaggtaagtgaggctgttttggcaataaacacgagcaagttcccaagcatgtacatccctgtgggccaagtcaccgattacggatttttaaatctaggtggcaccccaacaaagagaatgctcatgtacaacttccctaccagagcgggacagtgtggtggtgtccttatgtcaacaggaaaggtccttggcatacacgtgggaggaaatggtcaccaaggcttctctgctgctctcctcagacactacttcaacgaggaacagggcgaaatagagtttattgagagctctaaagatgcaggatttcctgtgatcaacacccctaataaaaccaaactggaaccaagtgtgtttcatcaggtttttgagggcaacaaagaaccagcagtcctaagaaacggagacccgcgacttaaagccaactttgaggaagcgatattttccaagtacatcggaaatgtgaacacacatgtggacgagtacatgatagaagctgttgatcactacgctggacagctggcaactctggacatcagtacagaacctatgaagcttgaggatgctgtttatggcactgaaggcttggaagcattggacttgaccactagcgcaggatatccttatgtcgccttgggcatcaagaaaagggatatcctctccaagaagactaaagatctcaccaagctgagggaatgcatggacaagtatggtctaaatctgccgatggtgacctacgtgaaggatgaactcaggtccgctgagaaagtagccaagggaaaatccagacttatagaagcttctagtctcaatgactcagtggccatgaggcagacatttgggaacctatacaagacattccacctcaacccaggcattgtcactggtagtgctgttgggtgcgacccagatgtgttttggagcaaaatacccgtgatgcttgacgggcaccttatagcttttgattactctggctacgacgctagcttgagcccagtgtggtttgcttgtttgaaactcctcctagggaaactagggtatactcataaggaaaccaattacatagactacctctgcaactcccatcacttatacagagataaacactatttcgtgaggggtggtatgccatcaggatgttcaggcaccagtatattcaacaccatgatcaacaacatcattattaggacccttatgctaaaggtctacaaaggtattgacctggatcagtttagaatgatcgcttacggggacgatgtgatagcctcttacccgtggcctattgatgcctcactactagcagaagcgggaaaggattatggtttgatcatgaccccagcagataaaggagagtgttttaatgaggtaacctggacaaatgtaaccttcttgaaaaggtactttagagctgatgaacaatatccattcttggtgcaccccgtgatgcccatgaaagacatacacgaatccattagatggaccaaagacccaaagaacactcaagatcatgtgcgctcgttatgcctattggcttggcacaatggggagcacgaatatgaggaatttatccgaaagatcagaagcgtgcctgttggacgctgtttgaccctcccggtgttctcaacactacgcaggaaatggttagattccttctaaaattagagtgcaatcaatgaactatgattggcttaaccctaccgcatgaaccgaactagacaaaagtgcggtaggggtaaattctccgcattcggtgcggaaaaaaaaaaaaaaaaaaaaaaaaaaaaaaaaaaaaaaaaaaaaaaaaaa

SEQ ID NO: 136 - RNA, 3815 nt, synthetic construct
  source 1..3815: mol_type = other RNA
  misc_feature 1..3815: note = H3N2_H3N8 mRNA construct
gagaataaactagtattcttctggtccccacagactcaatgaaaaccgtgatcgccctcagttacatcttctgcctcgcctttggacagaatctcctcggaaacgaaaacaacgctgccacactctgcctgggacaccacgccgtgcccaacggcacaatggtgaagaccatcaccgacgatcagatcgaggtgaccaatgccaccgagctggtgcagaacagctccaccggcaaaatctgcaacaatccccacaagatcctggacggcagggattgcaccctgatcgacgctctgctgggcgaccctcactgcgacgtgttccagaatgagacatgggatctgttcgtggagaggagcaatgccttctccaactgctacccctacgacgtgcctgattacgccagcctgcggtccatcgtggccagctccggcaccctggagttcatcaccgagggcttcacctgggctggagtgacccagaacggaggcagcggagcttgcaagaggggacccgccaatagcttcttctcccggctgaactggctgaccaagtccggcaatacctaccccgtgctgaacgtgaccatgcctaacaataacaatttcgacaagctgtacatctggggcgtgcaccaccctagcaccgatcaggagcagaccagcctgtacatccaggcctccggcagggtgaccgtgagcaccaggcggtcccagcagaccatcatccccaacatcggctccaggcctctggtgcggggacagagcggccggatctccgtgtactggaccatcgtgaagcccggcgacatcctggtcatcaacagcaatggcaacctgatcgcccctcgcggctacttcaagatgcacatcggcaagagcagcatcatgagatccgacgcccccatcgatacctgcatcagcgagtgcatcacccctaatggctccatccccaacgagaagcctttccagaatgtgaacaagatcacctacggcgcctgccccaagtacgtgaagcagaataccctgaagctggccaccggcatgcgcaacgtgcctgagagacagaccgtgggcctgttcggagctatcgctggcttcatcgagaatggctgggagggcatggtggacggctggtacggcttccgccaccagaacagcgagggcaccggacaggctgccgacctgaagtccacccaggccgccatcgatcagatcaatggcaagctgaacagagtgatcgagaagaccaacgagaagttccaccagatcgagaaggagttcagcgaggtggagggacgcatccaggacctggagaggtacgtggaggacaccaagatcgatctgtggagctacaatgccgagctgctggtggccctggagaatcagaacaccatcgacctgaccgattccgagatgaacaagctgttcgagaagacccgcagacagctgcgcgagaatgccgaggacatgggcaacggctgcttcaaaatctaccacaagtgcgataacgcctgcatcgagagcatcagaaatggcacctacgaccacaacatctaccgcgatgaggccgtgaacaatagattccagatcaagggcgtggagctgaagtccggctacaaggactggattctgtggatcagcttcgccatctcctgcttcctgctgtgcgtggtgctgctggggtttattatgtgggcttgtcagagggggaacatcaggtgtaacatttgtattctcgaggctttgttccaaggaccaccagtatacaggatgaaaacaactattatcctcatcctgctcactcactgggcttactctcagaaccctatctccggcaacaacaccgctacactgtgcctgggacaccacgctgtggctaatggcaccctggtgaagaccatgtccgacgatcagatcgaggtgaccaacgccaccgagctggtgcagagcatcagcatgggcaaaatctgcaataagagctaccgcgtgctggacggcagaaactgcaccctgatcgatgctatgctgggcgacccccagtgcgatgctttccagtacgagtcctgggacctgttcatcgagaggagcaatgccttcagcaactgctacccctacgacatccctgattacgccagcctgagatccatcgtggccagctccggcaccgtggagttcaccgctgagggcttcacctggaccggagtgacccagaatggcaggtccggagcttgcaagaggggcagcgccgactccttcttcagcaggctgaactggctgaccaagagcggcagctcctaccccaccctgaatgtgaccatgcctaacaataagaacttcgataagctgtacatctggggcatccaccaccccagctccaaccaggagcagaccaagctgtacatccaggagtccggccgcgtgaccgtgtccaccaagagaagccagcagaccatcatcccccacatcggcagccgccctctgatcagaggacagtccggccggatcagcatctactggaccatcgtgaagcccggcgacatcctgatgatcaacagcaatggcaacctggtggcccccaggggctacttcaagctgaaccctggcaagagcagcgtgatccggtccgacgtgcctatcgacatctgcgtgagcgagtgcatcacccccaatggcagcatctccaacgataagcctttccagaatgtgaacaaggtgacctacggcaagtgccccaagtacatccgccagaataccctgaagctggccaccggcatgagaaacgtgcctgagaagcagaccgtgggaatcttcggagctatcgctggcttcatcgagaatggctgggagggcatggtggacggctggtacggcttccgctaccagaactccgagggcaccggacaggctgccgacctgaagagcacccaggccgccatcgatcagatcaatggcaagctgaaccgcgtgatcgagcggaccaacgagaagttccaccagatcgagaaggagttctccgaggtggagggcagaatccaggatctggagaagtacgtggaggacaccaagatcgatctgtggagctacaatgccgagctgctggtggccctggagaaccagcacaccatcgacctgaccgatgccgagatgaataagctgttcgagaagaccaggcggcagctgagggagaatgccgaggacatgggcaacggctgcttcaaaatctaccacaagtgcgataacgcctgcatcgagtccatccggaccggcacctacgaccactacatctacagggatgaggccatcaacaatcggttccagatcaagggcgtggagctgaagagcggctacaaggactggattctgtggatctccttcgccatcagctgcttcctgatctgcgtggtgctcctcgggttcattatgtgggcttgccagaagggaaacattcgctgtaacatttgtatctaactcgagctggtactgcatgcacgcaatgctagctgcccctttcccgtcctgggtaccccgagtctcccccgacctcgggtcccaggtatgctcccacctccacctgccccactcaccacctctgctagttccagacacctcccaagcacgcagcaatgcagctcaaaacgcttagcctagccacacccccacgggaaacagcagtgattaacctttagcaataaacgaaagtttaactaagctatactaaccccagggttggtcaatttcgtgccagccacaccctggagctagcaaaaaaaaaaaaaaaaaaaaaaaaaaaaaaaaaaaaaaaaaaaaaaaaaa

SEQ ID NO: 137 - RNA, 8392 nt, synthetic construct
  source 1..8392: mol_type = other RNA
  misc_feature 1..8392: note = H3N2_H3N8 saRNA construct
ttaaaacagcctgtgggttgtacccacccacagggcccactgggcgctagcactctggtatcacggtacctttgtgtgcctgttttatatcccctttccccgattgtaacttagaagatgtacacactgatcaatagcgggcatagcacaccagctatgtcttgatcaagcactcctgtatccccggaccaagtatcaatagactgctcacgcggttgaaggagaaaacgttcgtcacccggctaactacttcgagaaacccagtagtatcatgaaagttgcgaggcgtttcgttcagcacacccccagtgtagatcgggtcgatgagtcaccgcatcccccacgggcgaccgtggcggtggctgcgctggcggcctgcctacggggcaacccgtaggacgcttcaatacagacatggtgcgaagagtcgattgagctagttagtagtcctccggcccctgaatgcggctaatcctaactgcggagcacatgccctcaacccagggggtattgtgtcgtaacgggcaactctgcagcggaaccgactactttgggtgtccgtgtttccttttatccttatactggctgcttatggtgacaattgaaagattgttgccatatagctattggattggccatccagtgtctaatagagctgttatttacctctttgttggatttataccactcaacctaaaagaagttaaaacactacagctcattttacaactgaatacagcaaaccaccatgaaaaccgtgatcgccctcagttacatcttctgcctcgcctttggacagaatctcctcggaaacgaaaacaacgctgccacactctgcctgggacaccacgccgtgcccaacggcacaatggtgaagaccatcaccgacgatcagatcgaggtgaccaatgccaccgagctggtgcagaacagctccaccggcaaaatctgcaacaatccccacaagatcctggacggcagggattgcaccctgatcgacgctctgctgggcgaccctcactgcgacgtgttccagaatgagacatgggatctgttcgtggagaggagcaatgccttctccaactgctacccctacgacgtgcctgattacgccagcctgcggtccatcgtggccagctccggcaccctggagttcatcaccgagggcttcacctgggctggagtgacccagaacggaggcagcggagcttgcaagaggggacccgccaatagcttcttctcccggctgaactggctgaccaagtccggcaatacctaccccgtgctgaacgtgaccatgcctaacaataacaatttcgacaagctgtacatctggggcgtgcaccaccctagcaccgatcaggagcagaccagcctgtacatccaggcctccggcagggtgaccgtgagcaccaggcggtcccagcagaccatcatccccaacatcggctccaggcctctggtgcggggacagagcggccggatctccgtgtactggaccatcgtgaagcccggcgacatcctggtcatcaacagcaatggcaacctgatcgcccctcgcggctacttcaagatgcacatcggcaagagcagcatcatgagatccgacgcccccatcgatacctgcatcagcgagtgcatcacccctaatggctccatccccaacgagaagcctttccagaatgtgaacaagatcacctacggcgcctgccccaagtacgtgaagcagaataccctgaagctggccaccggcatgcgcaacgtgcctgagagacagaccgtgggcctgttcggagctatcgctggcttcatcgagaatggctgggagggcatggtggacggctggtacggcttccgccaccagaacagcgagggcaccggacaggctgccgacctgaagtccacccaggccgccatcgatcagatcaatggcaagctgaacagagtgatcgagaagaccaacgagaagttccaccagatcgagaaggagttcagcgaggtggagggacgcatccaggacctggagaggtacgtggaggacaccaagatcgatctgtggagctacaatgccgagctgctggtggccctggagaatcagaacaccatcgacctgaccgattccgagatgaacaagctgttcgagaagacccgcagacagctgcgcgagaatgccgaggacatgggcaacggctgcttcaaaatctaccacaagtgcgataacgcctgcatcgagagcatcagaaatggcacctacgaccacaacatctaccgcgatgaggccgtgaacaatagattccagatcaagggcgtggagctgaagtccggctacaaggactggattctgtggatcagcttcgccatctcctgcttcctgctgtgcgtggtgctgctggggtttattatgtgggcttgtcagagggggaacatcaggtgtaacatttgtattctcgaggctttgttccaaggaccaccagtatacaggatgaaaacaactattatcctcatcctgctcactcactgggcttactctcagaaccctatctccggcaacaacaccgctacactgtgcctgggacaccacgctgtggctaatggcaccctggtgaagaccatgtccgacgatcagatcgaggtgaccaacgccaccgagctggtgcagagcatcagcatgggcaaaatctgcaataagagctaccgcgtgctggacggcagaaactgcaccctgatcgatgctatgctgggcgacccccagtgcgatgctttccagtacgagtcctgggacctgttcatcgagaggagcaatgccttcagcaactgctacccctacgacatccctgattacgccagcctgagatccatcgtggccagctccggcaccgtggagttcaccgctgagggcttcacctggaccggagtgacccagaatggcaggtccggagcttgcaagaggggcagcgccgactccttcttcagcaggctgaactggctgaccaagagcggcagctcctaccccaccctgaatgtgaccatgcctaacaataagaacttcgataagctgtacatctggggcatccaccaccccagctccaaccaggagcagaccaagctgtacatccaggagtccggccgcgtgaccgtgtccaccaagagaagccagcagaccatcatcccccacatcggcagccgccctctgatcagaggacagtccggccggatcagcatctactggaccatcgtgaagcccggcgacatcctgatgatcaacagcaatggcaacctggtggcccccaggggctacttcaagctgaaccctggcaagagcagcgtgatccggtccgacgtgcctatcgacatctgcgtgagcgagtgcatcacccccaatggcagcatctccaacgataagcctttccagaatgtgaacaaggtgacctacggcaagtgccccaagtacatccgccagaataccctgaagctggccaccggcatgagaaacgtgcctgagaagcagaccgtgggaatcttcggagctatcgctggcttcatcgagaatggctgggagggcatggtggacggctggtacggcttccgctaccagaactccgagggcaccggacaggctgccgacctgaagagcacccaggccgccatcgatcagatcaatggcaagctgaaccgcgtgatcgagcggaccaacgagaagttccaccagatcgagaaggagttctccgaggtggagggcagaatccaggatctggagaagtacgtggaggacaccaagatcgatctgtggagctacaatgccgagctgctggtggccctggagaaccagcacaccatcgacctgaccgatgccgagatgaataagctgttcgagaagaccaggcggcagctgagggagaatgccgaggacatgggcaacggctgcttcaaaatctaccacaagtgcgataacgcctgcatcgagtccatccggaccggcacctacgaccactacatctacagggatgaggccatcaacaatcggttccagatcaagggcgtggagctgaagagcggctacaaggactggattctgtggatctccttcgccatcagctgcttcctgatctgcgtggtgctcctcgggttcattatgtgggcttgccagaagggaaacattcgctgtaacatttgtatcaactttgagccaacaggggtgacggagtcccgcactgaaattacggcaatgcagaccaccggttcatgtgggcaacaatcaggagctgtgtacgtgggcaattacaggattgtaaacagacacctggcaacgagccacgattggcaaaattgcgtgtgggaggactacaacagggatctcctggtcagcacaacaactgctcatggttgtgatactatagcacggtgccaatgtactgctggcgtgtacttttgtgcatctagaaacaagcactacccagtgagcttcgagggtccaggtctagtgaaagttcaggagggcgagtactaccccgagagataccagtcgcacgtactccttgcagttggattttcagaaccgggtgattgtggaggtattttgaggtgtgaacatggagtcattgggctcgttaccatgggtggtgagggtgtagtaggcttcgctgacgtgcgggatcttttgtggttggaagacgacgccatggagcagggtgttagagattatgtagagcaactgggaaatgcatttggctcaggtttcactaaccaaatctgtgagcaagttaacctccttaaagaatctctgatagggcaggattccatattggaaaaatccctgaaggccctggttaaaatcatatcagccctggtgatagtggttaggaaccacgacgacctgattacagtgactgccacactagctttaatcggttgcgcatcatctccatggcgatggctcaaacaaaaagtgtgtcaatactacggaatccccatggcagaaaggcagaataacggttggttaaagaaattcactgaaatgaccaacgcctgcaagggcatggagtggattgctgttaaaattcaaaagttcatcgagtggctcaaagtaaagattctgcctgaagtgaaggagaaacatgagttccttaccagattgaagcaattgccactccttgaaagtcaaattgccaccattgagcaaagcgcaccctcacaaagtgatcaagagcagcttttttcgaatgttcagtacttcgcccattactgcaggaagtatgcacctctgtatgctgccgaagcaaaaagagtgttctcattagaaaagaaaatgagtaattacatacagttcaagtccaaatgccgcattgagcctgtatgcttactccttcacggtagtccaggggctggcaagtcagtagctaccaacctgatagggagatcccttgcagagaagctcaatagctctgtgtactctttaccaccagatccagatcattttgatgggtacaaacagcaggcagtggtgatcatggatgatctctgtcaaaaccccgatgggaaggacgtgtccttgttttgccaaatggtgtctagtgtagattttgtgccacccatggcggcgctggaagaaaaaggcattctctttacgtccccgtttgtgttggcatcaaccaacgcggggtccatcaatgcaccaacagtgtcagacagcagagcacttgccagaaggtttcactttgacatgaatattgaggtgatttcgatgtacagccagaatggtaaaattaacatgcccatgtctgttaagacatgtgatgatgaatgctgcccggtcaatttcaaaaagtgttgcccactagtgtgtggcaaggccatccagtttattgacaggagaaaccaagttagatattcactggacatgctggttactgagatgtttagagagtacaaccacagacacagtgtgggtgctaccctcgaggctttgttccaaggaccaccagtatacagggaaatcaaaatcagtgtggccccggaaacaccccctccaccagcaattgctgaccttctaaaatctgtagacagtgaggcaataagggagtactgcaaggaaaggggttggcttgtgccagaggtcagctccactctacaaattgaaaaacatgttagcagggcatttatttgcttgcaagcgctaactacatttgtttcagtggctggtataatctacatcatttacaagttgtttgccggctttcagggtgcatacactggaatgcccaaccagaaacccaaggtgcccaccttaagacaagctaaggtgcaaggtccggcatttgaatttgccgtagcaatgatgaaaaggaacgccagcacagtcaagacagaatacggtgagttcacgatgcttggcatctatgataaatgggcagtgctgccgcgccacgccaagcctggaccaactattttaatgaatgatcaggaggttggtgtgctcgatgccaaagagttagttgataaagacggaaccaacctggagctgacactattgaagcttaaccgcaatgaaaagttcagagacatcagaggttttcttgcaagggaagaagttgaggtaagtgaggctgttttggcaataaacacgagcaagttcccaagcatgtacatccctgtgggccaagtcaccgattacggatttttaaatctaggtggcaccccaacaaagagaatgctcatgtacaacttccctaccagagcgggacagtgtggtggtgtccttatgtcaacaggaaaggtccttggcatacacgtgggaggaaatggtcaccaaggcttctctgctgctctcctcagacactacttcaacgaggaacagggcgaaatagagtttattgagagctctaaagatgcaggatttcctgtgatcaacacccctaataaaaccaaactggaaccaagtgtgtttcatcaggtttttgagggcaacaaagaaccagcagtcctaagaaacggagacccgcgacttaaagccaactttgaggaagcgatattttccaagtacatcggaaatgtgaacacacatgtggacgagtacatgatagaagctgttgatcactacgctggacagctggcaactctggacatcagtacagaacctatgaagcttgaggatgctgtttatggcactgaaggcttggaagcattggacttgaccactagcgcaggatatccttatgtcgccttgggcatcaagaaaagggatatcctctccaagaagactaaagatctcaccaagctgagggaatgcatggacaagtatggtctaaatctgccgatggtgacctacgtgaaggatgaactcaggtccgctgagaaagtagccaagggaaaatccagacttatagaagcttctagtctcaatgactcagtggccatgaggcagacatttgggaacctatacaagacattccacctcaacccaggcattgtcactggtagtgctgttgggtgcgacccagatgtgttttggagcaaaatacccgtgatgcttgacgggcaccttatagcttttgattactctggctacgacgctagcttgagcccagtgtggtttgcttgtttgaaactcctcctagggaaactagggtatactcataaggaaaccaattacatagactacctctgcaactcccatcacttatacagagataaacactatttcgtgaggggtggtatgccatcaggatgttcaggcaccagtatattcaacaccatgatcaacaacatcattattaggacccttatgctaaaggtctacaaaggtattgacctggatcagtttagaatgatcgcttacggggacgatgtgatagcctcttacccgtggcctattgatgcctcactactagcagaagcgggaaaggattatggtttgatcatgaccccagcagataaaggagagtgttttaatgaggtaacctggacaaatgtaaccttcttgaaaaggtactttagagctgatgaacaatatccattcttggtgcaccccgtgatgcccatgaaagacatacacgaatccattagatggaccaaagacccaaagaacactcaagatcatgtgcgctcgttatgcctattggcttggcacaatggggagcacgaatatgaggaatttatccgaaagatcagaagcgtgcctgttggacgctgtttgaccctcccggtgttctcaacactacgcaggaaatggttagattccttctaaaattagagtgcaatcaatgaactatgattggcttaaccctaccgcatgaaccgaactagacaaaagtgcggtaggggtaaattctccgcattcggtgcggaaaaaaaaaaaaaaaaaaaaaaaaaaaaaaaaaaaaaaaaaaaaaaaaaa

SEQ ID NO: 138 - DNA, 8392 bp, synthetic construct
  source 1..8392: mol_type = other DNA
  misc_feature 1..8392: note = H3N2_H3N8 DNA vector construct
ttaaaacagcctgtgggttgtacccacccacagggcccactgggcgctagcactctggtatcacggtacctttgtgtgcctgttttatatcccctttccccgattgtaacttagaagatgtacacactgatcaatagcgggcatagcacaccagctatgtcttgatcaagcactcctgtatccccggaccaagtatcaatagactgctcacgcggttgaaggagaaaacgttcgtcacccggctaactacttcgagaaacccagtagtatcatgaaagttgcgaggcgtttcgttcagcacacccccagtgtagatcgggtcgatgagtcaccgcatcccccacgggcgaccgtggcggtggctgcgctggcggcctgcctacggggcaacccgtaggacgcttcaatacagacatggtgcgaagagtcgattgagctagttagtagtcctccggcccctgaatgcggctaatcctaactgcggagcacatgccctcaacccagggggtattgtgtcgtaacgggcaactctgcagcggaaccgactactttgggtgtccgtgtttccttttatccttatactggctgcttatggtgacaattgaaagattgttgccatatagctattggattggccatccagtgtctaatagagctgttatttacctctttgttggatttataccactcaacctaaaagaagttaaaacactacagctcattttacaactgaatacagcaaaccaccatgaaaaccgtgatcgccctcagttacatcttctgcctcgcctttggacagaatctcctcggaaacgaaaacaacgctgccacactctgcctgggacaccacgccgtgcccaacggcacaatggtgaagaccatcaccgacgatcagatcgaggtgaccaatgccaccgagctggtgcagaacagctccaccggcaaaatctgcaacaatccccacaagatcctggacggcagggattgcaccctgatcgacgctctgctgggcgaccctcactgcgacgtgttccagaatgagacatgggatctgttcgtggagaggagcaatgccttctccaactgctacccctacgacgtgcctgattacgccagcctgcggtccatcgtggccagctccggcaccctggagttcatcaccgagggcttcacctgggctggagtgacccagaacggaggcagcggagcttgcaagaggggacccgccaatagcttcttctcccggctgaactggctgaccaagtccggcaatacctaccccgtgctgaacgtgaccatgcctaacaataacaatttcgacaagctgtacatctggggcgtgcaccaccctagcaccgatcaggagcagaccagcctgtacatccaggcctccggcagggtgaccgtgagcaccaggcggtcccagcagaccatcatccccaacatcggctccaggcctctggtgcggggacagagcggccggatctccgtgtactggaccatcgtgaagcccggcgacatcctggtcatcaacagcaatggcaacctgatcgcccctcgcggctacttcaagatgcacatcggcaagagcagcatcatgagatccgacgcccccatcgatacctgcatcagcgagtgcatcacccctaatggctccatccccaacgagaagcctttccagaatgtgaacaagatcacctacggcgcctgccccaagtacgtgaagcagaataccctgaagctggccaccggcatgcgcaacgtgcctgagagacagaccgtgggcctgttcggagctatcgctggcttcatcgagaatggctgggagggcatggtggacggctggtacggcttccgccaccagaacagcgagggcaccggacaggctgccgacctgaagtccacccaggccgccatcgatcagatcaatggcaagctgaacagagtgatcgagaagaccaacgagaagttccaccagatcgagaaggagttcagcgaggtggagggacgcatccaggacctggagaggtacgtggaggacaccaagatcgatctgtggagctacaatgccgagctgctggtggccctggagaatcagaacaccatcgacctgaccgattccgagatgaacaagctgttcgagaagacccgcagacagctgcgcgagaatgccgaggacatgggcaacggctgcttcaaaatctaccacaagtgcgataacgcctgcatcgagagcatcagaaatggcacctacgaccacaacatctaccgcgatgaggccgtgaacaatagattccagatcaagggcgtggagctgaagtccggctacaaggactggattctgtggatcagcttcgccatctcctgcttcctgctgtgcgtggtgctgctggggtttattatgtgggcttgtcagagggggaacatcaggtgtaacatttgtattctcgaggctttgttccaaggaccaccagtatacaggatgaaaacaactattatcctcatcctgctcactcactgggcttactctcagaaccctatctccggcaacaacaccgctacactgtgcctgggacaccacgctgtggctaatggcaccctggtgaagaccatgtccgacgatcagatcgaggtgaccaacgccaccgagctggtgcagagcatcagcatgggcaaaatctgcaataagagctaccgcgtgctggacggcagaaactgcaccctgatcgatgctatgctgggcgacccccagtgcgatgctttccagtacgagtcctgggacctgttcatcgagaggagcaatgccttcagcaactgctacccctacgacatccctgattacgccagcctgagatccatcgtggccagctccggcaccgtggagttcaccgctgagggcttcacctggaccggagtgacccagaatggcaggtccggagcttgcaagaggggcagcgccgactccttcttcagcaggctgaactggctgaccaagagcggcagctcctaccccaccctgaatgtgaccatgcctaacaataagaacttcgataagctgtacatctggggcatccaccaccccagctccaaccaggagcagaccaagctgtacatccaggagtccggccgcgtgaccgtgtccaccaagagaagccagcagaccatcatcccccacatcggcagccgccctctgatcagaggacagtccggccggatcagcatctactggaccatcgtgaagcccggcgacatcctgatgatcaacagcaatggcaacctggtggcccccaggggctacttcaagctgaaccctggcaagagcagcgtgatccggtccgacgtgcctatcgacatctgcgtgagcgagtgcatcacccccaatggcagcatctccaacgataagcctttccagaatgtgaacaaggtgacctacggcaagtgccccaagtacatccgccagaataccctgaagctggccaccggcatgagaaacgtgcctgagaagcagaccgtgggaatcttcggagctatcgctggcttcatcgagaatggctgggagggcatggtggacggctggtacggcttccgctaccagaactccgagggcaccggacaggctgccgacctgaagagcacccaggccgccatcgatcagatcaatggcaagctgaaccgcgtgatcgagcggaccaacgagaagttccaccagatcgagaaggagttctccgaggtggagggcagaatccaggatctggagaagtacgtggaggacaccaagatcgatctgtggagctacaatgccgagctgctggtggccctggagaaccagcacaccatcgacctgaccgatgccgagatgaataagctgttcgagaagaccaggcggcagctgagggagaatgccgaggacatgggcaacggctgcttcaaaatctaccacaagtgcgataacgcctgcatcgagtccatccggaccggcacctacgaccactacatctacagggatgaggccatcaacaatcggttccagatcaagggcgtggagctgaagagcggctacaaggactggattctgtggatctccttcgccatcagctgcttcctgatctgcgtggtgctcctcgggttcattatgtgggcttgccagaagggaaacattcgctgtaacatttgtatcaactttgagccaacaggggtgacggagtcccgcactgaaattacggcaatgcagaccaccggttcatgtgggcaacaatcaggagctgtgtacgtgggcaattacaggattgtaaacagacacctggcaacgagccacgattggcaaaattgcgtgtgggaggactacaacagggatctcctggtcagcacaacaactgctcatggttgtgatactatagcacggtgccaatgtactgctggcgtgtacttttgtgcatctagaaacaagcactacccagtgagcttcgagggtccaggtctagtgaaagttcaggagggcgagtactaccccgagagataccagtcgcacgtactccttgcagttggattttcagaaccgggtgattgtggaggtattttgaggtgtgaacatggagtcattgggctcgttaccatgggtggtgagggtgtagtaggcttcgctgacgtgcgggatcttttgtggttggaagacgacgccatggagcagggtgttagagattatgtagagcaactgggaaatgcatttggctcaggtttcactaaccaaatctgtgagcaagttaacctccttaaagaatctctgatagggcaggattccatattggaaaaatccctgaaggccctggttaaaatcatatcagccctggtgatagtggttaggaaccacgacgacctgattacagtgactgccacactagctttaatcggttgcgcatcatctccatggcgatggctcaaacaaaaagtgtgtcaatactacggaatccccatggcagaaaggcagaataacggttggttaaagaaattcactgaaatgaccaacgcctgcaagggcatggagtggattgctgttaaaattcaaaagttcatcgagtggctcaaagtaaagattctgcctgaagtgaaggagaaacatgagttccttaccagattgaagcaattgccactccttgaaagtcaaattgccaccattgagcaaagcgcaccctcacaaagtgatcaagagcagcttttttcgaatgttcagtacttcgcccattactgcaggaagtatgcacctctgtatgctgccgaagcaaaaagagtgttctcattagaaaagaaaatgagtaattacatacagttcaagtccaaatgccgcattgagcctgtatgcttactccttcacggtagtccaggggctggcaagtcagtagctaccaacctgatagggagatcccttgcagagaagctcaatagctctgtgtactctttaccaccagatccagatcattttgatgggtacaaacagcaggcagtggtgatcatggatgatctctgtcaaaaccccgatgggaaggacgtgtccttgttttgccaaatggtgtctagtgtagattttgtgccacccatggcggcgctggaagaaaaaggcattctctttacgtccccgtttgtgttggcatcaaccaacgcggggtccatcaatgcaccaacagtgtcagacagcagagcacttgccagaaggtttcactttgacatgaatattgaggtgatttcgatgtacagccagaatggtaaaattaacatgcccatgtctgttaagacatgtgatgatgaatgctgcccggtcaatttcaaaaagtgttgcccactagtgtgtggcaaggccatccagtttattgacaggagaaaccaagttagatattcactggacatgctggttactgagatgtttagagagtacaaccacagacacagtgtgggtgctaccctcgaggctttgttccaaggaccaccagtatacagggaaatcaaaatcagtgtggccccggaaacaccccctccaccagcaattgctgaccttctaaaatctgtagacagtgaggcaataagggagtactgcaaggaaaggggttggcttgtgccagaggtcagctccactctacaaattgaaaaacatgttagcagggcatttatttgcttgcaagcgctaactacatttgtttcagtggctggtataatctacatcatttacaagttgtttgccggctttcagggtgcatacactggaatgcccaaccagaaacccaaggtgcccaccttaagacaagctaaggtgcaaggtccggcatttgaatttgccgtagcaatgatgaaaaggaacgccagcacagtcaagacagaatacggtgagttcacgatgcttggcatctatgataaatgggcagtgctgccgcgccacgccaagcctggaccaactattttaatgaatgatcaggaggttggtgtgctcgatgccaaagagttagttgataaagacggaaccaacctggagctgacactattgaagcttaaccgcaatgaaaagttcagagacatcagaggttttcttgcaagggaagaagttgaggtaagtgaggctgttttggcaataaacacgagcaagttcccaagcatgtacatccctgtgggccaagtcaccgattacggatttttaaatctaggtggcaccccaacaaagagaatgctcatgtacaacttccctaccagagcgggacagtgtggtggtgtccttatgtcaacaggaaaggtccttggcatacacgtgggaggaaatggtcaccaaggcttctctgctgctctcctcagacactacttcaacgaggaacagggcgaaatagagtttattgagagctctaaagatgcaggatttcctgtgatcaacacccctaataaaaccaaactggaaccaagtgtgtttcatcaggtttttgagggcaacaaagaaccagcagtcctaagaaacggagacccgcgacttaaagccaactttgaggaagcgatattttccaagtacatcggaaatgtgaacacacatgtggacgagtacatgatagaagctgttgatcactacgctggacagctggcaactctggacatcagtacagaacctatgaagcttgaggatgctgtttatggcactgaaggcttggaagcattggacttgaccactagcgcaggatatccttatgtcgccttgggcatcaagaaaagggatatcctctccaagaagactaaagatctcaccaagctgagggaatgcatggacaagtatggtctaaatctgccgatggtgacctacgtgaaggatgaactcaggtccgctgagaaagtagccaagggaaaatccagacttatagaagcttctagtctcaatgactcagtggccatgaggcagacatttgggaacctatacaagacattccacctcaacccaggcattgtcactggtagtgctgttgggtgcgacccagatgtgttttggagcaaaatacccgtgatgcttgacgggcaccttatagcttttgattactctggctacgacgctagcttgagcccagtgtggtttgcttgtttgaaactcctcctagggaaactagggtatactcataaggaaaccaattacatagactacctctgcaactcccatcacttatacagagataaacactatttcgtgaggggtggtatgccatcaggatgttcaggcaccagtatattcaacaccatgatcaacaacatcattattaggacccttatgctaaaggtctacaaaggtattgacctggatcagtttagaatgatcgcttacggggacgatgtgatagcctcttacccgtggcctattgatgcctcactactagcagaagcgggaaaggattatggtttgatcatgaccccagcagataaaggagagtgttttaatgaggtaacctggacaaatgtaaccttcttgaaaaggtactttagagctgatgaacaatatccattcttggtgcaccccgtgatgcccatgaaagacatacacgaatccattagatggaccaaagacccaaagaacactcaagatcatgtgcgctcgttatgcctattggcttggcacaatggggagcacgaatatgaggaatttatccgaaagatcagaagcgtgcctgttggacgctgtttgaccctcccggtgttctcaacactacgcaggaaatggttagattccttctaaaattagagtgcaatcaatgaactatgattggcttaaccctaccgcatgaaccgaactagacaaaagtgcggtaggggtaaattctccgcattcggtgcggaaaaaaaaaaaaaaaaaaaaaaaaaaaaaaaaaaaaaaaaaaaaaaaaaa

SEQ ID NO: 139 - protein, 271 aa, synthetic construct
  REGION 1..271: note = human papilloma virus E6_E7 domain antigen
MHQKRTAMFQDPQERPRKLPQLCTELQTTIHDIILECVYCKQQLLRREVYDFAFRDLCIVYRDGNPYAVCDKCLKFYSKISEYRHYCYSLYGTTLEQQYNKPLCDLLIRCINCQKPLCPEEKQRHLDKKQRFHNIRGRWTGRCMSCCRSSRTRRETQLGGGGSGGGGSGGGGSMHGDTPTLHEYMLDLQPETTDLYCYEQLNDSSEEEDEIDGPAGQAEPDRAHYNIVTFCCKCDSTLRLCVQSTHVDIRTLEDLLMGTLGIVCPICSQKP

SEQ ID NO: 140 - RNA, 813 nt, synthetic construct
  source 1..813: mol_type = other RNA
  misc_feature 1..813: note = human papilloma virus E6_E7 domain antigen
atgcaccagaaaagaaccgccatgttccaggacccccaggagcggcctagaaagctgcctcagctgtgcaccgagctgcagaccaccatccacgacatcatcctggaatgcgtgtattgtaaacaacagctcctgagaagagaagtctacgacttcgcttttagagacctgtgcatcgtgtaccgggacggcaatccttacgccgtgtgcgataagtgcctgaagttctacagcaagatcagcgagtacagacactactgctactctctgtacggcacaaccctggaacagcagtacaacaagccactgtgtgatctgctgatccggtgcattaactgccagaagcccctgtgtcctgaggaaaagcaaaggcatctggacaagaagcagagattccacaacatcagaggcagatggacaggaagatgtatgagctgctgccgctccagccggaccagaagagagacacagctgggtggaggcggttcaggcggaggtggctctggcggtggcggatcaatgcacggcgacacccctaccctgcacgagtacatgctggacctgcaacctgagacaacagacctgtattgttacgagcagctgaacgactccagcgaggaagaagatgagatcgacggacctgctggccaggccgagccagatagagcccactacaacatcgtgaccttctgctgcaagtgcgactctacactcagactgtgtgtgcagagcacccatgtggacatccggaccctggaggacctgctgatgggcaccctgggcatcgtctgccccatctgcagccagaagccc

SEQ ID NO: 141 - DNA, 813 bp, synthetic construct
  source 1..813: mol_type = other DNA
  misc_feature 1..813: note = human papilloma virus E6_E7 domain antigen
atgcaccagaaaagaaccgccatgttccaggacccccaggagcggcctagaaagctgcctcagctgtgcaccgagctgcagaccaccatccacgacatcatcctggaatgcgtgtattgtaaacaacagctcctgagaagagaagtctacgacttcgcttttagagacctgtgcatcgtgtaccgggacggcaatccttacgccgtgtgcgataagtgcctgaagttctacagcaagatcagcgagtacagacactactgctactctctgtacggcacaaccctggaacagcagtacaacaagccactgtgtgatctgctgatccggtgcattaactgccagaagcccctgtgtcctgaggaaaagcaaaggcatctggacaagaagcagagattccacaacatcagaggcagatggacaggaagatgtatgagctgctgccgctccagccggaccagaagagagacacagctgggtggaggcggttcaggcggaggtggctctggcggtggcggatcaatgcacggcgacacccctaccctgcacgagtacatgctggacctgcaacctgagacaacagacctgtattgttacgagcagctgaacgactccagcgaggaagaagatgagatcgacggacctgctggccaggccgagccagatagagcccactacaacatcgtgaccttctgctgcaagtgcgactctacactcagactgtgtgtgcagagcacccatgtggacatccggaccctggaggacctgctgatgggcaccctgggcatcgtctgccccatctgcagccagaagccc

SEQ ID NO: 142 - protein, 424 aa, synthetic construct
  REGION 1..424: note = human papilloma virus continuous antigen
MKLPQLCTELQTTIHDIILECVYCKQQTTIHDIILECVYCKQQLLRREVYDFAFRDLCIVYQQLLRREVYDFAFRDLCIVYRDGNPYAVCEVYDFAFRDLCIVYRDGNPYAVCDKCLKFYSKPYAVCDKCLKFYSKISEYRHYCYSLYGEYRHYCYSLYGTTLEQQYNKPLCDLLIRCINCQKPLCPEEKNKPLCDLLIRCINCQKPLCPEEKQRHLDKKQRFHNIRGRWTGRCLDKKQRFHNIRGRWTGRCMSCCRSSRTPTLHEYMLDLQPETTDHEYMLDLQPETTDLYCYEQLNDSSECYEQLNDSSEEEDEIDGPAGQADEIDGPAGQAEPDRAHYNIVTFCCKCDSTPDRAHYNIVTFCCKCDSTLRLCVLRLCVQSTHVDIRTLEDLLMGTLGTHVDIRTLEDLLMGTLGIVCPICS

SEQ ID NO: 143 - RNA, 1272 nt, synthetic construct
  source 1..1272: mol_type = other RNA
  misc_feature 1..1272: note = human papilloma virus continuous antigen
atgaagctgcctcagctgtgcaccgagctgcagaccaccatccacgacatcatcctggaatgcgtgtattgtaaacaacagaccaccatccacgacatcatcctggaatgcgtgtattgtaaacaacagctcctgagaagagaagtctacgacttcgcttttagagacctgtgcatcgtgtaccaacagctcctgagaagagaagtctacgacttcgcttttagagacctgtgcatcgtgtaccgggacggcaatccttacgccgtgtgcgaagtctacgacttcgcttttagagacctgtgcatcgtgtaccgggacggcaatccttacgccgtgtgcgataagtgcctgaagttctacagcaagccttacgccgtgtgcgataagtgcctgaagttctacagcaagatcagcgagtacagacactactgctactctctgtacggcgagtacagacactactgctactctctgtacggcacaaccctggaacagcagtacaacaagccactgtgtgatctgctgatccggtgcattaactgccagaagcccctgtgtcctgaggaaaagaacaagccactgtgtgatctgctgatccggtgcattaactgccagaagcccctgtgtcctgaggaaaagcaaaggcatctggacaagaagcagagattccacaacatcagaggcagatggacaggaagatgtctggacaagaagcagagattccacaacatcagaggcagatggacaggaagatgtatgagctgctgccgctccagccggacccctaccctgcacgagtacatgctggacctgcaacctgagacaacagaccacgagtacatgctggacctgcaacctgagacaacagacctgtattgttacgagcagctgaacgactccagcgagtgttacgagcagctgaacgactccagcgaggaagaagatgagatcgacggacctgctggccaggccgatgagatcgacggacctgctggccaggccgagccagatagagcccactacaacatcgtgaccttctgctgcaagtgcgactctacaccagatagagcccactacaacatcgtgaccttctgctgcaagtgcgactctacactcagactgtgtgtgctcagactgtgtgtgcagagcacccatgtggacatccggaccctggaggacctgctgatgggcaccctgggcacccatgtggacatccggaccctggaggacctgctgatgggcaccctgggcatcgtctgccccatctgcagc

SEQ ID NO: 144 - DNA, 1272 bp, synthetic construct
  source 1..1272: mol_type = other DNA
  misc_feature 1..1272: note = human papilloma virus continuous antigen
atgaagctgcctcagctgtgcaccgagctgcagaccaccatccacgacatcatcctggaatgcgtgtattgtaaacaacagaccaccatccacgacatcatcctggaatgcgtgtattgtaaacaacagctcctgagaagagaagtctacgacttcgcttttagagacctgtgcatcgtgtaccaacagctcctgagaagagaagtctacgacttcgcttttagagacctgtgcatcgtgtaccgggacggcaatccttacgccgtgtgcgaagtctacgacttcgcttttagagacctgtgcatcgtgtaccgggacggcaatccttacgccgtgtgcgataagtgcctgaagttctacagcaagccttacgccgtgtgcgataagtgcctgaagttctacagcaagatcagcgagtacagacactactgctactctctgtacggcgagtacagacactactgctactctctgtacggcacaaccctggaacagcagtacaacaagccactgtgtgatctgctgatccggtgcattaactgccagaagcccctgtgtcctgaggaaaagaacaagccactgtgtgatctgctgatccggtgcattaactgccagaagcccctgtgtcctgaggaaaagcaaaggcatctggacaagaagcagagattccacaacatcagaggcagatggacaggaagatgtctggacaagaagcagagattccacaacatcagaggcagatggacaggaagatgtatgagctgctgccgctccagccggacccctaccctgcacgagtacatgctggacctgcaacctgagacaacagaccacgagtacatgctggacctgcaacctgagacaacagacctgtattgttacgagcagctgaacgactccagcgagtgttacgagcagctgaacgactccagcgaggaagaagatgagatcgacggacctgctggccaggccgatgagatcgacggacctgctggccaggccgagccagatagagcccactacaacatcgtgaccttctgctgcaagtgcgactctacaccagatagagcccactacaacatcgtgaccttctgctgcaagtgcgactctacactcagactgtgtgtgctcagactgtgtgtgcagagcacccatgtggacatccggaccctggaggacctgctgatgggcaccctgggcacccatgtggacatccggaccctggaggacctgctgatgggcaccctgggcatcgtctgccccatctgcagc

SEQ ID NO: 145 - protein, 424 aa, synthetic construct
  REGION 1..424: note = human papilloma cross over antigen
MKLPQLCTELQTTIHDIILECVYCKQQTPTLHEYMLDLQPETTDTTIHDIILECVYCKQQLLRREVYDFAFRDLCIVYHEYMLDLQPETTDLYCYEQLNDSSEQQLLRREVYDFAFRDLCIVYRDGNPYAVCCYEQLNDSSEEEDEIDGPAGQAEVYDFAFRDLCIVYRDGNPYAVCDKCLKFYSKDEIDGPAGQAEPDRAHYNIVTFCCKCDSTPYAVCDKCLKFYSKISEYRHYCYSLYGPDRAHYNIVTFCCKCDSTLRLCVEYRHYCYSLYGTTLEQQYNKPLCDLLIRCINCQKPLCPEEKLRLCVQSTHVDIRTLEDLLMGTLGNKPLCDLLIRCINCQKPLCPEEKQRHLDKKQRFHNIRGRWTGRCTHVDIRTLEDLLMGTLGIVCPICSLDKKQRFHNIRGRWTGRCMSCCRSSR

SEQ ID NO: 146 - RNA, 1272 nt, synthetic construct
  source 1..1272: mol_type = other RNA
  misc_feature 1..1272: note = human papilloma cross over antigen
atgaagctgcctcagctgtgcaccgagctgcagaccaccatccacgacatcatcctggaatgcgtgtattgtaaacaacagacccctaccctgcacgagtacatgctggacctgcaacctgagacaacagacaccaccatccacgacatcatcctggaatgcgtgtattgtaaacaacagctcctgagaagagaagtctacgacttcgcttttagagacctgtgcatcgtgtaccacgagtacatgctggacctgcaacctgagacaacagacctgtattgttacgagcagctgaacgactccagcgagcaacagctcctgagaagagaagtctacgacttcgcttttagagacctgtgcatcgtgtaccgggacggcaatccttacgccgtgtgctgttacgagcagctgaacgactccagcgaggaagaagatgagatcgacggacctgctggccaggccgaagtctacgacttcgcttttagagacctgtgcatcgtgtaccgggacggcaatccttacgccgtgtgcgataagtgcctgaagttctacagcaaggatgagatcgacggacctgctggccaggccgagccagatagagcccactacaacatcgtgaccttctgctgcaagtgcgactctacaccttacgccgtgtgcgataagtgcctgaagttctacagcaagatcagcgagtacagacactactgctactctctgtacggcccagatagagcccactacaacatcgtgaccttctgctgcaagtgcgactctacactcagactgtgtgtggagtacagacactactgctactctctgtacggcacaaccctggaacagcagtacaacaagccactgtgtgatctgctgatccggtgcattaactgccagaagcccctgtgtcctgaggaaaagctcagactgtgtgtgcagagcacccatgtggacatccggaccctggaggacctgctgatgggcaccctgggcaacaagccactgtgtgatctgctgatccggtgcattaactgccagaagcccctgtgtcctgaggaaaagcaaaggcatctggacaagaagcagagattccacaacatcagaggcagatggacaggaagatgtacccatgtggacatccggaccctggaggacctgctgatgggcaccctgggcatcgtctgccccatctgcagcctggacaagaagcagagattccacaacatcagaggcagatggacaggaagatgtatgagctgctgccgctccagccgg

SEQ ID NO: 147 - DNA, 1272 bp, synthetic construct
  source 1..1272: mol_type = other DNA
  misc_feature 1..1272: note = human papilloma cross over antigen
atgaagctgcctcagctgtgcaccgagctgcagaccaccatccacgacatcatcctggaatgcgtgtattgtaaacaacagacccctaccctgcacgagtacatgctggacctgcaacctgagacaacagacaccaccatccacgacatcatcctggaatgcgtgtattgtaaacaacagctcctgagaagagaagtctacgacttcgcttttagagacctgtgcatcgtgtaccacgagtacatgctggacctgcaacctgagacaacagacctgtattgttacgagcagctgaacgactccagcgagcaacagctcctgagaagagaagtctacgacttcgcttttagagacctgtgcatcgtgtaccgggacggcaatccttacgccgtgtgctgttacgagcagctgaacgactccagcgaggaagaagatgagatcgacggacctgctggccaggccgaagtctacgacttcgcttttagagacctgtgcatcgtgtaccgggacggcaatccttacgccgtgtgcgataagtgcctgaagttctacagcaaggatgagatcgacggacctgctggccaggccgagccagatagagcccactacaacatcgtgaccttctgctgcaagtgcgactctacaccttacgccgtgtgcgataagtgcctgaagttctacagcaagatcagcgagtacagacactactgctactctctgtacggcccagatagagcccactacaacatcgtgaccttctgctgcaagtgcgactctacactcagactgtgtgtggagtacagacactactgctactctctgtacggcacaaccctggaacagcagtacaacaagccactgtgtgatctgctgatccggtgcattaactgccagaagcccctgtgtcctgaggaaaagctcagactgtgtgtgcagagcacccatgtggacatccggaccctggaggacctgctgatgggcaccctgggcaacaagccactgtgtgatctgctgatccggtgcattaactgccagaagcccctgtgtcctgaggaaaagcaaaggcatctggacaagaagcagagattccacaacatcagaggcagatggacaggaagatgtacccatgtggacatccggaccctggaggacctgctgatgggcaccctgggcatcgtctgccccatctgcagcctggacaagaagcagagattccacaacatcagaggcagatggacaggaagatgtatgagctgctgccgctccagccgg

SEQ ID NO: 148 - protein, 424 aa, synthetic construct
  REGION 1..424: note = human papilloma Odd-Even antigen
MKLPQLCTELQTTIHDIILECVYCKQQQQLLRREVYDFAFRDLCIVYRDGNPYAVCPYAVCDKCLKFYSKISEYRHYCYSLYGNKPLCDLLIRCINCQKPLCPEEKQRHLDKKQRFHNIRGRWTGRCTTIHDIILECVYCKQQLLRREVYDFAFRDLCIVYEVYDFAFRDLCIVYRDGNPYAVCDKCLKFYSKEYRHYCYSLYGTTLEQQYNKPLCDLLIRCINCQKPLCPEEKLDKKQRFHNIRGRWTGRCMSCCRSSRTPTLHEYMLDLQPETTDCYEQLNDSSEEEDEIDGPAGQAPDRAHYNIVTFCCKCDSTLRLCVTHVDIRTLEDLLMGTLGIVCPICSHEYMLDLQPETTDLYCYEQLNDSSEDEIDGPAGQAEPDRAHYNIVTFCCKCDSTLRLCVQSTHVDIRTLEDLLMGTLG

SEQ ID NO: 149 - RNA, 1272 nt, synthetic construct
  source 1..1272: mol_type = other RNA
  misc_feature 1..1272: note = human papilloma Odd-Even antigen
atgaagctgcctcagctgtgcaccgagctgcagaccaccatccacgacatcatcctggaatgcgtgtattgtaaacaacagcaacagctcctgagaagagaagtctacgacttcgcttttagagacctgtgcatcgtgtaccgggacggcaatccttacgccgtgtgcccttacgccgtgtgcgataagtgcctgaagttctacagcaagatcagcgagtacagacactactgctactctctgtacggcaacaagccactgtgtgatctgctgatccggtgcattaactgccagaagcccctgtgtcctgaggaaaagcaaaggcatctggacaagaagcagagattccacaacatcagaggcagatggacaggaagatgtaccaccatccacgacatcatcctggaatgcgtgtattgtaaacaacagctcctgagaagagaagtctacgacttcgcttttagagacctgtgcatcgtgtacgaagtctacgacttcgcttttagagacctgtgcatcgtgtaccgggacggcaatccttacgccgtgtgcgataagtgcctgaagttctacagcaaggagtacagacactactgctactctctgtacggcacaaccctggaacagcagtacaacaagccactgtgtgatctgctgatccggtgcattaactgccagaagcccctgtgtcctgaggaaaagctggacaagaagcagagattccacaacatcagaggcagatggacaggaagatgtatgagctgctgccgctccagccggacccctaccctgcacgagtacatgctggacctgcaacctgagacaacagactgttacgagcagctgaacgactccagcgaggaagaagatgagatcgacggacctgctggccaggccccagatagagcccactacaacatcgtgaccttctgctgcaagtgcgactctacactcagactgtgtgtgacccatgtggacatccggaccctggaggacctgctgatgggcaccctgggcatcgtctgccccatctgcagccacgagtacatgctggacctgcaacctgagacaacagacctgtattgttacgagcagctgaacgactccagcgaggatgagatcgacggacctgctggccaggccgagccagatagagcccactacaacatcgtgaccttctgctgcaagtgcgactctacactcagactgtgtgtgcagagcacccatgtggacatccggaccctggaggacctgctgatgggcaccctgggc

SEQ ID NO: 150 - DNA, 1272 bp, synthetic construct
  source 1..1272: mol_type = other DNA
  misc_feature 1..1272: note = human papilloma Odd-Even antigen
atgaagctgcctcagctgtgcaccgagctgcagaccaccatccacgacatcatcctggaatgcgtgtattgtaaacaacagcaacagctcctgagaagagaagtctacgacttcgcttttagagacctgtgcatcgtgtaccgggacggcaatccttacgccgtgtgcccttacgccgtgtgcgataagtgcctgaagttctacagcaagatcagcgagtacagacactactgctactctctgtacggcaacaagccactgtgtgatctgctgatccggtgcattaactgccagaagcccctgtgtcctgaggaaaagcaaaggcatctggacaagaagcagagattccacaacatcagaggcagatggacaggaagatgtaccaccatccacgacatcatcctggaatgcgtgtattgtaaacaacagctcctgagaagagaagtctacgacttcgcttttagagacctgtgcatcgtgtacgaagtctacgacttcgcttttagagacctgtgcatcgtgtaccgggacggcaatccttacgccgtgtgcgataagtgcctgaagttctacagcaaggagtacagacactactgctactctctgtacggcacaaccctggaacagcagtacaacaagccactgtgtgatctgctgatccggtgcattaactgccagaagcccctgtgtcctgaggaaaagctggacaagaagcagagattccacaacatcagaggcagatggacaggaagatgtatgagctgctgccgctccagccggacccctaccctgcacgagtacatgctggacctgcaacctgagacaacagactgttacgagcagctgaacgactccagcgaggaagaagatgagatcgacggacctgctggccaggccccagatagagcccactacaacatcgtgaccttctgctgcaagtgcgactctacactcagactgtgtgtgacccatgtggacatccggaccctggaggacctgctgatgggcaccctgggcatcgtctgccccatctgcagccacgagtacatgctggacctgcaacctgagacaacagacctgtattgttacgagcagctgaacgactccagcgaggatgagatcgacggacctgctggccaggccgagccagatagagcccactacaacatcgtgaccttctgctgcaagtgcgactctacactcagactgtgtgtgcagagcacccatgtggacatccggaccctggaggacctgctgatgggcaccctgggc

SEQ ID NO: 151 - RNA, 5852 nt, synthetic construct
  source 1..5852: mol_type = other RNA
  misc_feature 1..5852: note = G1 saRNA construct
ttaaaacagcctgtgggttgtacccacccacagggcccactgggcgctagcactctggtatcacggtacctttgtgtgcctgttttatatcccctttccccgattgtaacttagaagatgtacacactgatcaatagcgggcatagcacaccagctatgtcttgatcaagcactcctgtatccccggaccaagtatcaatagactgctcacgcggttgaaggagaaaacgttcgttacccggctaactacttcgagaaacccagtagtatcatgaaagttgcgaggcgtttcgttcagcacacccccagtgtagatcgggtcgatgagtcaccgcatcccccacgggcgaccgtggcggtggctgcgctggcggcctgcctacggggcaacccgtaggacgcttcaatacagacatggtgcgaagagtcgattgagctagttagtagtcctccggcccctgaatgcggctaatcctaactgcggagcacatgccctcaacccagggggtattgtgtcgtaacgggcaactctgcagcggaaccgactactttgggtgtccgtgtttccttttatccttatactggctgcttatggtgacaattgaaagattgttgccatatagctattggattggccatccagtgtctaatagagctgttatttacctctttgttggatttataccactcaacctaaaagaagttaaaacactacagctcattttacaactgaatacagcaaaccaccatgcaccagaaaagaaccgccatgttccaggacccccaggagcggcctagaaagctgcctcagctgtgcaccgagctgcagaccaccatccacgacatcatcctggaatgcgtgtattgtaaacaacagctcctgagaagagaagtctacgacttcgcttttagagacctgtgcatcgtgtaccgggacggcaatccttacgccgtgtgcgataagtgcctgaagttctacagcaagatcagcgagtacagacactactgctactctctgtacggcacaaccctggaacagcagtacaacaagccactgtgtgatctgctgatccggtgcattaactgccagaagcccctgtgtcctgaggaaaagcaaaggcatctggacaagaagcagagattccacaacatcagaggcagatggacaggaagatgtatgagctgctgccgctccagccggaccagaagagagacacagctgggtggaggcggttcaggcggaggtggctctggcggtggcggatcaatgcacggcgacacccctaccctgcacgagtacatgctggacctgcaacctgagacaacagacctgtattgttacgagcagctgaacgactccagcgaggaagaagatgagatcgacggacctgctggccaggccgagccagatagagcccactacaacatcgtgaccttctgctgcaagtgcgactctacactcagactgtgtgtgcagagcacccatgtggacatccggaccctggaggacctgctgatgggcaccctgggcatcgtctgccccatctgcagccagaagcccaactttgagccaacaggggtgacggagtcccgcactgaaattacggcaatgcagaccaccggttcatgtgggcaacaatcaggagctgtgtacgtgggcaattacaggattgtaaacagacacctggcaacgagccacgattggcaaaattgcgtgtgggaggactacaacagggatctcctggtcagcacaacaactgctcatggttgtgatactatagcacggtgccaatgtactgctggcgtgtacttttgtgcatctagaaacaagcactacccagtgagcttcgagggtccaggtctagtgaaagttcaggagagcgagtactaccccgagagataccagtcgcacgtactccttgcagttggattttcagaaccgggtgattgtggaggtattttgaggtgtgaacatggagtcattgggctcgttaccatgggtggtgagggtgtagtaggcttcgctgacgtgcgggatcttttgtggttggaagacgacgccatggagcagggtgttagagattatgtagagcaactgggaaatgcatttggctcaggtttcactaaccaaatctgtgagcaagttaacctccttaaagaatctctgatagggcaggattccatattggaaaaatccctgaaggccctggttaaaatcatatcagccctggtgatagtggttaggaaccacgacgacctgattacagtgactgccacactagctttaatcggttgcgcatcatctccatggcgatggctcaaacaaaaagtgtgtcaatactacggaatccccatggcagaaaggcagaataacggttggttaaagaaattcactgaaatgaccaacgcctgcaagggcatggagtggattgctgttaaaattcaaaagttcatcgagtggctcaaagtaaagattctgcctgaagtgaaggagaaacatgagttccttaccagattgaagcaattgccactccttgaaagtcaaattgccaccattgagcaaagcgcaccctcacaaagtgatcaagagcagcttttttcgaatgttcagtacttcgcccattactgcaggaagtatgcacctctgtatgctgccgaagcaaaaagagtgttctcattagaaaagaaaatgagtaattacatacagttcaagtccaaatgccgcattgagcctgtatgcttactccttcacggtagtccaggggctggcaagtcagtagctaccaacctgatagggagatcccttgcagagaagctcaatagctctgtgtactctttaccaccagatccagatcattttgatgggtacaaacagcaggcagtggtgatcatggatgatctctgtcaaaaccccgatgggaaggacgtgtccttgttttgccaaatggtgtctagtgtagattttgtgccacccatggcggcgctggaagaaaaaggcattctctttacgtccccgtttgtgttggcatcaaccaacgcggggtccatcaatgcaccaacagtgtcagacagcagagcacttgccagaaggtttcactttgacatgaatattgaggtgatttcgatgtacagccagaatggtaaaattaacatgcccatgtctgttaagacatgtgatgatgaatgctgcccggtcaatttcaaaaagtgttgcccactagtgtgtggcaaggccatccagtttattgacaggagaaaccaagttagatattcactggacatgctggttactgagatgtttagagagtacaaccacagacacagtgtgggtgctaccctcgaggctttgttccaaggaccaccagtatacagggaaatcaaaatcagtgtggccccggaaacaccccctccaccagcaattgctgaccttctaaaatctgtagacagtgaggcaataagggagtactgcaaggaaaggggttggcttgtgccagaggtcagctccactctacaaattgaaaaacatgttagcagggcatttatttgcttgcaagcgctaactacatttgtttcagtggctggtataatctacatcatttacaagttgtttgccggctttcagggtgcatacactggaatgcccaaccagaaacccaaggtgcccaccttaagacaagctaaggtgcaaggtccggcatttgaatttgccgtagcaatgatgaaaaggaacgccagcacagtcaagacagaatacggtgagttcacgatgcttggcatctatgataaatgggcagtgctgccgcgccacgccaagcctggaccaactattttaatgaatgatcaggaggttggtgtgctcgatgccaaagagttagttgataaagacggaaccaacctggagctgacactattgaagcttaaccgcaatgaaaagttcagagacatcagaggttttcttgcaagggaagaagttgaggtaagtgaggctgttttggcaataaacacgagcaagttcccaagcatgtacatccctgtgggccaagtcaccgattacggatttttaaatctaggtggcaccccaacaaagagaatgctcatgtacaacttccctaccagagcgggacagtgtggtggtgtccttatgtcaacaggaaaggtccttggcatacacgtgggaggaaatggtcaccaaggcttctctgctgctctcctcagacactacttcaacgaggaacagggcgaaatagagtttattgagagctctaaagatgcaggatttcctgtgatcaacacccctaataaaaccaaactggaaccaagtgtgtttcatcaggtttttgagggcaacaaagaaccagcagtcctaagaaacggagacccgcgacttaaagccaactttgaggaagcgatattttccaagtacatcggaaatgtgaacacacatgtggacgagtacatgatagaagctgttgatcactacgctggacagctggcaactctggacatcagtacagaacctatgaagcttgaggatgctgtttatggcactgaaggcttggaagcattggacttgaccactagcgcaggatatccttatgtcgccttgggcatcaagaaaagggatatcctctccaagaagactaaagatctcaccaagctgagggaatgcatggacaagtatggtctaaatctgccgatggtgacctacgtgaaggatgaactcaggtccgctgagaaagtagccaagggaaaatccagacttatagaagcttctagtctcaatgactcagtggccatgaggcagacatttgggaacctatacaagacattccacctcaacccaggcattgtcactggtagtgctgttgggtgcgacccagatgtgttttggagcaaaatacccgtgatgcttgacgggcaccttatagcttttgattactctggctacgacgctagcttgagcccagtgtggtttgcttgtttgaaactcctcctagggaaactagggtatactcataaggaaaccaattacatagactacctctgcaactcccatcacttatacagagataaacactatttcgtgaggggtggtatgccatcaggatgttcaggcaccagtatattcaacaccatgatcaacaacatcattattaggacccttatgctaaaggtctacaaaggtattgacctggatcagtttagaatgatcgcttacggggacgatgtgatagcctcttacccgtggcctattgatgcctcactactagcagaagcgggaaaggattatggtttgatcatgaccccagcagataaaggagagtgttttaatgaggtaacctggacaaatgtaaccttcttgaaaaggtactttagagctgatgaacaatatccattcttggtgcaccccgtgatgcccatgaaagacatacacgaatccattagatggaccaaagacccaaagaacactcaagatcatgtgcgctcgttatgcctattggcttggcacaatggggagcacgaatatgaggaatttatccgaaagatcagaagcgtgcctgttggacgctgtttgaccctcccggtgttctcaacactacgcaggaaatggttagattccttctgataatagaattagagtgcaatcaatgaactatgattggcttaaccctaccgcatgaaccgaactagacaaaagtgcggtaggggtaaattctccgcattcggtgcggaaaaaaaaaaaaaaaaaaaaaaaaaaaaaaaaaaaaaaaaaaaaaaaaaaaaaaaaaaaaaaaaaaaaaaaaaaaaaaaaaaaaaaaaaaaaaaaaaaaaaaaaaaaaaaaaaaaaaaaa

SEQ ID NO: 152 - DNA, 5852 bp, synthetic construct
  source 1..5852: mol_type = other DNA
  misc_feature 1..5852: note = G1 DNA vector construct
ttaaaacagcctgtgggttgtacccacccacagggcccactgggcgctagcactctggtatcacggtacctttgtgtgcctgttttatatcccctttccccgattgtaacttagaagatgtacacactgatcaatagcgggcatagcacaccagctatgtcttgatcaagcactcctgtatccccggaccaagtatcaatagactgctcacgcggttgaaggagaaaacgttcgttacccggctaactacttcgagaaacccagtagtatcatgaaagttgcgaggcgtttcgttcagcacacccccagtgtagatcgggtcgatgagtcaccgcatcccccacgggcgaccgtggcggtggctgcgctggcggcctgcctacggggcaacccgtaggacgcttcaatacagacatggtgcgaagagtcgattgagctagttagtagtcctccggcccctgaatgcggctaatcctaactgcggagcacatgccctcaacccagggggtattgtgtcgtaacgggcaactctgcagcggaaccgactactttgggtgtccgtgtttccttttatccttatactggctgcttatggtgacaattgaaagattgttgccatatagctattggattggccatccagtgtctaatagagctgttatttacctctttgttggatttataccactcaacctaaaagaagttaaaacactacagctcattttacaactgaatacagcaaaccaccatgcaccagaaaagaaccgccatgttccaggacccccaggagcggcctagaaagctgcctcagctgtgcaccgagctgcagaccaccatccacgacatcatcctggaatgcgtgtattgtaaacaacagctcctgagaagagaagtctacgacttcgcttttagagacctgtgcatcgtgtaccgggacggcaatccttacgccgtgtgcgataagtgcctgaagttctacagcaagatcagcgagtacagacactactgctactctctgtacggcacaaccctggaacagcagtacaacaagccactgtgtgatctgctgatccggtgcattaactgccagaagcccctgtgtcctgaggaaaagcaaaggcatctggacaagaagcagagattccacaacatcagaggcagatggacaggaagatgtatgagctgctgccgctccagccggaccagaagagagacacagctgggtggaggcggttcaggcggaggtggctctggcggtggcggatcaatgcacggcgacacccctaccctgcacgagtacatgctggacctgcaacctgagacaacagacctgtattgttacgagcagctgaacgactccagcgaggaagaagatgagatcgacggacctgctggccaggccgagccagatagagcccactacaacatcgtgaccttctgctgcaagtgcgactctacactcagactgtgtgtgcagagcacccatgtggacatccggaccctggaggacctgctgatgggcaccctgggcatcgtctgccccatctgcagccagaagcccaactttgagccaacaggggtgacggagtcccgcactgaaattacggcaatgcagaccaccggttcatgtgggcaacaatcaggagctgtgtacgtgggcaattacaggattgtaaacagacacctggcaacgagccacgattggcaaaattgcgtgtgggaggactacaacagggatctcctggtcagcacaacaactgctcatggttgtgatactatagcacggtgccaatgtactgctggcgtgtacttttgtgcatctagaaacaagcactacccagtgagcttcgagggtccaggtctagtgaaagttcaggagagcgagtactaccccgagagataccagtcgcacgtactccttgcagttggattttcagaaccgggtgattgtggaggtattttgaggtgtgaacatggagtcattgggctcgttaccatgggtggtgagggtgtagtaggcttcgctgacgtgcgggatcttttgtggttggaagacgacgccatggagcagggtgttagagattatgtagagcaactgggaaatgcatttggctcaggtttcactaaccaaatctgtgagcaagttaacctccttaaagaatctctgatagggcaggattccatattggaaaaatccctgaaggccctggttaaaatcatatcagccctggtgatagtggttaggaaccacgacgacctgattacagtgactgccacactagctttaatcggttgcgcatcatctccatggcgatggctcaaacaaaaagtgtgtcaatactacggaatccccatggcagaaaggcagaataacggttggttaaagaaattcactgaaatgaccaacgcctgcaagggcatggagtggattgctgttaaaattcaaaagttcatcgagtggctcaaagtaaagattctgcctgaagtgaaggagaaacatgagttccttaccagattgaagcaattgccactccttgaaagtcaaattgccaccattgagcaaagcgcaccctcacaaagtgatcaagagcagcttttttcgaatgttcagtacttcgcccattactgcaggaagtatgcacctctgtatgctgccgaagcaaaaagagtgttctcattagaaaagaaaatgagtaattacatacagttcaagtccaaatgccgcattgagcctgtatgcttactccttcacggtagtccaggggctggcaagtcagtagctaccaacctgatagggagatcccttgcagagaagctcaatagctctgtgtactctttaccaccagatccagatcattttgatgggtacaaacagcaggcagtggtgatcatggatgatctctgtcaaaaccccgatgggaaggacgtgtccttgttttgccaaatggtgtctagtgtagattttgtgccacccatggcggcgctggaagaaaaaggcattctctttacgtccccgtttgtgttggcatcaaccaacgcggggtccatcaatgcaccaacagtgtcagacagcagagcacttgccagaaggtttcactttgacatgaatattgaggtgatttcgatgtacagccagaatggtaaaattaacatgcccatgtctgttaagacatgtgatgatgaatgctgcccggtcaatttcaaaaagtgttgcccactagtgtgtggcaaggccatccagtttattgacaggagaaaccaagttagatattcactggacatgctggttactgagatgtttagagagtacaaccacagacacagtgtgggtgctaccctcgaggctttgttccaaggaccaccagtatacagggaaatcaaaatcagtgtggccccggaaacaccccctccaccagcaattgctgaccttctaaaatctgtagacagtgaggcaataagggagtactgcaaggaaaggggttggcttgtgccagaggtcagctccactctacaaattgaaaaacatgttagcagggcatttatttgcttgcaagcgctaactacatttgtttcagtggctggtataatctacatcatttacaagttgtttgccggctttcagggtgcatacactggaatgcccaaccagaaacccaaggtgcccaccttaagacaagctaaggtgcaaggtccggcatttgaatttgccgtagcaatgatgaaaaggaacgccagcacagtcaagacagaatacggtgagttcacgatgcttggcatctatgataaatgggcagtgctgccgcgccacgccaagcctggaccaactattttaatgaatgatcaggaggttggtgtgctcgatgccaaagagttagttgataaagacggaaccaacctggagctgacactattgaagcttaaccgcaatgaaaagttcagagacatcagaggttttcttgcaagggaagaagttgaggtaagtgaggctgttttggcaataaacacgagcaagttcccaagcatgtacatccctgtgggccaagtcaccgattacggatttttaaatctaggtggcaccccaacaaagagaatgctcatgtacaacttccctaccagagcgggacagtgtggtggtgtccttatgtcaacaggaaaggtccttggcatacacgtgggaggaaatggtcaccaaggcttctctgctgctctcctcagacactacttcaacgaggaacagggcgaaatagagtttattgagagctctaaagatgcaggatttcctgtgatcaacacccctaataaaaccaaactggaaccaagtgtgtttcatcaggtttttgagggcaacaaagaaccagcagtcctaagaaacggagacccgcgacttaaagccaactttgaggaagcgatattttccaagtacatcggaaatgtgaacacacatgtggacgagtacatgatagaagctgttgatcactacgctggacagctggcaactctggacatcagtacagaacctatgaagcttgaggatgctgtttatggcactgaaggcttggaagcattggacttgaccactagcgcaggatatccttatgtcgccttgggcatcaagaaaagggatatcctctccaagaagactaaagatctcaccaagctgagggaatgcatggacaagtatggtctaaatctgccgatggtgacctacgtgaaggatgaactcaggtccgctgagaaagtagccaagggaaaatccagacttatagaagcttctagtctcaatgactcagtggccatgaggcagacatttgggaacctatacaagacattccacctcaacccaggcattgtcactggtagtgctgttgggtgcgacccagatgtgttttggagcaaaatacccgtgatgcttgacgggcaccttatagcttttgattactctggctacgacgctagcttgagcccagtgtggtttgcttgtttgaaactcctcctagggaaactagggtatactcataaggaaaccaattacatagactacctctgcaactcccatcacttatacagagataaacactatttcgtgaggggtggtatgccatcaggatgttcaggcaccagtatattcaacaccatgatcaacaacatcattattaggacccttatgctaaaggtctacaaaggtattgacctggatcagtttagaatgatcgcttacggggacgatgtgatagcctcttacccgtggcctattgatgcctcactactagcagaagcgggaaaggattatggtttgatcatgaccccagcagataaaggagagtgttttaatgaggtaacctggacaaatgtaaccttcttgaaaaggtactttagagctgatgaacaatatccattcttggtgcaccccgtgatgcccatgaaagacatacacgaatccattagatggaccaaagacccaaagaacactcaagatcatgtgcgctcgttatgcctattggcttggcacaatggggagcacgaatatgaggaatttatccgaaagatcagaagcgtgcctgttggacgctgtttgaccctcccggtgttctcaacactacgcaggaaatggttagattccttctgataatagaattagagtgcaatcaatgaactatgattggcttaaccctaccgcatgaaccgaactagacaaaagtgcggtaggggtaaattctccgcattcggtgcggaaaaaaaaaaaaaaaaaaaaaaaaaaaaaaaaaaaaaaaaaaaaaaaaaaaaaaaaaaaaaaaaaaaaaaaaaaaaaaaaaaaaaaaaaaaaaaaaaaaaaaaaaaaaaaaaaaaaaaaa

SEQ ID NO: 153 - RNA, 6257 nt, synthetic construct
  source 1..6257: mol_type = other RNA
  misc_feature 1..6257: note = G2 saRNA construct
ttaaaacagcctgtgggttgtacccacccacagggcccactgggcgctagcactctggtatcacggtacctttgtgtgcctgttttatatcccctttccccgattgtaacttagaagatgtacacactgatcaatagcgggcatagcacaccagctatgtcttgatcaagcactcctgtatccccggaccaagtatcaatagactgctcacgcggttgaaggagaaaacgttcgttacccggctaactacttcgagaaacccagtagtatcatgaaagttgcgaggcgtttcgttcagcacacccccagtgtagatcgggtcgatgagtcaccgcatcccccacgggcgaccgtggcggtggctgcgctggcggcctgcctacggggcaacccgtaggacgcttcaatacagacatggtgcgaagagtcgattgagctagttagtagtcctccggcccctgaatgcggctaatcctaactgcggagcacatgccctcaacccagggggtattgtgtcgtaacgggcaactctgcagcggaaccgactactttgggtgtccgtgtttccttttatccttatactggctgcttatggtgacaattgaaagattgttgccatatagctattggattggccatccagtgtctaatagagctgttatttacctctttgttggatttataccactcaacctaaaagaagttaaaacactacagctcattttacaactgaatacagcaaaccaccatgaaactgcctcagctgtgcaccgagctgcagactaccatccacgacatcatcctggaatgtgtgtactgcaaacagcagaccaccattcacgacatcatcctggaatgcgtgtattgcaagcagcagctgctgcggagagaggtgtacgacttcgctttcagagacctgtgtatcgtttaccagcaactgctgagaagggaagtgtacgacttcgcctttcgggacctgtgtattgtgtacagagatggaaacccctacgccgtgtgcgaggtgtacgatttcgccttccgggacctgtgcatcgtgtatcgggatggaaatccttacgccgtgtgcgacaagtgcctgaagttctacagcaagccatacgccgtgtgcgacaagtgtctgaagttctacagcaagatcagcgagtaccggcactactgttacagcctgtacggcgagtacagacactactgctactccctgtacggcaccacactggaacagcaatacaacaagcccctgtgtgacctgctgatccggtgcatcaactgccagaagcctctgtgcccagaggaaaagctgagactgtgcgtgcagtctacccacgtggacatcagaacccttgaggacctgctgatgggaacactcggcctggacaaaaagcagagattccacaacatccgcggcagatggaccggcaggtgcatgagctgttgtagaagcagcagaacccctacactgcacgagtacatgctggatctgcagcctgaaaccacagaccacgaatacatgctggacctgcaacctgagacaaccgacctgtacgactgctatgagcaactcaacgactcttccgaatgctacgagcagctgaatgattccagcgaggaagaggacgagatcgacggccctgccggccaggccgacgagatcgacggccccgctggccaggctgagcctgacagagcccattataacatcgtgaccttttgttgcaagtgcgacagcacccctgatagagcccattacaacatcgtcaccttctgctgcaagtgtgatagcacactgagactgtgcgtcctgctgcaggtgcggctgtacacccagacagtgtgcgccgagcacccctgcggccaccccgaccccggcggacctacccacgtggacatcagaaccctggaggacctcctgatgggcaccctgggcatcgtgtgtcctatctgcagcaactttgagccaacaggggtgacggagtcccgcactgaaattacggcaatgcagaccaccggttcatgtgggcaacaatcaggagctgtgtacgtgggcaattacaggattgtaaacagacacctggcaacgagccacgattggcaaaattgcgtgtgggaggactacaacagggatctcctggtcagcacaacaactgctcatggttgtgatactatagcacggtgccaatgtactgctggcgtgtacttttgtgcatctagaaacaagcactacccagtgagcttcgagggtccaggtctagtgaaagttcaggagagcgagtactaccccgagagataccagtcgcacgtactccttgcagttggattttcagaaccgggtgattgtggaggtattttgaggtgtgaacatggagtcattgggctcgttaccatgggtggtgagggtgtagtaggcttcgctgacgtgcgggatcttttgtggttggaagacgacgccatggagcagggtgttagagattatgtagagcaactgggaaatgcatttggctcaggtttcactaaccaaatctgtgagcaagttaacctccttaaagaatctctgatagggcaggattccatattggaaaaatccctgaaggccctggttaaaatcatatcagccctggtgatagtggttaggaaccacgacgacctgattacagtgactgccacactagctttaatcggttgcgcatcatctccatggcgatggctcaaacaaaaagtgtgtcaatactacggaatccccatggcagaaaggcagaataacggttggttaaagaaattcactgaaatgaccaacgcctgcaagggcatggagtggattgctgttaaaattcaaaagttcatcgagtggctcaaagtaaagattctgcctgaagtgaaggagaaacatgagttccttaccagattgaagcaattgccactccttgaaagtcaaattgccaccattgagcaaagcgcaccctcacaaagtgatcaagagcagcttttttcgaatgttcagtacttcgcccattactgcaggaagtatgcacctctgtatgctgccgaagcaaaaagagtgttctcattagaaaagaaaatgagtaattacatacagttcaagtccaaatgccgcattgagcctgtatgcttactccttcacggtagtccaggggctggcaagtcagtagctaccaacctgatagggagatcccttgcagagaagctcaatagctctgtgtactctttaccaccagatccagatcattttgatgggtacaaacagcaggcagtggtgatcatggatgatctctgtcaaaaccccgatgggaaggacgtgtccttgttttgccaaatggtgtctagtgtagattttgtgccacccatggcggcgctggaagaaaaaggcattctctttacgtccccgtttgtgttggcatcaaccaacgcggggtccatcaatgcaccaacagtgtcagacagcagagcacttgccagaaggtttcactttgacatgaatattgaggtgatttcgatgtacagccagaatggtaaaattaacatgcccatgtctgttaagacatgtgatgatgaatgctgcccggtcaatttcaaaaagtgttgcccactagtgtgtggcaaggccatccagtttattgacaggagaaaccaagttagatattcactggacatgctggttactgagatgtttagagagtacaaccacagacacagtgtgggtgctaccctcgaggctttgttccaaggaccaccagtatacagggaaatcaaaatcagtgtggccccggaaacaccccctccaccagcaattgctgaccttctaaaatctgtagacagtgaggcaataagggagtactgcaaggaaaggggttggcttgtgccagaggtcagctccactctacaaattgaaaaacatgttagcagggcatttatttgcttgcaagcgctaactacatttgtttcagtggctggtataatctacatcatttacaagttgtttgccggctttcagggtgcatacactggaatgcccaaccagaaacccaaggtgcccaccttaagacaagctaaggtgcaaggtccggcatttgaatttgccgtagcaatgatgaaaaggaacgccagcacagtcaagacagaatacggtgagttcacgatgcttggcatctatgataaatgggcagtgctgccgcgccacgccaagcctggaccaactattttaatgaatgatcaggaggttggtgtgctcgatgccaaagagttagttgataaagacggaaccaacctggagctgacactattgaagcttaaccgcaatgaaaagttcagagacatcagaggttttcttgcaagggaagaagttgaggtaagtgaggctgttttggcaataaacacgagcaagttcccaagcatgtacatccctgtgggccaagtcaccgattacggatttttaaatctaggtggcaccccaacaaagagaatgctcatgtacaacttccctaccagagcgggacagtgtggtggtgtccttatgtcaacaggaaaggtccttggcatacacgtgggaggaaatggtcaccaaggcttctctgctgctctcctcagacactacttcaacgaggaacagggcgaaatagagtttattgagagctctaaagatgcaggatttcctgtgatcaacacccctaataaaaccaaactggaaccaagtgtgtttcatcaggtttttgagggcaacaaagaaccagcagtcctaagaaacggagacccgcgacttaaagccaactttgaggaagcgatattttccaagtacatcggaaatgtgaacacacatgtggacgagtacatgatagaagctgttgatcactacgctggacagctggcaactctggacatcagtacagaacctatgaagcttgaggatgctgtttatggcactgaaggcttggaagcattggacttgaccactagcgcaggatatccttatgtcgccttgggcatcaagaaaagggatatcctctccaagaagactaaagatctcaccaagctgagggaatgcatggacaagtatggtctaaatctgccgatggtgacctacgtgaaggatgaactcaggtccgctgagaaagtagccaagggaaaatccagacttatagaagcttctagtctcaatgactcagtggccatgaggcagacatttgggaacctatacaagacattccacctcaacccaggcattgtcactggtagtgctgttgggtgcgacccagatgtgttttggagcaaaatacccgtgatgcttgacgggcaccttatagcttttgattactctggctacgacgctagcttgagcccagtgtggtttgcttgtttgaaactcctcctagggaaactagggtatactcataaggaaaccaattacatagactacctctgcaactcccatcacttatacagagataaacactatttcgtgaggggtggtatgccatcaggatgttcaggcaccagtatattcaacaccatgatcaacaacatcattattaggacccttatgctaaaggtctacaaaggtattgacctggatcagtttagaatgatcgcttacggggacgatgtgatagcctcttacccgtggcctattgatgcctcactactagcagaagcgggaaaggattatggtttgatcatgaccccagcagataaaggagagtgttttaatgaggtaacctggacaaatgtaaccttcttgaaaaggtactttagagctgatgaacaatatccattcttggtgcaccccgtgatgcccatgaaagacatacacgaatccattagatggaccaaagacccaaagaacactcaagatcatgtgcgctcgttatgcctattggcttggcacaatggggagcacgaatatgaggaatttatccgaaagatcagaagcgtgcctgttggacgctgtttgaccctcccggtgttctcaacactacgcaggaaatggttagattccttctgataatagaattagagtgcaatcaatgaactatgattggcttaaccctaccgcatgaaccgaactagacaaaagtgcggtaggggtaaattctccgcattcggtgcggaaaaaaaaaaaaaaaaaaaaaaaaaaaaaaaaaaaaaaaaaaaaaaaaaaaaaaaaaaaaaaaaaaaaaaaaaaaaaaaaaaaaaaaaaaaaaaaaaaaaaaaaaaaaaaaaaaaaaaaa

SEQ ID NO: 154 - DNA, 6257 bp, synthetic construct
  source 1..6257: mol_type = other DNA
  misc_feature 1..6257: note = G2 DNA vector construct
ttaaaacagcctgtgggttgtacccacccacagggcccactgggcgctagcactctggtatcacggtacctttgtgtgcctgttttatatcccctttccccgattgtaacttagaagatgtacacactgatcaatagcgggcatagcacaccagctatgtcttgatcaagcactcctgtatccccggaccaagtatcaatagactgctcacgcggttgaaggagaaaacgttcgttacccggctaactacttcgagaaacccagtagtatcatgaaagttgcgaggcgtttcgttcagcacacccccagtgtagatcgggtcgatgagtcaccgcatcccccacgggcgaccgtggcggtggctgcgctggcggcctgcctacggggcaacccgtaggacgcttcaatacagacatggtgcgaagagtcgattgagctagttagtagtcctccggcccctgaatgcggctaatcctaactgcggagcacatgccctcaacccagggggtattgtgtcgtaacgggcaactctgcagcggaaccgactactttgggtgtccgtgtttccttttatccttatactggctgcttatggtgacaattgaaagattgttgccatatagctattggattggccatccagtgtctaatagagctgttatttacctctttgttggatttataccactcaacctaaaagaagttaaaacactacagctcattttacaactgaatacagcaaaccaccatgaaactgcctcagctgtgcaccgagctgcagactaccatccacgacatcatcctggaatgtgtgtactgcaaacagcagaccaccattcacgacatcatcctggaatgcgtgtattgcaagcagcagctgctgcggagagaggtgtacgacttcgctttcagagacctgtgtatcgtttaccagcaactgctgagaagggaagtgtacgacttcgcctttcgggacctgtgtattgtgtacagagatggaaacccctacgccgtgtgcgaggtgtacgatttcgccttccgggacctgtgcatcgtgtatcgggatggaaatccttacgccgtgtgcgacaagtgcctgaagttctacagcaagccatacgccgtgtgcgacaagtgtctgaagttctacagcaagatcagcgagtaccggcactactgttacagcctgtacggcgagtacagacactactgctactccctgtacggcaccacactggaacagcaatacaacaagcccctgtgtgacctgctgatccggtgcatcaactgccagaagcctctgtgcccagaggaaaagctgagactgtgcgtgcagtctacccacgtggacatcagaacccttgaggacctgctgatgggaacactcggcctggacaaaaagcagagattccacaacatccgcggcagatggaccggcaggtgcatgagctgttgtagaagcagcagaacccctacactgcacgagtacatgctggatctgcagcctgaaaccacagaccacgaatacatgctggacctgcaacctgagacaaccgacctgtacgactgctatgagcaactcaacgactcttccgaatgctacgagcagctgaatgattccagcgaggaagaggacgagatcgacggccctgccggccaggccgacgagatcgacggccccgctggccaggctgagcctgacagagcccattataacatcgtgaccttttgttgcaagtgcgacagcacccctgatagagcccattacaacatcgtcaccttctgctgcaagtgtgatagcacactgagactgtgcgtcctgctgcaggtgcggctgtacacccagacagtgtgcgccgagcacccctgcggccaccccgaccccggcggacctacccacgtggacatcagaaccctggaggacctcctgatgggcaccctgggcatcgtgtgtcctatctgcagcaactttgagccaacaggggtgacggagtcccgcactgaaattacggcaatgcagaccaccggttcatgtgggcaacaatcaggagctgtgtacgtgggcaattacaggattgtaaacagacacctggcaacgagccacgattggcaaaattgcgtgtgggaggactacaacagggatctcctggtcagcacaacaactgctcatggttgtgatactatagcacggtgccaatgtactgctggcgtgtacttttgtgcatctagaaacaagcactacccagtgagcttcgagggtccaggtctagtgaaagttcaggagagcgagtactaccccgagagataccagtcgcacgtactccttgcagttggattttcagaaccgggtgattgtggaggtattttgaggtgtgaacatggagtcattgggctcgttaccatgggtggtgagggtgtagtaggcttcgctgacgtgcgggatcttttgtggttggaagacgacgccatggagcagggtgttagagattatgtagagcaactgggaaatgcatttggctcaggtttcactaaccaaatctgtgagcaagttaacctccttaaagaatctctgatagggcaggattccatattggaaaaatccctgaaggccctggttaaaatcatatcagccctggtgatagtggttaggaaccacgacgacctgattacagtgactgccacactagctttaatcggttgcgcatcatctccatggcgatggctcaaacaaaaagtgtgtcaatactacggaatccccatggcagaaaggcagaataacggttggttaaagaaattcactgaaatgaccaacgcctgcaagggcatggagtggattgctgttaaaattcaaaagttcatcgagtggctcaaagtaaagattctgcctgaagtgaaggagaaacatgagttccttaccagattgaagcaattgccactccttgaaagtcaaattgccaccattgagcaaagcgcaccctcacaaagtgatcaagagcagcttttttcgaatgttcagtacttcgcccattactgcaggaagtatgcacctctgtatgctgccgaagcaaaaagagtgttctcattagaaaagaaaatgagtaattacatacagttcaagtccaaatgccgcattgagcctgtatgcttactccttcacggtagtccaggggctggcaagtcagtagctaccaacctgatagggagatcccttgcagagaagctcaatagctctgtgtactctttaccaccagatccagatcattttgatgggtacaaacagcaggcagtggtgatcatggatgatctctgtcaaaaccccgatgggaaggacgtgtccttgttttgccaaatggtgtctagtgtagattttgtgccacccatggcggcgctggaagaaaaaggcattctctttacgtccccgtttgtgttggcatcaaccaacgcggggtccatcaatgcaccaacagtgtcagacagcagagcacttgccagaaggtttcactttgacatgaatattgaggtgatttcgatgtacagccagaatggtaaaattaacatgcccatgtctgttaagacatgtgatgatgaatgctgcccggtcaatttcaaaaagtgttgcccactagtgtgtggcaaggccatccagtttattgacaggagaaaccaagttagatattcactggacatgctggttactgagatgtttagagagtacaaccacagacacagtgtgggtgctaccctcgaggctttgttccaaggaccaccagtatacagggaaatcaaaatcagtgtggccccggaaacaccccctccaccagcaattgctgaccttctaaaatctgtagacagtgaggcaataagggagtactgcaaggaaaggggttggcttgtgccagaggtcagctccactctacaaattgaaaaacatgttagcagggcatttatttgcttgcaagcgctaactacatttgtttcagtggctggtataatctacatcatttacaagttgtttgccggctttcagggtgcatacactggaatgcccaaccagaaacccaaggtgcccaccttaagacaagctaaggtgcaaggtccggcatttgaatttgccgtagcaatgatgaaaaggaacgccagcacagtcaagacagaatacggtgagttcacgatgcttggcatctatgataaatgggcagtgctgccgcgccacgccaagcctggaccaactattttaatgaatgatcaggaggttggtgtgctcgatgccaaagagttagttgataaagacggaaccaacctggagctgacactattgaagcttaaccgcaatgaaaagttcagagacatcagaggttttcttgcaagggaagaagttgaggtaagtgaggctgttttggcaataaacacgagcaagttcccaagcatgtacatccctgtgggccaagtcaccgattacggatttttaaatctaggtggcaccccaacaaagagaatgctcatgtacaacttccctaccagagcgggacagtgtggtggtgtccttatgtcaacaggaaaggtccttggcatacacgtgggaggaaatggtcaccaaggcttctctgctgctctcctcagacactacttcaacgaggaacagggcgaaatagagtttattgagagctctaaagatgcaggatttcctgtgatcaacacccctaataaaaccaaactggaaccaagtgtgtttcatcaggtttttgagggcaacaaagaaccagcagtcctaagaaacggagacccgcgacttaaagccaactttgaggaagcgatattttccaagtacatcggaaatgtgaacacacatgtggacgagtacatgatagaagctgttgatcactacgctggacagctggcaactctggacatcagtacagaacctatgaagcttgaggatgctgtttatggcactgaaggcttggaagcattggacttgaccactagcgcaggatatccttatgtcgccttgggcatcaagaaaagggatatcctctccaagaagactaaagatctcaccaagctgagggaatgcatggacaagtatggtctaaatctgccgatggtgacctacgtgaaggatgaactcaggtccgctgagaaagtagccaagggaaaatccagacttatagaagcttctagtctcaatgactcagtggccatgaggcagacatttgggaacctatacaagacattccacctcaacccaggcattgtcactggtagtgctgttgggtgcgacccagatgtgttttggagcaaaatacccgtgatgcttgacgggcaccttatagcttttgattactctggctacgacgctagcttgagcccagtgtggtttgcttgtttgaaactcctcctagggaaactagggtatactcataaggaaaccaattacatagactacctctgcaactcccatcacttatacagagataaacactatttcgtgaggggtggtatgccatcaggatgttcaggcaccagtatattcaacaccatgatcaacaacatcattattaggacccttatgctaaaggtctacaaaggtattgacctggatcagtttagaatgatcgcttacggggacgatgtgatagcctcttacccgtggcctattgatgcctcactactagcagaagcgggaaaggattatggtttgatcatgaccccagcagataaaggagagtgttttaatgaggtaacctggacaaatgtaaccttcttgaaaaggtactttagagctgatgaacaatatccattcttggtgcaccccgtgatgcccatgaaagacatacacgaatccattagatggaccaaagacccaaagaacactcaagatcatgtgcgctcgttatgcctattggcttggcacaatggggagcacgaatatgaggaatttatccgaaagatcagaagcgtgcctgttggacgctgtttgaccctcccggtgttctcaacactacgcaggaaatggttagattccttctgataatagaattagagtgcaatcaatgaactatgattggcttaaccctaccgcatgaaccgaactagacaaaagtgcggtaggggtaaattctccgcattcggtgcggaaaaaaaaaaaaaaaaaaaaaaaaaaaaaaaaaaaaaaaaaaaaaaaaaaaaaaaaaaaaaaaaaaaaaaaaaaaaaaaaaaaaaaaaaaaaaaaaaaaaaaaaaaaaaaaaaaaaaaaa

SEQ ID NO: 155 - RNA, 6254 nt, synthetic construct
  source 1..6254: mol_type = other RNA
  misc_feature 1..6254: note = G3 saRNA construct
ttaaaacagcctgtgggttgtacccacccacagggcccactgggcgctagcactctggtatcacggtacctttgtgtgcctgttttatatcccctttccccgattgtaacttagaagatgtacacactgatcaatagcgggcatagcacaccagctatgtcttgatcaagcactcctgtatccccggaccaagtatcaatagactgctcacgcggttgaaggagaaaacgttcgttacccggctaactacttcgagaaacccagtagtatcatgaaagttgcgaggcgtttcgttcagcacacccccagtgtagatcgggtcgatgagtcaccgcatcccccacgggcgaccgtggcggtggctgcgctggcggcctgcctacggggcaacccgtaggacgcttcaatacagacatggtgcgaagagtcgattgagctagttagtagtcctccggcccctgaatgcggctaatcctaactgcggagcacatgccctcaacccagggggtattgtgtcgtaacgggcaactctgcagcggaaccgactactttgggtgtccgtgtttccttttatccttatactggctgcttatggtgacaattgaaagattgttgccatatagctattggattggccatccagtgtctaatagagctgttatttacctctttgttggatttataccactcaacctaaaagaagttaaaacactacagctcattttacaactgaatacagcaaaccaccatgaagctgccccagctgtgtaccgagctgcagaccacaatccacgacattatcctggaatgtgtgtactgcaagcagcaaacccccaccctgcacgagtacatgctggatctgcaacctgagacaaccgacaccacaatccatgacatcatcctggaatgtgtgtactgcaaacagcagctgctgcggagagaagtgtatgacttcgccttccgcgacctgtgtatcgtgtaccacgagtatatgcttgatctgcagcctgagacaacagacctgtactgttatgagcagctgaacgacagctctgaacagcagctgctgagaagagaggtgtacgatttcgcctttcgggacctgtgcatcgtctatcgggacggcaacccatacgccgtgtgttgctacgagcaactcaatgactcttctgaagaggaggatgagatcgatggccctgccggccaggccgaggtctacgacttcgccttcagagacctgtgcatcgtgtaccgggacggcaatccctacgccgtgtgcgataagtgcctgaaattctactccaaggacgagatcgacggcccagctggccaggccgaacccgatagagcccactacaacatcgtgacattctgctgcaagtgcgacagcacaccttacgctgtgtgcgacaagtgtctgaagttctacagcaagatcagcgagtaccggcactactgctactccctgtacggccctgacagagcccactacaacatcgtgaccttttgctgtaaatgtgacagcaccctgagactgtgcgtggaataccggcactactgttactccctgtacggcaccaccctggaacagcagtacaacaagcctctgtgcgacttgctgatccggtgcattaactgccagaaacctctgtgccccgaggaaaagctactgcaggtgcggctgtacacccagactgtttgcgccgagcacccgtgcggccaccctgatcctggcggacctctgaggctgtgtgtgcagagcacccatgtggacatccgaacactggaggacctgctgatgggaaccctgggcacccacgtggacatcagaaccctggaggacctgctgatgggcacactgggaatcgtgtgccctatctgcagcctggacaagaagcaaagattccacaacatcagaggaagatggaccggcagatgcatgagctgctgcagaagcagcagaaactttgagccaacaggggtgacggagtcccgcactgaaattacggcaatgcagaccaccggttcatgtgggcaacaatcaggagctgtgtacgtgggcaattacaggattgtaaacagacacctggcaacgagccacgattggcaaaattgcgtgtgggaggactacaacagggatctcctggtcagcacaacaactgctcatggttgtgatactatagcacggtgccaatgtactgctggcgtgtacttttgtgcatctagaaacaagcactacccagtgagcttcgagggtccaggtctagtgaaagttcaggagagcgagtactaccccgagagataccagtcgcacgtactccttgcagttggattttcagaaccgggtgattgtggaggtattttgaggtgtgaacatggagtcattgggctcgttaccatgggtggtgagggtgtagtaggcttcgctgacgtgcgggatcttttgtggttggaagacgacgccatggagcagggtgttagagattatgtagagcaactgggaaatgcatttggctcaggtttcactaaccaaatctgtgagcaagttaacctccttaaagaatctctgatagggcaggattccatattggaaaaatccctgaaggccctggttaaaatcatatcagccctggtgatagtggttaggaaccacgacgacctgattacagtgactgccacactagctttaatcggttgcgcatcatctccatggcgatggctcaaacaaaaagtgtgtcaatactacggaatccccatggcagaaaggcagaataacggttggttaaagaaattcactgaaatgaccaacgcctgcaagggcatggagtggattgctgttaaaattcaaaagttcatcgagtggctcaaagtaaagattctgcctgaagtgaaggagaaacatgagttccttaccagattgaagcaattgccactccttgaaagtcaaattgccaccattgagcaaagcgcaccctcacaaagtgatcaagagcagcttttttcgaatgttcagtacttcgcccattactgcaggaagtatgcacctctgtatgctgccgaagcaaaaagagtgttctcattagaaaagaaaatgagtaattacatacagttcaagtccaaatgccgcattgagcctgtatgcttactccttcacggtagtccaggggctggcaagtcagtagctaccaacctgatagggagatcccttgcagagaagctcaatagctctgtgtactctttaccaccagatccagatcattttgatgggtacaaacagcaggcagtggtgatcatggatgatctctgtcaaaaccccgatgggaaggacgtgtccttgttttgccaaatggtgtctagtgtagattttgtgccacccatggcggcgctggaagaaaaaggcattctctttacgtccccgtttgtgttggcatcaaccaacgcggggtccatcaatgcaccaacagtgtcagacagcagagcacttgccagaaggtttcactttgacatgaatattgaggtgatttcgatgtacagccagaatggtaaaattaacatgcccatgtctgttaagacatgtgatgatgaatgctgcccggtcaatttcaaaaagtgttgcccactagtgtgtggcaaggccatccagtttattgacaggagaaaccaagttagatattcactggacatgctggttactgagatgtttagagagtacaaccacagacacagtgtgggtgctaccctcgaggctttgttccaaggaccaccagtatacagggaaatcaaaatcagtgtggccccggaaacaccccctccaccagcaattgctgaccttctaaaatctgtagacagtgaggcaataagggagtactgcaaggaaaggggttggcttgtgccagaggtcagctccactctacaaattgaaaaacatgttagcagggcatttatttgcttgcaagcgctaactacatttgtttcagtggctggtataatctacatcatttacaagttgtttgccggctttcagggtgcatacactggaatgcccaaccagaaacccaaggtgcccaccttaagacaagctaaggtgcaaggtccggcatttgaatttgccgtagcaatgatgaaaaggaacgccagcacagtcaagacagaatacggtgagttcacgatgcttggcatctatgataaatgggcagtgctgccgcgccacgccaagcctggaccaactattttaatgaatgatcaggaggttggtgtgctcgatgccaaagagttagttgataaagacggaaccaacctggagctgacactattgaagcttaaccgcaatgaaaagttcagagacatcagaggttttcttgcaagggaagaagttgaggtaagtgaggctgttttggcaataaacacgagcaagttcccaagcatgtacatccctgtgggccaagtcaccgattacggatttttaaatctaggtggcaccccaacaaagagaatgctcatgtacaacttccctaccagagcgggacagtgtggtggtgtccttatgtcaacaggaaaggtccttggcatacacgtgggaggaaatggtcaccaaggcttctctgctgctctcctcagacactacttcaacgaggaacagggcgaaatagagtttattgagagctctaaagatgcaggatttcctgtgatcaacacccctaataaaaccaaactggaaccaagtgtgtttcatcaggtttttgagggcaacaaagaaccagcagtcctaagaaacggagacccgcgacttaaagccaactttgaggaagcgatattttccaagtacatcggaaatgtgaacacacatgtggacgagtacatgatagaagctgttgatcactacgctggacagctggcaactctggacatcagtacagaacctatgaagcttgaggatgctgtttatggcactgaaggcttggaagcattggacttgaccactagcgcaggatatccttatgtcgccttgggcatcaagaaaagggatatcctctccaagaagactaaagatctcaccaagctgagggaatgcatggacaagtatggtctaaatctgccgatggtgacctacgtgaaggatgaactcaggtccgctgagaaagtagccaagggaaaatccagacttatagaagcttctagtctcaatgactcagtggccatgaggcagacatttgggaacctatacaagacattccacctcaacccaggcattgtcactggtagtgctgttgggtgcgacccagatgtgttttggagcaaaatacccgtgatgcttgacgggcaccttatagcttttgattactctggctacgacgctagcttgagcccagtgtggtttgcttgtttgaaactcctcctagggaaactagggtatactcataaggaaaccaattacatagactacctctgcaactcccatcacttatacagagataaacactatttcgtgaggggtggtatgccatcaggatgttcaggcaccagtatattcaacaccatgatcaacaacatcattattaggacccttatgctaaaggtctacaaaggtattgacctggatcagtttagaatgatcgcttacggggacgatgtgatagcctcttacccgtggcctattgatgcctcactactagcagaagcgggaaaggattatggtttgatcatgaccccagcagataaaggagagtgttttaatgaggtaacctggacaaatgtaaccttcttgaaaaggtactttagagctgatgaacaatatccattcttggtgcaccccgtgatgcccatgaaagacatacacgaatccattagatggaccaaagacccaaagaacactcaagatcatgtgcgctcgttatgcctattggcttggcacaatggggagcacgaatatgaggaatttatccgaaagatcagaagcgtgcctgttggacgctgtttgaccctcccggtgttctcaacactacgcaggaaatggttagattccttctgataatagaattagagtgcaatcaatgaactatgattggcttaaccctaccgcatgaaccgaactagacaaaagtgcggtaggggtaaattctccgcattcggtgcggaaaaaaaaaaaaaaaaaaaaaaaaaaaaaaaaaaaaaaaaaaaaaaaaaaaaaaaaaaaaaaaaaaaaaaaaaaaaaaaaaaaaaaaaaaaaaaaaaaaaaaaaaaaaaaaaaaaaaaaa

SEQ ID NO: 156 - DNA, 6254 bp, synthetic construct
  source 1..6254: mol_type = other DNA
  misc_feature 1..6254: note = G3 DNA vector construct
ttaaaacagcctgtgggttgtacccacccacagggcccactgggcgctagcactctggtatcacggtacctttgtgtgcctgttttatatcccctttccccgattgtaacttagaagatgtacacactgatcaatagcgggcatagcacaccagctatgtcttgatcaagcactcctgtatccccggaccaagtatcaatagactgctcacgcggttgaaggagaaaacgttcgttacccggctaactacttcgagaaacccagtagtatcatgaaagttgcgaggcgtttcgttcagcacacccccagtgtagatcgggtcgatgagtcaccgcatcccccacgggcgaccgtggcggtggctgcgctggcggcctgcctacggggcaacccgtaggacgcttcaatacagacatggtgcgaagagtcgattgagctagttagtagtcctccggcccctgaatgcggctaatcctaactgcggagcacatgccctcaacccagggggtattgtgtcgtaacgggcaactctgcagcggaaccgactactttgggtgtccgtgtttccttttatccttatactggctgcttatggtgacaattgaaagattgttgccatatagctattggattggccatccagtgtctaatagagctgttatttacctctttgttggatttataccactcaacctaaaagaagttaaaacactacagctcattttacaactgaatacagcaaaccaccatgaagctgccccagctgtgtaccgagctgcagaccacaatccacgacattatcctggaatgtgtgtactgcaagcagcaaacccccaccctgcacgagtacatgctggatctgcaacctgagacaaccgacaccacaatccatgacatcatcctggaatgtgtgtactgcaaacagcagctgctgcggagagaagtgtatgacttcgccttccgcgacctgtgtatcgtgtaccacgagtatatgcttgatctgcagcctgagacaacagacctgtactgttatgagcagctgaacgacagctctgaacagcagctgctgagaagagaggtgtacgatttcgcctttcgggacctgtgcatcgtctatcgggacggcaacccatacgccgtgtgttgctacgagcaactcaatgactcttctgaagaggaggatgagatcgatggccctgccggccaggccgaggtctacgacttcgccttcagagacctgtgcatcgtgtaccgggacggcaatccctacgccgtgtgcgataagtgcctgaaattctactccaaggacgagatcgacggcccagctggccaggccgaacccgatagagcccactacaacatcgtgacattctgctgcaagtgcgacagcacaccttacgctgtgtgcgacaagtgtctgaagttctacagcaagatcagcgagtaccggcactactgctactccctgtacggccctgacagagcccactacaacatcgtgaccttttgctgtaaatgtgacagcaccctgagactgtgcgtggaataccggcactactgttactccctgtacggcaccaccctggaacagcagtacaacaagcctctgtgcgacttgctgatccggtgcattaactgccagaaacctctgtgccccgaggaaaagctactgcaggtgcggctgtacacccagactgtttgcgccgagcacccgtgcggccaccctgatcctggcggacctctgaggctgtgtgtgcagagcacccatgtggacatccgaacactggaggacctgctgatgggaaccctgggcacccacgtggacatcagaaccctggaggacctgctgatgggcacactgggaatcgtgtgccctatctgcagcctggacaagaagcaaagattccacaacatcagaggaagatggaccggcagatgcatgagctgctgcagaagcagcagaaactttgagccaacaggggtgacggagtcccgcactgaaattacggcaatgcagaccaccggttcatgtgggcaacaatcaggagctgtgtacgtgggcaattacaggattgtaaacagacacctggcaacgagccacgattggcaaaattgcgtgtgggaggactacaacagggatctcctggtcagcacaacaactgctcatggttgtgatactatagcacggtgccaatgtactgctggcgtgtacttttgtgcatctagaaacaagcactacccagtgagcttcgagggtccaggtctagtgaaagttcaggagagcgagtactaccccgagagataccagtcgcacgtactccttgcagttggattttcagaaccgggtgattgtggaggtattttgaggtgtgaacatggagtcattgggctcgttaccatgggtggtgagggtgtagtaggcttcgctgacgtgcgggatcttttgtggttggaagacgacgccatggagcagggtgttagagattatgtagagcaactgggaaatgcatttggctcaggtttcactaaccaaatctgtgagcaagttaacctccttaaagaatctctgatagggcaggattccatattggaaaaatccctgaaggccctggttaaaatcatatcagccctggtgatagtggttaggaaccacgacgacctgattacagtgactgccacactagctttaatcggttgcgcatcatctccatggcgatggctcaaacaaaaagtgtgtcaatactacggaatccccatggcagaaaggcagaataacggttggttaaagaaattcactgaaatgaccaacgcctgcaagggcatggagtggattgctgttaaaattcaaaagttcatcgagtggctcaaagtaaagattctgcctgaagtgaaggagaaacatgagttccttaccagattgaagcaattgccactccttgaaagtcaaattgccaccattgagcaaagcgcaccctcacaaagtgatcaagagcagcttttttcgaatgttcagtacttcgcccattactgcaggaagtatgcacctctgtatgctgccgaagcaaaaagagtgttctcattagaaaagaaaatgagtaattacatacagttcaagtccaaatgccgcattgagcctgtatgcttactccttcacggtagtccaggggctggcaagtcagtagctaccaacctgatagggagatcccttgcagagaagctcaatagctctgtgtactctttaccaccagatccagatcattttgatgggtacaaacagcaggcagtggtgatcatggatgatctctgtcaaaaccccgatgggaaggacgtgtccttgttttgccaaatggtgtctagtgtagattttgtgccacccatggcggcgctggaagaaaaaggcattctctttacgtccccgtttgtgttggcatcaaccaacgcggggtccatcaatgcaccaacagtgtcagacagcagagcacttgccagaaggtttcactttgacatgaatattgaggtgatttcgatgtacagccagaatggtaaaattaacatgcccatgtctgttaagacatgtgatgatgaatgctgcccggtcaatttcaaaaagtgttgcccactagtgtgtggcaaggccatccagtttattgacaggagaaaccaagttagatattcactggacatgctggttactgagatgtttagagagtacaaccacagacacagtgtgggtgctaccctcgaggctttgttccaaggaccaccagtatacagggaaatcaaaatcagtgtggccccggaaacaccccctccaccagcaattgctgaccttctaaaatctgtagacagtgaggcaataagggagtactgcaaggaaaggggttggcttgtgccagaggtcagctccactctacaaattgaaaaacatgttagcagggcatttatttgcttgcaagcgctaactacatttgtttcagtggctggtataatctacatcatttacaagttgtttgccggctttcagggtgcatacactggaatgcccaaccagaaacccaaggtgcccaccttaagacaagctaaggtgcaaggtccggcatttgaatttgccgtagcaatgatgaaaaggaacgccagcacagtcaagacagaatacggtgagttcacgatgcttggcatctatgataaatgggcagtgctgccgcgccacgccaagcctggaccaactattttaatgaatgatcaggaggttggtgtgctcgatgccaaagagttagttgataaagacggaaccaacctggagctgacactattgaagcttaaccgcaatgaaaagttcagagacatcagaggttttcttgcaagggaagaagttgaggtaagtgaggctgttttggcaataaacacgagcaagttcccaagcatgtacatccctgtgggccaagtcaccgattacggatttttaaatctaggtggcaccccaacaaagagaatgctcatgtacaacttccctaccagagcgggacagtgtggtggtgtccttatgtcaacaggaaaggtccttggcatacacgtgggaggaaatggtcaccaaggcttctctgctgctctcctcagacactacttcaacgaggaacagggcgaaatagagtttattgagagctctaaagatgcaggatttcctgtgatcaacacccctaataaaaccaaactggaaccaagtgtgtttcatcaggtttttgagggcaacaaagaaccagcagtcctaagaaacggagacccgcgacttaaagccaactttgaggaagcgatattttccaagtacatcggaaatgtgaacacacatgtggacgagtacatgatagaagctgttgatcactacgctggacagctggcaactctggacatcagtacagaacctatgaagcttgaggatgctgtttatggcactgaaggcttggaagcattggacttgaccactagcgcaggatatccttatgtcgccttgggcatcaagaaaagggatatcctctccaagaagactaaagatctcaccaagctgagggaatgcatggacaagtatggtctaaatctgccgatggtgacctacgtgaaggatgaactcaggtccgctgagaaagtagccaagggaaaatccagacttatagaagcttctagtctcaatgactcagtggccatgaggcagacatttgggaacctatacaagacattccacctcaacccaggcattgtcactggtagtgctgttgggtgcgacccagatgtgttttggagcaaaatacccgtgatgcttgacgggcaccttatagcttttgattactctggctacgacgctagcttgagcccagtgtggtttgcttgtttgaaactcctcctagggaaactagggtatactcataaggaaaccaattacatagactacctctgcaactcccatcacttatacagagataaacactatttcgtgaggggtggtatgccatcaggatgttcaggcaccagtatattcaacaccatgatcaacaacatcattattaggacccttatgctaaaggtctacaaaggtattgacctggatcagtttagaatgatcgcttacggggacgatgtgatagcctcttacccgtggcctattgatgcctcactactagcagaagcgggaaaggattatggtttgatcatgaccccagcagataaaggagagtgttttaatgaggtaacctggacaaatgtaaccttcttgaaaaggtactttagagctgatgaacaatatccattcttggtgcaccccgtgatgcccatgaaagacatacacgaatccattagatggaccaaagacccaaagaacactcaagatcatgtgcgctcgttatgcctattggcttggcacaatggggagcacgaatatgaggaatttatccgaaagatcagaagcgtgcctgttggacgctgtttgaccctcccggtgttctcaacactacgcaggaaatggttagattccttctgataatagaattagagtgcaatcaatgaactatgattggcttaaccctaccgcatgaaccgaactagacaaaagtgcggtaggggtaaattctccgcattcggtgcggaaaaaaaaaaaaaaaaaaaaaaaaaaaaaaaaaaaaaaaaaaaaaaaaaaaaaaaaaaaaaaaaaaaaaaaaaaaaaaaaaaaaaaaaaaaaaaaaaaaaaaaaaaaaaaaaaaaaaaaa

SEQ ID NO: 157 - RNA, 6254 nt, synthetic construct
  source 1..6254: mol_type = other RNA
  misc_feature 1..6254: note = G4 saRNA construct
ttaaaacagcctgtgggttgtacccacccacagggcccactgggcgctagcactctggtatcacggtacctttgtgtgcctgttttatatcccctttccccgattgtaacttagaagatgtacacactgatcaatagcgggcatagcacaccagctatgtcttgatcaagcactcctgtatccccggaccaagtatcaatagactgctcacgcggttgaaggagaaaacgttcgttacccggctaactacttcgagaaacccagtagtatcatgaaagttgcgaggcgtttcgttcagcacacccccagtgtagatcgggtcgatgagtcaccgcatcccccacgggcgaccgtggcggtggctgcgctggcggcctgcctacggggcaacccgtaggacgcttcaatacagacatggtgcgaagagtcgattgagctagttagtagtcctccggcccctgaatgcggctaatcctaactgcggagcacatgccctcaacccagggggtattgtgtcgtaacgggcaactctgcagcggaaccgactactttgggtgtccgtgtttccttttatccttatactggctgcttatggtgacaattgaaagattgttgccatatagctattggattggccatccagtgtctaatagagctgttatttacctctttgttggatttataccactcaacctaaaagaagttaaaacactacagctcattttacaactgaatacagcaaaccaccatgaaactgcctcagctgtgcacagagctgcagacaacaatccacgacatcattctggagtgcgtctactgcaagcagcagcagcagctgctgagaagggaagtgtacgattttgcctttagagacctgtgcattgtgtaccgggacggcaatccttacgctgtgtgcccttacgccgtgtgcgacaagtgtctgaaattctactctaagatcagcgagtaccggcactactgttacagcctgtacggcctgcggctgtgtgtgcagtctacccacgtggacatcagaacactggaggacctgctcatgggcacactgggcaccaccatccacgacatcatcctggaatgcgtctactgcaagcaacagctgctgcggagggaggtgtacgacttcgccttccgggacctgtgcatcgtttatgaggtgtatgacttcgccttcagagacctgtgcatcgtgtatagagatggcaacccctacgccgtgtgcgacaagtgcctgaagttctactccaaggaatacagacactactgctatagcctgtacggcaccacccttgaacaacaatacaacaagcccctgtgcgatctgctgatccgatgtatcaactgccagaagcctctgtgtcccgaagagaagctggacaaaaagcaacggttccacaacatccggggaagatggaccggccggtgtatgagctgctgcagaagcagcagaacccctaccctgcacgagtacatgctggacctccagcctgaaaccaccgactgttacgagcagctgaacgacagttccgaggaggaagatgagatcgacggacctgccggccaggcccctgatagagcccattacaacatcgtgaccttctgttgcaagtgcgacagcacacttagactgtgtgtgacccacgtggacatcagaacactggaggacctgctgatgggcaccctgggcatcgtgtgccccatctgcagccacgagtacatgctggacctgcagcctgagacaaccgacctgtactgctacgagcagctgaatgacagcagcgaagacgagatcgatggaccagctggccaggccgagccagatagagcccactacaacatcgtgacattctgctgcaaatgtgacagcaccctgctccaggtgagactgtacacccagaccgtgtgtgccgaacacccctgcggtcatcctgaccccggcggccctaactttgagccaacaggggtgacggagtcccgcactgaaattacggcaatgcagaccaccggttcatgtgggcaacaatcaggagctgtgtacgtgggcaattacaggattgtaaacagacacctggcaacgagccacgattggcaaaattgcgtgtgggaggactacaacagggatctcctggtcagcacaacaactgctcatggttgtgatactatagcacggtgccaatgtactgctggcgtgtacttttgtgcatctagaaacaagcactacccagtgagcttcgagggtccaggtctagtgaaagttcaggagagcgagtactaccccgagagataccagtcgcacgtactccttgcagttggattttcagaaccgggtgattgtggaggtattttgaggtgtgaacatggagtcattgggctcgttaccatgggtggtgagggtgtagtaggcttcgctgacgtgcgggatcttttgtggttggaagacgacgccatggagcagggtgttagagattatgtagagcaactgggaaatgcatttggctcaggtttcactaaccaaatctgtgagcaagttaacctccttaaagaatctctgatagggcaggattccatattggaaaaatccctgaaggccctggttaaaatcatatcagccctggtgatagtggttaggaaccacgacgacctgattacagtgactgccacactagctttaatcggttgcgcatcatctccatggcgatggctcaaacaaaaagtgtgtcaatactacggaatccccatggcagaaaggcagaataacggttggttaaagaaattcactgaaatgaccaacgcctgcaagggcatggagtggattgctgttaaaattcaaaagttcatcgagtggctcaaagtaaagattctgcctgaagtgaaggagaaacatgagttccttaccagattgaagcaattgccactccttgaaagtcaaattgccaccattgagcaaagcgcaccctcacaaagtgatcaagagcagcttttttcgaatgttcagtacttcgcccattactgcaggaagtatgcacctctgtatgctgccgaagcaaaaagagtgttctcattagaaaagaaaatgagtaattacatacagttcaagtccaaatgccgcattgagcctgtatgcttactccttcacggtagtccaggggctggcaagtcagtagctaccaacctgatagggagatcccttgcagagaagctcaatagctctgtgtactctttaccaccagatccagatcattttgatgggtacaaacagcaggcagtggtgatcatggatgatctctgtcaaaaccccgatgggaaggacgtgtccttgttttgccaaatggtgtctagtgtagattttgtgccacccatggcggcgctggaagaaaaaggcattctctttacgtccccgtttgtgttggcatcaaccaacgcggggtccatcaatgcaccaacagtgtcagacagcagagcacttgccagaaggtttcactttgacatgaatattgaggtgatttcgatgtacagccagaatggtaaaattaacatgcccatgtctgttaagacatgtgatgatgaatgctgcccggtcaatttcaaaaagtgttgcccactagtgtgtggcaaggccatccagtttattgacaggagaaaccaagttagatattcactggacatgctggttactgagatgtttagagagtacaaccacagacacagtgtgggtgctaccctcgaggctttgttccaaggaccaccagtatacagggaaatcaaaatcagtgtggccccggaaacaccccctccaccagcaattgctgaccttctaaaatctgtagacagtgaggcaataagggagtactgcaaggaaaggggttggcttgtgccagaggtcagctccactctacaaattgaaaaacatgttagcagggcatttatttgcttgcaagcgctaactacatttgtttcagtggctggtataatctacatcatttacaagttgtttgccggctttcagggtgcatacactggaatgcccaaccagaaacccaaggtgcccaccttaagacaagctaaggtgcaaggtccggcatttgaatttgccgtagcaatgatgaaaaggaacgccagcacagtcaagacagaatacggtgagttcacgatgcttggcatctatgataaatgggcagtgctgccgcgccacgccaagcctggaccaactattttaatgaatgatcaggaggttggtgtgctcgatgccaaagagttagttgataaagacggaaccaacctggagctgacactattgaagcttaaccgcaatgaaaagttcagagacatcagaggttttcttgcaagggaagaagttgaggtaagtgaggctgttttggcaataaacacgagcaagttcccaagcatgtacatccctgtgggccaagtcaccgattacggatttttaaatctaggtggcaccccaacaaagagaatgctcatgtacaacttccctaccagagcgggacagtgtggtggtgtccttatgtcaacaggaaaggtccttggcatacacgtgggaggaaatggtcaccaaggcttctctgctgctctcctcagacactacttcaacgaggaacagggcgaaatagagtttattgagagctctaaagatgcaggatttcctgtgatcaacacccctaataaaaccaaactggaaccaagtgtgtttcatcaggtttttgagggcaacaaagaaccagcagtcctaagaaacggagacccgcgacttaaagccaactttgaggaagcgatattttccaagtacatcggaaatgtgaacacacatgtggacgagtacatgatagaagctgttgatcactacgctggacagctggcaactctggacatcagtacagaacctatgaagcttgaggatgctgtttatggcactgaaggcttggaagcattggacttgaccactagcgcaggatatccttatgtcgccttgggcatcaagaaaagggatatcctctccaagaagactaaagatctcaccaagctgagggaatgcatggacaagtatggtctaaatctgccgatggtgacctacgtgaaggatgaactcaggtccgctgagaaagtagccaagggaaaatccagacttatagaagcttctagtctcaatgactcagtggccatgaggcagacatttgggaacctatacaagacattccacctcaacccaggcattgtcactggtagtgctgttgggtgcgacccagatgtgttttggagcaaaatacccgtgatgcttgacgggcaccttatagcttttgattactctggctacgacgctagcttgagcccagtgtggtttgcttgtttgaaactcctcctagggaaactagggtatactcataaggaaaccaattacatagactacctctgcaactcccatcacttatacagagataaacactatttcgtgaggggtggtatgccatcaggatgttcaggcaccagtatattcaacaccatgatcaacaacatcattattaggacccttatgctaaaggtctacaaaggtattgacctggatcagtttagaatgatcgcttacggggacgatgtgatagcctcttacccgtggcctattgatgcctcactactagcagaagcgggaaaggattatggtttgatcatgaccccagcagataaaggagagtgttttaatgaggtaacctggacaaatgtaaccttcttgaaaaggtactttagagctgatgaacaatatccattcttggtgcaccccgtgatgcccatgaaagacatacacgaatccattagatggaccaaagacccaaagaacactcaagatcatgtgcgctcgttatgcctattggcttggcacaatggggagcacgaatatgaggaatttatccgaaagatcagaagcgtgcctgttggacgctgtttgaccctcccggtgttctcaacactacgcaggaaatggttagattccttctgataatagaattagagtgcaatcaatgaactatgattggcttaaccctaccgcatgaaccgaactagacaaaagtgcggtaggggtaaattctccgcattcggtgcggaaaaaaaaaaaaaaaaaaaaaaaaaaaaaaaaaaaaaaaaaaaaaaaaaaaaaaaaaaaaaaaaaaaaaaaaaaaaaaaaaaaaaaaaaaaaaaaaaaaaaaaaaaaaaaaaaaaaaaaa

SEQ ID NO: 158 - DNA, 6254 bp, synthetic construct
  source 1..6254: mol_type = other DNA
  misc_feature 1..6254: note = G4 DNA vector construct
ttaaaacagcctgtgggttgtacccacccacagggcccactgggcgctagcactctggtatcacggtacctttgtgtgcctgttttatatcccctttccccgattgtaacttagaagatgtacacactgatcaatagcgggcatagcacaccagctatgtcttgatcaagcactcctgtatccccggaccaagtatcaatagactgctcacgcggttgaaggagaaaacgttcgttacccggctaactacttcgagaaacccagtagtatcatgaaagttgcgaggcgtttcgttcagcacacccccagtgtagatcgggtcgatgagtcaccgcatcccccacgggcgaccgtggcggtggctgcgctggcggcctgcctacggggcaacccgtaggacgcttcaatacagacatggtgcgaagagtcgattgagctagttagtagtcctccggcccctgaatgcggctaatcctaactgcggagcacatgccctcaacccagggggtattgtgtcgtaacgggcaactctgcagcggaaccgactactttgggtgtccgtgtttccttttatccttatactggctgcttatggtgacaattgaaagattgttgccatatagctattggattggccatccagtgtctaatagagctgttatttacctctttgttggatttataccactcaacctaaaagaagttaaaacactacagctcattttacaactgaatacagcaaaccaccatgaaactgcctcagctgtgcacagagctgcagacaacaatccacgacatcattctggagtgcgtctactgcaagcagcagcagcagctgctgagaagggaagtgtacgattttgcctttagagacctgtgcattgtgtaccgggacggcaatccttacgctgtgtgcccttacgccgtgtgcgacaagtgtctgaaattctactctaagatcagcgagtaccggcactactgttacagcctgtacggcctgcggctgtgtgtgcagtctacccacgtggacatcagaacactggaggacctgctcatgggcacactgggcaccaccatccacgacatcatcctggaatgcgtctactgcaagcaacagctgctgcggagggaggtgtacgacttcgccttccgggacctgtgcatcgtttatgaggtgtatgacttcgccttcagagacctgtgcatcgtgtatagagatggcaacccctacgccgtgtgcgacaagtgcctgaagttctactccaaggaatacagacactactgctatagcctgtacggcaccacccttgaacaacaatacaacaagcccctgtgcgatctgctgatccgatgtatcaactgccagaagcctctgtgtcccgaagagaagctggacaaaaagcaacggttccacaacatccggggaagatggaccggccggtgtatgagctgctgcagaagcagcagaacccctaccctgcacgagtacatgctggacctccagcctgaaaccaccgactgttacgagcagctgaacgacagttccgaggaggaagatgagatcgacggacctgccggccaggcccctgatagagcccattacaacatcgtgaccttctgttgcaagtgcgacagcacacttagactgtgtgtgacccacgtggacatcagaacactggaggacctgctgatgggcaccctgggcatcgtgtgccccatctgcagccacgagtacatgctggacctgcagcctgagacaaccgacctgtactgctacgagcagctgaatgacagcagcgaagacgagatcgatggaccagctggccaggccgagccagatagagcccactacaacatcgtgacattctgctgcaaatgtgacagcaccctgctccaggtgagactgtacacccagaccgtgtgtgccgaacacccctgcggtcatcctgaccccggcggccctaactttgagccaacaggggtgacggagtcccgcactgaaattacggcaatgcagaccaccggttcatgtgggcaacaatcaggagctgtgtacgtgggcaattacaggattgtaaacagacacctggcaacgagccacgattggcaaaattgcgtgtgggaggactacaacagggatctcctggtcagcacaacaactgctcatggttgtgatactatagcacggtgccaatgtactgctggcgtgtacttttgtgcatctagaaacaagcactacccagtgagcttcgagggtccaggtctagtgaaagttcaggagagcgagtactaccccgagagataccagtcgcacgtactccttgcagttggattttcagaaccgggtgattgtggaggtattttgaggtgtgaacatggagtcattgggctcgttaccatgggtggtgagggtgtagtaggcttcgctgacgtgcgggatcttttgtggttggaagacgacgccatggagcagggtgttagagattatgtagagcaactgggaaatgcatttggctcaggtttcactaaccaaatctgtgagcaagttaacctccttaaagaatctctgatagggcaggattccatattggaaaaatccctgaaggccctggttaaaatcatatcagccctggtgatagtggttaggaaccacgacgacctgattacagtgactgccacactagctttaatcggttgcgcatcatctccatggcgatggctcaaacaaaaagtgtgtcaatactacggaatccccatggcagaaaggcagaataacggttggttaaagaaattcactgaaatgaccaacgcctgcaagggcatggagtggattgctgttaaaattcaaaagttcatcgagtggctcaaagtaaagattctgcctgaagtgaaggagaaacatgagttccttaccagattgaagcaattgccactccttgaaagtcaaattgccaccattgagcaaagcgcaccctcacaaagtgatcaagagcagcttttttcgaatgttcagtacttcgcccattactgcaggaagtatgcacctctgtatgctgccgaagcaaaaagagtgttctcattagaaaagaaaatgagtaattacatacagttcaagtccaaatgccgcattgagcctgtatgcttactccttcacggtagtccaggggctggcaagtcagtagctaccaacctgatagggagatcccttgcagagaagctcaatagctctgtgtactctttaccaccagatccagatcattttgatgggtacaaacagcaggcagtggtgatcatggatgatctctgtcaaaaccccgatgggaaggacgtgtccttgttttgccaaatggtgtctagtgtagattttgtgccacccatggcggcgctggaagaaaaaggcattctctttacgtccccgtttgtgttggcatcaaccaacgcggggtccatcaatgcaccaacagtgtcagacagcagagcacttgccagaaggtttcactttgacatgaatattgaggtgatttcgatgtacagccagaatggtaaaattaacatgcccatgtctgttaagacatgtgatgatgaatgctgcccggtcaatttcaaaaagtgttgcccactagtgtgtggcaaggccatccagtttattgacaggagaaaccaagttagatattcactggacatgctggttactgagatgtttagagagtacaaccacagacacagtgtgggtgctaccctcgaggctttgttccaaggaccaccagtatacagggaaatcaaaatcagtgtggccccggaaacaccccctccaccagcaattgctgaccttctaaaatctgtagacagtgaggcaataagggagtactgcaaggaaaggggttggcttgtgccagaggtcagctccactctacaaattgaaaaacatgttagcagggcatttatttgcttgcaagcgctaactacatttgtttcagtggctggtataatctacatcatttacaagttgtttgccggctttcagggtgcatacactggaatgcccaaccagaaacccaaggtgcccaccttaagacaagctaaggtgcaaggtccggcatttgaatttgccgtagcaatgatgaaaaggaacgccagcacagtcaagacagaatacggtgagttcacgatgcttggcatctatgataaatgggcagtgctgccgcgccacgccaagcctggaccaactattttaatgaatgatcaggaggttggtgtgctcgatgccaaagagttagttgataaagacggaaccaacctggagctgacactattgaagcttaaccgcaatgaaaagttcagagacatcagaggttttcttgcaagggaagaagttgaggtaagtgaggctgttttggcaataaacacgagcaagttcccaagcatgtacatccctgtgggccaagtcaccgattacggatttttaaatctaggtggcaccccaacaaagagaatgctcatgtacaacttccctaccagagcgggacagtgtggtggtgtccttatgtcaacaggaaaggtccttggcatacacgtgggaggaaatggtcaccaaggcttctctgctgctctcctcagacactacttcaacgaggaacagggcgaaatagagtttattgagagctctaaagatgcaggatttcctgtgatcaacacccctaataaaaccaaactggaaccaagtgtgtttcatcaggtttttgagggcaacaaagaaccagcagtcctaagaaacggagacccgcgacttaaagccaactttgaggaagcgatattttccaagtacatcggaaatgtgaacacacatgtggacgagtacatgatagaagctgttgatcactacgctggacagctggcaactctggacatcagtacagaacctatgaagcttgaggatgctgtttatggcactgaaggcttggaagcattggacttgaccactagcgcaggatatccttatgtcgccttgggcatcaagaaaagggatatcctctccaagaagactaaagatctcaccaagctgagggaatgcatggacaagtatggtctaaatctgccgatggtgacctacgtgaaggatgaactcaggtccgctgagaaagtagccaagggaaaatccagacttatagaagcttctagtctcaatgactcagtggccatgaggcagacatttgggaacctatacaagacattccacctcaacccaggcattgtcactggtagtgctgttgggtgcgacccagatgtgttttggagcaaaatacccgtgatgcttgacgggcaccttatagcttttgattactctggctacgacgctagcttgagcccagtgtggtttgcttgtttgaaactcctcctagggaaactagggtatactcataaggaaaccaattacatagactacctctgcaactcccatcacttatacagagataaacactatttcgtgaggggtggtatgccatcaggatgttcaggcaccagtatattcaacaccatgatcaacaacatcattattaggacccttatgctaaaggtctacaaaggtattgacctggatcagtttagaatgatcgcttacggggacgatgtgatagcctcttacccgtggcctattgatgcctcactactagcagaagcgggaaaggattatggtttgatcatgaccccagcagataaaggagagtgttttaatgaggtaacctggacaaatgtaaccttcttgaaaaggtactttagagctgatgaacaatatccattcttggtgcaccccgtgatgcccatgaaagacatacacgaatccattagatggaccaaagacccaaagaacactcaagatcatgtgcgctcgttatgcctattggcttggcacaatggggagcacgaatatgaggaatttatccgaaagatcagaagcgtgcctgttggacgctgtttgaccctcccggtgttctcaacactacgcaggaaatggttagattccttctgataatagaattagagtgcaatcaatgaactatgattggcttaaccctaccgcatgaaccgaactagacaaaagtgcggtaggggtaaattctccgcattcggtgcggaaaaaaaaaaaaaaaaaaaaaaaaaaaaaaaaaaaaaaaaaaaaaaaaaaaaaaaaaaaaaaaaaaaaaaaaaaaaaaaaaaaaaaaaaaaaaaaaaaaaaaaaaaaaaaaaaaaaaaaa

SEQ ID NO: 159 - protein, 158 aa, synthetic construct
  REGION 1..158: note = HPV 16 E6 domain
MHQKRTAMFQDPQERPRKLPQLCTELQTTIHDIILECVYCKQQLLRREVYDFAFRDLCIVYRDGNPYAVCDKCLKFYSKISEYRHYCYSLYGTTLEQQYNKPLCDLLIRCINCQKPLCPEEKQRHLDKKQRFHNIRGRWTGRCMSCCRSSRTRRETQL

SEQ ID NO: 160 - protein, 98 aa, synthetic construct
  REGION 1..98: note = HPV 16 E7 domain
MHGDTPTLHEYMLDLQPETTDLYCYEQLNDSSEEEDEIDGPAGQAEPDRAHYNIVTFCCKCDSTLRLCVQSTHVDIRTLEDLLMGTLGIVCPICSQKP

SEQ ID NO: 161 - DNA, 3605 bp, synthetic construct
  source 1..3605: mol_type = other DNA
  misc_feature 1..3605: note = SFTS B DNA construct
gagaataaactagtattcttctggtccccacagactcaatgatgaaggtgatctggttcagctcccttatctgtctggtgattcagtgttctggcgacaccggccctatcatctgtgccggacccatccatagcaacaagagcgccaatatcccccacctgctgggctacagtgagaaaatctgccagatcgacagactgatccacgtgagcagctggctgagaaaccactctcaatttcagggctacgtaggtcagagaggcggtcggagccaggtgagctactaccctgccgagaactcttatagccggtggtctggattgctgtcgccttgcgacgccgattggctggggatgctggtcgtgaaaaaggccaagggcagcgatatgatcgtgccaggcccttcttataaaggcaaggtgttcttcgaaagacctacatttgacggatatgtgggatggggctgcggctccggcaagagcagaacagaatccggcgagctgtgcagctctgattctggaaccagcagcggactgctgccttctgatagagtgctgtggatcggcgatgtggcctgccagcctatgacccctatacccgaggaaacattcctggaactgaaaagttttagccagagcgagtttcctgacatctgcaagatcgacggaatcgtgtttaaccagtgcgagtctgagagccttcctcagcctttcgacgtggcctggatggatgtgggccacagccacaagatcatcatgagagagcacaagaccaagtgggtgcaggagagcagcagcaaagacttcgtctgctacaaggaaggcaccggcccatgctctgagagcgaggaaaagacctgtaaaaccagtggctcttgcaggggcgacatgcagttctgtaaggttgccgggtgcgaacacggcgaggaggcctctgaggccaagtgcagatgctccctggtgcacaaacctggggaggtggtggtgagctacggcggcatgcgggtgcggcccaagtgctacggcttctccagaatgatggccaccctggaagtgaatcctccagagcagcggatcggccagtgtacaggctgccacctggaatgcattaacggcggagtcaggctgattacactaacctccgagctgaagtctgccacagtgtgcgcgagccacttctgcagcagcgccacaagcggcaagaagtctacagagatccagttccacagcggcagcctggtgggcaagaccgccatccatgtgaagggcgccctggtggacggcacagagttcacctttgagggctcctgcatgttccccgatggctgtgatgccgtggactgcaccttctgcagagagttcctgaagaacccacagtgttaccctgccaagaagtggctgttcatcatcatcgtgatcctgctcggctacgccggactgatgttgctgaccaacgtgctgaaggccatcggcgtgtggggctcctgggtcatcgcccccgtcaagctgatgttcgccatcatcaagaagctgatgcgcagcgtgtcgtgcctgatgggcaagctcatggatagaggcagacaggtgattcacgaggagatcggcgagaacagagagggaaaccaagacgatgtgcggatcgaaatggccagacctcggagagtgcggcactggatgtacagccctgtgatccttacaatcctggccatcggcctggccgaaggctgtgacgagatggtgcacgccgactccaagctggtctcttgcaaacagggctccggaaatatgaaggagtgtgtgaccaccggaagagccctgctgcctgccgtgaaccctggacaggaggcttgcctgcatttcaccgcccctggtagccctgacagcaaatgtctgaaaatcaaagtgaaacgaatcaacctgaagtgcaaaaagtcaagctcttacttcgtgcccgacgcacgatctcggtgtaccagcgttcggcggtgcagatgggccggcgattgccagagcggctgtccttcccatttcacaagcaacagcttcagtgacgactgggccggcaagatggatagagccggcctggggttctccggctgttccgacggctgcggaggagctgcttgtggctgcttcaacgccgctccaagctgcatcttctggagaaagtgggtggaaaatcctcacggcatcatctggaaggtgagcccatgcgctgcctgggtgccctcggctgtcatcgagctgacaatgccttctggcgaagtgcggacatttcaccccatgagcggcatccccacccaggttttcaagggggtgagcgtgacctacctgggcagcgacatggaagtgagcggcctgacagacctgtgcgagatcgaggaactgaaaagcaagaagctggccctggctccttgcaaccaggccggaatgggcgtggtgggaaaggtgggagaaatccaatgtagctccgaagaaagcgccagaaccattaagaaggacgggtgcatctggaacgctgatctggtcggtattgaactgcgagtggacgacgccgtgtgctactccaaaatcaccagtgttgaggccgtcgccaattacagcgccattcccaccactatcggcggactgaggttcgagagaagccacgactctcagggcaagatcagcggcagcccactggacatcacagccatcagaggctcattctccgtgaactaccggggcttgagactgtctctgagcgaaatcaccgccacctgcaccggcgaggtgacaaacgtgtccggctgctacagctgtatgaccggcgccaaggtgtctatcaagctgcactccagcaagaacagcaccgcccacgtgagatgtaaaggcgacgagacagctttcagcgtgctggagggcgtacacagctacaccgtgtccctgagcttcgaccacgccgtggtggacgagcagtgccagctaaactgcggaggccacgaaagccaagtgaccctgaagggcaacctgatcttcctggatgtgcctaagttcgtggacggcagctacatgcaaacataccacagctcagtgcctacgggcgccaacatcccttctccaaccgactggctgaacgctctgtttggcaatggactgagcaggtggattctgggcgtgatcggggtgctgctgggcggcctggccctgttcttcctgataatgagcctgtttaagctgggcaccaagcaggtgttcagatccagaaccaagctggcttgactcgagctggtactgcatgcacgcaatgctagctgcccctttcccgtcctgggtaccccgagtctcccccgacctcgggtcccaggtatgctcccacctccacctgccccactcaccacctctgctagttccagacacctcccaagcacgcagcaatgcagctcaaaacgcttagcctagccacacccccacgggaaacagcagtgattaacctttagcaataaacgaaagtttaactaagctatactaaccccagggttggtcaatttcgtgccagccacaccctggagctagcaaaaaaaaaaaaaaaaaaaaaaaaaaaaaaaaaaaaaaaaaaaaaaaaaa

SEQ ID NO: 162 - RNA, 8858 nt, synthetic construct
  source 1..8858: mol_type = other RNA
  misc_feature 1..8858: note = SARS saRNA construct
ttaaaacagcctgtgggttgtacccacccacagggcccactgggcgctagcactctggtatcacggtacctttgtgtgcctgttttatatcccctttccccgattgtaacttagaagatgtacacactgatcaatagcgggcatagcacaccagctatgtcttgatcaagcactcctgtatccccggaccaagtatcaatagactgctcacgcggttgaaggagaaaacgttcgttacccggctaactacttcgagaaacccagtagtatcatgaaagttgcgaggcgtttcgttcagcacacccccagtgtagatcgggtcgatgagtcaccgcatcccccacgggcgaccgtggcggtggctgcgctggcggcctgcctacggggcaacccgtaggacgcttcaatacagacatggtgcgaagagtcgattgagctagttagtagtcctccggcccctgaatgcggctaatcctaactgcggagcacatgccctcaacccagggggtattgtgtcgtaacgggcaactctgcagcggaaccgactactttgggtgtccgtgtttccttttatccttatactggctgcttatggtgacaattgaaagattgttgccatatagctattggattggccatccagtgtctaatagagctgttatttacctctttgttggatttataccactcaacctaaaagaagttaaaacactacagctcattttacaactgaatacagcaaaccaccatgtttgtgttcctggtgctgctgccactggtgtccagccagtgtgtgaacctgaccaccaggacccaacttcctcctgcctacaccaactccttcaccaggggagtctactaccctgacaaggtgttcaggtcctctgtgctgcacagcacccaggacctgttcctgccattcttcagcaatgtgacctggttccatgccatccatgtgtctggcaccaatggcaccaagaggtttgacaaccctgtgctgccattcaatgatggagtctactttgccagcacagagaagagcaacatcatcaggggctggatttttggcaccaccctggacagcaagacccagtccctgctgattgtgaacaatgccaccaatgtggtgattaaggtgtgtgagttccagttctgtaatgacccattcctgggagtctactaccacaagaacaacaagtcctggatggagtctgagttcagggtctactcctctgccaacaactgtacctttgaatatgtgagccaaccattcctgatggacttggagggcaagcagggcaacttcaagaacctgagggagtttgtgttcaagaacattgatggctacttcaagatttacagcaaacacacaccaatcaacctggtgagggacctgccacagggcttctctgccttggaaccactggtggacctgccaattggcatcaacatcaccaggttccagaccctgctggctctgcacaggtcctacctgacacctggagactcctcctctggctggacagcaggagcagcagcctactatgtgggctacctccaaccaaggaccttcctgctgaaatacaatgagaatggcaccatcacagatgctgtggactgtgccctggacccactgtctgagaccaagtgtaccctgaaatccttcacagtggagaagggcatctaccagaccagcaacttcagggtccaaccaacagagagcattgtgaggtttccaaacatcaccaacctgtgtccatttggagaggtgttcaatgccaccaggtttgcctctgtctatgcctggaacaggaagaggattagcaactgtgtggctgactactctgtgctctacaactctgcctccttcagcaccttcaagtgttatggagtgagcccaaccaaactgaatgacctgtgtttcaccaatgtctatgctgactcctttgtgattaggggagatgaggtgagacagattgcccctggacaaacaggcaagattgctgactacaactacaaactgcctgatgacttcacaggctgtgtgattgcctggaacagcaacaacctggacagcaaggtgggaggcaactacaactacctctacagactgttcaggaagagcaacctgaaaccatttgagagggacatcagcacagagatttaccaggctggcagcacaccatgtaatggagtggagggcttcaactgttactttccactccaatcctatggcttccaaccaaccaatggagtgggctaccaaccatacagggtggtggtgctgtcctttgaactgctccatgcccctgccacagtgtgtggaccaaagaagagcaccaacctggtgaagaacaagtgtgtgaacttcaacttcaatggactgacaggcacaggagtgctgacagagagcaacaagaagttcctgccattccaacagtttggcagggacattgctgacaccacagatgctgtgagggacccacagaccttggagattctggacatcacaccatgttcctttggaggagtgtctgtgattacacctggcaccaacaccagcaaccaggtggctgtgctctaccaggatgtgaactgtactgaggtgcctgtggctatccatgctgaccaacttacaccaacctggagggtctacagcacaggcagcaatgtgttccagaccagggctggctgtctgattggagcagagcatgtgaacaactcctatgagtgtgacatcccaattggagcaggcatctgtgcctcctaccagacccagaccaacagcccaaggagggcaaggtctgtggcaagccagagcatcattgcctacacaatgagtctgggagcagagaactctgtggcttacagcaacaacagcattgccatcccaaccaacttcaccatctctgtgaccacagagattctgcctgtgagtatgaccaagacctctgtggactgtacaatgtatatctgtggagacagcacagagtgtagcaacctgctgctccaatatggctccttctgtacccaacttaacagggctctgacaggcattgctgtggaacaggacaagaacacccaggaggtgtttgcccaggtgaagcagatttacaagacacctccaatcaaggactttggaggcttcaacttcagccagattctgcctgacccaagcaagccaagcaagaggtccttcattgaggacctgctgttcaacaaggtgaccctggctgatgctggcttcatcaagcaatatggagactgtctgggagacattgctgccagggacctgatttgtgcccagaagttcaatggactgacagtgctgcctccactgctgacagatgagatgattgcccaatacacctctgccctgctggctggcaccatcacctctggctggacctttggagcaggagcagccctccaaatcccatttgctatgcagatggcttacaggttcaatggcattggagtgacccagaatgtgctctatgagaaccagaaactgattgccaaccagttcaactctgccattggcaagattcaggactccctgtccagcacagcctctgccctgggcaaactccaagatgtggtgaaccagaatgcccaggctctgaacaccctggtgaagcaactttccagcaactttggagccatctcctctgtgctgaatgacatcctgagcagactggaccctcccgaggctgaggtccagattgacagactgattacaggcagactccaatccctccaaacctatgtgacccaacaacttatcagggctgctgagattagggcatctgccaacctggctgccaccaagatgagtgagtgtgtgctgggacaaagcaagagggtggacttctgtggcaagggctaccacctgatgagttttccacagtctgcccctcatggagtggtgttcctgcatgtgacctatgtgcctgcccaggagaagaacttcaccacagcccctgccatctgccatgatggcaaggctcactttccaagggagggagtgtttgtgagcaatggcacccactggtttgtgacccagaggaacttctatgaaccacagattatcaccacagacaacacctttgtgtctggcaactgtgatgtggtgattggcattgtgaacaacacagtctatgacccactccaacctgaactggactccttcaaggaggaactggacaaatacttcaagaaccacaccagccctgatgtggacctgggagacatctctggcatcaatgcctctgtggtgaacatccagaaggagattgacagactgaatgaggtggctaagaacctgaatgagtccctgattgacctccaagaactgggcaaatatgaacaatacatcaagtggccatggtacatctggctgggcttcattgctggactgattgccattgtgatggtgaccataatgctgtgttgtatgacctcctgttgttcctgtctgaaaggctgttgttcctgtggctcctgttgtaagtttgatgaggatgactctgaacctgtgctgaaaggagtgaaactgcactacaccaactttgagccaacaggggtgacggagtcccgcactgaaattacggcaatgcagaccaccggttcatgtgggcaacaatcaggagctgtgtacgtgggcaattacaggattgtaaacagacacctggcaacgagccacgattggcaaaattgcgtgtgggaggactacaacagggatctcctggtcagcacaacaactgctcatggttgtgatactatagcacggtgccaatgtactgctggcgtgtacttttgtgcatctagaaacaagcactacccagtgagcttcgagggtccaggtctagtgaaagttcaggagagcgagtactaccccgagagataccagtcgcacgtactccttgcagttggattttcagaaccgggtgattgtggaggtattttgaggtgtgaacatggagtcattgggctcgttaccatgggtggtgagggtgtagtaggcttcgctgacgtgcgggatcttttgtggttggaagacgacgccatggagcagggtgttagagattatgtagagcaactgggaaatgcatttggctcaggtttcactaaccaaatctgtgagcaagttaacctccttaaagaatctctgatagggcaggattccatattggaaaaatccctgaaggccctggttaaaatcatatcagccctggtgatagtggttaggaaccacgacgacctgattacagtgactgccacactagctttaatcggttgcgcatcatctccatggcgatggctcaaacaaaaagtgtgtcaatactacggaatccccatggcagaaaggcagaataacggttggttaaagaaattcactgaaatgaccaacgcctgcaagggcatggagtggattgctgttaaaattcaaaagttcatcgagtggctcaaagtaaagattctgcctgaagtgaaggagaaacatgagttccttaccagattgaagcaattgccactccttgaaagtcaaattgccaccattgagcaaagcgcaccctcacaaagtgatcaagagcagcttttttcgaatgttcagtacttcgcccattactgcaggaagtatgcacctctgtatgctgccgaagcaaaaagagtgttctcattagaaaagaaaatgagtaattacatacagttcaagtccaaatgccgcattgagcctgtatgcttactccttcacggtagtccaggggctggcaagtcagtagctaccaacctgatagggagatcccttgcagagaagctcaatagctctgtgtactctttaccaccagatccagatcattttgatgggtacaaacagcaggcagtggtgatcatggatgatctctgtcaaaaccccgatgggaaggacgtgtccttgttttgccaaatggtgtctagtgtagattttgtgccacccatggcggcgctggaagaaaaaggcattctctttacgtccccgtttgtgttggcatcaaccaacgcggggtccatcaatgcaccaacagtgtcagacagcagagcacttgccagaaggtttcactttgacatgaatattgaggtgatttcgatgtacagccagaatggtaaaattaacatgcccatgtctgttaagacatgtgatgatgaatgctgcccggtcaatttcaaaaagtgttgcccactagtgtgtggcaaggccatccagtttattgacaggagaaaccaagttagatattcactggacatgctggttactgagatgtttagagagtacaaccacagacacagtgtgggtgctaccctcgaggctttgttccaaggaccaccagtatacagggaaatcaaaatcagtgtggccccggaaacaccccctccaccagcaattgctgaccttctaaaatctgtagacagtgaggcaataagggagtactgcaaggaaaggggttggcttgtgccagaggtcagctccactctacaaattgaaaaacatgttagcagggcatttatttgcttgcaagcgctaactacatttgtttcagtggctggtataatctacatcatttacaagttgtttgccggctttcagggtgcatacactggaatgcccaaccagaaacccaaggtgcccaccttaagacaagctaaggtgcaaggtccggcatttgaatttgccgtagcaatgatgaaaaggaacgccagcacagtcaagacagaatacggtgagttcacgatgcttggcatctatgataaatgggcagtgctgccgcgccacgccaagcctggaccaactattttaatgaatgatcaggaggttggtgtgctcgatgccaaagagttagttgataaagacggaaccaacctggagctgacactattgaagcttaaccgcaatgaaaagttcagagacatcagaggttttcttgcaagggaagaagttgaggtaagtgaggctgttttggcaataaacacgagcaagttcccaagcatgtacatccctgtgggccaagtcaccgattacggatttttaaatctaggtggcaccccaacaaagagaatgctcatgtacaacttccctaccagagcgggacagtgtggtggtgtccttatgtcaacaggaaaggtccttggcatacacgtgggaggaaatggtcaccaaggcttctctgctgctctcctcagacactacttcaacgaggaacagggcgaaatagagtttattgagagctctaaagatgcaggatttcctgtgatcaacacccctaataaaaccaaactggaaccaagtgtgtttcatcaggtttttgagggcaacaaagaaccagcagtcctaagaaacggagacccgcgacttaaagccaactttgaggaagcgatattttccaagtacatcggaaatgtgaacacacatgtggacgagtacatgatagaagctgttgatcactacgctggacagctggcaactctggacatcagtacagaacctatgaagcttgaggatgctgtttatggcactgaaggcttggaagcattggacttgaccactagcgcaggatatccttatgtcgccttgggcatcaagaaaagggatatcctctccaagaagactaaagatctcaccaagctgagggaatgcatggacaagtatggtctaaatctgccgatggtgacctacgtgaaggatgaactcaggtccgctgagaaagtagccaagggaaaatccagacttatagaagcttctagtctcaatgactcagtggccatgaggcagacatttgggaacctatacaagacattccacctcaacccaggcattgtcactggtagtgctgttgggtgcgacccagatgtgttttggagcaaaatacccgtgatgcttgacgggcaccttatagcttttgattactctggctacgacgctagcttgagcccagtgtggtttgcttgtttgaaactcctcctagggaaactagggtatactcataaggaaaccaattacatagactacctctgcaactcccatcacttatacagagataaacactatttcgtgaggggtggtatgccatcaggatgttcaggcaccagtatattcaacaccatgatcaacaacatcattattaggacccttatgctaaaggtctacaaaggtattgacctggatcagtttagaatgatcgcttacggggacgatgtgatagcctcttacccgtggcctattgatgcctcactactagcagaagcgggaaaggattatggtttgatcatgaccccagcagataaaggagagtgttttaatgaggtaacctggacaaatgtaaccttcttgaaaaggtactttagagctgatgaacaatatccattcttggtgcaccccgtgatgcccatgaaagacatacacgaatccattagatggaccaaagacccaaagaacactcaagatcatgtgcgctcgttatgcctattggcttggcacaatggggagcacgaatatgaggaatttatccgaaagatcagaagcgtgcctgttggacgctgtttgaccctcccggtgttctcaacactacgcaggaaatggttagattccttctgataatagaattagagtgcaatcaatgaactatgattggcttaaccctaccgcatgaaccgaactagacaaaagtgcggtaggggtaaattctccgcattcggtgcggaaaaaaaaaaaaaaaaaaaaaaaaaaaaaaaaaaaaaaaaaaaaaaaaaaaaaaaaaaaaaaaaaaaaaaaaaaaaaaaaaaaaaaaaaaaaaaaaaaaaaaaaaaaaaaaaaaaaaaaa

SEQ ID NO: 163 - DNA, 8858 bp, synthetic construct
  source 1..8858: mol_type = other DNA
  misc_feature 1..8858: note = SARS DNA vector construct
ttaaaacagcctgtgggttgtacccacccacagggcccactgggcgctagcactctggtatcacggtacctttgtgtgcctgttttatatcccctttccccgattgtaacttagaagatgtacacactgatcaatagcgggcatagcacaccagctatgtcttgatcaagcactcctgtatccccggaccaagtatcaatagactgctcacgcggttgaaggagaaaacgttcgttacccggctaactacttcgagaaacccagtagtatcatgaaagttgcgaggcgtttcgttcagcacacccccagtgtagatcgggtcgatgagtcaccgcatcccccacgggcgaccgtggcggtggctgcgctggcggcctgcctacggggcaacccgtaggacgcttcaatacagacatggtgcgaagagtcgattgagctagttagtagtcctccggcccctgaatgcggctaatcctaactgcggagcacatgccctcaacccagggggtattgtgtcgtaacgggcaactctgcagcggaaccgactactttgggtgtccgtgtttccttttatccttatactggctgcttatggtgacaattgaaagattgttgccatatagctattggattggccatccagtgtctaatagagctgttatttacctctttgttggatttataccactcaacctaaaagaagttaaaacactacagctcattttacaactgaatacagcaaaccaccatgtttgtgttcctggtgctgctgccactggtgtccagccagtgtgtgaacctgaccaccaggacccaacttcctcctgcctacaccaactccttcaccaggggagtctactaccctgacaaggtgttcaggtcctctgtgctgcacagcacccaggacctgttcctgccattcttcagcaatgtgacctggttccatgccatccatgtgtctggcaccaatggcaccaagaggtttgacaaccctgtgctgccattcaatgatggagtctactttgccagcacagagaagagcaacatcatcaggggctggatttttggcaccaccctggacagcaagacccagtccctgctgattgtgaacaatgccaccaatgtggtgattaaggtgtgtgagttccagttctgtaatgacccattcctgggagtctactaccacaagaacaacaagtcctggatggagtctgagttcagggtctactcctctgccaacaactgtacctttgaatatgtgagccaaccattcctgatggacttggagggcaagcagggcaacttcaagaacctgagggagtttgtgttcaagaacattgatggctacttcaagatttacagcaaacacacaccaatcaacctggtgagggacctgccacagggcttctctgccttggaaccactggtggacctgccaattggcatcaacatcaccaggttccagaccctgctggctctgcacaggtcctacctgacacctggagactcctcctctggctggacagcaggagcagcagcctactatgtgggctacctccaaccaaggaccttcctgctgaaatacaatgagaatggcaccatcacagatgctgtggactgtgccctggacccactgtctgagaccaagtgtaccctgaaatccttcacagtggagaagggcatctaccagaccagcaacttcagggtccaaccaacagagagcattgtgaggtttccaaacatcaccaacctgtgtccatttggagaggtgttcaatgccaccaggtttgcctctgtctatgcctggaacaggaagaggattagcaactgtgtggctgactactctgtgctctacaactctgcctccttcagcaccttcaagtgttatggagtgagcccaaccaaactgaatgacctgtgtttcaccaatgtctatgctgactcctttgtgattaggggagatgaggtgagacagattgcccctggacaaacaggcaagattgctgactacaactacaaactgcctgatgacttcacaggctgtgtgattgcctggaacagcaacaacctggacagcaaggtgggaggcaactacaactacctctacagactgttcaggaagagcaacctgaaaccatttgagagggacatcagcacagagatttaccaggctggcagcacaccatgtaatggagtggagggcttcaactgttactttccactccaatcctatggcttccaaccaaccaatggagtgggctaccaaccatacagggtggtggtgctgtcctttgaactgctccatgcccctgccacagtgtgtggaccaaagaagagcaccaacctggtgaagaacaagtgtgtgaacttcaacttcaatggactgacaggcacaggagtgctgacagagagcaacaagaagttcctgccattccaacagtttggcagggacattgctgacaccacagatgctgtgagggacccacagaccttggagattctggacatcacaccatgttcctttggaggagtgtctgtgattacacctggcaccaacaccagcaaccaggtggctgtgctctaccaggatgtgaactgtactgaggtgcctgtggctatccatgctgaccaacttacaccaacctggagggtctacagcacaggcagcaatgtgttccagaccagggctggctgtctgattggagcagagcatgtgaacaactcctatgagtgtgacatcccaattggagcaggcatctgtgcctcctaccagacccagaccaacagcccaaggagggcaaggtctgtggcaagccagagcatcattgcctacacaatgagtctgggagcagagaactctgtggcttacagcaacaacagcattgccatcccaaccaacttcaccatctctgtgaccacagagattctgcctgtgagtatgaccaagacctctgtggactgtacaatgtatatctgtggagacagcacagagtgtagcaacctgctgctccaatatggctccttctgtacccaacttaacagggctctgacaggcattgctgtggaacaggacaagaacacccaggaggtgtttgcccaggtgaagcagatttacaagacacctccaatcaaggactttggaggcttcaacttcagccagattctgcctgacccaagcaagccaagcaagaggtccttcattgaggacctgctgttcaacaaggtgaccctggctgatgctggcttcatcaagcaatatggagactgtctgggagacattgctgccagggacctgatttgtgcccagaagttcaatggactgacagtgctgcctccactgctgacagatgagatgattgcccaatacacctctgccctgctggctggcaccatcacctctggctggacctttggagcaggagcagccctccaaatcccatttgctatgcagatggcttacaggttcaatggcattggagtgacccagaatgtgctctatgagaaccagaaactgattgccaaccagttcaactctgccattggcaagattcaggactccctgtccagcacagcctctgccctgggcaaactccaagatgtggtgaaccagaatgcccaggctctgaacaccctggtgaagcaactttccagcaactttggagccatctcctctgtgctgaatgacatcctgagcagactggaccctcccgaggctgaggtccagattgacagactgattacaggcagactccaatccctccaaacctatgtgacccaacaacttatcagggctgctgagattagggcatctgccaacctggctgccaccaagatgagtgagtgtgtgctgggacaaagcaagagggtggacttctgtggcaagggctaccacctgatgagttttccacagtctgcccctcatggagtggtgttcctgcatgtgacctatgtgcctgcccaggagaagaacttcaccacagcccctgccatctgccatgatggcaaggctcactttccaagggagggagtgtttgtgagcaatggcacccactggtttgtgacccagaggaacttctatgaaccacagattatcaccacagacaacacctttgtgtctggcaactgtgatgtggtgattggcattgtgaacaacacagtctatgacccactccaacctgaactggactccttcaaggaggaactggacaaatacttcaagaaccacaccagccctgatgtggacctgggagacatctctggcatcaatgcctctgtggtgaacatccagaaggagattgacagactgaatgaggtggctaagaacctgaatgagtccctgattgacctccaagaactgggcaaatatgaacaatacatcaagtggccatggtacatctggctgggcttcattgctggactgattgccattgtgatggtgaccataatgctgtgttgtatgacctcctgttgttcctgtctgaaaggctgttgttcctgtggctcctgttgtaagtttgatgaggatgactctgaacctgtgctgaaaggagtgaaactgcactacaccaactttgagccaacaggggtgacggagtcccgcactgaaattacggcaatgcagaccaccggttcatgtgggcaacaatcaggagctgtgtacgtgggcaattacaggattgtaaacagacacctggcaacgagccacgattggcaaaattgcgtgtgggaggactacaacagggatctcctggtcagcacaacaactgctcatggttgtgatactatagcacggtgccaatgtactgctggcgtgtacttttgtgcatctagaaacaagcactacccagtgagcttcgagggtccaggtctagtgaaagttcaggagagcgagtactaccccgagagataccagtcgcacgtactccttgcagttggattttcagaaccgggtgattgtggaggtattttgaggtgtgaacatggagtcattgggctcgttaccatgggtggtgagggtgtagtaggcttcgctgacgtgcgggatcttttgtggttggaagacgacgccatggagcagggtgttagagattatgtagagcaactgggaaatgcatttggctcaggtttcactaaccaaatctgtgagcaagttaacctccttaaagaatctctgatagggcaggattccatattggaaaaatccctgaaggccctggttaaaatcatatcagccctggtgatagtggttaggaaccacgacgacctgattacagtgactgccacactagctttaatcggttgcgcatcatctccatggcgatggctcaaacaaaaagtgtgtcaatactacggaatccccatggcagaaaggcagaataacggttggttaaagaaattcactgaaatgaccaacgcctgcaagggcatggagtggattgctgttaaaattcaaaagttcatcgagtggctcaaagtaaagattctgcctgaagtgaaggagaaacatgagttccttaccagattgaagcaattgccactccttgaaagtcaaattgccaccattgagcaaagcgcaccctcacaaagtgatcaagagcagcttttttcgaatgttcagtacttcgcccattactgcaggaagtatgcacctctgtatgctgccgaagcaaaaagagtgttctcattagaaaagaaaatgagtaattacatacagttcaagtccaaatgccgcattgagcctgtatgcttactccttcacggtagtccaggggctggcaagtcagtagctaccaacctgatagggagatcccttgcagagaagctcaatagctctgtgtactctttaccaccagatccagatcattttgatgggtacaaacagcaggcagtggtgatcatggatgatctctgtcaaaaccccgatgggaaggacgtgtccttgttttgccaaatggtgtctagtgtagattttgtgccacccatggcggcgctggaagaaaaaggcattctctttacgtccccgtttgtgttggcatcaaccaacgcggggtccatcaatgcaccaacagtgtcagacagcagagcacttgccagaaggtttcactttgacatgaatattgaggtgatttcgatgtacagccagaatggtaaaattaacatgcccatgtctgttaagacatgtgatgatgaatgctgcccggtcaatttcaaaaagtgttgcccactagtgtgtggcaaggccatccagtttattgacaggagaaaccaagttagatattcactggacatgctggttactgagatgtttagagagtacaaccacagacacagtgtgggtgctaccctcgaggctttgttccaaggaccaccagtatacagggaaatcaaaatcagtgtggccccggaaacaccccctccaccagcaattgctgaccttctaaaatctgtagacagtgaggcaataagggagtactgcaaggaaaggggttggcttgtgccagaggtcagctccactctacaaattgaaaaacatgttagcagggcatttatttgcttgcaagcgctaactacatttgtttcagtggctggtataatctacatcatttacaagttgtttgccggctttcagggtgcatacactggaatgcccaaccagaaacccaaggtgcccaccttaagacaagctaaggtgcaaggtccggcatttgaatttgccgtagcaatgatgaaaaggaacgccagcacagtcaagacagaatacggtgagttcacgatgcttggcatctatgataaatgggcagtgctgccgcgccacgccaagcctggaccaactattttaatgaatgatcaggaggttggtgtgctcgatgccaaagagttagttgataaagacggaaccaacctggagctgacactattgaagcttaaccgcaatgaaaagttcagagacatcagaggttttcttgcaagggaagaagttgaggtaagtgaggctgttttggcaataaacacgagcaagttcccaagcatgtacatccctgtgggccaagtcaccgattacggatttttaaatctaggtggcaccccaacaaagagaatgctcatgtacaacttccctaccagagcgggacagtgtggtggtgtccttatgtcaacaggaaaggtccttggcatacacgtgggaggaaatggtcaccaaggcttctctgctgctctcctcagacactacttcaacgaggaacagggcgaaatagagtttattgagagctctaaagatgcaggatttcctgtgatcaacacccctaataaaaccaaactggaaccaagtgtgtttcatcaggtttttgagggcaacaaagaaccagcagtcctaagaaacggagacccgcgacttaaagccaactttgaggaagcgatattttccaagtacatcggaaatgtgaacacacatgtggacgagtacatgatagaagctgttgatcactacgctggacagctggcaactctggacatcagtacagaacctatgaagcttgaggatgctgtttatggcactgaaggcttggaagcattggacttgaccactagcgcaggatatccttatgtcgccttgggcatcaagaaaagggatatcctctccaagaagactaaagatctcaccaagctgagggaatgcatggacaagtatggtctaaatctgccgatggtgacctacgtgaaggatgaactcaggtccgctgagaaagtagccaagggaaaatccagacttatagaagcttctagtctcaatgactcagtggccatgaggcagacatttgggaacctatacaagacattccacctcaacccaggcattgtcactggtagtgctgttgggtgcgacccagatgtgttttggagcaaaatacccgtgatgcttgacgggcaccttatagcttttgattactctggctacgacgctagcttgagcccagtgtggtttgcttgtttgaaactcctcctagggaaactagggtatactcataaggaaaccaattacatagactacctctgcaactcccatcacttatacagagataaacactatttcgtgaggggtggtatgccatcaggatgttcaggcaccagtatattcaacaccatgatcaacaacatcattattaggacccttatgctaaaggtctacaaaggtattgacctggatcagtttagaatgatcgcttacggggacgatgtgatagcctcttacccgtggcctattgatgcctcactactagcagaagcgggaaaggattatggtttgatcatgaccccagcagataaaggagagtgttttaatgaggtaacctggacaaatgtaaccttcttgaaaaggtactttagagctgatgaacaatatccattcttggtgcaccccgtgatgcccatgaaagacatacacgaatccattagatggaccaaagacccaaagaacactcaagatcatgtgcgctcgttatgcctattggcttggcacaatggggagcacgaatatgaggaatttatccgaaagatcagaagcgtgcctgttggacgctgtttgaccctcccggtgttctcaacactacgcaggaaatggttagattccttctgataatagaattagagtgcaatcaatgaactatgattggcttaaccctaccgcatgaaccgaactagacaaaagtgcggtaggggtaaattctccgcattcggtgcggaaaaaaaaaaaaaaaaaaaaaaaaaaaaaaaaaaaaaaaaaaaaaaaaaaaaaaaaaaaaaaaaaaaaaaaaaaaaaaaaaaaaaaaaaaaaaaaaaaaaaaaaaaaaaaaaaaaaaaaa

SEQ ID NO: 164 - RNA, 4205 nt, synthetic construct
  source 1..4205: mol_type = other RNA
  misc_feature 1..4205: note = SARS mRNA construct
gagaataaactagtattcttctggtccccacagactcaatgtttgtgttcctggtgctgctgccactggtgtccagccagtgtgtgaacctgaccaccaggacccaacttcctcctgcctacaccaactccttcaccaggggagtctactaccctgacaaggtgttcaggtcctctgtgctgcacagcacccaggacctgttcctgccattcttcagcaatgtgacctggttccatgccatccatgtgtctggcaccaatggcaccaagaggtttgacaaccctgtgctgccattcaatgatggagtctactttgccagcacagagaagagcaacatcatcaggggctggatttttggcaccaccctggacagcaagacccagtccctgctgattgtgaacaatgccaccaatgtggtgattaaggtgtgtgagttccagttctgtaatgacccattcctgggagtctactaccacaagaacaacaagtcctggatggagtctgagttcagggtctactcctctgccaacaactgtacctttgaatatgtgagccaaccattcctgatggacttggagggcaagcagggcaacttcaagaacctgagggagtttgtgttcaagaacattgatggctacttcaagatttacagcaaacacacaccaatcaacctggtgagggacctgccacagggcttctctgccttggaaccactggtggacctgccaattggcatcaacatcaccaggttccagaccctgctggctctgcacaggtcctacctgacacctggagactcctcctctggctggacagcaggagcagcagcctactatgtgggctacctccaaccaaggaccttcctgctgaaatacaatgagaatggcaccatcacagatgctgtggactgtgccctggacccactgtctgagaccaagtgtaccctgaaatccttcacagtggagaagggcatctaccagaccagcaacttcagggtccaaccaacagagagcattgtgaggtttccaaacatcaccaacctgtgtccatttggagaggtgttcaatgccaccaggtttgcctctgtctatgcctggaacaggaagaggattagcaactgtgtggctgactactctgtgctctacaactctgcctccttcagcaccttcaagtgttatggagtgagcccaaccaaactgaatgacctgtgtttcaccaatgtctatgctgactcctttgtgattaggggagatgaggtgagacagattgcccctggacaaacaggcaagattgctgactacaactacaaactgcctgatgacttcacaggctgtgtgattgcctggaacagcaacaacctggacagcaaggtgggaggcaactacaactacctctacagactgttcaggaagagcaacctgaaaccatttgagagggacatcagcacagagatttaccaggctggcagcacaccatgtaatggagtggagggcttcaactgttactttccactccaatcctatggcttccaaccaaccaatggagtgggctaccaaccatacagggtggtggtgctgtcctttgaactgctccatgcccctgccacagtgtgtggaccaaagaagagcaccaacctggtgaagaacaagtgtgtgaacttcaacttcaatggactgacaggcacaggagtgctgacagagagcaacaagaagttcctgccattccaacagtttggcagggacattgctgacaccacagatgctgtgagggacccacagaccttggagattctggacatcacaccatgttcctttggaggagtgtctgtgattacacctggcaccaacaccagcaaccaggtggctgtgctctaccaggatgtgaactgtactgaggtgcctgtggctatccatgctgaccaacttacaccaacctggagggtctacagcacaggcagcaatgtgttccagaccagggctggctgtctgattggagcagagcatgtgaacaactcctatgagtgtgacatcccaattggagcaggcatctgtgcctcctaccagacccagaccaacagcccaaggagggcaaggtctgtggcaagccagagcatcattgcctacacaatgagtctgggagcagagaactctgtggcttacagcaacaacagcattgccatcccaaccaacttcaccatctctgtgaccacagagattctgcctgtgagtatgaccaagacctctgtggactgtacaatgtatatctgtggagacagcacagagtgtagcaacctgctgctccaatatggctccttctgtacccaacttaacagggctctgacaggcattgctgtggaacaggacaagaacacccaggaggtgtttgcccaggtgaagcagatttacaagacacctccaatcaaggactttggaggcttcaacttcagccagattctgcctgacccaagcaagccaagcaagaggtccttcattgaggacctgctgttcaacaaggtgaccctggctgatgctggcttcatcaagcaatatggagactgtctgggagacattgctgccagggacctgatttgtgcccagaagttcaatggactgacagtgctgcctccactgctgacagatgagatgattgcccaatacacctctgccctgctggctggcaccatcacctctggctggacctttggagcaggagcagccctccaaatcccatttgctatgcagatggcttacaggttcaatggcattggagtgacccagaatgtgctctatgagaaccagaaactgattgccaaccagttcaactctgccattggcaagattcaggactccctgtccagcacagcctctgccctgggcaaactccaagatgtggtgaaccagaatgcccaggctctgaacaccctggtgaagcaactttccagcaactttggagccatctcctctgtgctgaatgacatcctgagcagactggaccctcccgaggctgaggtccagattgacagactgattacaggcagactccaatccctccaaacctatgtgacccaacaacttatcagggctgctgagattagggcatctgccaacctggctgccaccaagatgagtgagtgtgtgctgggacaaagcaagagggtggacttctgtggcaagggctaccacctgatgagttttccacagtctgcccctcatggagtggtgttcctgcatgtgacctatgtgcctgcccaggagaagaacttcaccacagcccctgccatctgccatgatggcaaggctcactttccaagggagggagtgtttgtgagcaatggcacccactggtttgtgacccagaggaacttctatgaaccacagattatcaccacagacaacacctttgtgtctggcaactgtgatgtggtgattggcattgtgaacaacacagtctatgacccactccaacctgaactggactccttcaaggaggaactggacaaatacttcaagaaccacaccagccctgatgtggacctgggagacatctctggcatcaatgcctctgtggtgaacatccagaaggagattgacagactgaatgaggtggctaagaacctgaatgagtccctgattgacctccaagaactgggcaaatatgaacaatacatcaagtggccatggtacatctggctgggcttcattgctggactgattgccattgtgatggtgaccataatgctgtgttgtatgacctcctgttgttcctgtctgaaaggctgttgttcctgtggctcctgttgtaagtttgatgaggatgactctgaacctgtgctgaaaggagtgaaactgcactacacctaactcgagctggtactgcatgcacgcaatgctagctgcccctttcccgtcctgggtaccccgagtctcccccgacctcgggtcccaggtatgctcccacctccacctgccccactcaccacctctgctagttccagacacctcccaagcacgcagcaatgcagctcaaaacgcttagcctagccacacccccacgggaaacagcagtgattaacctttagcaataaacgaaagtttaactaagctatactaaccccagggttggtcaatttcgtgccagccacaccctggagctagcaaaaaaaaaaaaaaaaaaaaaaaaaaaaaaaaaaaaaaaaaaaaaaaaaa

SEQ ID NO: 165 - DNA, 4205 bp, synthetic construct
  source 1..4205: mol_type = other DNA
  misc_feature 1..4205: note = SARS DNA construct
gagaataaactagtattcttctggtccccacagactcaatgtttgtgttcctggtgctgctgccactggtgtccagccagtgtgtgaacctgaccaccaggacccaacttcctcctgcctacaccaactccttcaccaggggagtctactaccctgacaaggtgttcaggtcctctgtgctgcacagcacccaggacctgttcctgccattcttcagcaatgtgacctggttccatgccatccatgtgtctggcaccaatggcaccaagaggtttgacaaccctgtgctgccattcaatgatggagtctactttgccagcacagagaagagcaacatcatcaggggctggatttttggcaccaccctggacagcaagacccagtccctgctgattgtgaacaatgccaccaatgtggtgattaaggtgtgtgagttccagttctgtaatgacccattcctgggagtctactaccacaagaacaacaagtcctggatggagtctgagttcagggtctactcctctgccaacaactgtacctttgaatatgtgagccaaccattcctgatggacttggagggcaagcagggcaacttcaagaacctgagggagtttgtgttcaagaacattgatggctacttcaagatttacagcaaacacacaccaatcaacctggtgagggacctgccacagggcttctctgccttggaaccactggtggacctgccaattggcatcaacatcaccaggttccagaccctgctggctctgcacaggtcctacctgacacctggagactcctcctctggctggacagcaggagcagcagcctactatgtgggctacctccaaccaaggaccttcctgctgaaatacaatgagaatggcaccatcacagatgctgtggactgtgccctggacccactgtctgagaccaagtgtaccctgaaatccttcacagtggagaagggcatctaccagaccagcaacttcagggtccaaccaacagagagcattgtgaggtttccaaacatcaccaacctgtgtccatttggagaggtgttcaatgccaccaggtttgcctctgtctatgcctggaacaggaagaggattagcaactgtgtggctgactactctgtgctctacaactctgcctccttcagcaccttcaagtgttatggagtgagcccaaccaaactgaatgacctgtgtttcaccaatgtctatgctgactcctttgtgattaggggagatgaggtgagacagattgcccctggacaaacaggcaagattgctgactacaactacaaactgcctgatgacttcacaggctgtgtgattgcctggaacagcaacaacctggacagcaaggtgggaggcaactacaactacctctacagactgttcaggaagagcaacctgaaaccatttgagagggacatcagcacagagatttaccaggctggcagcacaccatgtaatggagtggagggcttcaactgttactttccactccaatcctatggcttccaaccaaccaatggagtgggctaccaaccatacagggtggtggtgctgtcctttgaactgctccatgcccctgccacagtgtgtggaccaaagaagagcaccaacctggtgaagaacaagtgtgtgaacttcaacttcaatggactgacaggcacaggagtgctgacagagagcaacaagaagttcctgccattccaacagtttggcagggacattgctgacaccacagatgctgtgagggacccacagaccttggagattctggacatcacaccatgttcctttggaggagtgtctgtgattacacctggcaccaacaccagcaaccaggtggctgtgctctaccaggatgtgaactgtactgaggtgcctgtggctatccatgctgaccaacttacaccaacctggagggtctacagcacaggcagcaatgtgttccagaccagggctggctgtctgattggagcagagcatgtgaacaactcctatgagtgtgacatcccaattggagcaggcatctgtgcctcctaccagacccagaccaacagcccaaggagggcaaggtctgtggcaagccagagcatcattgcctacacaatgagtctgggagcagagaactctgtggcttacagcaacaacagcattgccatcccaaccaacttcaccatctctgtgaccacagagattctgcctgtgagtatgaccaagacctctgtggactgtacaatgtatatctgtggagacagcacagagtgtagcaacctgctgctccaatatggctccttctgtacccaacttaacagggctctgacaggcattgctgtggaacaggacaagaacacccaggaggtgtttgcccaggtgaagcagatttacaagacacctccaatcaaggactttggaggcttcaacttcagccagattctgcctgacccaagcaagccaagcaagaggtccttcattgaggacctgctgttcaacaaggtgaccctggctgatgctggcttcatcaagcaatatggagactgtctgggagacattgctgccagggacctgatttgtgcccagaagttcaatggactgacagtgctgcctccactgctgacagatgagatgattgcccaatacacctctgccctgctggctggcaccatcacctctggctggacctttggagcaggagcagccctccaaatcccatttgctatgcagatggcttacaggttcaatggcattggagtgacccagaatgtgctctatgagaaccagaaactgattgccaaccagttcaactctgccattggcaagattcaggactccctgtccagcacagcctctgccctgggcaaactccaagatgtggtgaaccagaatgcccaggctctgaacaccctggtgaagcaactttccagcaactttggagccatctcctctgtgctgaatgacatcctgagcagactggaccctcccgaggctgaggtccagattgacagactgattacaggcagactccaatccctccaaacctatgtgacccaacaacttatcagggctgctgagattagggcatctgccaacctggctgccaccaagatgagtgagtgtgtgctgggacaaagcaagagggtggacttctgtggcaagggctaccacctgatgagttttccacagtctgcccctcatggagtggtgttcctgcatgtgacctatgtgcctgcccaggagaagaacttcaccacagcccctgccatctgccatgatggcaaggctcactttccaagggagggagtgtttgtgagcaatggcacccactggtttgtgacccagaggaacttctatgaaccacagattatcaccacagacaacacctttgtgtctggcaactgtgatgtggtgattggcattgtgaacaacacagtctatgacccactccaacctgaactggactccttcaaggaggaactggacaaatacttcaagaaccacaccagccctgatgtggacctgggagacatctctggcatcaatgcctctgtggtgaacatccagaaggagattgacagactgaatgaggtggctaagaacctgaatgagtccctgattgacctccaagaactgggcaaatatgaacaatacatcaagtggccatggtacatctggctgggcttcattgctggactgattgccattgtgatggtgaccataatgctgtgttgtatgacctcctgttgttcctgtctgaaaggctgttgttcctgtggctcctgttgtaagtttgatgaggatgactctgaacctgtgctgaaaggagtgaaactgcactacacctaactcgagctggtactgcatgcacgcaatgctagctgcccctttcccgtcctgggtaccccgagtctcccccgacctcgggtcccaggtatgctcccacctccacctgccccactcaccacctctgctagttccagacacctcccaagcacgcagcaatgcagctcaaaacgcttagcctagccacacccccacgggaaacagcagtgattaacctttagcaataaacgaaagtttaactaagctatactaaccccagggttggtcaatttcgtgccagccacaccctggagctagcaaaaaaaaaaaaaaaaaaaaaaaaaaaaaaaaaaaaaaaaaaaaaaaaaa

SEQ ID NO: 166 - DNA, 6731 bp, synthetic construct
  source 1..6731: mol_type = other DNA
  misc_feature 1..6731: note = H5N8 DNA vector construct
ttaaaacagcctgtgggttgtacccacccacagggcccactgggcgctagcactctggtatcacggtacctttgtgtgcctgttttatatcccctttccccgattgtaacttagaagatgtacacactgatcaatagcgggcatagcacaccagctatgtcttgatcaagcactcctgtatccccggaccaagtatcaatagactgctcacgcggttgaaggagaaaacgttcgttacccggctaactacttcgagaaacccagtagtatcatgaaagttgcgaggcgtttcgttcagcacacccccagtgtagatcgggtcgatgagtcaccgcatcccccacgggcgaccgtggcggtggctgcgctggcggcctgcctacggggcaacccgtaggacgcttcaatacagacatggtgcgaagagtcgattgagctagttagtagtcctccggcccctgaatgcggctaatcctaactgcggagcacatgccctcaacccagggggtattgtgtcgtaacgggcaactctgcagcggaaccgactactttgggtgtccgtgtttccttttatccttatactggctgcttatggtgacaattgaaagattgttgccatatagctattggattggccatccagtgtctaatagagctgttatttacctctttgttggatttataccactcaacctaaaagaagttaaaacactacagctcattttacaactgaatacagcaaaccaccatggaaaagatcgtgctgctgctggccgtggtgtccctggtcaaaagcgaccagatctgcatcggctaccacgccaacaacagcaccaaacaggtggacaccatcatggaaaaaaacgtgaccgtgacacacgcccaggacatcctggaaaagacccacaacggcaagctgtgcgacctgaacggcgtgaagcctctgatcctgaaggactgttctgtggccggatggctgctgggcaaccctatgtgtgacgagttcatcagagtgcccgagtggtcctacatcgtggaaagagctaaccccgccaacgacctgtgctaccctggcacactgaacgactacgaggaactgaagcacctcctgagcagaatcaaccacttcgagaaaaccctgatcatccccaagagcagctggcccaaccacgagacatctctgggagtgtctgccgcatgtccataccagggcgctcccagcttcttcagaaacgtcgtgtggctgatcaagaagaacgacgcttaccccaccatcaagatcagctacaacaacaccaaccgcgaggacctgctgatcctgtggggaatccaccactctaacaacgccgccgagcagaccaacctgtacaagaaccctgacacctacgtgtccgtgggcacaagcaccctgaaccagagactggtgcccaagatcgccaccagatctcaagtgaacggccagaggggcagaatggacttcttctggaccatcctgaagcctaacgacgccatccactttgagagcaacggcaactttatcgcccctgagtacgcctacaagatcgtgaagaagggcgacagcacaatcatgaagtccgagatggaatacggccactgcaacaccaagtgtcagacccctatcggcgccatcaactccagcatgcccttccacaacatccatcctctgaccatcggcgagtgccccaaatacgtgaagtccaacaagctggtgctggccaccggcctgagaaactctccactgagagagacggtaggcctgtttggcgctatcgccggctttattgaaggcggctggcaaggcatggtggacggatggtacggctatcaccacagcaacgagcaaggctctggctacgccgctgacaaagagagcacccagaaagccatcgacggcgtgaccaacaaagtgaacagcatcatcgacaagatgaacacccagttcgaggccgtgggcagagagttcaacaacctggaaagaaggatcgagaacctcaacaagaaaatggaagatggcttcctggacgtgtggacctacaacgctgagctgctggtcctgatggaaaacgagagaaccctggacttccacgacagcaacgtgaagaacctgtacgacaaagtgcggctgcagctgagagacaacgccaaagaactcggcaacggctgcttcgagttctaccacaagtgcgacaacgagtgcatggaaagcgtgcggaacggcacctacgactaccccaagtacagcgaggaagccagactgaagagagaagagatcagcggagtgaagctggaatccatcggcacataccagatcctgagcatctacagcaccgtggcctcttctctggccctggctatcattgtggctggcctgagcctgtggatgtgcagcaatggcagcctgcagtgcagaatctgcatcaactttgagccaacaggggtgacggagtcccgcactgaaattacggcaatgcagaccaccggttcatgtgggcaacaatcaggagctgtgtacgtgggcaattacaggattgtaaacagacacctggcaacgagccacgattggcaaaattgcgtgtgggaggactacaacagggatctcctggtcagcacaacaactgctcatggttgtgatactatagcacggtgccaatgtactgctggcgtgtacttttgtgcatctagaaacaagcactacccagtgagcttcgagggtccaggtctagtgaaagttcaggagagcgagtactaccccgagagataccagtcgcacgtactccttgcagttggattttcagaaccgggtgattgtggaggtattttgaggtgtgaacatggagtcattgggctcgttaccatgggtggtgagggtgtagtaggcttcgctgacgtgcgggatcttttgtggttggaagacgacgccatggagcagggtgttagagattatgtagagcaactgggaaatgcatttggctcaggtttcactaaccaaatctgtgagcaagttaacctccttaaagaatctctgatagggcaggattccatattggaaaaatccctgaaggccctggttaaaatcatatcagccctggtgatagtggttaggaaccacgacgacctgattacagtgactgccacactagctttaatcggttgcgcatcatctccatggcgatggctcaaacaaaaagtgtgtcaatactacggaatccccatggcagaaaggcagaataacggttggttaaagaaattcactgaaatgaccaacgcctgcaagggcatggagtggattgctgttaaaattcaaaagttcatcgagtggctcaaagtaaagattctgcctgaagtgaaggagaaacatgagttccttaccagattgaagcaattgccactccttgaaagtcaaattgccaccattgagcaaagcgcaccctcacaaagtgatcaagagcagcttttttcgaatgttcagtacttcgcccattactgcaggaagtatgcacctctgtatgctgccgaagcaaaaagagtgttctcattagaaaagaaaatgagtaattacatacagttcaagtccaaatgccgcattgagcctgtatgcttactccttcacggtagtccaggggctggcaagtcagtagctaccaacctgatagggagatcccttgcagagaagctcaatagctctgtgtactctttaccaccagatccagatcattttgatgggtacaaacagcaggcagtggtgatcatggatgatctctgtcaaaaccccgatgggaaggacgtgtccttgttttgccaaatggtgtctagtgtagattttgtgccacccatggcggcgctggaagaaaaaggcattctctttacgtccccgtttgtgttggcatcaaccaacgcggggtccatcaatgcaccaacagtgtcagacagcagagcacttgccagaaggtttcactttgacatgaatattgaggtgatttcgatgtacagccagaatggtaaaattaacatgcccatgtctgttaagacatgtgatgatgaatgctgcccggtcaatttcaaaaagtgttgcccactagtgtgtggcaaggccatccagtttattgacaggagaaaccaagttagatattcactggacatgctggttactgagatgtttagagagtacaaccacagacacagtgtgggtgctaccctcgaggctttgttccaaggaccaccagtatacagggaaatcaaaatcagtgtggccccggaaacaccccctccaccagcaattgctgaccttctaaaatctgtagacagtgaggcaataagggagtactgcaaggaaaggggttggcttgtgccagaggtcagctccactctacaaattgaaaaacatgttagcagggcatttatttgcttgcaagcgctaactacatttgtttcagtggctggtataatctacatcatttacaagttgtttgccggctttcagggtgcatacactggaatgcccaaccagaaacccaaggtgcccaccttaagacaagctaaggtgcaaggtccggcatttgaatttgccgtagcaatgatgaaaaggaacgccagcacagtcaagacagaatacggtgagttcacgatgcttggcatctatgataaatgggcagtgctgccgcgccacgccaagcctggaccaactattttaatgaatgatcaggaggttggtgtgctcgatgccaaagagttagttgataaagacggaaccaacctggagctgacactattgaagcttaaccgcaatgaaaagttcagagacatcagaggttttcttgcaagggaagaagttgaggtaagtgaggctgttttggcaataaacacgagcaagttcccaagcatgtacatccctgtgggccaagtcaccgattacggatttttaaatctaggtggcaccccaacaaagagaatgctcatgtacaacttccctaccagagcgggacagtgtggtggtgtccttatgtcaacaggaaaggtccttggcatacacgtgggaggaaatggtcaccaaggcttctctgctgctctcctcagacactacttcaacgaggaacagggcgaaatagagtttattgagagctctaaagatgcaggatttcctgtgatcaacacccctaataaaaccaaactggaaccaagtgtgtttcatcaggtttttgagggcaacaaagaaccagcagtcctaagaaacggagacccgcgacttaaagccaactttgaggaagcgatattttccaagtacatcggaaatgtgaacacacatgtggacgagtacatgatagaagctgttgatcactacgctggacagctggcaactctggacatcagtacagaacctatgaagcttgaggatgctgtttatggcactgaaggcttggaagcattggacttgaccactagcgcaggatatccttatgtcgccttgggcatcaagaaaagggatatcctctccaagaagactaaagatctcaccaagctgagggaatgcatggacaagtatggtctaaatctgccgatggtgacctacgtgaaggatgaactcaggtccgctgagaaagtagccaagggaaaatccagacttatagaagcttctagtctcaatgactcagtggccatgaggcagacatttgggaacctatacaagacattccacctcaacccaggcattgtcactggtagtgctgttgggtgcgacccagatgtgttttggagcaaaatacccgtgatgcttgacgggcaccttatagcttttgattactctggctacgacgctagcttgagcccagtgtggtttgcttgtttgaaactcctcctagggaaactagggtatactcataaggaaaccaattacatagactacctctgcaactcccatcacttatacagagataaacactatttcgtgaggggtggtatgccatcaggatgttcaggcaccagtatattcaacaccatgatcaacaacatcattattaggacccttatgctaaaggtctacaaaggtattgacctggatcagtttagaatgatcgcttacggggacgatgtgatagcctcttacccgtggcctattgatgcctcactactagcagaagcgggaaaggattatggtttgatcatgaccccagcagataaaggagagtgttttaatgaggtaacctggacaaatgtaaccttcttgaaaaggtactttagagctgatgaacaatatccattcttggtgcaccccgtgatgcccatgaaagacatacacgaatccattagatggaccaaagacccaaagaacactcaagatcatgtgcgctcgttatgcctattggcttggcacaatggggagcacgaatatgaggaatttatccgaaagatcagaagcgtgcctgttggacgctgtttgaccctcccggtgttctcaacactacgcaggaaatggttagattccttctgataatagaattagagtgcaatcaatgaactatgattggcttaaccctaccgcatgaaccgaactagacaaaagtgcggtaggggtaaattctccgcattcggtgcggaaaaaaaaaaaaaaaaaaaaaaaaaaaaaaaaaaaaaaaaaaaaaaaaaaaaaaaaaaaaaaaaaaaaaaaaaaaaaaaaaaaaaaaaaaaaaaaaaaaaaaaaaaaaaaaaaaaaaaaa

SEQ ID NO: 167 - DNA, 6146 bp, synthetic construct
  source 1..6146: mol_type = other DNA
  misc_feature 1..6146: note = H5N8 DNA construct
gagaataaactagtattcttctggtccccacagactcaatggaaaagatcgtgctgctgctggccgtggtgtccctggtcaaaagcgaccagatctgcatcggctaccacgccaacaacagcaccaaacaggtggacaccatcatggaaaaaaacgtgaccgtgacacacgcccaggacatcctggaaaagacccacaacggcaagctgtgcgacctgaacggcgtgaagcctctgatcctgaaggactgttctgtggccggatggctgctgggcaaccctatgtgtgacgagttcatcagagtgcccgagtggtcctacatcgtggaaagagctaaccccgccaacgacctgtgctaccctggcacactgaacgactacgaggaactgaagcacctcctgagcagaatcaaccacttcgagaaaaccctgatcatccccaagagcagctggcccaaccacgagacatctctgggagtgtctgccgcatgtccataccagggcgctcccagcttcttcagaaacgtcgtgtggctgatcaagaagaacgacgcttaccccaccatcaagatcagctacaacaacaccaaccgcgaggacctgctgatcctgtggggaatccaccactctaacaacgccgccgagcagaccaacctgtacaagaaccctgacacctacgtgtccgtgggcacaagcaccctgaaccagagactggtgcccaagatcgccaccagatctcaagtgaacggccagaggggcagaatggacttcttctggaccatcctgaagcctaacgacgccatccactttgagagcaacggcaactttatcgcccctgagtacgcctacaagatcgtgaagaagggcgacagcacaatcatgaagtccgagatggaatacggccactgcaacaccaagtgtcagacccctatcggcgccatcaactccagcatgcccttccacaacatccatcctctgaccatcggcgagtgccccaaatacgtgaagtccaacaagctggtgctggccaccggcctgagaaactctccactgagagagacggtaggcctgtttggcgctatcgccggctttattgaaggcggctggcaaggcatggtggacggatggtacggctatcaccacagcaacgagcaaggctctggctacgccgctgacaaagagagcacccagaaagccatcgacggcgtgaccaacaaagtgaacagcatcatcgacaagatgaacacccagttcgaggccgtgggcagagagttcaacaacctggaaagaaggatcgagaacctcaacaagaaaatggaagatggcttcctggacgtgtggacctacaacgctgagctgctggtcctgatggaaaacgagagaaccctggacttccacgacagcaacgtgaagaacctgtacgacaaagtgcggctgcagctgagagacaacgccaaagaactcggcaacggctgcttcgagttctaccacaagtgcgacaacgagtgcatggaaagcgtgcggaacggcacctacgactaccccaagtacagcgaggaagccagactgaagagagaagagatcagcggagtgaagctggaatccatcggcacataccagatcctgagcatctacagcaccgtggcctcttctctggccctggctatcattgtggctggcctgagcctgtggatgtgcagcaatggcagcctgcagtgcagaatctgcatcaactttgagccaacaggggtgacggagtcccgcactgaaattacggcaatgcagaccaccggttcatgtgggcaacaatcaggagctgtgtacgtgggcaattacaggattgtaaacagacacctggcaacgagccacgattggcaaaattgcgtgtgggaggactacaacagggatctcctggtcagcacaacaactgctcatggttgtgatactatagcacggtgccaatgtactgctggcgtgtacttttgtgcatctagaaacaagcactacccagtgagcttcgagggtccaggtctagtgaaagttcaggagggcgagtactaccccgagagataccagtcgcacgtactccttgcagttggattttcagaaccgggtgattgtggaggtattttgaggtgtgaacatggagtcattgggctcgttaccatgggtggtgagggtgtagtaggcttcgctgacgtgcgggatcttttgtggttggaagacgacgccatggagcagggtgttagagattatgtagagcaactgggaaatgcatttggctcaggtttcactaaccaaatctgtgagcaagttaacctccttaaagaatctctgatagggcaggattccatattggaaaaatccctgaaggccctggttaaaatcatatcagccctggtgatagtggttaggaaccacgacgacctgattacagtgactgccacactagctttaatcggttgcgcatcatctccatggcgatggctcaaacaaaaagtgtgtcaatactacggaatccccatggcagaaaggcagaataacggttggttaaagaaattcactgaaatgaccaacgcctgcaagggcatggagtggattgctgttaaaattcaaaagttcatcgagtggctcaaagtaaagattctgcctgaagtgaaggagaaacatgagttccttaccagattgaagcaattgccactccttgaaagtcaaattgccaccattgagcaaagcgcaccctcacaaagtgatcaagagcagcttttttcgaatgttcagtacttcgcccattactgcaggaagtatgcacctctgtatgctgccgaagcaaaaagagtgttctcattagaaaagaaaatgagtaattacatacagttcaagtccaaatgccgcattgagcctgtatgcttactccttcacggtagtccaggggctggcaagtcagtagctaccaacctgatagggagatcccttgcagagaagctcaatagctctgtgtactctttaccaccagatccagatcattttgatgggtacaaacagcaggcagtggtgatcatggatgatctctgtcaaaaccccgatgggaaggacgtgtccttgttttgccaaatggtgtctagtgtagattttgtgccacccatggcggcgctggaagaaaaaggcattctctttacgtccccgtttgtgttggcatcaaccaacgcggggtccatcaatgcaccaacagtgtcagacagcagagcacttgccagaaggtttcactttgacatgaatattgaggtgatttcgatgtacagccagaatggtaaaattaacatgcccatgtctgttaagacatgtgatgatgaatgctgcccggtcaatttcaaaaagtgttgcccactagtgtgtggcaaggccatccagtttattgacaggagaaaccaagttagatattcactggacatgctggttactgagatgtttagagagtacaaccacagacacagtgtgggtgctaccctcgaggctttgttccaaggaccaccagtatacagggaaatcaaaatcagtgtggccccggaaacaccccctccaccagcaattgctgaccttctaaaatctgtagacagtgaggcaataagggagtactgcaaggaaaggggttggcttgtgccagaggtcagctccactctacaaattgaaaaacatgttagcagggcatttatttgcttgcaagcgctaactacatttgtttcagtggctggtataatctacatcatttacaagttgtttgccggctttcagggtgcatacactggaatgcccaaccagaaacccaaggtgcccaccttaagacaagctaaggtgcaaggtccggcatttgaatttgccgtagcaatgatgaaaaggaacgccagcacagtcaagacagaatacggtgagttcacgatgcttggcatctatgataaatgggcagtgctgccgcgccacgccaagcctggaccaactattttaatgaatgatcaggaggttggtgtgctcgatgccaaagagttagttgataaagacggaaccaacctggagctgacactattgaagcttaaccgcaatgaaaagttcagagacatcagaggttttcttgcaagggaagaagttgaggtaagtgaggctgttttggcaataaacacgagcaagttcccaagcatgtacatccctgtgggccaagtcaccgattacggatttttaaatctaggtggcaccccaacaaagagaatgctcatgtacaacttccctaccagagcgggacagtgtggtggtgtccttatgtcaacaggaaaggtccttggcatacacgtgggaggaaatggtcaccaaggcttctctgctgctctcctcagacactacttcaacgaggaacagggcgaaatagagtttattgagagctctaaagatgcaggatttcctgtgatcaacacccctaataaaaccaaactggaaccaagtgtgtttcatcaggtttttgagggcaacaaagaaccagcagtcctaagaaacggagacccgcgacttaaagccaactttgaggaagcgatattttccaagtacatcggaaatgtgaacacacatgtggacgagtacatgatagaagctgttgatcactacgctggacagctggcaactctggacatcagtacagaacctatgaagcttgaggatgctgtttatggcactgaaggcttggaagcattggacttgaccactagcgcaggatatccttatgtcgccttgggcatcaagaaaagggatatcctctccaagaagactaaagatctcaccaagctgagggaatgcatggacaagtatggtctaaatctgccgatggtgacctacgtgaaggatgaactcaggtccgctgagaaagtagccaagggaaaatccagacttatagaagcttctagtctcaatgactcagtggccatgaggcagacatttgggaacctatacaagacattccacctcaacccaggcattgtcactggtagtgctgttgggtgcgacccagatgtgttttggagcaaaatacccgtgatgcttgacgggcaccttatagcttttgattactctggctacgacgctagcttgagcccagtgtggtttgcttgtttgaaactcctcctagggaaactagggtatactcataaggaaaccaattacatagactacctctgcaactcccatcacttatacagagataaacactatttcgtgaggggtggtatgccatcaggatgttcaggcaccagtatattcaacaccatgatcaacaacatcattattaggacccttatgctaaaggtctacaaaggtattgacctggatcagtttagaatgatcgcttacggggacgatgtgatagcctcttacccgtggcctattgatgcctcactactagcagaagcgggaaaggattatggtttgatcatgaccccagcagataaaggagagtgttttaatgaggtaacctggacaaatgtaaccttcttgaaaaggtactttagagctgatgaacaatatccattcttggtgcaccccgtgatgcccatgaaagacatacacgaatccattagatggaccaaagacccaaagaacactcaagatcatgtgcgctcgttatgcctattggcttggcacaatggggagcacgaatatgaggaatttatccgaaagatcagaagcgtgcctgttggacgctgtttgaccctcccggtgttctcaacactacgcaggaaatggttagattccttctgataatagctcgagctggtactgcatgcacgcaatgctagctgcccctttcccgtcctgggtaccccgagtctcccccgacctcgggtcccaggtatgctcccacctccacctgccccactcaccacctctgctagttccagacacctcccaagcacgcagcaatgcagctcaaaacgcttagcctagccacacccccacgggaaacagcagtgattaacctttagcaataaacgaaagtttaactaagctatactaaccccagggttggtcaatttcgtgccagccacaccctggagctagcaaaaaaaaaaaaaaaaaaaaaaaaaaaaaaaaaaaaaaaaaaaaaaaaaa

SEQ ID NO: 168 - DNA, 1698 bp, synthetic construct; identical to SEQ ID NO: 51
  source 1..1698: mol_type = other DNA
  misc_feature 1..1698: note = H3N2 DNA construct

SEQ ID NO: 169 - DNA, 2280 bp, synthetic construct
  source 1..2280: mol_type = other DNA
  misc_feature 1..2280: note = nucleotide sequence coding PB2
atggaaagaataaaagaactacgaaatctaatgtcgcagtctcgcacccgcgagatactcacaaaaaccaccgtggaccatatggccataatcaagaagtacacatcaggaagacaggagaagaacccagcacttaggatgaaatggatgatggcaatgaaatatccaattacagcagacaagaggataacggaaatgattcctgagagaaatgagcaaggacaaactttatggagtaaaatgaatgatgccggatcagaccgagtgatggtatcacctctggctgtgacatggtggaataggaatggaccaataacaaatacagttcattatccaaaaatctacaaaacttattttgaaagagtcgaaaggctaaagcatggaacctttggccctgtccattttagaaaccaagtcaaaatacgtcggagagttgacataaatcctggtcatgcagatctcagtgccaaggaggcacaggatgtaatcatggaagttgttttccctaacgaagtgggagccaggatactaacatcggaatcgcaactaacgataaccaaagagaagaaagaagaactccaggattgcaaaatttctcctttgatggttgcatacatgttggagagagaactggtccgcaaaacgagattcctcccagtggctggtggaacaagcagtgtgtacattgaagtgttgcatttgactcaaggaacatgctgggaacagatgtatactccaggaggggaagtgaggaatgatgatgttgatcaaagcttgattattgctgctaggaacatagtgagaagagctgcagtatcagcagatccactagcatctttattggagatgtgccacagcacacagattggtggaattaggatggtagacatccttaggcagaacccaacagaagagcaagccgtggatatatgcaaggctgcaatgggactgagaattagctcatccttcagttttggtggattcacatttaagagaacaagcggatcatcagtcaagagagaggaagaggtgcttacgggcaatcttcaaacattgaagataagagtgcatgagggatatgaagagttcacaatggttgggagaagagcaacagccatactcagaaaagcaaccaggagattgattcagctgatagtgagtgggagagacgaacagtcgattgccgaagcaataattgtggccatggtattttcacaagaggattgtatgataaaagcagtcagaggtgatctgaatttcgtcaatagggcgaatcaacgattgaatcctatgcatcaacttttaagacattttcagaaggatgcgaaagtgctttttcaaaattggggagttgaacctatcgacaatgtgatgggaatgattgggatattgcccgacatgactccaagcatcgagatgtcaatgagaggagtgagaatcagcaaaatgggtgtagatgagtactccagcacggagagggtagtggtgagcattgaccgttttttgagaatccgggaccaacgaggaaatgtactactgtctcccgaggaggtcagtgaaacacagggaacagagaaactgacaataacttactcatcgtcaatgatgtgggagattaatggtcctgaatcagtgttggtcaatacctatcaatggatcatcagaaactgggaaactgttaaaattcagtggtcccagaaccctacaatgctatacaataaaatggaatttgaaccatttcagtctttagtacctaaggccattagaggccaatacagtgggtttgtaagaactctgttccaacaaatgagggatgtgcttgggacatttgataccgcacagataataaaacttcttcccttcgcagccgctccaccaaagcaaagtagaatgcagttctcctcatttactgtgaatgtgaggggatcaggaatgagaatacttgtaaggggcaattctcctgtattcaactataacaaggccacgaagagactcacagttctcggaaaggatgctggcactttaactgaagacccagatgaaggcacagctggagtggagtccgctgttctgaggggattcctcattctgggcaaagaagacaagagatatgggccagcactaagcatcaatgaactgagcaaccttgcgaaaggagagaaggctaatgtgctaattgggcaaggagacgtggtgttggtaatgaaacggaaacgggactctagcatacttactgacagccagacagcgaccaaaagaattcggatggccatcaattag

SEQ ID NO: 170 - protein, 759 aa, synthetic construct
  REGION 1..759: note = PB2
MERIKELRNLMSQSRTREILTKTTVDHMAIIKKYTSGRQEKNPALRMKWMMAMKYPITADKRITEMIPERNEQGQTLWSKMNDAGSDRVMVSPLAVTWWNRNGPITNTVHYPKIYKTYFERVERLKHGTFGPVHFRNQVKIRRRVDINPGHADLSAKEAQDVIMEVVFPNEVGARILTSESQLTITKEKKEELQDCKISPLMVAYMLERELVRKTRFLPVAGGTSSVYIEVLHLTQGTCWEQMYTPGGEVRNDDVDQSLIIAARNIVRRAAVSADPLASLLEMCHSTQIGGIRMVDILRQNPTEEQAVDICKAAMGLRISSSFSFGGFTFKRTSGSSVKREEEVLTGNLQTLKIRVHEGYEEFTMVGRRATAILRKATRRLIQLIVSGRDEQSIAEAIIVAMVFSQEDCMIKAVRGDLNFVNRANQRLNPMHQLLRHFQKDAKVLFQNWGVEPIDNVMGMIGILPDMTPSIEMSMRGVRISKMGVDEYSSTERVVVSIDRFLRIRDQRGNVLLSPEEVSETQGTEKLTITYSSSMMWEINGPESVLVNTYQWIIRNWETVKIQWSQNPTMLYNKMEFEPFQSLVPKAIRGQYSGFVRTLFQQMRDVLGTFDTAQIIKLLPFAAAPPKQSRMQFSSFTVNVRGSGMRILVRGNSPVFNYNKATKRLTVLGKDAGTLTEDPDEGTAGVESAVLRGFLILGKEDKRYGPALSINELSNLAKGEKANVLIGQGDVVLVMKRKRDSSILTDSQTATKRIRMAIN

SEQ ID NO: 171 - DNA, 2274 bp, synthetic construct
  source 1..2274: mol_type = other DNA
  misc_feature 1..2274: note = nucleotide sequence codign PB1
atggatgtcaatccgaccttacttttcttaaaagtgccagcacaaaatgctataagcacaactttcccttatactggagaccctccttacagccatgggacaggaacaggatacaccatggatactgtcaacaggacacatcagtactcagaaaagggaagatggacaacaaacaccgaaactggagcaccgcaactcaacccgattgatgggccactgccagaagacaatgaaccaagtggttatgcccaaacagattgtgtattggaggcgatggctttccttgaggaatcccatcctggtatttttgaaaactcgtgtattgaaacgatggaggttgttcagcaaacacgagtagacaagctgacacaaggccgacagacctatgactggactctaaatagaaaccaacctgctgcaacagcattggccaacacaatagaagtgttcagatcaaatggcctcacggccaatgagtctggaaggctcatagacttccttaaggatgtaatggagtcaatgaacaaagaagaaatggggatcacaactcattttcagagaaagagacgggtgagagacaatatgactaagaaaatgataacacagagaacaatgggtaaaaagaagcagagattgaacaaaaggagttatctaattagagcattgaccctgaacacaatgaccaaagatgctgagagagggaagctaaaacggagagcaattgcaaccccagggatgcaaataagggggtttgtatactttgttgagacactggcaaggagtatatgtgagaaacttgaacaatcagggttgccagttggaggcaatgagaagaaagcaaagttggcaaatgttgtaaggaagatgatgaccaattctcaggacaccgaactttctttcaccatcactggagataacaccaaatggaacgaaaatcagaatcctcggatgtttttggccatgatcacatatatgaccagaaatcagcccgaatggttcagaaatgttctaagtattgctccaataatgttctcaaacaaaatggcgagactgggaaaagggtatatgtttgagagcaagagtatgaaacttagaactcaaatacctgcagaaatgctagcaagcatcgatttgaaatatttcaatgattcaacaagaaagaagattgaaaaaatccgaccgctcttaatagaggggactgcatcattgagccctggaatgatgatgggcatgttcaatatgttaagcactgtattaggcgtctccatcctgaatcttggacaaaagagatacaccaagactacttactggtgggatggtcttcaatcctctgacgattttgctctgattgtgaatgcacccaatcatgaagggattcaagccggagtcgacaggttttatcgaacctgtaagctacttggaatcaatatgagcaagaaaaagtcttacataaacagaacaggtacatttgaattcacaagttttttctatcgttatgggtttgttgccaatttcagcatggagcttcccagttttggggtgtctgggatcaacgagtcagcggacatgagtattggagttactgtcatcaaaaacaatatgataaacaatgatcttggtccagcaacagctcaaatggcccttcagttgttcatcaaagattacaggtacacgtaccgatgccatataggtgacacacaaatacaaacccgaagatcatttgaaataaagaaactgtgggagcaaacccgttccaaagctggactgctggtctccgacggaggcccaaatttatacaacattagaaatctccacattcctgaagtctgcctaaaatgggaattgatggatgaggattaccaggggcgtttatgcaacccactgaacccatttgtcagccataaagaaattgaatcaatgaacaatgcagtgatgatgccagcacatggtccagccaaaaacatggagtatgatgctgttgcaacaacacactcctggatccccaaaagaaatcgatccatcttgaatacaagtcaaagaggagtacttgaggatgaacaaatgtaccaaaggtgctgcaatttatttgaaaaattcttccccagcagttcatacagaagaccagtcgggatatccagtatggtggaggctatggtttccagagcccgaattgatgcacggattgatttcgaatctggaaggataaagaaagaagagttcactgagatcatgaagatctgttccaccattgaagagctcagacggcaaaaatag

SEQ ID NO: 172 - protein, 757 aa, synthetic construct
  REGION 1..757: note = PB1
MDVNPTLLFLKVPAQNAISTTFPYTGDPPYSHGTGTGYTMDTVNRTHQYSEKGRWTTNTETGAPQLNPIDGPLPEDNEPSGYAQTDCVLEAMAFLEESHPGIFENSCIETMEVVQQTRVDKLTQGRQTYDWTLNRNQPAATALANTIEVFRSNGLTANESGRLIDFLKDVMESMNKEEMGITTHFQRKRRVRDNMTKKMITQRTMGKKKQRLNKRSYLIRALTLNTMTKDAERGKLKRRAIATPGMQIRGFVYFVETLARSICEKLEQSGLPVGGNEKKAKLANVVRKMMTNSQDTELSFTITGDNTKWNENQNPRMFLAMITYMTRNQPEWFRNVLSIAPIMFSNKMARLGKGYMFESKSMKLRTQIPAEMLASIDLKYFNDSTRKKIEKIRPLLIEGTASLSPGMMMGMFNMLSTVLGVSILNLGQKRYTKTTYWWDGLQSSDDFALIVNAPNHEGIQAGVDRFYRTCKLLGINMSKKKSYINRTGTFEFTSFFYRYGFVANFSMELPSFGVSGINESADMSIGVTVIKNNMINNDLGPATAQMALQLFIKDYRYTYRCHIGDTQIQTRRSFEIKKLWEQTRSKAGLLVSDGGPNLYNIRNLHIPEVCLKWELMDEDYQGRLCNPLNPFVSHKEIESMNNAVMMPAHGPAKNMEYDAVATTHSWIPKRNRSILNTSQRGVLEDEQMYQRCCNLFEKFFPSSSYRRPVGISSMVEAMVSRARIDARIDFESGRIKKEEFTEIMKICSTIEELRRQK

SEQ ID NO: 173 - DNA, 2151 bp, synthetic construct
  source 1..2151: mol_type = other DNA
  misc_feature 1..2151: note = nucleotide sequence coding PA
atggaagattttgtgcgacaatgcttcaatccgatgattgtcgagcttgcggaaaaaacaatgaaagagtatggggaggacctgaaaatcgaaacaaacaaatttgcagcaatatgcactcacttggaagtatgcttcatgtattcagattttcacttcatcaatgagcaaggcgagtcaataatcgtagaacttggtgatccaaatgcacttttgaagcacagatttgaaataatcgagggaagagatcgcacaatggcctggacagtagtaaacagtatttgcaacactacaggggctgagaaaccaaagtttctaccagatttgtatgattacaaggagaatagattcatcgaaattggagtaacaaggagagaagttcacatatactatctggaaaaggccaataaaattaaatctgagaaaacacacatccacattttctcgttcactggggaagaaatggccacaaaggcagactacactctcgatgaagaaagcagggctaggatcaaaaccagactattcaccataagacaagaaatggccagcagaggcctctgggattcctttcgtcagtccgagagaggagaagagacaattgaagaaaggtttgaaatcacaggaacaatgcgtaagcttgccgaccaaagtctcccgccgaacttctccagccttgaaaattttagagcctatgtggatggattcgaaccgaacggctacattgagggcaagctgtctcaaatgtccaaagaagtaaatgctagaattgaaccttttttgaaaacaacaccacgaccacttagacttccgaatgggcctccctgttctcagcggtccaaattcctgctgatggatgccttaaaattaagcattgaggacccaagtcatgaaggagagggaataccgctatatgatgcaatcaaatgcatgagaacattctttggatggaaggaacccaatgttgttaaaccacacgaaaagggaataaatccaaattatcttctgtcatggaagcaagtactggcagaactgcaggacattgagaatgaggagaaaattccaaagactaaaaatatgaagaaaacaagtcagctaaagtgggcacttggtgagaacatggcaccagaaaaggtagactttgacgactgtaaagatgtaggtgatttgaagcaatatgatagtgatgaaccagaattgaggtcgcttgcaagttggattcagaatgagtttaacaaggcatgcgaactgacagattcaagctggatagagctcgatgagattggagaagatgtggctccaattgaacacattgcaagcatgagaaggaattatttcacatcagaggtgtctcactgcagagccacagaatacataatgaagggagtgtacatcaatactgccttgcttaatgcatcttgtgcagcaatggatgatttccaattaattccaatgataagcaagtgtagaactaaggagggaaggcgaaagaccaacttgtatggtttcatcataaaaggaagatcccacttaaggaatgacaccgacgtggtaaactttgtgagcatggagttttctctcactgacccaagacttgaaccacataaatgggagaagtactgtgttcttgagataggagatatgcttataagaagtgccataggccaggtttcaaggcccatgttcttgtatgtgagaacaaatggaacctcaaaaattaaaatgaaatggggaatggagatgaggcgttgcctcctccagtcacttcaacaaattgagagtatgattgaagctgagtcctctgtcaaagagaaagacatgaccaaagagttctttgagaacaaatcagaaacatggcccattggagagtcccccaaaggagtggaggaaagttccattgggaaggtctgcaggactttattagcaaagtcggtattcaacagcttgtatgcatctccacaactagaaggattttcagctgaatcaagaaaactgcttcttatcgttcaggctcttagggacaacctggaacctgggacctttgatcttggggggctatatgaagcaattgaggagtgcctgattaatgatccctgggttttgcttaatgcttcttggttcaactccttccttacacatgcattgagttag

SEQ ID NO: 174 - protein, 716 aa, synthetic construct
  REGION 1..716: note = PA
MEDFVRQCFNPMIVELAEKTMKEYGEDLKIETNKFAAICTHLEVCFMYSDFHFINEQGESIIVELGDPNALLKHRFEIIEGRDRTMAWTVVNSICNTTGAEKPKFLPDLYDYKENRFIEIGVTRREVHIYYLEKANKIKSEKTHIHIFSFTGEEMATKADYTLDEESRARIKTRLFTIRQEMASRGLWDSFRQSERGEETIEERFEITGTMRKLADQSLPPNFSSLENFRAYVDGFEPNGYIEGKLSQMSKEVNARIEPFLKTTPRPLRLPNGPPCSQRSKFLLMDALKLSIEDPSHEGEGIPLYDAIKCMRTFFGWKEPNVVKPHEKGINPNYLLSWKQVLAELQDIENEEKIPKTKNMKKTSQLKWALGENMAPEKVDFDDCKDVGDLKQYDSDEPELRSLASWIQNEFNKACELTDSSWIELDEIGEDVAPIEHIASMRRNYFTSEVSHCRATEYIMKGVYINTALLNASCAAMDDFQLIPMISKCRTKEGRRKTNLYGFIIKGRSHLRNDTDVVNFVSMEFSLTDPRLEPHKWEKYCVLEIGDMLIRSAIGQVSRPMFLYVRTNGTSKIKMKWGMEMRRCLLQSLQQIESMIEAESSVKEKDMTKEFFENKSETWPIGESPKGVEESSIGKVCRTLLAKSVFNSLYASPQLEGFSAESRKLLLIVQALRDNLEPGTFDLGGLYEAIEECLINDPWVLLNASWFNSFLTHALS

SEQ ID NO: 175 - DNA, 693 bp, synthetic construct
  source 1..693: mol_type = other DNA
  misc_feature 1..693: note = nucleotide sequence coding NS
atggatccaaacactgtgtcaagctttcaggtagattgctttctttggcatgtccgcaaacgagttgcagaccaagaactaggcgatgccccattccttgatcggcttcgccgagatcagaaatccctaagaggaaggggcagtactctcggtctggacatcaagacagccacacgtgctggaaagcagatagtggagcggattctgaaagaagaatccgatgaggcacttaaaatgaccatggcctctgtacctgcgtcgcgttacctaactgacatgactcttgaggaaatgtcaagggactggtccatgctcatacccaagcagaaagtggcaggccctctttgtatcagaatggaccaggcgatcatggataagaacatcatactgaaagcgaacttcagtgtgatttttgaccggctggagactctaatattgctaagggctttcaccgaagagggagcaattgttggcgaaatttcaccattgccttctcttccaggacatactgctgaggatgtcaaaaatgcagttggagtcctcatcggaggacttgaatggaatgataacacagttcgagtctctgaaactctacagagattcgcttggagaagcagtaatgagaatgggagacctccactcactccaaaacagaaacgagaaatggcgggaacaattaggtcagaagtttga

SEQ ID NO: 176 - protein, 230 aa, synthetic construct
  REGION 1..230: note = NS
MDPNTVSSFQVDCFLWHVRKRVADQELGDAPFLDRLRRDQKSLRGRGSTLGLDIKTATRAGKQIVERILKEESDEALKMTMASVPASRYLTDMTLEEMSRDWSMLIPKQKVAGPLCIRMDQAIMDKNIILKANFSVIFDRLETLILLRAFTEEGAIVGEISPLPSLPGHTAEDVKNAVGVLIGGLEWNDNTVRVSETLQRFAWRSSNENGRPPLTPKQKREMAGTIRSEV

SEQ ID NO: 177 - DNA, 1497 bp, synthetic construct
  source 1..1497: mol_type = other DNA
  misc_feature 1..1497: note = nucleotide sequence coding NP
atggcgtctcaaggcaccaaacgatcttacgaacagatggagactgatggagaacgccagaatgccactgaaatcagagcatccgtcggaaaaatgattggtggaattggacgattctacatccaaatgtgcaccgaactcaaactcagtgattatgagggacggttgatccaaaacagcttaacaatagagagaatggtgctctctgcttttgacgaaaggagaaataaataccttgaagaacatcccagtgcggggaaagatcctaagaaaactggaggacctatatacaggagagtaaacggaaagtggatgagagaactcatcctttatgacaaagaagaaataaggcgaatctggcgccaagctaataatggtgacgatgcaacggctggtctgactcacatgatgatctggcattccaatttgaatgatgcaacttatcagaggacaagagctcttgttcgcaccggaatggatcccaggatgtgctctctgatgcaaggttcaactctccctaggaggtctggagccgcaggtgctgcagtcaaaggagttggaacaatggtgatggaattggtcagaatgatcaaacgtgggatcaatgatcggaacttctggaggggtgagaatggacgaaaaacaagaattgcttatgaaagaatgtgcaacattctcaaagggaaatttcaaactgctgcacaaaaagcaatgatggatcaagtgagagagagccggaacccagggaatgctgagttcgaagatctcacttttctagcacggtctgcactcatattgagagggtcggttgctcacaagtcctgcctgcctgcctgtgtgtatggacctgccgtagccagtgggtacgactttgaaagggagggatactctctagtcggaatagaccctttcagactgcttcaaaacagccaagtgtacagcctaatcagaccaaatgagaatccagcacacaagagtcaactggtgtggatggcatgccattctgccgcatttgaagatctaagagtattaagcttcatcaaagggacgaaggtgctcccaagagggaagctttccactagaggagttcaaattgcttccaatgaaaatatggagactatggaatcaagtacacttgaactgagaagcaggtactgggccataaggaccagaagtggaggaaacaccaatcaacagagggcatctgcgggccaaatcagcatacaacctacgttctcagtacagagaaatctcccttttgacagaacaaccattatggcagcattcaatgggaatacagaggggagaacatctgacatgaggaccgaaatcataaggatgatggaaagtgcaagaccagaagatgtgtctttccaggggcggggagtcttcgagctctcggacgaaaaggcagcgagcccgatcgtgccttcctttgacatgagtaatgaaggatcttatttcttcggagacaatgcagaggagtacgacaattaa

SEQ ID NO: 178 - protein, 498 aa, synthetic construct
  REGION 1..498: note = NP
MASQGTKRSYEQMETDGERQNATEIRASVGKMIGGIGRFYIQMCTELKLSDYEGRLIQNSLTIERMVLSAFDERRNKYLEEHPSAGKDPKKTGGPIYRRVNGKWMRELILYDKEEIRRIWRQANNGDDATAGLTHMMIWHSNLNDATYQRTRALVRTGMDPRMCSLMQGSTLPRRSGAAGAAVKGVGTMVMELVRMIKRGINDRNFWRGENGRKTRIAYERMCNILKGKFQTAAQKAMMDQVRESRNPGNAEFEDLTFLARSALILRGSVAHKSCLPACVYGPAVASGYDFEREGYSLVGIDPFRLLQNSQVYSLIRPNENPAHKSQLVWMACHSAAFEDLRVLSFIKGTKVLPRGKLSTRGVQIASNENMETMESSTLELRSRYWAIRTRSGGNTNQQRASAGQISIQPTFSVQRNLPFDRTTIMAAFNGNTEGRTSDMRTEIIRMMESARPEDVSFQGRGVFELSDEKAASPIVPSFDMSNEGSYFFGDNAEEYDN

SEQ ID NO: 179 - DNA, 1365 bp, synthetic construct
  source 1..1365: mol_type = other DNA
  misc_feature 1..1365: note = nucleotide sequence coding NA
atgaatccaaatcagaaaataataaccattggatcaatctgtctggtagtcggactaattagcctaatattgcaaatagggaatataatctcaatatggattagccattcaattcaaactggaagtcaaaaccatactggaatatgcaaccaaaacatcattacctataaaaatagcacctgggtaaaggacacaacttcagtgatattaaccggcaattcatctctttgtcccatccgtgggtgggctatatacagcaaagacaatagcataagaattggttccaaaggagacgtttttgtcataagagagccctttatttcatgttctcacttggaatgcaggaccttttttctgacccaaggtgccttactgaatgacaagcattcaagtgggactgttaaggacagaagcccttatagggccttaatgagctgccctgtcggtgaagctccgtccccgtacaattcaagatttgaatcggttgcttggtcagcaagtgcatgtcatgatggcatgggctggctaacaatcggaatttcaggtccagataatggagcagtggctgtattaaaatacaacggcataataactgaaaccataaaaagttggaggaagaaaatattgaggacacaagagtctgaatgtgcctgtgtaaatggttcatgttttactataatgactgatggcccgagtgatgggctggcctcgtacaaaattttcaagatcgaaaaggggaaggttactaaatcaatagagttgaatgcacctaattctcactatgaggaatgttcctgttaccctgataccggcaaagtgatgtgtgtgtgcagagacaattggcatggttcgaaccggccatgggtgtctttcgatcaaaacctggattatcaaataggatacatctgcagtggggttttcggtgacaacccgcgtcccgaagatggaacaggcagctgtggtccagtgtatgttgatggagcaaacggagtaaagggattttcatataggtatggtaatggtgtttggataggaaggaccaaaggtcacagttccagacatgggtttgagatgatttgggatcctaatggatggacagagactgatagtaagttctctgtgaggcaagatgttgtggcaatgactgattggtcagggtatagcggaagtttcgttcaacatcctgagctgacagggctagactgtatgaggccgtgcttctgggttgaattaatcaggggacgacctaaagaaaaaacaatctggactagtgcgagcagcatttctttttgtggcgtgaatagtgatactgtagattggtcttggccagacggtgctgagttgccattcagcattgacaagtag

SEQ ID NO: 180 - protein, 454 aa, synthetic construct
  REGION 1..454: note = NA
MNPNQKIITIGSICLVVGLISLILQIGNIISIWISHSIQTGSQNHTGICNQNIITYKNSTWVKDTTSVILTGNSSLCPIRGWAIYSKDNSIRIGSKGDVFVIREPFISCSHLECRTFFLTQGALLNDKHSSGTVKDRSPYRALMSCPVGEAPSPYNSRFESVAWSASACHDGMGWLTIGISGPDNGAVAVLKYNGIITETIKSWRKKILRTQESECACVNGSCFTIMTDGPSDGLASYKIFKIEKGKVTKSIELNAPNSHYEECSCYPDTGKVMCVCRDNWHGSNRPWVSFDQNLDYQIGYICSGVFGDNPRPEDGTGSCGPVYVDGANGVKGFSYRYGNGVWIGRTKGHSSRHGFEMIWDPNGWTETDSKFSVRQDVVAMTDWSGYSGSFVQHPELTGLDCMRPCFWVELIRGRPKEKTIWTSASSISFCGVNSDTVDWSWPDGAELPFSIDK

SEQ ID NO: 181 - DNA, 759 bp, synthetic construct
  source 1..759: mol_type = other DNA
  misc_feature 1..759: note = nucleotide sequence coding M
atgagtcttctaaccgaggtcgaaacgtacgtactctctatcatcccgtcaggccccctcaaagccgagatcgcacagagacttgaagatgtctttgcagggaagaacaccgatcttgaggttctcatggaatggctaaagacaagaccaatcctgtcacctctgactaaggggattttaggatttgtgttcacgctcaccgtgcccagtgagcgaggactgcagcgtagacgctttgtccaaaatgcccttaatgggaacggggatccaaataacatggacaaagcagttaaactgtataggaagctcaagagggagataacattccatggggccaaagaaatctcactcagttattctgctggtgcacttgccagttgtatgggcctcatatacaacaggatgggggctgtgaccactgaagtggcatttggcctggtatgtgcaacctgtgaacagattgctgactcccagcatcggtctcataggcaaatggtgacaacaaccaatccactaatcagacatgagaacagaatggttttagccagcactacagctaaggctatggagcaaatggctggatcgagtgagcaagcagcagaggccatggaggttgctagtcaggctagacaaatggtgcaagcgatgagaaccattgggactcatcctagctccagtgctggtctgaaaaatgatcttcttgaaaatttgcaggcctatcagaaacgaatgggggtgcagatgcaacggttcaagtga

SEQ ID NO: 182 - protein, 252 aa, synthetic construct
  REGION 1..252: note = M
MSLLTEVETYVLSIIPSGPLKAEIAQRLEDVFAGKNTDLEVLMEWLKTRPILSPLTKGILGFVFTLTVPSERGLQRRRFVQNALNGNGDPNNMDKAVKLYRKLKREITFHGAKEISLSYSAGALASCMGLIYNRMGAVTTEVAFGLVCATCEQIADSQHRSHRQMVTTTNPLIRHENRMVLASTTAKAMEQMAGSSEQAAEAMEVASQARQMVQAMRTIGTHPSSSAGLKNDLLENLQAYQKRMGVQMQRFK

SEQ ID NO: 183 - DNA, 1701 bp, synthetic construct
  source 1..1701: mol_type = other DNA
  misc_feature 1..1701: note = nucleotide sequence coding H3N2_HA
atgaaaaccgttattgctttaagctacattttctgcctggcttttggtcagaatcttccaggaaatgaaaataatgctgcaacactatgcctgggacatcatgcagtgccgaacgggacaatagtgaaaactatcacagacgatcaaattgaggtgaccaacgccaccgagctagtccaaaactcctcaacagggaaaatatgcaacaatccccacaagattcttgatgggagggactgcacactaatagatgccctactaggggacccgcactgtgacgtcttccaaaatgagacatgggacctttttgtggaacgaagcaatgcttttagcaattgttacccttatgatgtaccagactatgcatcccttcgatccatagttgcatcatcaggcacattggagttcatcactgaaggtttcacttgggcaggagtaattcaaaatggaggaagcggtgcttgtaaaaggggacctgctaatggtttcttcagtagattgaattggttaactaagtcaggaaatacatatccagtattgaatgtgactatgccaaacaataacaatttcgacaaattatacatttggggagttcatcacccaagcactaatcaagaacaaaccagcctgtatattcaggcctcaggaagagtcgcagtctctaccaggagaagccaacagaccataatcccaaacattggatctagacccttggtaaggggccaatctggcagaataagcgtatattggacaatagtcaaacctggagacgtactggtaataaacagtaatggaaacctaatcgctcctcgaggctacttcaaaatgcacattgggaaaagctcaataatgagatcagatgcacctattgacacctgcatttccgaatgtatcactccgaacgggagcatccccaatgaaaagcccttccaaaatgtaaacaagatcacatacggagcatgtcccaaatatgttaagcaaaacaccttgaaactggcaacaggaatgcggaatgtccctgagaggcaaaccagaggcctgttcggcgcaatagcaggcttcatagaaaatggatgggaagggatggtagacggttggtatggcttcaggcaccaaaattccgaaggtacaggacaagcagcagaccttaaaagcactcaggcagccattgaccagattaatgggaaattgaacagagtgattgaaaaaacgaatgagaagttccatcaaatcgaaaaggagttttccgaagtagaagggaggattcaagaccttgagagatacgttgaagacacaaaagtagatctttggtcttacaatgccgagcttcttgttgctttagaaaaccagaacacaattgatttaactgattcagaaatgaacaaattgtttgaaaagactaggaggcaattgagggaaaatgctgaagacatgggcaatggctgcttcaagatataccacaagtgtgacaatgcttgcatagaatcgattagaaacggaacttatgaccataacatatatagagatgaggcagtgaacaatcggttccagatcaaaggtgttgagctaaagtctggatacaaagactggatcttgtggatttcctttgccatatcatgctttttgctttgtgttgtcttgctgggtttcattatgtgggcctgccagagaggcaacattaggtgcaacatttgcatttga

SEQ ID NO: 184 - protein, 566 aa, synthetic construct
  REGION 1..566: note = H3N2_HA
MKTVIALSYIFCLAFGQNLPGNENNAATLCLGHHAVPNGTIVKTITDDQIEVTNATELVQNSSTGKICNNPHKILDGRDCTLIDALLGDPHCDVFQNETWDLFVERSNAFSNCYPYDVPDYASLRSIVASSGTLEFITEGFTWAGVIQNGGSGACKRGPANGFFSRLNWLTKSGNTYPVLNVTMPNNNNFDKLYIWGVHHPSTNQEQTSLYIQASGRVAVSTRRSQQTIIPNIGSRPLVRGQSGRISVYWTIVKPGDVLVINSNGNLIAPRGYFKMHIGKSSIMRSDAPIDTCISECITPNGSIPNEKPFQNVNKITYGACPKYVKQNTLKLATGMRNVPERQTRGLFGAIAGFIENGWEGMVDGWYGFRHQNSEGTGQAADLKSTQAAIDQINGKLNRVIEKTNEKFHQIEKEFSEVEGRIQDLERYVEDTKVDLWSYNAELLVALENQNTIDLTDSEMNKLFEKTRRQLRENAEDMGNGCFKIYHKCDNACIESIRNGTYDHNIYRDEAVNNRFQIKGVELKSGYKDWILWISFAISCFLLCVVLLGFIMWACQRGNIRCNICI

SEQ ID NO: 185 - DNA, 1698 bp, synthetic construct
  source 1..1698: mol_type = other DNA
  misc_feature 1..1698: note = nucleotide sequence coding H3N8_HA
atgaaaacaaccattattttaatactactgacccattgggcctacagtcaaaacccaatcagtggcaataacacagccacactgtgtctgggacaccatgcagtagcaaatggaacattgatcaagacaatgagtgatgatcaaattgaagtgacaaatgctacagaattagttcagagcatttcaatggggaaaatatgcaacaaatcatatagagttctagatggaagaaattgcacattaatagatgcaatgctaggagacccccagtgtgacgcctttcagtatgagagttgggacctctttatagaaagaagcaacgctttcagcaattgctacccatatgacatccctgattatgcatcgctccgatccattgtagcatcctcaggaacagtggaattcacagcagagggattcacatggacaggtgtcactcaaaacggaaaaagtggagcttgcaaaaggggatcagccgatagtttctttagccgactgaattggctaacaaaatctggaagctcttaccccacattgaatgtaacaatgcctaacaataaaaatttcgacaagctatacatctgggggattcatcacccgagctcgaatcaagagcagacaaaattgtacattcaagaatcaggacgagtaacagtctcaacaaaaagaagtcaacaaacaataatccctcacatcggatctagaccgttgatcagaggtcaatcaggcaggataagcatatactggaccattgtaaaacctggagatatcctaatgataaacagtaatggcaacttagttgcaccgcggggatatttcaaattgaatccaggaaaaagctctgtaattagatccgatgtacccatagacatttgtgtgtctgaatgtattacaccaaatggaagcatctccaacgacaagccattccaaaatgtgaacaaagttacatatggaaaatgccccaagtatatcaagcaaaacactttaaagttggctactgggatgaggaatgtgccagaaaagcaaaccagaggaatctttggggcgatagcgggattcatcgaaaacggctgggaaggaatggttgatgggtggtatgggttccgatatcaaaactctgaaggaacagggcaagctgcagatctaaagagtactcaagcagccatcgaccagattaatggaaagttaaacagggtgattgaaagaaccaatgagaaattccatcaaatagagaaggaattctcagaagtagaaggaagaattcaggacttggagaaatatgtagaagacaccaaaatagacctatggtcctacaatgcagaactactggtggctctagaaaatcaacatacaattgacttaacagatgcagaaatgaataaattatttgagaagactagacgccagttaagagaaaatgcagaagacatgggaaatggatgtttcaagatttaccacaagtgtgataatgcatgcattgagtcaataagaactggaacatatgaccattacatatacagagatgaagcaataaacaaccgatttcagatcaaaggtgtagaattgaaatcaggctacaaagattggatactgtggatttcattcgccatatcatgcttcttaatttgcgttgttctattgggtttcattatgtgggcttgccaaaaaggcaacatcagatgcaacatttgcatttga

SEQ ID NO: 186 - protein, 565 aa, synthetic construct
  REGION 1..565: note = H3N8_HA
MKTTIILILLTHWAYSQNPISGNNTATLCLGHHAVANGTLIKTMSDDQIEVTNATELVQSISMGKICNKSYRVLDGRNCTLIDAMLGDPQCDAFQYESWDLFIERSNAFSNCYPYDIPDYASLRSIVASSGTVEFTAEGFTWTGVTQNGKSGACKRGSADSFFSRLNWLTKSGSSYPTLNVTMPNNKNFDKLYIWGIHHPSSNQEQTKLYIQESGRVTVSTKRSQQTIIPHIGSRPLIRGQSGRISIYWTIVKPGDILMINSNGNLVAPRGYFKLNPGKSSVIRSDVPIDICVSECITPNGSISNDKPFQNVNKVTYGKCPKYIKQNTLKLATGMRNVPEKQTRGIFGAIAGFIENGWEGMVDGWYGFRYQNSEGTGQAADLKSTQAAIDQINGKLNRVIERTNEKFHQIEKEFSEVEGRIQDLEKYVEDTKIDLWSYNAELLVALENQHTIDLTDAEMNKLFEKTRRQLRENAEDMGNGCFKIYHKCDNACIESIRTGTYDHYIYRDEAINNRFQIKGVELKSGYKDWILWISFAISCFLICVVLLGFIMWACQKGNIRCNICI

SEQ ID NO: 187 - protein, 18 aa, synthetic construct
  REGION 1..18: note = P2A
ATNFSLLKQAGDVEENPG

SEQ ID NO: 188 - skipped

SEQ ID NO: 189 - protein, 5 aa, synthetic construct
  REGION 1..5: note = linker
GGGGS

SEQ ID NO: 190 - RNA, 8377 nt, synthetic construct
  source 1..8377: mol_type = other RNA
  misc_feature 1..8377: note = H3N2_P2A_Luci saRNA construct
ttaaaacagcctgtgggttgtacccacccacagggcccactgggcgctagcactctggtatcacggtacctttgtgtgcctgttttatatcccctttccccgattgtaacttagaagatgtacacactgatcaatagcgggcatagcacaccagctatgtcttgatcaagcactcctgtatccccggaccaagtatcaatagactgctcacgcggttgaaggagaaaacgttcgtcacccggctaactacttcgagaaacccagtagtatcatgaaagttgcgaggcgtttcgttcagcacacccccagtgtagatcgggtcgatgagtcaccgcatcccccacgggcgaccgtggcggtggctgcgctggcggcctgcctacggggcaacccgtaggacgcttcaatacagacatggtgcgaagagtcgattgagctagttagtagtcctccggcccctgaatgcggctaatcctaactgcggagcacatgccctcaacccagggggtattgtgtcgtaacgggcaactctgcagcggaaccgactactttgggtgtccgtgtttccttttatccttatactggctgcttatggtgacaattgaaagattgttgccatatagctattggattggccatccagtgtctaatagagctgttatttacctctttgttggatttataccactcaacctaaaagaagttaaaacactacagctcattttacaactgaatacagcaaaccaccatgaaaaccgtgatcgccctcagttacatcttctgcctcgcctttggacagaatctcctcggaaacgaaaacaacgctgccacactctgcctgggacaccacgccgtgcccaacggcacaatggtgaagaccatcaccgacgatcagatcgaggtgaccaatgccaccgagctggtgcagaacagctccaccggcaaaatctgcaacaatccccacaagatcctggacggcagggattgcaccctgatcgacgctctgctgggcgaccctcactgcgacgtgttccagaatgagacatgggatctgttcgtggagaggagcaatgccttctccaactgctacccctacgacgtgcctgattacgccagcctgcggtccatcgtggccagctccggcaccctggagttcatcaccgagggcttcacctgggctggagtgacccagaacggaggcagcggagcttgcaagaggggacccgccaatagcttcttctcccggctgaactggctgaccaagtccggcaatacctaccccgtgctgaacgtgaccatgcctaacaataacaatttcgacaagctgtacatctggggcgtgcatcaccctagcaccgatcaggagcagaccagcctgtacatccaggcctccggcagggtgaccgtgagcaccaggcggtcccagcagaccatcatccccaacatcggctccaggcctctggtgcggggacagagcggccggatctccgtgtactggaccatcgtgaagcccggcgacatcctggtcatcaacagcaatggcaacctgatcgcccctcgcggctacttcaagatgcacatcggcaagagcagcatcatgagatccgacgcccccatcgatacctgcatcagcgagtgcatcacccctaatggctccatccccaacgagaagcctttccagaatgtgaacaagatcacctacggcgcctgccccaagtacgtgaagcagaataccctgaagctggccaccggcatgcgcaacgtgcctgagagacagaccgtgggcctgttcggagctatcgctggcttcatcgagaatggctgggagggcatggtggacggctggtacggcttccgccaccagaacagcgagggcaccggacaggctgccgacctgaagtccacccaggccgccatcgatcagatcaatggcaagctgaacagagtgatcgagaagaccaacgagaagttccaccagatcgagaaggagttcagcgaggtggagggacgcatccaggacctggagaggtacgtggaggacaccaagatcgatctgtggagctacaatgccgagctgctggtggccctggagaatcagaacaccatcgacctgaccgattccgagatgaacaagctgttcgagaagacccgcagacagctgcgcgagaatgccgaggacatgggcaacggctgcttcaaaatctaccacaagtgcgataacgcctgcatcgagagcatcagaaatggcacctacgaccacaacatctaccgcgatgaggccgtgaacaatagattccagatcaagggcgtggagctgaagtccggctacaaggactggattctgtggatcagcttcgccatctcctgcttcctgctgtgcgtggtgctgctggggtttattatgtgggcttgtcagagggggaacatcaggtgtaacatttgtattggaagcggagctactaacttcagcctgctgaagcaggctggacaggtggaggagaaccctggacctatggaagacgccaaaaacataaagaaaggcccggcgccattctatccgctggaagatggaaccgctggagagcaactgcataaggctatgaagagatacgccctggttcctggaacaattgcttttacagatgcacatatcgaggtggacatcacttacgctgagtacttcgaaatgtccgttcggttggcagaagctatgaaacgatatgggctgaatacaaatcacagaatcgtcgtatgcagtgaaaactctcttcaattctttatgccggtgttgggcgcgttatttatcggagttgcagttgcgcccgcgaacgacatttataatgaacgtgaattgctcaacagtatgggcatttcgcagcctaccgtggtgttcgtttccaaaaaggggttgcaaaaaattttgaacgtgcaaaaaaagctcccaatcatccaaaaaattattatcatggattctaaaacggattaccagggatttcagtcgatgtacacgttcgtcacatctcatctacctcccggttttaatgaatacgattttgtgccagagtccttcgatagggacaagacaattgcactgatcatgaactcctctggatctactggtctgcctaaaggtgtcgctctgcctcatagaactgcctgcgtgagattctcgcatgccagagatcctatttttggcaatcaaatcattccggatactgcgattttaagtgttgttccattccatcacggttttggaatgtttactacactcggatatttgatatgtggatttcgagtcgtcttaatgtatagatttgaagaagagctgtttctgaggagccttcaggattacaagattcaaagtgcgctgctggtgccaaccctattctccttcttcgccaaaagcactctgattgacaaatacgatttatctaatttacacgaaattgcttctggtggcgctcccctctctaaggaagtcggggaagcggttgccaagaggttccatctgccaggtatcaggcaaggatatgggctcactgagactacatcagctattctgattacacccgagggggatgataaaccgggcgcggtcggtaaagttgttccattttttgaagcgaaggttgtggatctggataccgggaaaacgctgggcgttaatcaaagaggcgaactgtgtgtgagaggtcctatgattatgtccggttatgtaaacaatccggaagcgaccaacgccttgattgacaaggatggatggctacattctggagacatagcttactgggacgaagacgaacacttcttcatcgttgaccgcctgaagtctctgattaagtacaaaggctatcaggtggctcccgctgaattggaatccatcttgctccaacaccccaacatcttcgacgcaggtgtcgcaggtcttcccgacgatgacgccggtgaacttcccgccgccgttgttgttttggagcacggaaagacgatgacggaaaaagagatcgtggattacgtcgccagtcaagtaacaaccgcgaaaaagttgcgcggaggagttgtgtttgtggacgaagtaccgaaaggtcttaccggaaaactcgacgcaagaaaaatcagagagatcctcataaaggccaagaagggcggaaagatcgccgtgaactttgagccaacaggggtgacggagtcccgcactgaaattacggcaatgcagaccaccggttcatgtgggcaacaatcaggagctgtgtacgtgggcaattacaggattgtaaacagacacctggcaacgagccacgattggcaaaattgcgtgtgggaggactacaacagggatctcctggtcagcacaacaactgctcatggttgtgatactatagcacggtgccaatgtactgctggcgtgtacttttgtgcatctagaaacaagcactacccagtgagcttcgagggtccaggtctagtgaaagttcaggagggcgagtactaccccgagagataccagtcgcacgtactccttgcagttggattttcagaaccgggtgattgtggaggtattttgaggtgtgaacatggagtcattgggctcgttaccatgggtggtgagggtgtagtaggcttcgctgacgtgcgggatcttttgtggttggaagacgacgccatggagcagggtgttagagattatgtagagcaactgggaaatgcatttggctcaggtttcactaaccaaatctgtgagcaagttaacctccttaaagaatctctgatagggcaggattccatattggaaaaatccctgaaggccctggttaaaatcatatcagccctggtgatagtggttaggaaccacgacgacctgattacagtgactgccacactagctttaatcggttgcgcatcatctccatggcgatggctcaaacaaaaagtgtgtcaatactacggaatccccatggcagaaaggcagaataacggttggttaaagaaattcactgaaatgaccaacgcctgcaagggcatggagtggattgctgttaaaattcaaaagttcatcgagtggctcaaagtaaagattctgcctgaagtgaaggagaaacatgagttccttaccagattgaagcaattgccactccttgaaagtcaaattgccaccattgagcaaagcgcaccctcacaaagtgatcaagagcagcttttttcgaatgttcagtacttcgcccattactgcaggaagtatgcacctctgtatgctgccgaagcaaaaagagtgttctcattagaaaagaaaatgagtaattacatacagttcaagtccaaatgccgcattgagcctgtatgcttactccttcacggtagtccaggggctggcaagtcagtagctaccaacctgatagggagatcccttgcagagaagctcaatagctctgtgtactctttaccaccagatccagatcattttgatgggtacaaacagcaggcagtggtgatcatggatgatctctgtcaaaaccccgatgggaaggacgtgtccttgttttgccaaatggtgtctagtgtagattttgtgccacccatggcggcgctggaagaaaaaggcattctctttacgtccccgtttgtgttggcatcaaccaacgcggggtccatcaatgcaccaacagtgtcagacagcagagcacttgccagaaggtttcactttgacatgaatattgaggtgatttcgatgtacagccagaatggtaaaattaacatgcccatgtctgttaagacatgtgatgatgaatgctgcccggtcaatttcaaaaagtgttgcccactagtgtgtggcaaggccatccagtttattgacaggagaaaccaagttagatattcactggacatgctggttactgagatgtttagagagtacaaccacagacacagtgtgggtgctaccctcgaggctttgttccaaggaccaccagtatacagggaaatcaaaatcagtgtggccccggaaacaccccctccaccagcaattgctgaccttctaaaatctgtagacagtgaggcaataagggagtactgcaaggaaaggggttggcttgtgccagaggtcagctccactctacaaattgaaaaacatgttagcagggcatttatttgcttgcaagcgctaactacatttgtttcagtggctggtataatctacatcatttacaagttgtttgccggctttcagggtgcatacactggaatgcccaaccagaaacccaaggtgcccaccttaagacaagctaaggtgcaaggtccggcatttgaatttgccgtagcaatgatgaaaaggaacgccagcacagtcaagacagaatacggtgagttcacgatgcttggcatctatgataaatgggcagtgctgccgcgccacgccaagcctggaccaactattttaatgaatgatcaggaggttggtgtgctcgatgccaaagagttagttgataaagacggaaccaacctggagctgacactattgaagcttaaccgcaatgaaaagttcagagacatcagaggttttcttgcaagggaagaagttgaggtaagtgaggctgttttggcaataaacacgagcaagttcccaagcatgtacatccctgtgggccaagtcaccgattacggatttttaaatctaggtggcaccccaacaaagagaatgctcatgtacaacttccctaccagagcgggacagtgtggtggtgtccttatgtcaacaggaaaggtccttggcatacacgtgggaggaaatggtcaccaaggcttctctgctgctctcctcagacactacttcaacgaggaacagggcgaaatagagtttattgagagctctaaagatgcaggatttcctgtgatcaacacccctaataaaaccaaactggaaccaagtgtgtttcatcaggtttttgagggcaacaaagaaccagcagtcctaagaaacggagacccgcgacttaaagccaactttgaggaagcgatattttccaagtacatcggaaatgtgaacacacatgtggacgagtacatgatagaagctgttgatcactacgctggacagctggcaactctggacatcagtacagaacctatgaagcttgaggatgctgtttatggcactgaaggcttggaagcattggacttgaccactagcgcaggatatccttatgtcgccttgggcatcaagaaaagggatatcctctccaagaagactaaagatctcaccaagctgagggaatgcatggacaagtatggtctaaatctgccgatggtgacctacgtgaaggatgaactcaggtccgctgagaaagtagccaagggaaaatccagacttatagaagcttctagtctcaatgactcagtggccatgaggcagacatttgggaacctatacaagacattccacctcaacccaggcattgtcactggtagtgctgttgggtgcgacccagatgtgttttggagcaaaatacccgtgatgcttgacgggcaccttatagcttttgattactctggctacgacgctagcttgagcccagtgtggtttgcttgtttgaaactcctcctagggaaactagggtatactcataaggaaaccaattacatagactacctctgcaactcccatcacttatacagagataaacactatttcgtgaggggtggtatgccatcaggatgttcaggcaccagtatattcaacaccatgatcaacaacatcattattaggacccttatgctaaaggtctacaaaggtattgacctggatcagtttagaatgatcgcttacggggacgatgtgatagcctcttacccgtggcctattgatgcctcactactagcagaagcgggaaaggattatggtttgatcatgaccccagcagataaaggagagtgttttaatgaggtaacctggacaaatgtaaccttcttgaaaaggtactttagagctgatgaacaatatccattcttggtgcaccccgtgatgcccatgaaagacatacacgaatccattagatggaccaaagacccaaagaacactcaagatcatgtgcgctcgttatgcctattggcttggcacaatggggagcacgaatatgaggaatttatccgaaagatcagaagcgtgcctgttggacgctgtttgaccctcccggtgttctcaacactacgcaggaaatggttagattccttctaaaattagagtgcaatcaatgaactatgattggcttaaccctaccgcatgaaccgaactagacaaaagtgcggtaggggtaaattctccgcattcggtgcggaaaaaaaaaaaaaaaaaaaaaaaaaaaaaaaaaaaaaaaaaaaaaaaaaa

SEQ ID NO: 191 - DNA, 8377 bp, synthetic construct
  source 1..8377: mol_type = other DNA
  misc_feature 1..8377: note = H3N2_P2A_Luci DNA vector construct
ttaaaacagcctgtgggttgtacccacccacagggcccactgggcgctagcactctggtatcacggtacctttgtgtgcctgttttatatcccctttccccgattgtaacttagaagatgtacacactgatcaatagcgggcatagcacaccagctatgtcttgatcaagcactcctgtatccccggaccaagtatcaatagactgctcacgcggttgaaggagaaaacgttcgtcacccggctaactacttcgagaaacccagtagtatcatgaaagttgcgaggcgtttcgttcagcacacccccagtgtagatcgggtcgatgagtcaccgcatcccccacgggcgaccgtggcggtggctgcgctggcggcctgcctacggggcaacccgtaggacgcttcaatacagacatggtgcgaagagtcgattgagctagttagtagtcctccggcccctgaatgcggctaatcctaactgcggagcacatgccctcaacccagggggtattgtgtcgtaacgggcaactctgcagcggaaccgactactttgggtgtccgtgtttccttttatccttatactggctgcttatggtgacaattgaaagattgttgccatatagctattggattggccatccagtgtctaatagagctgttatttacctctttgttggatttataccactcaacctaaaagaagttaaaacactacagctcattttacaactgaatacagcaaaccaccatgaaaaccgtgatcgccctcagttacatcttctgcctcgcctttggacagaatctcctcggaaacgaaaacaacgctgccacactctgcctgggacaccacgccgtgcccaacggcacaatggtgaagaccatcaccgacgatcagatcgaggtgaccaatgccaccgagctggtgcagaacagctccaccggcaaaatctgcaacaatccccacaagatcctggacggcagggattgcaccctgatcgacgctctgctgggcgaccctcactgcgacgtgttccagaatgagacatgggatctgttcgtggagaggagcaatgccttctccaactgctacccctacgacgtgcctgattacgccagcctgcggtccatcgtggccagctccggcaccctggagttcatcaccgagggcttcacctgggctggagtgacccagaacggaggcagcggagcttgcaagaggggacccgccaatagcttcttctcccggctgaactggctgaccaagtccggcaatacctaccccgtgctgaacgtgaccatgcctaacaataacaatttcgacaagctgtacatctggggcgtgcatcaccctagcaccgatcaggagcagaccagcctgtacatccaggcctccggcagggtgaccgtgagcaccaggcggtcccagcagaccatcatccccaacatcggctccaggcctctggtgcggggacagagcggccggatctccgtgtactggaccatcgtgaagcccggcgacatcctggtcatcaacagcaatggcaacctgatcgcccctcgcggctacttcaagatgcacatcggcaagagcagcatcatgagatccgacgcccccatcgatacctgcatcagcgagtgcatcacccctaatggctccatccccaacgagaagcctttccagaatgtgaacaagatcacctacggcgcctgccccaagtacgtgaagcagaataccctgaagctggccaccggcatgcgcaacgtgcctgagagacagaccgtgggcctgttcggagctatcgctggcttcatcgagaatggctgggagggcatggtggacggctggtacggcttccgccaccagaacagcgagggcaccggacaggctgccgacctgaagtccacccaggccgccatcgatcagatcaatggcaagctgaacagagtgatcgagaagaccaacgagaagttccaccagatcgagaaggagttcagcgaggtggagggacgcatccaggacctggagaggtacgtggaggacaccaagatcgatctgtggagctacaatgccgagctgctggtggccctggagaatcagaacaccatcgacctgaccgattccgagatgaacaagctgttcgagaagacccgcagacagctgcgcgagaatgccgaggacatgggcaacggctgcttcaaaatctaccacaagtgcgataacgcctgcatcgagagcatcagaaatggcacctacgaccacaacatctaccgcgatgaggccgtgaacaatagattccagatcaagggcgtggagctgaagtccggctacaaggactggattctgtggatcagcttcgccatctcctgcttcctgctgtgcgtggtgctgctggggtttattatgtgggcttgtcagagggggaacatcaggtgtaacatttgtattggaagcggagctactaacttcagcctgctgaagcaggctggacaggtggaggagaaccctggacctatggaagacgccaaaaacataaagaaaggcccggcgccattctatccgctggaagatggaaccgctggagagcaactgcataaggctatgaagagatacgccctggttcctggaacaattgcttttacagatgcacatatcgaggtggacatcacttacgctgagtacttcgaaatgtccgttcggttggcagaagctatgaaacgatatgggctgaatacaaatcacagaatcgtcgtatgcagtgaaaactctcttcaattctttatgccggtgttgggcgcgttatttatcggagttgcagttgcgcccgcgaacgacatttataatgaacgtgaattgctcaacagtatgggcatttcgcagcctaccgtggtgttcgtttccaaaaaggggttgcaaaaaattttgaacgtgcaaaaaaagctcccaatcatccaaaaaattattatcatggattctaaaacggattaccagggatttcagtcgatgtacacgttcgtcacatctcatctacctcccggttttaatgaatacgattttgtgccagagtccttcgatagggacaagacaattgcactgatcatgaactcctctggatctactggtctgcctaaaggtgtcgctctgcctcatagaactgcctgcgtgagattctcgcatgccagagatcctatttttggcaatcaaatcattccggatactgcgattttaagtgttgttccattccatcacggttttggaatgtttactacactcggatatttgatatgtggatttcgagtcgtcttaatgtatagatttgaagaagagctgtttctgaggagccttcaggattacaagattcaaagtgcgctgctggtgccaaccctattctccttcttcgccaaaagcactctgattgacaaatacgatttatctaatttacacgaaattgcttctggtggcgctcccctctctaaggaagtcggggaagcggttgccaagaggttccatctgccaggtatcaggcaaggatatgggctcactgagactacatcagctattctgattacacccgagggggatgataaaccgggcgcggtcggtaaagttgttccattttttgaagcgaaggttgtggatctggataccgggaaaacgctgggcgttaatcaaagaggcgaactgtgtgtgagaggtcctatgattatgtccggttatgtaaacaatccggaagcgaccaacgccttgattgacaaggatggatggctacattctggagacatagcttactgggacgaagacgaacacttcttcatcgttgaccgcctgaagtctctgattaagtacaaaggctatcaggtggctcccgctgaattggaatccatcttgctccaacaccccaacatcttcgacgcaggtgtcgcaggtcttcccgacgatgacgccggtgaacttcccgccgccgttgttgttttggagcacggaaagacgatgacggaaaaagagatcgtggattacgtcgccagtcaagtaacaaccgcgaaaaagttgcgcggaggagttgtgtttgtggacgaagtaccgaaaggtcttaccggaaaactcgacgcaagaaaaatcagagagatcctcataaaggccaagaagggcggaaagatcgccgtgaactttgagccaacaggggtgacggagtcccgcactgaaattacggcaatgcagaccaccggttcatgtgggcaacaatcaggagctgtgtacgtgggcaattacaggattgtaaacagacacctggcaacgagccacgattggcaaaattgcgtgtgggaggactacaacagggatctcctggtcagcacaacaactgctcatggttgtgatactatagcacggtgccaatgtactgctggcgtgtacttttgtgcatctagaaacaagcactacccagtgagcttcgagggtccaggtctagtgaaagttcaggagggcgagtactaccccgagagataccagtcgcacgtactccttgcagttggattttcagaaccgggtgattgtggaggtattttgaggtgtgaacatggagtcattgggctcgttaccatgggtggtgagggtgtagtaggcttcgctgacgtgcgggatcttttgtggttggaagacgacgccatggagcagggtgttagagattatgtagagcaactgggaaatgcatttggctcaggtttcactaaccaaatctgtgagcaagttaacctccttaaagaatctctgatagggcaggattccatattggaaaaatccctgaaggccctggttaaaatcatatcagccctggtgatagtggttaggaaccacgacgacctgattacagtgactgccacactagctttaatcggttgcgcatcatctccatggcgatggctcaaacaaaaagtgtgtcaatactacggaatccccatggcagaaaggcagaataacggttggttaaagaaattcactgaaatgaccaacgcctgcaagggcatggagtggattgctgttaaaattcaaaagttcatcgagtggctcaaagtaaagattctgcctgaagtgaaggagaaacatgagttccttaccagattgaagcaattgccactccttgaaagtcaaattgccaccattgagcaaagcgcaccctcacaaagtgatcaagagcagcttttttcgaatgttcagtacttcgcccattactgcaggaagtatgcacctctgtatgctgccgaagcaaaaagagtgttctcattagaaaagaaaatgagtaattacatacagttcaagtccaaatgccgcattgagcctgtatgcttactccttcacggtagtccaggggctggcaagtcagtagctaccaacctgatagggagatcccttgcagagaagctcaatagctctgtgtactctttaccaccagatccagatcattttgatgggtacaaacagcaggcagtggtgatcatggatgatctctgtcaaaaccccgatgggaaggacgtgtccttgttttgccaaatggtgtctagtgtagattttgtgccacccatggcggcgctggaagaaaaaggcattctctttacgtccccgtttgtgttggcatcaaccaacgcggggtccatcaatgcaccaacagtgtcagacagcagagcacttgccagaaggtttcactttgacatgaatattgaggtgatttcgatgtacagccagaatggtaaaattaacatgcccatgtctgttaagacatgtgatgatgaatgctgcccggtcaatttcaaaaagtgttgcccactagtgtgtggcaaggccatccagtttattgacaggagaaaccaagttagatattcactggacatgctggttactgagatgtttagagagtacaaccacagacacagtgtgggtgctaccctcgaggctttgttccaaggaccaccagtatacagggaaatcaaaatcagtgtggccccggaaacaccccctccaccagcaattgctgaccttctaaaatctgtagacagtgaggcaataagggagtactgcaaggaaaggggttggcttgtgccagaggtcagctccactctacaaattgaaaaacatgttagcagggcatttatttgcttgcaagcgctaactacatttgtttcagtggctggtataatctacatcatttacaagttgtttgccggctttcagggtgcatacactggaatgcccaaccagaaacccaaggtgcccaccttaagacaagctaaggtgcaaggtccggcatttgaatttgccgtagcaatgatgaaaaggaacgccagcacagtcaagacagaatacggtgagttcacgatgcttggcatctatgataaatgggcagtgctgccgcgccacgccaagcctggaccaactattttaatgaatgatcaggaggttggtgtgctcgatgccaaagagttagttgataaagacggaaccaacctggagctgacactattgaagcttaaccgcaatgaaaagttcagagacatcagaggttttcttgcaagggaagaagttgaggtaagtgaggctgttttggcaataaacacgagcaagttcccaagcatgtacatccctgtgggccaagtcaccgattacggatttttaaatctaggtggcaccccaacaaagagaatgctcatgtacaacttccctaccagagcgggacagtgtggtggtgtccttatgtcaacaggaaaggtccttggcatacacgtgggaggaaatggtcaccaaggcttctctgctgctctcctcagacactacttcaacgaggaacagggcgaaatagagtttattgagagctctaaagatgcaggatttcctgtgatcaacacccctaataaaaccaaactggaaccaagtgtgtttcatcaggtttttgagggcaacaaagaaccagcagtcctaagaaacggagacccgcgacttaaagccaactttgaggaagcgatattttccaagtacatcggaaatgtgaacacacatgtggacgagtacatgatagaagctgttgatcactacgctggacagctggcaactctggacatcagtacagaacctatgaagcttgaggatgctgtttatggcactgaaggcttggaagcattggacttgaccactagcgcaggatatccttatgtcgccttgggcatcaagaaaagggatatcctctccaagaagactaaagatctcaccaagctgagggaatgcatggacaagtatggtctaaatctgccgatggtgacctacgtgaaggatgaactcaggtccgctgagaaagtagccaagggaaaatccagacttatagaagcttctagtctcaatgactcagtggccatgaggcagacatttgggaacctatacaagacattccacctcaacccaggcattgtcactggtagtgctgttgggtgcgacccagatgtgttttggagcaaaatacccgtgatgcttgacgggcaccttatagcttttgattactctggctacgacgctagcttgagcccagtgtggtttgcttgtttgaaactcctcctagggaaactagggtatactcataaggaaaccaattacatagactacctctgcaactcccatcacttatacagagataaacactatttcgtgaggggtggtatgccatcaggatgttcaggcaccagtatattcaacaccatgatcaacaacatcattattaggacccttatgctaaaggtctacaaaggtattgacctggatcagtttagaatgatcgcttacggggacgatgtgatagcctcttacccgtggcctattgatgcctcactactagcagaagcgggaaaggattatggtttgatcatgaccccagcagataaaggagagtgttttaatgaggtaacctggacaaatgtaaccttcttgaaaaggtactttagagctgatgaacaatatccattcttggtgcaccccgtgatgcccatgaaagacatacacgaatccattagatggaccaaagacccaaagaacactcaagatcatgtgcgctcgttatgcctattggcttggcacaatggggagcacgaatatgaggaatttatccgaaagatcagaagcgtgcctgttggacgctgtttgaccctcccggtgttctcaacactacgcaggaaatggttagattccttctaaaattagagtgcaatcaatgaactatgattggcttaaccctaccgcatgaaccgaactagacaaaagtgcggtaggggtaaattctccgcattcggtgcggaaaaaaaaaaaaaaaaaaaaaaaaaaaaaaaaaaaaaaaaaaaaaaaaaa

SEQ ID NO: 192 - RNA, 8347 nt, synthetic construct
  source 1..8347: mol_type = other RNA
  misc_feature 1..8347: note = H3N2_3C protease recognition region_Luci saRNA construct
ttaaaacagcctgtgggttgtacccacccacagggcccactgggcgctagcactctggtatcacggtacctttgtgtgcctgttttatatcccctttccccgattgtaacttagaagatgtacacactgatcaatagcgggcatagcacaccagctatgtcttgatcaagcactcctgtatccccggaccaagtatcaatagactgctcacgcggttgaaggagaaaacgttcgtcacccggctaactacttcgagaaacccagtagtatcatgaaagttgcgaggcgtttcgttcagcacacccccagtgtagatcgggtcgatgagtcaccgcatcccccacgggcgaccgtggcggtggctgcgctggcggcctgcctacggggcaacccgtaggacgcttcaatacagacatggtgcgaagagtcgattgagctagttagtagtcctccggcccctgaatgcggctaatcctaactgcggagcacatgccctcaacccagggggtattgtgtcgtaacgggcaactctgcagcggaaccgactactttgggtgtccgtgtttccttttatccttatactggctgcttatggtgacaattgaaagattgttgccatatagctattggattggccatccagtgtctaatagagctgttatttacctctttgttggatttataccactcaacctaaaagaagttaaaacactacagctcattttacaactgaatacagcaaaccaccatgaaaaccgtgatcgccctcagttacatcttctgcctcgcctttggacagaatctcctcggaaacgaaaacaacgctgccacactctgcctgggacaccacgccgtgcccaacggcacaatggtgaagaccatcaccgacgatcagatcgaggtgaccaatgccaccgagctggtgcagaacagctccaccggcaaaatctgcaacaatccccacaagatcctggacggcagggattgcaccctgatcgacgctctgctgggcgaccctcactgcgacgtgttccagaatgagacatgggatctgttcgtggagaggagcaatgccttctccaactgctacccctacgacgtgcctgattacgccagcctgcggtccatcgtggccagctccggcaccctggagttcatcaccgagggcttcacctgggctggagtgacccagaacggaggcagcggagcttgcaagaggggacccgccaatagcttcttctcccggctgaactggctgaccaagtccggcaatacctaccccgtgctgaacgtgaccatgcctaacaataacaatttcgacaagctgtacatctggggcgtgcaccaccctagcaccgatcaggagcagaccagcctgtacatccaggcctccggcagggtgaccgtgagcaccaggcggtcccagcagaccatcatccccaacatcggctccaggcctctggtgcggggacagagcggccggatctccgtgtactggaccatcgtgaagcccggcgacatcctggtcatcaacagcaatggcaacctgatcgcccctcgcggctacttcaagatgcacatcggcaagagcagcatcatgagatccgacgcccccatcgatacctgcatcagcgagtgcatcacccctaatggctccatccccaacgagaagcctttccagaatgtgaacaagatcacctacggcgcctgccccaagtacgtgaagcagaataccctgaagctggccaccggcatgcgcaacgtgcctgagagacagaccgtgggcctgttcggagctatcgctggcttcatcgagaatggctgggagggcatggtggacggctggtacggcttccgccaccagaacagcgagggcaccggacaggctgccgacctgaagtccacccaggccgccatcgatcagatcaatggcaagctgaacagagtgatcgagaagaccaacgagaagttccaccagatcgagaaggagttcagcgaggtggagggacgcatccaggacctggagaggtacgtggaggacaccaagatcgatctgtggagctacaatgccgagctgctggtggccctggagaatcagaacaccatcgacctgaccgattccgagatgaacaagctgttcgagaagacccgcagacagctgcgcgagaatgccgaggacatgggcaacggctgcttcaaaatctaccacaagtgcgataacgcctgcatcgagagcatcagaaatggcacctacgaccacaacatctaccgcgatgaggccgtgaacaatagattccagatcaagggcgtggagctgaagtccggctacaaggactggattctgtggatcagcttcgccatctcctgcttcctgctgtgcgtggtgctgctggggtttattatgtgggcttgtcagagggggaacatcaggtgtaacatttgtattcaggacaactttttccaaggaccacccggggaagctatggaagacgccaaaaacataaagaaaggcccggcgccattctatccgctggaagatggaaccgctggagagcaactgcataaggctatgaagagatacgccctggttcctggaacaattgcttttacagatgcacatatcgaggtggacatcacttacgctgagtacttcgaaatgtccgttcggttggcagaagctatgaaacgatatgggctgaatacaaatcacagaatcgtcgtatgcagtgaaaactctcttcaattctttatgccggtgttgggcgcgttatttatcggagttgcagttgcgcccgcgaacgacatttataatgaacgtgaattgctcaacagtatgggcatttcgcagcctaccgtggtgttcgtttccaaaaaggggttgcaaaaaattttgaacgtgcaaaaaaagctcccaatcatccaaaaaattattatcatggattctaaaacggattaccagggatttcagtcgatgtacacgttcgtcacatctcatctacctcccggttttaatgaatacgattttgtgccagagtccttcgatagggacaagacaattgcactgatcatgaactcctctggatctactggtctgcctaaaggtgtcgctctgcctcatagaactgcctgcgtgagattctcgcatgccagagatcctatttttggcaatcaaatcattccggatactgcgattttaagtgttgttccattccatcacggttttggaatgtttactacactcggatatttgatatgtggatttcgagtcgtcttaatgtatagatttgaagaagagctgtttctgaggagccttcaggattacaagattcaaagtgcgctgctggtgccaaccctattctccttcttcgccaaaagcactctgattgacaaatacgatttatctaatttacacgaaattgcttctggtggcgctcccctctctaaggaagtcggggaagcggttgccaagaggttccatctgccaggtatcaggcaaggatatgggctcactgagactacatcagctattctgattacacccgagggggatgataaaccgggcgcggtcggtaaagttgttccattttttgaagcgaaggttgtggatctggataccgggaaaacgctgggcgttaatcaaagaggcgaactgtgtgtgagaggtcctatgattatgtccggttatgtaaacaatccggaagcgaccaacgccttgattgacaaggatggatggctacattctggagacatagcttactgggacgaagacgaacacttcttcatcgttgaccgcctgaagtctctgattaagtacaaaggctatcaggtggctcccgctgaattggaatccatcttgctccaacaccccaacatcttcgacgcaggtgtcgcaggtcttcccgacgatgacgccggtgaacttcccgccgccgttgttgttttggagcacggaaagacgatgacggaaaaagagatcgtggattacgtcgccagtcaagtaacaaccgcgaaaaagttgcgcggaggagttgtgtttgtggacgaagtaccgaaaggtcttaccggaaaactcgacgcaagaaaaatcagagagatcctcataaaggccaagaagggcggaaagatcgccgtgaactttgagccaacaggggtgacggagtcccgcactgaaattacggcaatgcagaccaccggttcatgtgggcaacaatcaggagctgtgtacgtgggcaattacaggattgtaaacagacacctggcaacgagccacgattggcaaaattgcgtgtgggaggactacaacagggatctcctggtcagcacaacaactgctcatggttgtgatactatagcacggtgccaatgtactgctggcgtgtacttttgtgcatctagaaacaagcactacccagtgagcttcgagggtccaggtctagtgaaagttcaggagggcgagtactaccccgagagataccagtcgcacgtactccttgcagttggattttcagaaccgggtgattgtggaggtattttgaggtgtgaacatggagtcattgggctcgttaccatgggtggtgagggtgtagtaggcttcgctgacgtgcgggatcttttgtggttggaagacgacgccatggagcagggtgttagagattatgtagagcaactgggaaatgcatttggctcaggtttcactaaccaaatctgtgagcaagttaacctccttaaagaatctctgatagggcaggattccatattggaaaaatccctgaaggccctggttaaaatcatatcagccctggtgatagtggttaggaaccacgacgacctgattacagtgactgccacactagctttaatcggttgcgcatcatctccatggcgatggctcaaacaaaaagtgtgtcaatactacggaatccccatggcagaaaggcagaataacggttggttaaagaaattcactgaaatgaccaacgcctgcaagggcatggagtggattgctgttaaaattcaaaagttcatcgagtggctcaaagtaaagattctgcctgaagtgaaggagaaacatgagttccttaccagattgaagcaattgccactccttgaaagtcaaattgccaccattgagcaaagcgcaccctcacaaagtgatcaagagcagcttttttcgaatgttcagtacttcgcccattactgcaggaagtatgcacctctgtatgctgccgaagcaaaaagagtgttctcattagaaaagaaaatgagtaattacatacagttcaagtccaaatgccgcattgagcctgtatgcttactccttcacggtagtccaggggctggcaagtcagtagctaccaacctgatagggagatcccttgcagagaagctcaatagctctgtgtactctttaccaccagatccagatcattttgatgggtacaaacagcaggcagtggtgatcatggatgatctctgtcaaaaccccgatgggaaggacgtgtccttgttttgccaaatggtgtctagtgtagattttgtgccacccatggcggcgctggaagaaaaaggcattctctttacgtccccgtttgtgttggcatcaaccaacgcggggtccatcaatgcaccaacagtgtcagacagcagagcacttgccagaaggtttcactttgacatgaatattgaggtgatttcgatgtacagccagaatggtaaaattaacatgcccatgtctgttaagacatgtgatgatgaatgctgcccggtcaatttcaaaaagtgttgcccactagtgtgtggcaaggccatccagtttattgacaggagaaaccaagttagatattcactggacatgctggttactgagatgtttagagagtacaaccacagacacagtgtgggtgctaccctcgaggctttgttccaaggaccaccagtatacagggaaatcaaaatcagtgtggccccggaaacaccccctccaccagcaattgctgaccttctaaaatctgtagacagtgaggcaataagggagtactgcaaggaaaggggttggcttgtgccagaggtcagctccactctacaaattgaaaaacatgttagcagggcatttatttgcttgcaagcgctaactacatttgtttcagtggctggtataatctacatcatttacaagttgtttgccggctttcagggtgcatacactggaatgcccaaccagaaacccaaggtgcccaccttaagacaagctaaggtgcaaggtccggcatttgaatttgccgtagcaatgatgaaaaggaacgccagcacagtcaagacagaatacggtgagttcacgatgcttggcatctatgataaatgggcagtgctgccgcgccacgccaagcctggaccaactattttaatgaatgatcaggaggttggtgtgctcgatgccaaagagttagttgataaagacggaaccaacctggagctgacactattgaagcttaaccgcaatgaaaagttcagagacatcagaggttttcttgcaagggaagaagttgaggtaagtgaggctgttttggcaataaacacgagcaagttcccaagcatgtacatccctgtgggccaagtcaccgattacggatttttaaatctaggtggcaccccaacaaagagaatgctcatgtacaacttccctaccagagcgggacagtgtggtggtgtccttatgtcaacaggaaaggtccttggcatacacgtgggaggaaatggtcaccaaggcttctctgctgctctcctcagacactacttcaacgaggaacagggcgaaatagagtttattgagagctctaaagatgcaggatttcctgtgatcaacacccctaataaaaccaaactggaaccaagtgtgtttcatcaggtttttgagggcaacaaagaaccagcagtcctaagaaacggagacccgcgacttaaagccaactttgaggaagcgatattttccaagtacatcggaaatgtgaacacacatgtggacgagtacatgatagaagctgttgatcactacgctggacagctggcaactctggacatcagtacagaacctatgaagcttgaggatgctgtttatggcactgaaggcttggaagcattggacttgaccactagcgcaggatatccttatgtcgccttgggcatcaagaaaagggatatcctctccaagaagactaaagatctcaccaagctgagggaatgcatggacaagtatggtctaaatctgccgatggtgacctacgtgaaggatgaactcaggtccgctgagaaagtagccaagggaaaatccagacttatagaagcttctagtctcaatgactcagtggccatgaggcagacatttgggaacctatacaagacattccacctcaacccaggcattgtcactggtagtgctgttgggtgcgacccagatgtgttttggagcaaaatacccgtgatgcttgacgggcaccttatagcttttgattactctggctacgacgctagcttgagcccagtgtggtttgcttgtttgaaactcctcctagggaaactagggtatactcataaggaaaccaattacatagactacctctgcaactcccatcacttatacagagataaacactatttcgtgaggggtggtatgccatcaggatgttcaggcaccagtatattcaacaccatgatcaacaacatcattattaggacccttatgctaaaggtctacaaaggtattgacctggatcagtttagaatgatcgcttacggggacgatgtgatagcctcttacccgtggcctattgatgcctcactactagcagaagcgggaaaggattatggtttgatcatgaccccagcagataaaggagagtgttttaatgaggtaacctggacaaatgtaaccttcttgaaaaggtactttagagctgatgaacaatatccattcttggtgcaccccgtgatgcccatgaaagacatacacgaatccattagatggaccaaagacccaaagaacactcaagatcatgtgcgctcgttatgcctattggcttggcacaatggggagcacgaatatgaggaatttatccgaaagatcagaagcgtgcctgttggacgctgtttgaccctcccggtgttctcaacactacgcaggaaatggttagattccttctaaaattagagtgcaatcaatgaactatgattggcttaaccctaccgcatgaaccgaactagacaaaagtgcggtaggggtaaattctccgcattcggtgcggaaaaaaaaaaaaaaaaaaaaaaaaaaaaaaaaaaaaaaaaaaaaaaaaaa

SEQ ID NO: 193 - DNA, 8347 bp, synthetic construct
  source 1..8347: mol_type = other DNA
  misc_feature 1..8347: note = H3N2_3C protease recognition region_Luci DNA vector construct
ttaaaacagcctgtgggttgtacccacccacagggcccactgggcgctagcactctggtatcacggtacctttgtgtgcctgttttatatcccctttccccgattgtaacttagaagatgtacacactgatcaatagcgggcatagcacaccagctatgtcttgatcaagcactcctgtatccccggaccaagtatcaatagactgctcacgcggttgaaggagaaaacgttcgtcacccggctaactacttcgagaaacccagtagtatcatgaaagttgcgaggcgtttcgttcagcacacccccagtgtagatcgggtcgatgagtcaccgcatcccccacgggcgaccgtggcggtggctgcgctggcggcctgcctacggggcaacccgtaggacgcttcaatacagacatggtgcgaagagtcgattgagctagttagtagtcctccggcccctgaatgcggctaatcctaactgcggagcacatgccctcaacccagggggtattgtgtcgtaacgggcaactctgcagcggaaccgactactttgggtgtccgtgtttccttttatccttatactggctgcttatggtgacaattgaaagattgttgccatatagctattggattggccatccagtgtctaatagagctgttatttacctctttgttggatttataccactcaacctaaaagaagttaaaacactacagctcattttacaactgaatacagcaaaccaccatgaaaaccgtgatcgccctcagttacatcttctgcctcgcctttggacagaatctcctcggaaacgaaaacaacgctgccacactctgcctgggacaccacgccgtgcccaacggcacaatggtgaagaccatcaccgacgatcagatcgaggtgaccaatgccaccgagctggtgcagaacagctccaccggcaaaatctgcaacaatccccacaagatcctggacggcagggattgcaccctgatcgacgctctgctgggcgaccctcactgcgacgtgttccagaatgagacatgggatctgttcgtggagaggagcaatgccttctccaactgctacccctacgacgtgcctgattacgccagcctgcggtccatcgtggccagctccggcaccctggagttcatcaccgagggcttcacctgggctggagtgacccagaacggaggcagcggagcttgcaagaggggacccgccaatagcttcttctcccggctgaactggctgaccaagtccggcaatacctaccccgtgctgaacgtgaccatgcctaacaataacaatttcgacaagctgtacatctggggcgtgcaccaccctagcaccgatcaggagcagaccagcctgtacatccaggcctccggcagggtgaccgtgagcaccaggcggtcccagcagaccatcatccccaacatcggctccaggcctctggtgcggggacagagcggccggatctccgtgtactggaccatcgtgaagcccggcgacatcctggtcatcaacagcaatggcaacctgatcgcccctcgcggctacttcaagatgcacatcggcaagagcagcatcatgagatccgacgcccccatcgatacctgcatcagcgagtgcatcacccctaatggctccatccccaacgagaagcctttccagaatgtgaacaagatcacctacggcgcctgccccaagtacgtgaagcagaataccctgaagctggccaccggcatgcgcaacgtgcctgagagacagaccgtgggcctgttcggagctatcgctggcttcatcgagaatggctgggagggcatggtggacggctggtacggcttccgccaccagaacagcgagggcaccggacaggctgccgacctgaagtccacccaggccgccatcgatcagatcaatggcaagctgaacagagtgatcgagaagaccaacgagaagttccaccagatcgagaaggagttcagcgaggtggagggacgcatccaggacctggagaggtacgtggaggacaccaagatcgatctgtggagctacaatgccgagctgctggtggccctggagaatcagaacaccatcgacctgaccgattccgagatgaacaagctgttcgagaagacccgcagacagctgcgcgagaatgccgaggacatgggcaacggctgcttcaaaatctaccacaagtgcgataacgcctgcatcgagagcatcagaaatggcacctacgaccacaacatctaccgcgatgaggccgtgaacaatagattccagatcaagggcgtggagctgaagtccggctacaaggactggattctgtggatcagcttcgccatctcctgcttcctgctgtgcgtggtgctgctggggtttattatgtgggcttgtcagagggggaacatcaggtgtaacatttgtattcaggacaactttttccaaggaccacccggggaagctatggaagacgccaaaaacataaagaaaggcccggcgccattctatccgctggaagatggaaccgctggagagcaactgcataaggctatgaagagatacgccctggttcctggaacaattgcttttacagatgcacatatcgaggtggacatcacttacgctgagtacttcgaaatgtccgttcggttggcagaagctatgaaacgatatgggctgaatacaaatcacagaatcgtcgtatgcagtgaaaactctcttcaattctttatgccggtgttgggcgcgttatttatcggagttgcagttgcgcccgcgaacgacatttataatgaacgtgaattgctcaacagtatgggcatttcgcagcctaccgtggtgttcgtttccaaaaaggggttgcaaaaaattttgaacgtgcaaaaaaagctcccaatcatccaaaaaattattatcatggattctaaaacggattaccagggatttcagtcgatgtacacgttcgtcacatctcatctacctcccggttttaatgaatacgattttgtgccagagtccttcgatagggacaagacaattgcactgatcatgaactcctctggatctactggtctgcctaaaggtgtcgctctgcctcatagaactgcctgcgtgagattctcgcatgccagagatcctatttttggcaatcaaatcattccggatactgcgattttaagtgttgttccattccatcacggttttggaatgtttactacactcggatatttgatatgtggatttcgagtcgtcttaatgtatagatttgaagaagagctgtttctgaggagccttcaggattacaagattcaaagtgcgctgctggtgccaaccctattctccttcttcgccaaaagcactctgattgacaaatacgatttatctaatttacacgaaattgcttctggtggcgctcccctctctaaggaagtcggggaagcggttgccaagaggttccatctgccaggtatcaggcaaggatatgggctcactgagactacatcagctattctgattacacccgagggggatgataaaccgggcgcggtcggtaaagttgttccattttttgaagcgaaggttgtggatctggataccgggaaaacgctgggcgttaatcaaagaggcgaactgtgtgtgagaggtcctatgattatgtccggttatgtaaacaatccggaagcgaccaacgccttgattgacaaggatggatggctacattctggagacatagcttactgggacgaagacgaacacttcttcatcgttgaccgcctgaagtctctgattaagtacaaaggctatcaggtggctcccgctgaattggaatccatcttgctccaacaccccaacatcttcgacgcaggtgtcgcaggtcttcccgacgatgacgccggtgaacttcccgccgccgttgttgttttggagcacggaaagacgatgacggaaaaagagatcgtggattacgtcgccagtcaagtaacaaccgcgaaaaagttgcgcggaggagttgtgtttgtggacgaagtaccgaaaggtcttaccggaaaactcgacgcaagaaaaatcagagagatcctcataaaggccaagaagggcggaaagatcgccgtgaactttgagccaacaggggtgacggagtcccgcactgaaattacggcaatgcagaccaccggttcatgtgggcaacaatcaggagctgtgtacgtgggcaattacaggattgtaaacagacacctggcaacgagccacgattggcaaaattgcgtgtgggaggactacaacagggatctcctggtcagcacaacaactgctcatggttgtgatactatagcacggtgccaatgtactgctggcgtgtacttttgtgcatctagaaacaagcactacccagtgagcttcgagggtccaggtctagtgaaagttcaggagggcgagtactaccccgagagataccagtcgcacgtactccttgcagttggattttcagaaccgggtgattgtggaggtattttgaggtgtgaacatggagtcattgggctcgttaccatgggtggtgagggtgtagtaggcttcgctgacgtgcgggatcttttgtggttggaagacgacgccatggagcagggtgttagagattatgtagagcaactgggaaatgcatttggctcaggtttcactaaccaaatctgtgagcaagttaacctccttaaagaatctctgatagggcaggattccatattggaaaaatccctgaaggccctggttaaaatcatatcagccctggtgatagtggttaggaaccacgacgacctgattacagtgactgccacactagctttaatcggttgcgcatcatctccatggcgatggctcaaacaaaaagtgtgtcaatactacggaatccccatggcagaaaggcagaataacggttggttaaagaaattcactgaaatgaccaacgcctgcaagggcatggagtggattgctgttaaaattcaaaagttcatcgagtggctcaaagtaaagattctgcctgaagtgaaggagaaacatgagttccttaccagattgaagcaattgccactccttgaaagtcaaattgccaccattgagcaaagcgcaccctcacaaagtgatcaagagcagcttttttcgaatgttcagtacttcgcccattactgcaggaagtatgcacctctgtatgctgccgaagcaaaaagagtgttctcattagaaaagaaaatgagtaattacatacagttcaagtccaaatgccgcattgagcctgtatgcttactccttcacggtagtccaggggctggcaagtcagtagctaccaacctgatagggagatcccttgcagagaagctcaatagctctgtgtactctttaccaccagatccagatcattttgatgggtacaaacagcaggcagtggtgatcatggatgatctctgtcaaaaccccgatgggaaggacgtgtccttgttttgccaaatggtgtctagtgtagattttgtgccacccatggcggcgctggaagaaaaaggcattctctttacgtccccgtttgtgttggcatcaaccaacgcggggtccatcaatgcaccaacagtgtcagacagcagagcacttgccagaaggtttcactttgacatgaatattgaggtgatttcgatgtacagccagaatggtaaaattaacatgcccatgtctgttaagacatgtgatgatgaatgctgcccggtcaatttcaaaaagtgttgcccactagtgtgtggcaaggccatccagtttattgacaggagaaaccaagttagatattcactggacatgctggttactgagatgtttagagagtacaaccacagacacagtgtgggtgctaccctcgaggctttgttccaaggaccaccagtatacagggaaatcaaaatcagtgtggccccggaaacaccccctccaccagcaattgctgaccttctaaaatctgtagacagtgaggcaataagggagtactgcaaggaaaggggttggcttgtgccagaggtcagctccactctacaaattgaaaaacatgttagcagggcatttatttgcttgcaagcgctaactacatttgtttcagtggctggtataatctacatcatttacaagttgtttgccggctttcagggtgcatacactggaatgcccaaccagaaacccaaggtgcccaccttaagacaagctaaggtgcaaggtccggcatttgaatttgccgtagcaatgatgaaaaggaacgccagcacagtcaagacagaatacggtgagttcacgatgcttggcatctatgataaatgggcagtgctgccgcgccacgccaagcctggaccaactattttaatgaatgatcaggaggttggtgtgctcgatgccaaagagttagttgataaagacggaaccaacctggagctgacactattgaagcttaaccgcaatgaaaagttcagagacatcagaggttttcttgcaagggaagaagttgaggtaagtgaggctgttttggcaataaacacgagcaagttcccaagcatgtacatccctgtgggccaagtcaccgattacggatttttaaatctaggtggcaccccaacaaagagaatgctcatgtacaacttccctaccagagcgggacagtgtggtggtgtccttatgtcaacaggaaaggtccttggcatacacgtgggaggaaatggtcaccaaggcttctctgctgctctcctcagacactacttcaacgaggaacagggcgaaatagagtttattgagagctctaaagatgcaggatttcctgtgatcaacacccctaataaaaccaaactggaaccaagtgtgtttcatcaggtttttgagggcaacaaagaaccagcagtcctaagaaacggagacccgcgacttaaagccaactttgaggaagcgatattttccaagtacatcggaaatgtgaacacacatgtggacgagtacatgatagaagctgttgatcactacgctggacagctggcaactctggacatcagtacagaacctatgaagcttgaggatgctgtttatggcactgaaggcttggaagcattggacttgaccactagcgcaggatatccttatgtcgccttgggcatcaagaaaagggatatcctctccaagaagactaaagatctcaccaagctgagggaatgcatggacaagtatggtctaaatctgccgatggtgacctacgtgaaggatgaactcaggtccgctgagaaagtagccaagggaaaatccagacttatagaagcttctagtctcaatgactcagtggccatgaggcagacatttgggaacctatacaagacattccacctcaacccaggcattgtcactggtagtgctgttgggtgcgacccagatgtgttttggagcaaaatacccgtgatgcttgacgggcaccttatagcttttgattactctggctacgacgctagcttgagcccagtgtggtttgcttgtttgaaactcctcctagggaaactagggtatactcataaggaaaccaattacatagactacctctgcaactcccatcacttatacagagataaacactatttcgtgaggggtggtatgccatcaggatgttcaggcaccagtatattcaacaccatgatcaacaacatcattattaggacccttatgctaaaggtctacaaaggtattgacctggatcagtttagaatgatcgcttacggggacgatgtgatagcctcttacccgtggcctattgatgcctcactactagcagaagcgggaaaggattatggtttgatcatgaccccagcagataaaggagagtgttttaatgaggtaacctggacaaatgtaaccttcttgaaaaggtactttagagctgatgaacaatatccattcttggtgcaccccgtgatgcccatgaaagacatacacgaatccattagatggaccaaagacccaaagaacactcaagatcatgtgcgctcgttatgcctattggcttggcacaatggggagcacgaatatgaggaatttatccgaaagatcagaagcgtgcctgttggacgctgtttgaccctcccggtgttctcaacactacgcaggaaatggttagattccttctaaaattagagtgcaatcaatgaactatgattggcttaaccctaccgcatgaaccgaactagacaaaagtgcggtaggggtaaattctccgcattcggtgcggaaaaaaaaaaaaaaaaaaaaaaaaaaaaaaaaaaaaaaaaaaaaaaaaaa

SEQ ID NO: 194 - RNA, 8377 nt, synthetic construct
  source 1..8377: mol_type = other RNA
  misc_feature 1..8377: note = Luci_P2A_H3N2 saRNA construct
ttaaaacagcctgtgggttgtacccacccacagggcccactgggcgctagcactctggtatcacggtacctttgtgtgcctgttttatatcccctttccccgattgtaacttagaagatgtacacactgatcaatagcgggcatagcacaccagctatgtcttgatcaagcactcctgtatccccggaccaagtatcaatagactgctcacgcggttgaaggagaaaacgttcgtcacccggctaactacttcgagaaacccagtagtatcatgaaagttgcgaggcgtttcgttcagcacacccccagtgtagatcgggtcgatgagtcaccgcatcccccacgggcgaccgtggcggtggctgcgctggcggcctgcctacggggcaacccgtaggacgcttcaatacagacatggtgcgaagagtcgattgagctagttagtagtcctccggcccctgaatgcggctaatcctaactgcggagcacatgccctcaacccagggggtattgtgtcgtaacgggcaactctgcagcggaaccgactactttgggtgtccgtgtttccttttatccttatactggctgcttatggtgacaattgaaagattgttgccatatagctattggattggccatccagtgtctaatagagctgttatttacctctttgttggatttataccactcaacctaaaagaagttaaaacactacagctcattttacaactgaatacagcaaaccaccatggaagacgccaaaaacataaagaaaggcccggcgccattctatccgctggaagatggaaccgctggagagcaactgcataaggctatgaagagatacgccctggttcctggaacaattgcttttacagatgcacatatcgaggtggacatcacttacgctgagtacttcgaaatgtccgttcggttggcagaagctatgaaacgatatgggctgaatacaaatcacagaatcgtcgtatgcagtgaaaactctcttcaattctttatgccggtgttgggcgcgttatttatcggagttgcagttgcgcccgcgaacgacatttataatgaacgtgaattgctcaacagtatgggcatttcgcagcctaccgtggtgttcgtttccaaaaaggggttgcaaaaaattttgaacgtgcaaaaaaagctcccaatcatccaaaaaattattatcatggattctaaaacggattaccagggatttcagtcgatgtacacgttcgtcacatctcatctacctcccggttttaatgaatacgattttgtgccagagtccttcgatagggacaagacaattgcactgatcatgaactcctctggatctactggtctgcctaaaggtgtcgctctgcctcatagaactgcctgcgtgagattctcgcatgccagagatcctatttttggcaatcaaatcattccggatactgcgattttaagtgttgttccattccatcacggttttggaatgtttactacactcggatatttgatatgtggatttcgagtcgtcttaatgtatagatttgaagaagagctgtttctgaggagccttcaggattacaagattcaaagtgcgctgctggtgccaaccctattctccttcttcgccaaaagcactctgattgacaaatacgatttatctaatttacacgaaattgcttctggtggcgctcccctctctaaggaagtcggggaagcggttgccaagaggttccatctgccaggtatcaggcaaggatatgggctcactgagactacatcagctattctgattacacccgagggggatgataaaccgggcgcggtcggtaaagttgttccattttttgaagcgaaggttgtggatctggataccgggaaaacgctgggcgttaatcaaagaggcgaactgtgtgtgagaggtcctatgattatgtccggttatgtaaacaatccggaagcgaccaacgccttgattgacaaggatggatggctacattctggagacatagcttactgggacgaagacgaacacttcttcatcgttgaccgcctgaagtctctgattaagtacaaaggctatcaggtggctcccgctgaattggaatccatcttgctccaacaccccaacatcttcgacgcaggtgtcgcaggtcttcccgacgatgacgccggtgaacttcccgccgccgttgttgttttggagcacggaaagacgatgacggaaaaagagatcgtggattacgtcgccagtcaagtaacaaccgcgaaaaagttgcgcggaggagttgtgtttgtggacgaagtaccgaaaggtcttaccggaaaactcgacgcaagaaaaatcagagagatcctcataaaggccaagaagggcggaaagatcgccgtgtaaggaagcggagctactaacttcagcctgctgaagcaggctggacaggtggaggagaaccctggacctatgaaaaccgtgatcgccctcagttacatcttctgcctcgcctttggacagaatctcctcggaaacgaaaacaacgctgccacactctgcctgggacaccacgccgtgcccaacggcacaatggtgaagaccatcaccgacgatcagatcgaggtgaccaatgccaccgagctggtgcagaacagctccaccggcaaaatctgcaacaatccccacaagatcctggacggcagggattgcaccctgatcgacgctctgctgggcgaccctcactgcgacgtgttccagaatgagacatgggatctgttcgtggagaggagcaatgccttctccaactgctacccctacgacgtgcctgattacgccagcctgcggtccatcgtggccagctccggcaccctggagttcatcaccgagggcttcacctgggctggagtgacccagaacggaggcagcggagcttgcaagaggggacccgccaatagcttcttctcccggctgaactggctgaccaagtccggcaatacctaccccgtgctgaacgtgaccatgcctaacaataacaatttcgacaagctgtacatctggggcgtgcaccaccctagcaccgatcaggagcagaccagcctgtacatccaggcctccggcagggtgaccgtgagcaccaggcggtcccagcagaccatcatccccaacatcggctccaggcctctggtgcggggacagagcggccggatctccgtgtactggaccatcgtgaagcccggcgacatcctggtcatcaacagcaatggcaacctgatcgcccctcgcggctacttcaagatgcacatcggcaagagcagcatcatgagatccgacgcccccatcgatacctgcatcagcgagtgcatcacccctaatggctccatccccaacgagaagcctttccagaatgtgaacaagatcacctacggcgcctgccccaagtacgtgaagcagaataccctgaagctggccaccggcatgcgcaacgtgcctgagagacagaccgtgggcctgttcggagctatcgctggcttcatcgagaatggctgggagggcatggtggacggctggtacggcttccgccaccagaacagcgagggcaccggacaggctgccgacctgaagtccacccaggccgccatcgatcagatcaatggcaagctgaacagagtgatcgagaagaccaacgagaagttccaccagatcgagaaggagttcagcgaggtggagggacgcatccaggacctggagaggtacgtggaggacaccaagatcgatctgtggagctacaatgccgagctgctggtggccctggagaatcagaacaccatcgacctgaccgattccgagatgaacaagctgttcgagaagacccgcagacagctgcgcgagaatgccgaggacatgggcaacggctgcttcaaaatctaccacaagtgcgataacgcctgcatcgagagcatcagaaatggcacctacgaccacaacatctaccgcgatgaggccgtgaacaatagattccagatcaagggcgtggagctgaagtccggctacaaggactggattctgtggatcagcttcgccatctcctgcttcctgctgtgcgtggtgctgctggggtttattatgtgggcttgtcagagggggaacatcaggtgtaacatttgtaactttgagccaacaggggtgacggagtcccgcactgaaattacggcaatgcagaccaccggttcatgtgggcaacaatcaggagctgtgtacgtgggcaattacaggattgtaaacagacacctggcaacgagccacgattggcaaaattgcgtgtgggaggactacaacagggatctcctggtcagcacaacaactgctcatggttgtgatactatagcacggtgccaatgtactgctggcgtgtacttttgtgcatctagaaacaagcactacccagtgagcttcgagggtccaggtctagtgaaagttcaggagggcgagtactaccccgagagataccagtcgcacgtactccttgcagttggattttcagaaccgggtgattgtggaggtattttgaggtgtgaacatggagtcattgggctcgttaccatgggtggtgagggtgtagtaggcttcgctgacgtgcgggatcttttgtggttggaagacgacgccatggagcagggtgttagagattatgtagagcaactgggaaatgcatttggctcaggtttcactaaccaaatctgtgagcaagttaacctccttaaagaatctctgatagggcaggattccatattggaaaaatccctgaaggccctggttaaaatcatatcagccctggtgatagtggttaggaaccacgacgacctgattacagtgactgccacactagctttaatcggttgcgcatcatctccatggcgatggctcaaacaaaaagtgtgtcaatactacggaatccccatggcagaaaggcagaataacggttggttaaagaaattcactgaaatgaccaacgcctgcaagggcatggagtggattgctgttaaaattcaaaagttcatcgagtggctcaaagtaaagattctgcctgaagtgaaggagaaacatgagttccttaccagattgaagcaattgccactccttgaaagtcaaattgccaccattgagcaaagcgcaccctcacaaagtgatcaagagcagcttttttcgaatgttcagtacttcgcccattactgcaggaagtatgcacctctgtatgctgccgaagcaaaaagagtgttctcattagaaaagaaaatgagtaattacatacagttcaagtccaaatgccgcattgagcctgtatgcttactccttcacggtagtccaggggctggcaagtcagtagctaccaacctgatagggagatcccttgcagagaagctcaatagctctgtgtactctttaccaccagatccagatcattttgatgggtacaaacagcaggcagtggtgatcatggatgatctctgtcaaaaccccgatgggaaggacgtgtccttgttttgccaaatggtgtctagtgtagattttgtgccacccatggcggcgctggaagaaaaaggcattctctttacgtccccgtttgtgttggcatcaaccaacgcggggtccatcaatgcaccaacagtgtcagacagcagagcacttgccagaaggtttcactttgacatgaatattgaggtgatttcgatgtacagccagaatggtaaaattaacatgcccatgtctgttaagacatgtgatgatgaatgctgcccggtcaatttcaaaaagtgttgcccactagtgtgtggcaaggccatccagtttattgacaggagaaaccaagttagatattcactggacatgctggttactgagatgtttagagagtacaaccacagacacagtgtgggtgctaccctcgaggctttgttccaaggaccaccagtatacagggaaatcaaaatcagtgtggccccggaaacaccccctccaccagcaattgctgaccttctaaaatctgtagacagtgaggcaataagggagtactgcaaggaaaggggttggcttgtgccagaggtcagctccactctacaaattgaaaaacatgttagcagggcatttatttgcttgcaagcgctaactacatttgtttcagtggctggtataatctacatcatttacaagttgtttgccggctttcagggtgcatacactggaatgcccaaccagaaacccaaggtgcccaccttaagacaagctaaggtgcaaggtccggcatttgaatttgccgtagcaatgatgaaaaggaacgccagcacagtcaagacagaatacggtgagttcacgatgcttggcatctatgataaatgggcagtgctgccgcgccacgccaagcctggaccaactattttaatgaatgatcaggaggttggtgtgctcgatgccaaagagttagttgataaagacggaaccaacctggagctgacactattgaagcttaaccgcaatgaaaagttcagagacatcagaggttttcttgcaagggaagaagttgaggtaagtgaggctgttttggcaataaacacgagcaagttcccaagcatgtacatccctgtgggccaagtcaccgattacggatttttaaatctaggtggcaccccaacaaagagaatgctcatgtacaacttccctaccagagcgggacagtgtggtggtgtccttatgtcaacaggaaaggtccttggcatacacgtgggaggaaatggtcaccaaggcttctctgctgctctcctcagacactacttcaacgaggaacagggcgaaatagagtttattgagagctctaaagatgcaggatttcctgtgatcaacacccctaataaaaccaaactggaaccaagtgtgtttcatcaggtttttgagggcaacaaagaaccagcagtcctaagaaacggagacccgcgacttaaagccaactttgaggaagcgatattttccaagtacatcggaaatgtgaacacacatgtggacgagtacatgatagaagctgttgatcactacgctggacagctggcaactctggacatcagtacagaacctatgaagcttgaggatgctgtttatggcactgaaggcttggaagcattggacttgaccactagcgcaggatatccttatgtcgccttgggcatcaagaaaagggatatcctctccaagaagactaaagatctcaccaagctgagggaatgcatggacaagtatggtctaaatctgccgatggtgacctacgtgaaggatgaactcaggtccgctgagaaagtagccaagggaaaatccagacttatagaagcttctagtctcaatgactcagtggccatgaggcagacatttgggaacctatacaagacattccacctcaacccaggcattgtcactggtagtgctgttgggtgcgacccagatgtgttttggagcaaaatacccgtgatgcttgacgggcaccttatagcttttgattactctggctacgacgctagcttgagcccagtgtggtttgcttgtttgaaactcctcctagggaaactagggtatactcataaggaaaccaattacatagactacctctgcaactcccatcacttatacagagataaacactatttcgtgaggggtggtatgccatcaggatgttcaggcaccagtatattcaacaccatgatcaacaacatcattattaggacccttatgctaaaggtctacaaaggtattgacctggatcagtttagaatgatcgcttacggggacgatgtgatagcctcttacccgtggcctattgatgcctcactactagcagaagcgggaaaggattatggtttgatcatgaccccagcagataaaggagagtgttttaatgaggtaacctggacaaatgtaaccttcttgaaaaggtactttagagctgatgaacaatatccattcttggtgcaccccgtgatgcccatgaaagacatacacgaatccattagatggaccaaagacccaaagaacactcaagatcatgtgcgctcgttatgcctattggcttggcacaatggggagcacgaatatgaggaatttatccgaaagatcagaagcgtgcctgttggacgctgtttgaccctcccggtgttctcaacactacgcaggaaatggttagattccttctaaaattagagtgcaatcaatgaactatgattggcttaaccctaccgcatgaaccgaactagacaaaagtgcggtaggggtaaattctccgcattcggtgcggaaaaaaaaaaaaaaaaaaaaaaaaaaaaaaaaaaaaaaaaaaaaaaaaaa

SEQ ID NO: 195 - DNA, 8377 bp, synthetic construct
  source 1..8377: mol_type = other DNA
  misc_feature 1..8377: note = Luci_P2A_H3N2 DNA vector construct
ttaaaacagcctgtgggttgtacccacccacagggcccactgggcgctagcactctggtatcacggtacctttgtgtgcctgttttatatcccctttccccgattgtaacttagaagatgtacacactgatcaatagcgggcatagcacaccagctatgtcttgatcaagcactcctgtatccccggaccaagtatcaatagactgctcacgcggttgaaggagaaaacgttcgtcacccggctaactacttcgagaaacccagtagtatcatgaaagttgcgaggcgtttcgttcagcacacccccagtgtagatcgggtcgatgagtcaccgcatcccccacgggcgaccgtggcggtggctgcgctggcggcctgcctacggggcaacccgtaggacgcttcaatacagacatggtgcgaagagtcgattgagctagttagtagtcctccggcccctgaatgcggctaatcctaactgcggagcacatgccctcaacccagggggtattgtgtcgtaacgggcaactctgcagcggaaccgactactttgggtgtccgtgtttccttttatccttatactggctgcttatggtgacaattgaaagattgttgccatatagctattggattggccatccagtgtctaatagagctgttatttacctctttgttggatttataccactcaacctaaaagaagttaaaacactacagctcattttacaactgaatacagcaaaccaccatggaagacgccaaaaacataaagaaaggcccggcgccattctatccgctggaagatggaaccgctggagagcaactgcataaggctatgaagagatacgccctggttcctggaacaattgcttttacagatgcacatatcgaggtggacatcacttacgctgagtacttcgaaatgtccgttcggttggcagaagctatgaaacgatatgggctgaatacaaatcacagaatcgtcgtatgcagtgaaaactctcttcaattctttatgccggtgttgggcgcgttatttatcggagttgcagttgcgcccgcgaacgacatttataatgaacgtgaattgctcaacagtatgggcatttcgcagcctaccgtggtgttcgtttccaaaaaggggttgcaaaaaattttgaacgtgcaaaaaaagctcccaatcatccaaaaaattattatcatggattctaaaacggattaccagggatttcagtcgatgtacacgttcgtcacatctcatctacctcccggttttaatgaatacgattttgtgccagagtccttcgatagggacaagacaattgcactgatcatgaactcctctggatctactggtctgcctaaaggtgtcgctctgcctcatagaactgcctgcgtgagattctcgcatgccagagatcctatttttggcaatcaaatcattccggatactgcgattttaagtgttgttccattccatcacggttttggaatgtttactacactcggatatttgatatgtggatttcgagtcgtcttaatgtatagatttgaagaagagctgtttctgaggagccttcaggattacaagattcaaagtgcgctgctggtgccaaccctattctccttcttcgccaaaagcactctgattgacaaatacgatttatctaatttacacgaaattgcttctggtggcgctcccctctctaaggaagtcggggaagcggttgccaagaggttccatctgccaggtatcaggcaaggatatgggctcactgagactacatcagctattctgattacacccgagggggatgataaaccgggcgcggtcggtaaagttgttccattttttgaagcgaaggttgtggatctggataccgggaaaacgctgggcgttaatcaaagaggcgaactgtgtgtgagaggtcctatgattatgtccggttatgtaaacaatccggaagcgaccaacgccttgattgacaaggatggatggctacattctggagacatagcttactgggacgaagacgaacacttcttcatcgttgaccgcctgaagtctctgattaagtacaaaggctatcaggtggctcccgctgaattggaatccatcttgctccaacaccccaacatcttcgacgcaggtgtcgcaggtcttcccgacgatgacgccggtgaacttcccgccgccgttgttgttttggagcacggaaagacgatgacggaaaaagagatcgtggattacgtcgccagtcaagtaacaaccgcgaaaaagttgcgcggaggagttgtgtttgtggacgaagtaccgaaaggtcttaccggaaaactcgacgcaagaaaaatcagagagatcctcataaaggccaagaagggcggaaagatcgccgtgtaaggaagcggagctactaacttcagcctgctgaagcaggctggacaggtggaggagaaccctggacctatgaaaaccgtgatcgccctcagttacatcttctgcctcgcctttggacagaatctcctcggaaacgaaaacaacgctgccacactctgcctgggacaccacgccgtgcccaacggcacaatggtgaagaccatcaccgacgatcagatcgaggtgaccaatgccaccgagctggtgcagaacagctccaccggcaaaatctgcaacaatccccacaagatcctggacggcagggattgcaccctgatcgacgctctgctgggcgaccctcactgcgacgtgttccagaatgagacatgggatctgttcgtggagaggagcaatgccttctccaactgctacccctacgacgtgcctgattacgccagcctgcggtccatcgtggccagctccggcaccctggagttcatcaccgagggcttcacctgggctggagtgacccagaacggaggcagcggagcttgcaagaggggacccgccaatagcttcttctcccggctgaactggctgaccaagtccggcaatacctaccccgtgctgaacgtgaccatgcctaacaataacaatttcgacaagctgtacatctggggcgtgcaccaccctagcaccgatcaggagcagaccagcctgtacatccaggcctccggcagggtgaccgtgagcaccaggcggtcccagcagaccatcatccccaacatcggctccaggcctctggtgcggggacagagcggccggatctccgtgtactggaccatcgtgaagcccggcgacatcctggtcatcaacagcaatggcaacctgatcgcccctcgcggctacttcaagatgcacatcggcaagagcagcatcatgagatccgacgcccccatcgatacctgcatcagcgagtgcatcacccctaatggctccatccccaacgagaagcctttccagaatgtgaacaagatcacctacggcgcctgccccaagtacgtgaagcagaataccctgaagctggccaccggcatgcgcaacgtgcctgagagacagaccgtgggcctgttcggagctatcgctggcttcatcgagaatggctgggagggcatggtggacggctggtacggcttccgccaccagaacagcgagggcaccggacaggctgccgacctgaagtccacccaggccgccatcgatcagatcaatggcaagctgaacagagtgatcgagaagaccaacgagaagttccaccagatcgagaaggagttcagcgaggtggagggacgcatccaggacctggagaggtacgtggaggacaccaagatcgatctgtggagctacaatgccgagctgctggtggccctggagaatcagaacaccatcgacctgaccgattccgagatgaacaagctgttcgagaagacccgcagacagctgcgcgagaatgccgaggacatgggcaacggctgcttcaaaatctaccacaagtgcgataacgcctgcatcgagagcatcagaaatggcacctacgaccacaacatctaccgcgatgaggccgtgaacaatagattccagatcaagggcgtggagctgaagtccggctacaaggactggattctgtggatcagcttcgccatctcctgcttcctgctgtgcgtggtgctgctggggtttattatgtgggcttgtcagagggggaacatcaggtgtaacatttgtaactttgagccaacaggggtgacggagtcccgcactgaaattacggcaatgcagaccaccggttcatgtgggcaacaatcaggagctgtgtacgtgggcaattacaggattgtaaacagacacctggcaacgagccacgattggcaaaattgcgtgtgggaggactacaacagggatctcctggtcagcacaacaactgctcatggttgtgatactatagcacggtgccaatgtactgctggcgtgtacttttgtgcatctagaaacaagcactacccagtgagcttcgagggtccaggtctagtgaaagttcaggagggcgagtactaccccgagagataccagtcgcacgtactccttgcagttggattttcagaaccgggtgattgtggaggtattttgaggtgtgaacatggagtcattgggctcgttaccatgggtggtgagggtgtagtaggcttcgctgacgtgcgggatcttttgtggttggaagacgacgccatggagcagggtgttagagattatgtagagcaactgggaaatgcatttggctcaggtttcactaaccaaatctgtgagcaagttaacctccttaaagaatctctgatagggcaggattccatattggaaaaatccctgaaggccctggttaaaatcatatcagccctggtgatagtggttaggaaccacgacgacctgattacagtgactgccacactagctttaatcggttgcgcatcatctccatggcgatggctcaaacaaaaagtgtgtcaatactacggaatccccatggcagaaaggcagaataacggttggttaaagaaattcactgaaatgaccaacgcctgcaagggcatggagtggattgctgttaaaattcaaaagttcatcgagtggctcaaagtaaagattctgcctgaagtgaaggagaaacatgagttccttaccagattgaagcaattgccactccttgaaagtcaaattgccaccattgagcaaagcgcaccctcacaaagtgatcaagagcagcttttttcgaatgttcagtacttcgcccattactgcaggaagtatgcacctctgtatgctgccgaagcaaaaagagtgttctcattagaaaagaaaatgagtaattacatacagttcaagtccaaatgccgcattgagcctgtatgcttactccttcacggtagtccaggggctggcaagtcagtagctaccaacctgatagggagatcccttgcagagaagctcaatagctctgtgtactctttaccaccagatccagatcattttgatgggtacaaacagcaggcagtggtgatcatggatgatctctgtcaaaaccccgatgggaaggacgtgtccttgttttgccaaatggtgtctagtgtagattttgtgccacccatggcggcgctggaagaaaaaggcattctctttacgtccccgtttgtgttggcatcaaccaacgcggggtccatcaatgcaccaacagtgtcagacagcagagcacttgccagaaggtttcactttgacatgaatattgaggtgatttcgatgtacagccagaatggtaaaattaacatgcccatgtctgttaagacatgtgatgatgaatgctgcccggtcaatttcaaaaagtgttgcccactagtgtgtggcaaggccatccagtttattgacaggagaaaccaagttagatattcactggacatgctggttactgagatgtttagagagtacaaccacagacacagtgtgggtgctaccctcgaggctttgttccaaggaccaccagtatacagggaaatcaaaatcagtgtggccccggaaacaccccctccaccagcaattgctgaccttctaaaatctgtagacagtgaggcaataagggagtactgcaaggaaaggggttggcttgtgccagaggtcagctccactctacaaattgaaaaacatgttagcagggcatttatttgcttgcaagcgctaactacatttgtttcagtggctggtataatctacatcatttacaagttgtttgccggctttcagggtgcatacactggaatgcccaaccagaaacccaaggtgcccaccttaagacaagctaaggtgcaaggtccggcatttgaatttgccgtagcaatgatgaaaaggaacgccagcacagtcaagacagaatacggtgagttcacgatgcttggcatctatgataaatgggcagtgctgccgcgccacgccaagcctggaccaactattttaatgaatgatcaggaggttggtgtgctcgatgccaaagagttagttgataaagacggaaccaacctggagctgacactattgaagcttaaccgcaatgaaaagttcagagacatcagaggttttcttgcaagggaagaagttgaggtaagtgaggctgttttggcaataaacacgagcaagttcccaagcatgtacatccctgtgggccaagtcaccgattacggatttttaaatctaggtggcaccccaacaaagagaatgctcatgtacaacttccctaccagagcgggacagtgtggtggtgtccttatgtcaacaggaaaggtccttggcatacacgtgggaggaaatggtcaccaaggcttctctgctgctctcctcagacactacttcaacgaggaacagggcgaaatagagtttattgagagctctaaagatgcaggatttcctgtgatcaacacccctaataaaaccaaactggaaccaagtgtgtttcatcaggtttttgagggcaacaaagaaccagcagtcctaagaaacggagacccgcgacttaaagccaactttgaggaagcgatattttccaagtacatcggaaatgtgaacacacatgtggacgagtacatgatagaagctgttgatcactacgctggacagctggcaactctggacatcagtacagaacctatgaagcttgaggatgctgtttatggcactgaaggcttggaagcattggacttgaccactagcgcaggatatccttatgtcgccttgggcatcaagaaaagggatatcctctccaagaagactaaagatctcaccaagctgagggaatgcatggacaagtatggtctaaatctgccgatggtgacctacgtgaaggatgaactcaggtccgctgagaaagtagccaagggaaaatccagacttatagaagcttctagtctcaatgactcagtggccatgaggcagacatttgggaacctatacaagacattccacctcaacccaggcattgtcactggtagtgctgttgggtgcgacccagatgtgttttggagcaaaatacccgtgatgcttgacgggcaccttatagcttttgattactctggctacgacgctagcttgagcccagtgtggtttgcttgtttgaaactcctcctagggaaactagggtatactcataaggaaaccaattacatagactacctctgcaactcccatcacttatacagagataaacactatttcgtgaggggtggtatgccatcaggatgttcaggcaccagtatattcaacaccatgatcaacaacatcattattaggacccttatgctaaaggtctacaaaggtattgacctggatcagtttagaatgatcgcttacggggacgatgtgatagcctcttacccgtggcctattgatgcctcactactagcagaagcgggaaaggattatggtttgatcatgaccccagcagataaaggagagtgttttaatgaggtaacctggacaaatgtaaccttcttgaaaaggtactttagagctgatgaacaatatccattcttggtgcaccccgtgatgcccatgaaagacatacacgaatccattagatggaccaaagacccaaagaacactcaagatcatgtgcgctcgttatgcctattggcttggcacaatggggagcacgaatatgaggaatttatccgaaagatcagaagcgtgcctgttggacgctgtttgaccctcccggtgttctcaacactacgcaggaaatggttagattccttctaaaattagagtgcaatcaatgaactatgattggcttaaccctaccgcatgaaccgaactagacaaaagtgcggtaggggtaaattctccgcattcggtgcggaaaaaaaaaaaaaaaaaaaaaaaaaaaaaaaaaaaaaaaaaaaaaaaaaa

SEQ ID NO: 196 - RNA, 8347 nt, synthetic construct
  source 1..8347: mol_type = other RNA
  misc_feature 1..8347: note = Luci_3C protease recognition region_H3N2 saRNA construct
ttaaaacagcctgtgggttgtacccacccacagggcccactgggcgctagcactctggtatcacggtacctttgtgtgcctgttttatatcccctttccccgattgtaacttagaagatgtacacactgatcaatagcgggcatagcacaccagctatgtcttgatcaagcactcctgtatccccggaccaagtatcaatagactgctcacgcggttgaaggagaaaacgttcgtcacccggctaactacttcgagaaacccagtagtatcatgaaagttgcgaggcgtttcgttcagcacacccccagtgtagatcgggtcgatgagtcaccgcatcccccacgggcgaccgtggcggtggctgcgctggcggcctgcctacggggcaacccgtaggacgcttcaatacagacatggtgcgaagagtcgattgagctagttagtagtcctccggcccctgaatgcggctaatcctaactgcggagcacatgccctcaacccagggggtattgtgtcgtaacgggcaactctgcagcggaaccgactactttgggtgtccgtgtttccttttatccttatactggctgcttatggtgacaattgaaagattgttgccatatagctattggattggccatccagtgtctaatagagctgttatttacctctttgttggatttataccactcaacctaaaagaagttaaaacactacagctcattttacaactgaatacagcaaaccaccatggaagacgccaaaaacataaagaaaggcccggcgccattctatccgctggaagatggaaccgctggagagcaactgcataaggctatgaagagatacgccctggttcctggaacaattgcttttacagatgcacatatcgaggtggacatcacttacgctgagtacttcgaaatgtccgttcggttggcagaagctatgaaacgatatgggctgaatacaaatcacagaatcgtcgtatgcagtgaaaactctcttcaattctttatgccggtgttgggcgcgttatttatcggagttgcagttgcgcccgcgaacgacatttataatgaacgtgaattgctcaacagtatgggcatttcgcagcctaccgtggtgttcgtttccaaaaaggggttgcaaaaaattttgaacgtgcaaaaaaagctcccaatcatccaaaaaattattatcatggattctaaaacggattaccagggatttcagtcgatgtacacgttcgtcacatctcatctacctcccggttttaatgaatacgattttgtgccagagtccttcgatagggacaagacaattgcactgatcatgaactcctctggatctactggtctgcctaaaggtgtcgctctgcctcatagaactgcctgcgtgagattctcgcatgccagagatcctatttttggcaatcaaatcattccggatactgcgattttaagtgttgttccattccatcacggttttggaatgtttactacactcggatatttgatatgtggatttcgagtcgtcttaatgtatagatttgaagaagagctgtttctgaggagccttcaggattacaagattcaaagtgcgctgctggtgccaaccctattctccttcttcgccaaaagcactctgattgacaaatacgatttatctaatttacacgaaattgcttctggtggcgctcccctctctaaggaagtcggggaagcggttgccaagaggttccatctgccaggtatcaggcaaggatatgggctcactgagactacatcagctattctgattacacccgagggggatgataaaccgggcgcggtcggtaaagttgttccattttttgaagcgaaggttgtggatctggataccgggaaaacgctgggcgttaatcaaagaggcgaactgtgtgtgagaggtcctatgattatgtccggttatgtaaacaatccggaagcgaccaacgccttgattgacaaggatggatggctacattctggagacatagcttactgggacgaagacgaacacttcttcatcgttgaccgcctgaagtctctgattaagtacaaaggctatcaggtggctcccgctgaattggaatccatcttgctccaacaccccaacatcttcgacgcaggtgtcgcaggtcttcccgacgatgacgccggtgaacttcccgccgccgttgttgttttggagcacggaaagacgatgacggaaaaagagatcgtggattacgtcgccagtcaagtaacaaccgcgaaaaagttgcgcggaggagttgtgtttgtggacgaagtaccgaaaggtcttaccggaaaactcgacgcaagaaaaatcagagagatcctcataaaggccaagaagggcggaaagatcgccgtgtaacaggacaactttttccaaggaccacccggggaagctatgaaaaccgtgatcgccctcagttacatcttctgcctcgcctttggacagaatctcctcggaaacgaaaacaacgctgccacactctgcctgggacaccacgccgtgcccaacggcacaatggtgaagaccatcaccgacgatcagatcgaggtgaccaatgccaccgagctggtgcagaacagctccaccggcaaaatctgcaacaatccccacaagatcctggacggcagggattgcaccctgatcgacgctctgctgggcgaccctcactgcgacgtgttccagaatgagacatgggatctgttcgtggagaggagcaatgccttctccaactgctacccctacgacgtgcctgattacgccagcctgcggtccatcgtggccagctccggcaccctggagttcatcaccgagggcttcacctgggctggagtgacccagaacggaggcagcggagcttgcaagaggggacccgccaatagcttcttctcccggctgaactggctgaccaagtccggcaatacctaccccgtgctgaacgtgaccatgcctaacaataacaatttcgacaagctgtacatctggggcgtgcaccaccctagcaccgatcaggagcagaccagcctgtacatccaggcctccggcagggtgaccgtgagcaccaggcggtcccagcagaccatcatccccaacatcggctccaggcctctggtgcggggacagagcggccggatctccgtgtactggaccatcgtgaagcccggcgacatcctggtcatcaacagcaatggcaacctgatcgcccctcgcggctacttcaagatgcacatcggcaagagcagcatcatgagatccgacgcccccatcgatacctgcatcagcgagtgcatcacccctaatggctccatccccaacgagaagcctttccagaatgtgaacaagatcacctacggcgcctgccccaagtacgtgaagcagaataccctgaagctggccaccggcatgcgcaacgtgcctgagagacagaccgtgggcctgttcggagctatcgctggcttcatcgagaatggctgggagggcatggtggacggctggtacggcttccgccaccagaacagcgagggcaccggacaggctgccgacctgaagtccacccaggccgccatcgatcagatcaatggcaagctgaacagagtgatcgagaagaccaacgagaagttccaccagatcgagaaggagttcagcgaggtggagggacgcatccaggacctggagaggtacgtggaggacaccaagatcgatctgtggagctacaatgccgagctgctggtggccctggagaatcagaacaccatcgacctgaccgattccgagatgaacaagctgttcgagaagacccgcagacagctgcgcgagaatgccgaggacatgggcaacggctgcttcaaaatctaccacaagtgcgataacgcctgcatcgagagcatcagaaatggcacctacgaccacaacatctaccgcgatgaggccgtgaacaatagattccagatcaagggcgtggagctgaagtccggctacaaggactggattctgtggatcagcttcgccatctcctgcttcctgctgtgcgtggtgctgctggggtttattatgtgggcttgtcagagggggaacatcaggtgtaacatttgtaactttgagccaacaggggtgacggagtcccgcactgaaattacggcaatgcagaccaccggttcatgtgggcaacaatcaggagctgtgtacgtgggcaattacaggattgtaaacagacacctggcaacgagccacgattggcaaaattgcgtgtgggaggactacaacagggatctcctggtcagcacaacaactgctcatggttgtgatactatagcacggtgccaatgtactgctggcgtgtacttttgtgcatctagaaacaagcactacccagtgagcttcgagggtccaggtctagtgaaagttcaggagggcgagtactaccccgagagataccagtcgcacgtactccttgcagttggattttcagaaccgggtgattgtggaggtattttgaggtgtgaacatggagtcattgggctcgttaccatgggtggtgagggtgtagtaggcttcgctgacgtgcgggatcttttgtggttggaagacgacgccatggagcagggtgttagagattatgtagagcaactgggaaatgcatttggctcaggtttcactaaccaaatctgtgagcaagttaacctccttaaagaatctctgatagggcaggattccatattggaaaaatccctgaaggccctggttaaaatcatatcagccctggtgatagtggttaggaaccacgacgacctgattacagtgactgccacactagctttaatcggttgcgcatcatctccatggcgatggctcaaacaaaaagtgtgtcaatactacggaatccccatggcagaaaggcagaataacggttggttaaagaaattcactgaaatgaccaacgcctgcaagggcatggagtggattgctgttaaaattcaaaagttcatcgagtggctcaaagtaaagattctgcctgaagtgaaggagaaacatgagttccttaccagattgaagcaattgccactccttgaaagtcaaattgccaccattgagcaaagcgcaccctcacaaagtgatcaagagcagcttttttcgaatgttcagtacttcgcccattactgcaggaagtatgcacctctgtatgctgccgaagcaaaaagagtgttctcattagaaaagaaaatgagtaattacatacagttcaagtccaaatgccgcattgagcctgtatgcttactccttcacggtagtccaggggctggcaagtcagtagctaccaacctgatagggagatcccttgcagagaagctcaatagctctgtgtactctttaccaccagatccagatcattttgatgggtacaaacagcaggcagtggtgatcatggatgatctctgtcaaaaccccgatgggaaggacgtgtccttgttttgccaaatggtgtctagtgtagattttgtgccacccatggcggcgctggaagaaaaaggcattctctttacgtccccgtttgtgttggcatcaaccaacgcggggtccatcaatgcaccaacagtgtcagacagcagagcacttgccagaaggtttcactttgacatgaatattgaggtgatttcgatgtacagccagaatggtaaaattaacatgcccatgtctgttaagacatgtgatgatgaatgctgcccggtcaatttcaaaaagtgttgcccactagtgtgtggcaaggccatccagtttattgacaggagaaaccaagttagatattcactggacatgctggttactgagatgtttagagagtacaaccacagacacagtgtgggtgctaccctcgaggctttgttccaaggaccaccagtatacagggaaatcaaaatcagtgtggccccggaaacaccccctccaccagcaattgctgaccttctaaaatctgtagacagtgaggcaataagggagtactgcaaggaaaggggttggcttgtgccagaggtcagctccactctacaaattgaaaaacatgttagcagggcatttatttgcttgcaagcgctaactacatttgtttcagtggctggtataatctacatcatttacaagttgtttgccggctttcagggtgcatacactggaatgcccaaccagaaacccaaggtgcccaccttaagacaagctaaggtgcaaggtccggcatttgaatttgccgtagcaatgatgaaaaggaacgccagcacagtcaagacagaatacggtgagttcacgatgcttggcatctatgataaatgggcagtgctgccgcgccacgccaagcctggaccaactattttaatgaatgatcaggaggttggtgtgctcgatgccaaagagttagttgataaagacggaaccaacctggagctgacactattgaagcttaaccgcaatgaaaagttcagagacatcagaggttttcttgcaagggaagaagttgaggtaagtgaggctgttttggcaataaacacgagcaagttcccaagcatgtacatccctgtgggccaagtcaccgattacggatttttaaatctaggtggcaccccaacaaagagaatgctcatgtacaacttccctaccagagcgggacagtgtggtggtgtccttatgtcaacaggaaaggtccttggcatacacgtgggaggaaatggtcaccaaggcttctctgctgctctcctcagacactacttcaacgaggaacagggcgaaatagagtttattgagagctctaaagatgcaggatttcctgtgatcaacacccctaataaaaccaaactggaaccaagtgtgtttcatcaggtttttgagggcaacaaagaaccagcagtcctaagaaacggagacccgcgacttaaagccaactttgaggaagcgatattttccaagtacatcggaaatgtgaacacacatgtggacgagtacatgatagaagctgttgatcactacgctggacagctggcaactctggacatcagtacagaacctatgaagcttgaggatgctgtttatggcactgaaggcttggaagcattggacttgaccactagcgcaggatatccttatgtcgccttgggcatcaagaaaagggatatcctctccaagaagactaaagatctcaccaagctgagggaatgcatggacaagtatggtctaaatctgccgatggtgacctacgtgaaggatgaactcaggtccgctgagaaagtagccaagggaaaatccagacttatagaagcttctagtctcaatgactcagtggccatgaggcagacatttgggaacctatacaagacattccacctcaacccaggcattgtcactggtagtgctgttgggtgcgacccagatgtgttttggagcaaaatacccgtgatgcttgacgggcaccttatagcttttgattactctggctacgacgctagcttgagcccagtgtggtttgcttgtttgaaactcctcctagggaaactagggtatactcataaggaaaccaattacatagactacctctgcaactcccatcacttatacagagataaacactatttcgtgaggggtggtatgccatcaggatgttcaggcaccagtatattcaacaccatgatcaacaacatcattattaggacccttatgctaaaggtctacaaaggtattgacctggatcagtttagaatgatcgcttacggggacgatgtgatagcctcttacccgtggcctattgatgcctcactactagcagaagcgggaaaggattatggtttgatcatgaccccagcagataaaggagagtgttttaatgaggtaacctggacaaatgtaaccttcttgaaaaggtactttagagctgatgaacaatatccattcttggtgcaccccgtgatgcccatgaaagacatacacgaatccattagatggaccaaagacccaaagaacactcaagatcatgtgcgctcgttatgcctattggcttggcacaatggggagcacgaatatgaggaatttatccgaaagatcagaagcgtgcctgttggacgctgtttgaccctcccggtgttctcaacactacgcaggaaatggttagattccttctaaaattagagtgcaatcaatgaactatgattggcttaaccctaccgcatgaaccgaactagacaaaagtgcggtaggggtaaattctccgcattcggtgcggaaaaaaaaaaaaaaaaaaaaaaaaaaaaaaaaaaaaaaaaaaaaaaaaaa

SEQ ID NO: 197 - DNA, 8347 bp, synthetic construct
  source 1..8347: mol_type = other DNA
  misc_feature 1..8347: note = Luci_3C protease recognition region_H3N2 DNA vector construct
ttaaaacagcctgtgggttgtacccacccacagggcccactgggcgctagcactctggtatcacggtacctttgtgtgcctgttttatatcccctttccccgattgtaacttagaagatgtacacactgatcaatagcgggcatagcacaccagctatgtcttgatcaagcactcctgtatccccggaccaagtatcaatagactgctcacgcggttgaaggagaaaacgttcgtcacccggctaactacttcgagaaacccagtagtatcatgaaagttgcgaggcgtttcgttcagcacacccccagtgtagatcgggtcgatgagtcaccgcatcccccacgggcgaccgtggcggtggctgcgctggcggcctgcctacggggcaacccgtaggacgcttcaatacagacatggtgcgaagagtcgattgagctagttagtagtcctccggcccctgaatgcggctaatcctaactgcggagcacatgccctcaacccagggggtattgtgtcgtaacgggcaactctgcagcggaaccgactactttgggtgtccgtgtttccttttatccttatactggctgcttatggtgacaattgaaagattgttgccatatagctattggattggccatccagtgtctaatagagctgttatttacctctttgttggatttataccactcaacctaaaagaagttaaaacactacagctcattttacaactgaatacagcaaaccaccatggaagacgccaaaaacataaagaaaggcccggcgccattctatccgctggaagatggaaccgctggagagcaactgcataaggctatgaagagatacgccctggttcctggaacaattgcttttacagatgcacatatcgaggtggacatcacttacgctgagtacttcgaaatgtccgttcggttggcagaagctatgaaacgatatgggctgaatacaaatcacagaatcgtcgtatgcagtgaaaactctcttcaattctttatgccggtgttgggcgcgttatttatcggagttgcagttgcgcccgcgaacgacatttataatgaacgtgaattgctcaacagtatgggcatttcgcagcctaccgtggtgttcgtttccaaaaaggggttgcaaaaaattttgaacgtgcaaaaaaagctcccaatcatccaaaaaattattatcatggattctaaaacggattaccagggatttcagtcgatgtacacgttcgtcacatctcatctacctcccggttttaatgaatacgattttgtgccagagtccttcgatagggacaagacaattgcactgatcatgaactcctctggatctactggtctgcctaaaggtgtcgctctgcctcatagaactgcctgcgtgagattctcgcatgccagagatcctatttttggcaatcaaatcattccggatactgcgattttaagtgttgttccattccatcacggttttggaatgtttactacactcggatatttgatatgtggatttcgagtcgtcttaatgtatagatttgaagaagagctgtttctgaggagccttcaggattacaagattcaaagtgcgctgctggtgccaaccctattctccttcttcgccaaaagcactctgattgacaaatacgatttatctaatttacacgaaattgcttctggtggcgctcccctctctaaggaagtcggggaagcggttgccaagaggttccatctgccaggtatcaggcaaggatatgggctcactgagactacatcagctattctgattacacccgagggggatgataaaccgggcgcggtcggtaaagttgttccattttttgaagcgaaggttgtggatctggataccgggaaaacgctgggcgttaatcaaagaggcgaactgtgtgtgagaggtcctatgattatgtccggttatgtaaacaatccggaagcgaccaacgccttgattgacaaggatggatggctacattctggagacatagcttactgggacgaagacgaacacttcttcatcgttgaccgcctgaagtctctgattaagtacaaaggctatcaggtggctcccgctgaattggaatccatcttgctccaacaccccaacatcttcgacgcaggtgtcgcaggtcttcccgacgatgacgccggtgaacttcccgccgccgttgttgttttggagcacggaaagacgatgacggaaaaagagatcgtggattacgtcgccagtcaagtaacaaccgcgaaaaagttgcgcggaggagttgtgtttgtggacgaagtaccgaaaggtcttaccggaaaactcgacgcaagaaaaatcagagagatcctcataaaggccaagaagggcggaaagatcgccgtgtaacaggacaactttttccaaggaccacccggggaagctatgaaaaccgtgatcgccctcagttacatcttctgcctcgcctttggacagaatctcctcggaaacgaaaacaacgctgccacactctgcctgggacaccacgccgtgcccaacggcacaatggtgaagaccatcaccgacgatcagatcgaggtgaccaatgccaccgagctggtgcagaacagctccaccggcaaaatctgcaacaatccccacaagatcctggacggcagggattgcaccctgatcgacgctctgctgggcgaccctcactgcgacgtgttccagaatgagacatgggatctgttcgtggagaggagcaatgccttctccaactgctacccctacgacgtgcctgattacgccagcctgcggtccatcgtggccagctccggcaccctggagttcatcaccgagggcttcacctgggctggagtgacccagaacggaggcagcggagcttgcaagaggggacccgccaatagcttcttctcccggctgaactggctgaccaagtccggcaatacctaccccgtgctgaacgtgaccatgcctaacaataacaatttcgacaagctgtacatctggggcgtgcaccaccctagcaccgatcaggagcagaccagcctgtacatccaggcctccggcagggtgaccgtgagcaccaggcggtcccagcagaccatcatccccaacatcggctccaggcctctggtgcggggacagagcggccggatctccgtgtactggaccatcgtgaagcccggcgacatcctggtcatcaacagcaatggcaacctgatcgcccctcgcggctacttcaagatgcacatcggcaagagcagcatcatgagatccgacgcccccatcgatacctgcatcagcgagtgcatcacccctaatggctccatccccaacgagaagcctttccagaatgtgaacaagatcacctacggcgcctgccccaagtacgtgaagcagaataccctgaagctggccaccggcatgcgcaacgtgcctgagagacagaccgtgggcctgttcggagctatcgctggcttcatcgagaatggctgggagggcatggtggacggctggtacggcttccgccaccagaacagcgagggcaccggacaggctgccgacctgaagtccacccaggccgccatcgatcagatcaatggcaagctgaacagagtgatcgagaagaccaacgagaagttccaccagatcgagaaggagttcagcgaggtggagggacgcatccaggacctggagaggtacgtggaggacaccaagatcgatctgtggagctacaatgccgagctgctggtggccctggagaatcagaacaccatcgacctgaccgattccgagatgaacaagctgttcgagaagacccgcagacagctgcgcgagaatgccgaggacatgggcaacggctgcttcaaaatctaccacaagtgcgataacgcctgcatcgagagcatcagaaatggcacctacgaccacaacatctaccgcgatgaggccgtgaacaatagattccagatcaagggcgtggagctgaagtccggctacaaggactggattctgtggatcagcttcgccatctcctgcttcctgctgtgcgtggtgctgctggggtttattatgtgggcttgtcagagggggaacatcaggtgtaacatttgtaactttgagccaacaggggtgacggagtcccgcactgaaattacggcaatgcagaccaccggttcatgtgggcaacaatcaggagctgtgtacgtgggcaattacaggattgtaaacagacacctggcaacgagccacgattggcaaaattgcgtgtgggaggactacaacagggatctcctggtcagcacaacaactgctcatggttgtgatactatagcacggtgccaatgtactgctggcgtgtacttttgtgcatctagaaacaagcactacccagtgagcttcgagggtccaggtctagtgaaagttcaggagggcgagtactaccccgagagataccagtcgcacgtactccttgcagttggattttcagaaccgggtgattgtggaggtattttgaggtgtgaacatggagtcattgggctcgttaccatgggtggtgagggtgtagtaggcttcgctgacgtgcgggatcttttgtggttggaagacgacgccatggagcagggtgttagagattatgtagagcaactgggaaatgcatttggctcaggtttcactaaccaaatctgtgagcaagttaacctccttaaagaatctctgatagggcaggattccatattggaaaaatccctgaaggccctggttaaaatcatatcagccctggtgatagtggttaggaaccacgacgacctgattacagtgactgccacactagctttaatcggttgcgcatcatctccatggcgatggctcaaacaaaaagtgtgtcaatactacggaatccccatggcagaaaggcagaataacggttggttaaagaaattcactgaaatgaccaacgcctgcaagggcatggagtggattgctgttaaaattcaaaagttcatcgagtggctcaaagtaaagattctgcctgaagtgaaggagaaacatgagttccttaccagattgaagcaattgccactccttgaaagtcaaattgccaccattgagcaaagcgcaccctcacaaagtgatcaagagcagcttttttcgaatgttcagtacttcgcccattactgcaggaagtatgcacctctgtatgctgccgaagcaaaaagagtgttctcattagaaaagaaaatgagtaattacatacagttcaagtccaaatgccgcattgagcctgtatgcttactccttcacggtagtccaggggctggcaagtcagtagctaccaacctgatagggagatcccttgcagagaagctcaatagctctgtgtactctttaccaccagatccagatcattttgatgggtacaaacagcaggcagtggtgatcatggatgatctctgtcaaaaccccgatgggaaggacgtgtccttgttttgccaaatggtgtctagtgtagattttgtgccacccatggcggcgctggaagaaaaaggcattctctttacgtccccgtttgtgttggcatcaaccaacgcggggtccatcaatgcaccaacagtgtcagacagcagagcacttgccagaaggtttcactttgacatgaatattgaggtgatttcgatgtacagccagaatggtaaaattaacatgcccatgtctgttaagacatgtgatgatgaatgctgcccggtcaatttcaaaaagtgttgcccactagtgtgtggcaaggccatccagtttattgacaggagaaaccaagttagatattcactggacatgctggttactgagatgtttagagagtacaaccacagacacagtgtgggtgctaccctcgaggctttgttccaaggaccaccagtatacagggaaatcaaaatcagtgtggccccggaaacaccccctccaccagcaattgctgaccttctaaaatctgtagacagtgaggcaataagggagtactgcaaggaaaggggttggcttgtgccagaggtcagctccactctacaaattgaaaaacatgttagcagggcatttatttgcttgcaagcgctaactacatttgtttcagtggctggtataatctacatcatttacaagttgtttgccggctttcagggtgcatacactggaatgcccaaccagaaacccaaggtgcccaccttaagacaagctaaggtgcaaggtccggcatttgaatttgccgtagcaatgatgaaaaggaacgccagcacagtcaagacagaatacggtgagttcacgatgcttggcatctatgataaatgggcagtgctgccgcgccacgccaagcctggaccaactattttaatgaatgatcaggaggttggtgtgctcgatgccaaagagttagttgataaagacggaaccaacctggagctgacactattgaagcttaaccgcaatgaaaagttcagagacatcagaggttttcttgcaagggaagaagttgaggtaagtgaggctgttttggcaataaacacgagcaagttcccaagcatgtacatccctgtgggccaagtcaccgattacggatttttaaatctaggtggcaccccaacaaagagaatgctcatgtacaacttccctaccagagcgggacagtgtggtggtgtccttatgtcaacaggaaaggtccttggcatacacgtgggaggaaatggtcaccaaggcttctctgctgctctcctcagacactacttcaacgaggaacagggcgaaatagagtttattgagagctctaaagatgcaggatttcctgtgatcaacacccctaataaaaccaaactggaaccaagtgtgtttcatcaggtttttgagggcaacaaagaaccagcagtcctaagaaacggagacccgcgacttaaagccaactttgaggaagcgatattttccaagtacatcggaaatgtgaacacacatgtggacgagtacatgatagaagctgttgatcactacgctggacagctggcaactctggacatcagtacagaacctatgaagcttgaggatgctgtttatggcactgaaggcttggaagcattggacttgaccactagcgcaggatatccttatgtcgccttgggcatcaagaaaagggatatcctctccaagaagactaaagatctcaccaagctgagggaatgcatggacaagtatggtctaaatctgccgatggtgacctacgtgaaggatgaactcaggtccgctgagaaagtagccaagggaaaatccagacttatagaagcttctagtctcaatgactcagtggccatgaggcagacatttgggaacctatacaagacattccacctcaacccaggcattgtcactggtagtgctgttgggtgcgacccagatgtgttttggagcaaaatacccgtgatgcttgacgggcaccttatagcttttgattactctggctacgacgctagcttgagcccagtgtggtttgcttgtttgaaactcctcctagggaaactagggtatactcataaggaaaccaattacatagactacctctgcaactcccatcacttatacagagataaacactatttcgtgaggggtggtatgccatcaggatgttcaggcaccagtatattcaacaccatgatcaacaacatcattattaggacccttatgctaaaggtctacaaaggtattgacctggatcagtttagaatgatcgcttacggggacgatgtgatagcctcttacccgtggcctattgatgcctcactactagcagaagcgggaaaggattatggtttgatcatgaccccagcagataaaggagagtgttttaatgaggtaacctggacaaatgtaaccttcttgaaaaggtactttagagctgatgaacaatatccattcttggtgcaccccgtgatgcccatgaaagacatacacgaatccattagatggaccaaagacccaaagaacactcaagatcatgtgcgctcgttatgcctattggcttggcacaatggggagcacgaatatgaggaatttatccgaaagatcagaagcgtgcctgttggacgctgtttgaccctcccggtgttctcaacactacgcaggaaatggttagattccttctaaaattagagtgcaatcaatgaactatgattggcttaaccctaccgcatgaaccgaactagacaaaagtgcggtaggggtaaattctccgcattcggtgcggaaaaaaaaaaaaaaaaaaaaaaaaaaaaaaaaaaaaaaaaaaaaaaaaaa